European Patent Application EP 4 768 586 A1, published July 1, 2026. Title: NEW SIRNA, COMPOSITION COMPRISING SAME, AND USE. Applicant: CHANGCHUN GENESCIENCE PHARMACEUTICAL CO., LTD. The sequence listing filed with the application follows.

SEQUENCE LISTING (1446 sequences)

SEQ ID NO: 1 - RNA, 21 nt, synthetic construct
  source 1..21: mol_type = other RNA; note = GPSZRA001 antisense strand
gccatcctgcttccttccagg

SEQ ID NO: 2 - RNA, 21 nt, synthetic construct
  source 1..21: mol_type = other RNA; note = GPSZRA002 antisense strand
acagactgaggaccagcaccc

SEQ ID NO: 3 - RNA, 21 nt, synthetic construct
  source 1..21: mol_type = other RNA; note = GPSZRA003 antisense strand
cacagactgaggaccagcacc

SEQ ID NO: 4 - RNA, 21 nt, synthetic construct
  source 1..21: mol_type = other RNA; note = GPSZRA004 antisense strand
gttttgagcacctactactgc

SEQ ID NO: 5 - RNA, 21 nt, synthetic construct
  source 1..21: mol_type = other RNA; note = GPSZRA005 antisense strand
tgttttgagcacctactactg

SEQ ID NO: 6 - RNA, 21 nt, synthetic construct
  source 1..21: mol_type = other RNA; note = GPSZRA006 antisense strand
atgttttgagcacctactact

SEQ ID NO: 7 - RNA, 21 nt, synthetic construct
  source 1..21: mol_type = other RNA; note = GPSZRA007 antisense strand
gatgttttgagcacctactac

SEQ ID NO: 8 - RNA, 21 nt, synthetic construct
  source 1..21: mol_type = other RNA; note = GPSZRA008 antisense strand
tgatgttttgagcacctacta

SEQ ID NO: 9 - RNA, 21 nt, synthetic construct
  source 1..21: mol_type = other RNA; note = GPSZRA009 antisense strand
gtgatgttttgagcacctact

SEQ ID NO: 10 - RNA, 21 nt, synthetic construct
  source 1..21: mol_type = other RNA; note = GPSZRA010 antisense strand
tgtgatgttttgagcacctac

SEQ ID NO: 11 - RNA, 21 nt, synthetic construct
  source 1..21: mol_type = other RNA; note = GPSZRA011 antisense strand
ctgtgatgttttgagcaccta

SEQ ID NO: 12 - RNA, 21 nt, synthetic construct
  source 1..21: mol_type = other RNA; note = GPSZRA012 antisense strand
gctgtgatgttttgagcacct

SEQ ID NO: 13 - RNA, 21 nt, synthetic construct
  source 1..21: mol_type = other RNA; note = GPSZRA013 antisense strand
ggctgtgatgttttgagcacc

SEQ ID NO: 14 - RNA, 21 nt, synthetic construct
  source 1..21: mol_type = other RNA; note = GPSZRA014 antisense strand
gggctgtgatgttttgagcac

SEQ ID NO: 15 - RNA, 21 nt, synthetic construct
  source 1..21: mol_type = other RNA; note = GPSZRA015 antisense strand
cgggctgtgatgttttgagca

SEQ ID NO: 16 - RNA, 21 nt, synthetic construct
  source 1..21: mol_type = other RNA; note = GPSZRA016 antisense strand
ccgggctgtgatgttttgagc

SEQ ID NO: 17 - RNA, 21 nt, synthetic construct
  source 1..21: mol_type = other RNA; note = GPSZRA017 antisense strand
tccgggctgtgatgttttgag

SEQ ID NO: 18 - RNA, 21 nt, synthetic construct
  source 1..21: mol_type = other RNA; note = GPSZRA018 antisense strand
atccgggctgtgatgttttga

SEQ ID NO: 19 - RNA, 21 nt, synthetic construct
  source 1..21: mol_type = other RNA; note = GPSZRA019 antisense strand
acacttcagcaccagtggctc

SEQ ID NO: 20 - RNA, 21 nt, synthetic construct
  source 1..21: mol_type = other RNA; note = GPSZRA020 antisense strand
tacacttcagcaccagtggct

SEQ ID NO: 21 - RNA, 21 nt, synthetic construct
  source 1..21: mol_type = other RNA; note = GPSZRA021 antisense strand
ttacacttcagcaccagtggc

SEQ ID NO: 22 - RNA, 21 nt, synthetic construct
  source 1..21: mol_type = other RNA; note = GPSZRA022 antisense strand
cttacacttcagcaccagtgg

SEQ ID NO: 23 - RNA, 21 nt, synthetic construct
  source 1..21: mol_type = other RNA; note = GPSZRA023 antisense strand
ccttacacttcagcaccagtg

SEQ ID NO: 24 - RNA, 21 nt, synthetic construct
  source 1..21: mol_type = other RNA; note = GPSZRA024 antisense strand
cccttacacttcagcaccagt

SEQ ID NO: 25 - RNA, 21 nt, synthetic construct
  source 1..21: mol_type = other RNA; note = GPSZRA025 antisense strand
ccccttacacttcagcaccag

SEQ ID NO: 26 - RNA, 21 nt, synthetic construct
  source 1..21: mol_type = other RNA; note = GPSZRA026 antisense strand
cccccttacacttcagcacca

SEQ ID NO: 27 - RNA, 21 nt, synthetic construct
  source 1..21: mol_type = other RNA; note = GPSZRA027 antisense strand
gcccccttacacttcagcacc

SEQ ID NO: 28 - RNA, 21 nt, synthetic construct
  source 1..21: mol_type = other RNA; note = GPSZRA028 antisense strand
tttcttgggggcccccttaca

SEQ ID NO: 29 - RNA, 21 nt, synthetic construct
  source 1..21: mol_type = other RNA; note = GPSZRA029 antisense strand
ttccaagcttctgtccggcct

SEQ ID NO: 30 - RNA, 21 nt, synthetic construct
  source 1..21: mol_type = other RNA; note = GPSZRA030 antisense strand
cttccaagcttctgtccggcc

SEQ ID NO: 31 - RNA, 21 nt, synthetic construct
  source 1..21: mol_type = other RNA; note = GPSZRA031 antisense strand
ccttccaagcttctgtccggc

SEQ ID NO: 32 - RNA, 21 nt, synthetic construct
  source 1..21: mol_type = other RNA; note = GPSZRA032 antisense strand
accttccaagcttctgtccgg

SEQ ID NO: 33 - RNA, 21 nt, synthetic construct
  source 1..21: mol_type = other RNA; note = GPSZRA033 antisense strand
gaccttccaagcttctgtccg

SEQ ID NO: 34 - RNA, 21 nt, synthetic construct
  source 1..21: mol_type = other RNA; note = GPSZRA034 antisense strand
ggaccttccaagcttctgtcc

SEQ ID NO: 35 - RNA, 21 nt, synthetic construct
  source 1..21: mol_type = other RNA; note = GPSZRA035 antisense strand
aggaccttccaagcttctgtc

SEQ ID NO: 36 - RNA, 21 nt, synthetic construct
  source 1..21: mol_type = other RNA; note = GPSZRA036 antisense strand
ttgggaaggacacgagccaca

SEQ ID NO: 37 - RNA, 21 nt, synthetic construct
  source 1..21: mol_type = other RNA; note = GPSZRA037 antisense strand
aagagggagccgttgggaagg

SEQ ID NO: 38 - RNA, 21 nt, synthetic construct
  source 1..21: mol_type = other RNA; note = GPSZRA038 antisense strand
aaggaagagggagccgttggg

SEQ ID NO: 39 - RNA, 21 nt, synthetic construct
  source 1..21: mol_type = other RNA; note = GPSZRA039 antisense strand
gaaggaagagggagccgttgg

SEQ ID NO: 40 - RNA, 21 nt, synthetic construct
  source 1..21: mol_type = other RNA; note = GPSZRA040 antisense strand
tcatcctggatcccgacagcc

SEQ ID NO: 41 - RNA, 21 nt, synthetic construct
  source 1..21: mol_type = other RNA; note = GPSZRA041 antisense strand
ctcatcctggatcccgacagc

SEQ ID NO: 42 - RNA, 21 nt, synthetic construct
  source 1..21: mol_type = other RNA; note = GPSZRA042 antisense strand
atcccctcatcctggatcccg

SEQ ID NO: 43 - RNA, 21 nt, synthetic construct
  source 1..21: mol_type = other RNA; note = GPSZRA043 antisense strand
aatcccctcatcctggatccc

SEQ ID NO: 44 - RNA, 21 nt, synthetic construct
  source 1..21: mol_type = other RNA; note = GPSZRA044 antisense strand
aaatcccctcatcctggatcc

SEQ ID NO: 45 - RNA, 21 nt, synthetic construct
  source 1..21: mol_type = other RNA; note = GPSZRA045 antisense strand
aaaatcccctcatcctggatc

SEQ ID NO: 46 - RNA, 21 nt, synthetic construct
  source 1..21: mol_type = other RNA; note = GPSZRA046 antisense strand
gaaaatcccctcatcctggat

SEQ ID NO: 47 - RNA, 21 nt, synthetic construct
  source 1..21: mol_type = other RNA; note = GPSZRA047 antisense strand
ggaaaatcccctcatcctgga

SEQ ID NO: 48 - RNA, 21 nt, synthetic construct
  source 1..21: mol_type = other RNA; note = GPSZRA048 antisense strand
cggaaaatcccctcatcctgg

SEQ ID NO: 49 - RNA, 21 nt, synthetic construct
  source 1..21: mol_type = other RNA; note = GPSZRA049 antisense strand
ccggaaaatcccctcatcctg

SEQ ID NO: 50 - RNA, 21 nt, synthetic construct
  source 1..21: mol_type = other RNA; note = GPSZRA050 antisense strand
accggaaaatcccctcatcct

SEQ ID NO: 51 - RNA, 21 nt, synthetic construct
  source 1..21: mol_type = other RNA; note = GPSZRA051 antisense strand
caccggaaaatcccctcatcc

SEQ ID NO: 52 - RNA, 21 nt, synthetic construct
  source 1..21: mol_type = other RNA; note = GPSZRA052 antisense strand
gcaccggaaaatcccctcatc

SEQ ID NO: 53 - RNA, 21 nt, synthetic construct
  source 1..21: mol_type = other RNA; note = GPSZRA053 antisense strand
tggcaccggaaaatcccctca

SEQ ID NO: 54 - RNA, 21 nt, synthetic construct
  source 1..21: mol_type = other RNA; note = GPSZRA054 antisense strand
tgcctggcaccggaaaatccc

SEQ ID NO: 55 - RNA, 21 nt, synthetic construct
  source 1..21: mol_type = other RNA; note = GPSZRA055 antisense strand
ttgcctggcaccggaaaatcc

SEQ ID NO: 56 - RNA, 21 nt, synthetic construct
  source 1..21: mol_type = other RNA; note = GPSZRA056 antisense strand
attgcctggcaccggaaaatc

SEQ ID NO: 57 - RNA, 21 nt, synthetic construct
  source 1..21: mol_type = other RNA; note = GPSZRA057 antisense strand
cattgcctggcaccggaaaat

SEQ ID NO: 58 - RNA, 21 nt, synthetic construct
  source 1..21: mol_type = other RNA; note = GPSZRA058 antisense strand
tcattgcctggcaccggaaaa

SEQ ID NO: 59 - RNA, 21 nt, synthetic construct
  source 1..21: mol_type = other RNA; note = GPSZRA059 antisense strand
ttcattgcctggcaccggaaa

SEQ ID NO: 60 - RNA, 21 nt, synthetic construct
  source 1..21: mol_type = other RNA; note = GPSZRA060 antisense strand
tgttcattgcctggcaccgga

SEQ ID NO: 61 - RNA, 21 nt, synthetic construct
  source 1..21: mol_type = other RNA; note = GPSZRA061 antisense strand
ctgttcattgcctggcaccgg

SEQ ID NO: 62 - RNA, 21 nt, synthetic construct
  source 1..21: mol_type = other RNA; note = GPSZRA062 antisense strand
cctgttcattgcctggcaccg

SEQ ID NO: 63 - RNA, 21 nt, synthetic construct
  source 1..21: mol_type = other RNA; note = GPSZRA063 antisense strand
tcctgttcattgcctggcacc

SEQ ID NO: 64 - RNA, 21 nt, synthetic construct
  source 1..21: mol_type = other RNA; note = GPSZRA064 antisense strand
ttcctgttcattgcctggcac

SEQ ID NO: 65 - RNA, 21 nt, synthetic construct
  source 1..21: mol_type = other RNA; note = GPSZRA065 antisense strand
attcctgttcattgcctggca

SEQ ID NO: 66 - RNA, 21 nt, synthetic construct
  source 1..21: mol_type = other RNA; note = GPSZRA066 antisense strand
cattcctgttcattgcctggc

SEQ ID NO: 67 - RNA, 21 nt, synthetic construct
  source 1..21: mol_type = other RNA; note = GPSZRA067 antisense strand
ccattcctgttcattgcctgg

SEQ ID NO: 68 - RNA, 21 nt, synthetic construct
  source 1..21: mol_type = other RNA; note = GPSZRA068 antisense strand
tccattcctgttcattgcctg

SEQ ID NO: 69 - RNA, 21 nt, synthetic construct
  source 1..21: mol_type = other RNA; note = GPSZRA069 antisense strand
ttccattcctgttcattgcct

SEQ ID NO: 70 - RNA, 21 nt, synthetic construct
  source 1..21: mol_type = other RNA; note = GPSZRA070 antisense strand
tttccattcctgttcattgcc

SEQ ID NO: 71 - RNA, 21 nt, synthetic construct
  source 1..21: mol_type = other RNA; note = GPSZRA071 antisense strand
ctttccattcctgttcattgc

SEQ ID NO: 72 - RNA, 21 nt, synthetic construct
  source 1..21: mol_type = other RNA; note = GPSZRA072 antisense strand
cctttccattcctgttcattg

SEQ ID NO: 73 - RNA, 21 nt, synthetic construct
  source 1..21: mol_type = other RNA; note = GPSZRA073 antisense strand
tcctttccattcctgttcatt

SEQ ID NO: 74 - RNA, 21 nt, synthetic construct
  source 1..21: mol_type = other RNA; note = GPSZRA074 antisense strand
ctcctttccattcctgttcat

SEQ ID NO: 75 - RNA, 21 nt, synthetic construct
  source 1..21: mol_type = other RNA; note = GPSZRA075 antisense strand
tctcctttccattcctgttca

SEQ ID NO: 76 - RNA, 21 nt, synthetic construct
  source 1..21: mol_type = other RNA; note = GPSZRA076 antisense strand
gtctcctttccattcctgttc

SEQ ID NO: 77 - RNA, 21 nt, synthetic construct
  source 1..21: mol_type = other RNA; note = GPSZRA077 antisense strand
ggtctcctttccattcctgtt

SEQ ID NO: 78 - RNA, 21 nt, synthetic construct
  source 1..21: mol_type = other RNA; note = GPSZRA078 antisense strand
tggtctcctttccattcctgt

SEQ ID NO: 79 - RNA, 21 nt, synthetic construct
  source 1..21: mol_type = other RNA; note = GPSZRA079 antisense strand
ttggtctcctttccattcctg

SEQ ID NO: 80 - RNA, 21 nt, synthetic construct
  source 1..21: mol_type = other RNA; note = GPSZRA080 antisense strand
cttggtctcctttccattcct

SEQ ID NO: 81 - RNA, 21 nt, synthetic construct
  source 1..21: mol_type = other RNA; note = GPSZRA081 antisense strand
acttggtctcctttccattcc

SEQ ID NO: 82 - RNA, 21 nt, synthetic construct
  source 1..21: mol_type = other RNA; note = GPSZRA082 antisense strand
gacttggtctcctttccattc

SEQ ID NO: 83 - RNA, 21 nt, synthetic construct
  source 1..21: mol_type = other RNA; note = GPSZRA083 antisense strand
ggacttggtctcctttccatt

SEQ ID NO: 84 - RNA, 21 nt, synthetic construct
  source 1..21: mol_type = other RNA; note = GPSZRA084 antisense strand
tggacttggtctcctttccat

SEQ ID NO: 85 - RNA, 21 nt, synthetic construct
  source 1..21: mol_type = other RNA; note = GPSZRA085 antisense strand
ttggacttggtctcctttcca

SEQ ID NO: 86 - RNA, 21 nt, synthetic construct
  source 1..21: mol_type = other RNA; note = GPSZRA086 antisense strand
gttggacttggtctcctttcc

SEQ ID NO: 87 - RNA, 21 nt, synthetic construct
  source 1..21: mol_type = other RNA; note = GPSZRA087 antisense strand
agttggacttggtctcctttc

SEQ ID NO: 88 - RNA, 21 nt, synthetic construct
  source 1..21: mol_type = other RNA; note = GPSZRA088 antisense strand
tagttggacttggtctccttt

SEQ ID NO: 89 - RNA, 21 nt, synthetic construct
  source 1..21: mol_type = other RNA; note = GPSZRA089 antisense strand
gtagttggacttggtctcctt

SEQ ID NO: 90 - RNA, 21 nt, synthetic construct
  source 1..21: mol_type = other RNA; note = GPSZRA090 antisense strand
ggtagttggacttggtctcct

SEQ ID NO: 91 - RNA, 21 nt, synthetic construct
  source 1..21: mol_type = other RNA; note = GPSZRA091 antisense strand
cggtagttggacttggtctcc

SEQ ID NO: 92 - RNA, 21 nt, synthetic construct
  source 1..21: mol_type = other RNA; note = GPSZRA092 antisense strand
tcggtagttggacttggtctc

SEQ ID NO: 93 - RNA, 21 nt, synthetic construct
  source 1..21: mol_type = other RNA; note = GPSZRA093 antisense strand
ctcggtagttggacttggtct

SEQ ID NO: 94 - RNA, 21 nt, synthetic construct
  source 1..21: mol_type = other RNA; note = GPSZRA094 antisense strand
actcggtagttggacttggtc

SEQ ID NO: 95 - RNA, 21 nt, synthetic construct
  source 1..21: mol_type = other RNA; note = GPSZRA095 antisense strand
gactcggtagttggacttggt

SEQ ID NO: 96 - RNA, 21 nt, synthetic construct
  source 1..21: mol_type = other RNA; note = GPSZRA096 antisense strand
ggactcggtagttggacttgg

SEQ ID NO: 97 - RNA, 21 nt, synthetic construct
  source 1..21: mol_type = other RNA; note = GPSZRA097 antisense strand
cggactcggtagttggacttg

SEQ ID NO: 98 - RNA, 21 nt, synthetic construct
  source 1..21: mol_type = other RNA; note = GPSZRA098 antisense strand
acggactcggtagttggactt

SEQ ID NO: 99 - RNA, 21 nt, synthetic construct
  source 1..21: mol_type = other RNA; note = GPSZRA099 antisense strand
cacggactcggtagttggact

SEQ ID NO: 100 - RNA, 21 nt, synthetic construct
  source 1..21: mol_type = other RNA; note = GPSZRA100 antisense strand
acacggactcggtagttggac

SEQ ID NO: 101 - RNA, 21 nt, synthetic construct
  source 1..21: mol_type = other RNA; note = GPSZRA101 antisense strand
gacacggactcggtagttgga

SEQ ID NO: 102 - RNA, 21 nt, synthetic construct
  source 1..21: mol_type = other RNA; note = GPSZRA102 antisense strand
agacacggactcggtagttgg

SEQ ID NO: 103 - RNA, 21 nt, synthetic construct
  source 1..21: mol_type = other RNA; note = GPSZRA103 antisense strand
tagacacggactcggtagttg

SEQ ID NO: 104 - RNA, 21 nt, synthetic construct
  source 1..21: mol_type = other RNA; note = GPSZRA104 antisense strand
gtagacacggactcggtagtt

SEQ ID NO: 105 - RNA, 21 nt, synthetic construct
  source 1..21: mol_type = other RNA; note = GPSZRA105 antisense strand
ggtagacacggactcggtagt

SEQ ID NO: 106 - RNA, 21 nt, synthetic construct
  source 1..21: mol_type = other RNA; note = GPSZRA106 antisense strand
tggtagacacggactcggtag

SEQ ID NO: 107 - RNA, 21 nt, synthetic construct
  source 1..21: mol_type = other RNA; note = GPSZRA107 antisense strand
tctggtagacacggactcggt

SEQ ID NO: 108 - RNA, 21 nt, synthetic construct
  source 1..21: mol_type = other RNA; note = GPSZRA108 antisense strand
atctggtagacacggactcgg

SEQ ID NO: 109 - RNA, 21 nt, synthetic construct
  source 1..21: mol_type = other RNA; note = GPSZRA109 antisense strand
aatctggtagacacggactcg

SEQ ID NO: 110 - RNA, 21 nt, synthetic construct
  source 1..21: mol_type = other RNA; note = GPSZRA110 antisense strand
gaatctggtagacacggactc

SEQ ID NO: 111 - RNA, 21 nt, synthetic construct
  source 1..21: mol_type = other RNA; note = GPSZRA111 antisense strand
ggaatctggtagacacggact

SEQ ID NO: 112 - RNA, 21 nt, synthetic construct
  source 1..21: mol_type = other RNA; note = GPSZRA112 antisense strand
aggaatctggtagacacggac

SEQ ID NO: 113 - RNA, 21 nt, synthetic construct
  source 1..21: mol_type = other RNA; note = GPSZRA113 antisense strand
caggaatctggtagacacgga

SEQ ID NO: 114 - RNA, 21 nt, synthetic construct
  source 1..21: mol_type = other RNA; note = GPSZRA114 antisense strand
ccaggaatctggtagacacgg

SEQ ID NO: 115 - RNA, 21 nt, synthetic construct
  source 1..21: mol_type = other RNA; note = GPSZRA115 antisense strand
cccaggaatctggtagacacg

SEQ ID NO: 116 - RNA, 21 nt, synthetic construct
  source 1..21: mol_type = other RNA; note = GPSZRA116 antisense strand
tcccaggaatctggtagacac

SEQ ID NO: 117 - RNA, 21 nt, synthetic construct
  source 1..21: mol_type = other RNA; note = GPSZRA117 antisense strand
ttcccaggaatctggtagaca

SEQ ID NO: 118 - RNA, 21 nt, synthetic construct
  source 1..21: mol_type = other RNA; note = GPSZRA118 antisense strand
cttcccaggaatctggtagac

SEQ ID NO: 119 - RNA, 21 nt, synthetic construct
  source 1..21: mol_type = other RNA; note = GPSZRA119 antisense strand
gcttcccaggaatctggtaga

SEQ ID NO: 120 - RNA, 21 nt, synthetic construct
  source 1..21: mol_type = other RNA; note = GPSZRA120 antisense strand
ggcttcccaggaatctggtag

SEQ ID NO: 121 - RNA, 21 nt, synthetic construct
  source 1..21: mol_type = other RNA; note = GPSZRA121 antisense strand
tgagttcagaggcagaatcta

SEQ ID NO: 122 - RNA, 21 nt, synthetic construct
  source 1..21: mol_type = other RNA; note = GPSZRA122 antisense strand
gtgagttcagaggcagaatct

SEQ ID NO: 123 - RNA, 21 nt, synthetic construct
  source 1..21: mol_type = other RNA; note = GPSZRA123 antisense strand
cgtgagttcagaggcagaatc

SEQ ID NO: 124 - RNA, 21 nt, synthetic construct
  source 1..21: mol_type = other RNA; note = GPSZRA124 antisense strand
ccgtgagttcagaggcagaat

SEQ ID NO: 125 - RNA, 21 nt, synthetic construct
  source 1..21: mol_type = other RNA; note = GPSZRA125 antisense strand
agccgtgagttcagaggcaga

SEQ ID NO: 126 - RNA, 21 nt, synthetic construct
  source 1..21: mol_type = other RNA; note = GPSZRA126 antisense strand
accagccgtgagttcagaggc

SEQ ID NO: 127 - RNA, 21 nt, synthetic construct
  source 1..21: mol_type = other RNA; note = GPSZRA127 antisense strand
caccagccgtgagttcagagg

SEQ ID NO: 128 - RNA, 21 nt, synthetic construct
  source 1..21: mol_type = other RNA; note = GPSZRA128 antisense strand
acaccagccgtgagttcagag

SEQ ID NO: 129 - RNA, 21 nt, synthetic construct
  source 1..21: mol_type = other RNA; note = GPSZRA129 antisense strand
aacaccagccgtgagttcaga

SEQ ID NO: 130 - RNA, 21 nt, synthetic construct
  source 1..21: mol_type = other RNA; note = GPSZRA130 antisense strand
gaacaccagccgtgagttcag

SEQ ID NO: 131 - RNA, 21 nt, synthetic construct
  source 1..21: mol_type = other RNA; note = GPSZRA131 antisense strand
ggaacaccagccgtgagttca

SEQ ID NO: 132 - RNA, 21 nt, synthetic construct
  source 1..21: mol_type = other RNA; note = GPSZRA132 antisense strand
ttgggaacaccagccgtgagt

SEQ ID NO: 133 - RNA, 21 nt, synthetic construct
  source 1..21: mol_type = other RNA; note = GPSZRA133 antisense strand
attgggaacaccagccgtgag

SEQ ID NO: 134 - RNA, 21 nt, synthetic construct
  source 1..21: mol_type = other RNA; note = GPSZRA134 antisense strand
tattgggaacaccagccgtga

SEQ ID NO: 135 - RNA, 21 nt, synthetic construct
  source 1..21: mol_type = other RNA; note = GPSZRA135 antisense strand
ttattgggaacaccagccgtg

SEQ ID NO: 136 - RNA, 21 nt, synthetic construct
  source 1..21: mol_type = other RNA; note = GPSZRA136 antisense strand
cttattgggaacaccagccgt

SEQ ID NO: 137 - RNA, 21 nt, synthetic construct
  source 1..21: mol_type = other RNA; note = GPSZRA137 antisense strand
ccttattgggaacaccagccg

SEQ ID NO: 138 - RNA, 21 nt, synthetic construct
  source 1..21: mol_type = other RNA; note = GPSZRA138 antisense strand
accttattgggaacaccagcc

SEQ ID NO: 139 - RNA, 21 nt, synthetic construct
  source 1..21: mol_type = other RNA; note = GPSZRA139 antisense strand
caccttattgggaacaccagc

SEQ ID NO: 140 - RNA, 21 nt, synthetic construct
  source 1..21: mol_type = other RNA; note = GPSZRA140 antisense strand
ccaccttattgggaacaccag

SEQ ID NO: 141 - RNA, 21 nt, synthetic construct
  source 1..21: mol_type = other RNA; note = GPSZRA141 antisense strand
cccaccttattgggaacacca

SEQ ID NO: 142 - RNA, 21 nt, synthetic construct
  source 1..21: mol_type = other RNA; note = GPSZRA142 antisense strand
ccccaccttattgggaacacc

SEQ ID NO: 143 - RNA, 21 nt, synthetic construct
  source 1..21: mol_type = other RNA; note = GPSZRA143 antisense strand
tccccaccttattgggaacac

SEQ ID NO: 144 - RNA, 21 nt, synthetic construct
  source 1..21: mol_type = other RNA; note = GPSZRA144 antisense strand
gtccccaccttattgggaaca

SEQ ID NO: 145 - RNA, 21 nt, synthetic construct
  source 1..21: mol_type = other RNA; note = GPSZRA145 antisense strand
tgtccccaccttattgggaac

SEQ ID NO: 146 - RNA, 21 nt, synthetic construct
  source 1..21: mol_type = other RNA; note = GPSZRA146 antisense strand
atgtccccaccttattgggaa

SEQ ID NO: 147 - RNA, 21 nt, synthetic construct
  source 1..21: mol_type = other RNA; note = GPSZRA147 antisense strand
catgtccccaccttattggga

SEQ ID NO: 148 - RNA, 21 nt, synthetic construct
  source 1..21: mol_type = other RNA; note = GPSZRA148 antisense strand
acatgtccccaccttattggg

SEQ ID NO: 149 - RNA, 21 nt, synthetic construct
  source 1..21: mol_type = other RNA; note = GPSZRA149 antisense strand
cacatgtccccaccttattgg

SEQ ID NO: 150 - RNA, 21 nt, synthetic construct
  source 1..21: mol_type = other RNA; note = GPSZRA150 antisense strand
acacatgtccccaccttattg

SEQ ID NO: 151 - RNA, 21 nt, synthetic construct
  source 1..21: mol_type = other RNA; note = GPSZRA151 antisense strand
cacacatgtccccaccttatt

SEQ ID NO: 152 - RNA, 21 nt, synthetic construct
  source 1..21: mol_type = other RNA; note = GPSZRA152 antisense strand
acacacatgtccccaccttat

SEQ ID NO: 153 - RNA, 21 nt, synthetic construct
  source 1..21: mol_type = other RNA; note = GPSZRA153 antisense strand
gacacacatgtccccacctta

SEQ ID NO: 154 - RNA, 21 nt, synthetic construct
  source 1..21: mol_type = other RNA; note = GPSZRA154 antisense strand
tgacacacatgtccccacctt

SEQ ID NO: 155 - RNA, 21 nt, synthetic construct
  source 1..21: mol_type = other RNA; note = GPSZRA155 antisense strand
ctgacacacatgtccccacct

SEQ ID NO: 156 - RNA, 21 nt, synthetic construct
  source 1..21: mol_type = other RNA; note = GPSZRA156 antisense strand
tctgacacacatgtccccacc

SEQ ID NO: 157 - RNA, 21 nt, synthetic construct
  source 1..21: mol_type = other RNA; note = GPSZRA157 antisense strand
ctctgacacacatgtccccac

SEQ ID NO: 158 - RNA, 21 nt, synthetic construct
  source 1..21: mol_type = other RNA; note = GPSZRA158 antisense strand
cctctgacacacatgtcccca

SEQ ID NO: 159 - RNA, 21 nt, synthetic construct
  source 1..21: mol_type = other RNA; note = GPSZRA159 antisense strand
ccctctgacacacatgtcccc

SEQ ID NO: 160 - RNA, 21 nt, synthetic construct
  source 1..21: mol_type = other RNA; note = GPSZRA160 antisense strand
tccctctgacacacatgtccc

SEQ ID NO: 161 - RNA, 21 nt, synthetic construct
  source 1..21: mol_type = other RNA; note = GPSZRA161 antisense strand
ttccctctgacacacatgtcc

SEQ ID NO: 162 - RNA, 21 nt, synthetic construct
  source 1..21: mol_type = other RNA; note = GPSZRA162 antisense strand
cttccctctgacacacatgtc

SEQ ID NO: 163 - RNA, 21 nt, synthetic construct
  source 1..21: mol_type = other RNA; note = GPSZRA163 antisense strand
gcttccctctgacacacatgt

SEQ ID NO: 164 - RNA, 21 nt, synthetic construct
  source 1..21: mol_type = other RNA; note = GPSZRA164 antisense strand
agcttccctctgacacacatg

SEQ ID NO: 165 - RNA, 21 nt, synthetic construct
  source 1..21: mol_type = other RNA; note = GPSZRA165 antisense strand
tagcttccctctgacacacat

SEQ ID NO: 166 - RNA, 21 nt, synthetic construct
  source 1..21: mol_type = other RNA; note = GPSZRA166 antisense strand
gtagcttccctctgacacaca

SEQ ID NO: 167 - RNA, 21 nt, synthetic construct
  source 1..21: mol_type = other RNA; note = GPSZRA167 antisense strand
ggtagcttccctctgacacac

SEQ ID NO: 168 - RNA, 21 nt, synthetic construct
  source 1..21: mol_type = other RNA; note = GPSZRA168 antisense strand
gggtagcttccctctgacaca

SEQ ID NO: 169 - RNA, 21 nt, synthetic construct
  source 1..21: mol_type = other RNA; note = GPSZRA169 antisense strand
agggtagcttccctctgacac

SEQ ID NO: 170 - RNA, 21 nt, synthetic construct
  source 1..21: mol_type = other RNA; note = GPSZRA170 antisense strand
cagggtagcttccctctgaca

SEQ ID NO: 171 - RNA, 21 nt, synthetic construct
  source 1..21: mol_type = other RNA; note = GPSZRA171 antisense strand
tgcagggtagcttccctctga

SEQ ID NO: 172 - RNA, 21 nt, synthetic construct
  source 1..21: mol_type = other RNA; note = GPSZRA172 antisense strand
agtccctgcagggtagcttcc

SEQ ID NO: 173 - RNA, 21 nt, synthetic construct
  source 1..21: mol_type = other RNA; note = GPSZRA173 antisense strand
aagagtccctgcagggtagct

SEQ ID NO: 174 - RNA, 21 nt, synthetic construct
  source 1..21: mol_type = other RNA; note = GPSZRA174 antisense strand
taagagtccctgcagggtagc

SEQ ID NO: 175 - RNA, 21 nt, synthetic construct
  source 1..21: mol_type = other RNA; note = GPSZRA175 antisense strand
ctaagagtccctgcagggtag

SEQ ID NO: 176 - RNA, 21 nt, synthetic construct
  source 1..21: mol_type = other RNA; note = GPSZRA176 antisense strand
agctaagagtccctgcagggt

SEQ ID NO: 177 - RNA, 21 nt, synthetic construct
  source 1..21: mol_type = other RNA; note = GPSZRA177 antisense strand
cagctaagagtccctgcaggg

SEQ ID NO: 178 - RNA, 21 nt, synthetic construct
  source 1..21: mol_type = other RNA; note = GPSZRA178 antisense strand
ccagctaagagtccctgcagg

SEQ ID NO: 179 - RNA, 21 nt, synthetic construct
  source 1..21: mol_type = other RNA; note = GPSZRA179 antisense strand
tgccagctaagagtccctgca

SEQ ID NO: 180 - RNA, 21 nt, synthetic construct
  source 1..21: mol_type = other RNA; note = GPSZRA180 antisense strand
gtgccagctaagagtccctgc

SEQ ID NO: 181 - RNA, 21 nt, synthetic construct
  source 1..21: mol_type = other RNA; note = GPSZRA181 antisense strand
agtgccagctaagagtccctg

SEQ ID NO: 182 - RNA, 21 nt, synthetic construct
  source 1..21: mol_type = other RNA; note = GPSZRA182 antisense strand
aagtgccagctaagagtccct

SEQ ID NO: 183 - RNA, 21 nt, synthetic construct
  source 1..21: mol_type = other RNA; note = GPSZRA183 antisense strand
caagtgccagctaagagtccc

SEQ ID NO: 184 - RNA, 21 nt, synthetic construct
  source 1..21: mol_type = other RNA; note = GPSZRA184 antisense strand
ccaagtgccagctaagagtcc

SEQ ID NO: 185 - RNA, 21 nt, synthetic construct
  source 1..21: mol_type = other RNA; note = GPSZRA185 antisense strand
tccaagtgccagctaagagtc

SEQ ID NO: 186 - RNA, 21 nt, synthetic construct
  source 1..21: mol_type = other RNA; note = GPSZRA186 antisense strand
atccaagtgccagctaagagt

SEQ ID NO: 187 - RNA, 21 nt, synthetic construct
  source 1..21: mol_type = other RNA; note = GPSZRA187 antisense strand
catccaagtgccagctaagag

SEQ ID NO: 188 - RNA, 21 nt, synthetic construct
  source 1..21: mol_type = other RNA; note = GPSZRA188 antisense strand
ccatccaagtgccagctaaga

SEQ ID NO: 189 - RNA, 21 nt, synthetic construct
  source 1..21: mol_type = other RNA; note = GPSZRA189 antisense strand
cccatccaagtgccagctaag

SEQ ID NO: 190 - RNA, 21 nt, synthetic construct
  source 1..21: mol_type = other RNA; note = GPSZRA190 antisense strand
tcccatccaagtgccagctaa

SEQ ID NO: 191 - RNA, 21 nt, synthetic construct
  source 1..21: mol_type = other RNA; note = GPSZRA191 antisense strand
ttcccatccaagtgccagcta

SEQ ID NO: 192 - RNA, 21 nt, synthetic construct
  source 1..21: mol_type = other RNA; note = GPSZRA192 antisense strand
cttcccatccaagtgccagct

SEQ ID NO: 193 - RNA, 21 nt, synthetic construct
  source 1..21: mol_type = other RNA; note = GPSZRA193 antisense strand
gcttcccatccaagtgccagc

SEQ ID NO: 194 - RNA, 21 nt, synthetic construct
  source 1..21: mol_type = other RNA; note = GPSZRA194 antisense strand
aggggcttcccatccaagtgc

SEQ ID NO: 195 - RNA, 21 nt, synthetic construct
  source 1..21: mol_type = other RNA; note = GPSZRA195 antisense strand
attaggcaccaggggcttccc

SEQ ID NO: 196 - RNA, 21 nt, synthetic construct
  source 1..21: mol_type = other RNA; note = GPSZRA196 antisense strand
cattaggcaccaggggcttcc

SEQ ID NO: 197 - RNA, 21 nt, synthetic construct
  source 1..21: mol_type = other RNA; note = GPSZRA197 antisense strand
tcattaggcaccaggggcttc

SEQ ID NO: 198 - RNA, 21 nt, synthetic construct
  source 1..21: mol_type = other RNA; note = GPSZRA198 antisense strand
tctcattaggcaccaggggct

SEQ ID NO: 199 - RNA, 21 nt, synthetic construct
  source 1..21: mol_type = other RNA; note = GPSZRA199 antisense strand
ttctcattaggcaccaggggc

SEQ ID NO: 200 - RNA, 21 nt, synthetic construct
  source 1..21: mol_type = other RNA; note = GPSZRA200 antisense strand
cttctcattaggcaccagggg

SEQ ID NO: 201 - RNA, 21 nt, synthetic construct
  source 1..21: mol_type = other RNA; note = GPSZRA201 antisense strand
ccttctcattaggcaccaggg

SEQ ID NO: 202 - RNA, 21 nt, synthetic construct
  source 1..21: mol_type = other RNA; note = GPSZRA202 antisense strand
cccttctcattaggcaccagg

SEQ ID NO: 203 - RNA, 21 nt, synthetic construct
  source 1..21: mol_type = other RNA; note = GPSZRA203 antisense strand
tcccttctcattaggcaccag

SEQ ID NO: 204 - RNA, 21 nt, synthetic construct
  source 1..21: mol_type = other RNA; note = GPSZRA204 antisense strand
ctcccttctcattaggcacca

SEQ ID NO: 205 - RNA, 21 nt, synthetic construct
  source 1..21: mol_type = other RNA; note = GPSZRA205 antisense strand
actcccttctcattaggcacc

SEQ ID NO: 206 - RNA, 21 nt, synthetic construct
  source 1..21: mol_type = other RNA; note = GPSZRA206 antisense strand
tactcccttctcattaggcac

SEQ ID NO: 207 - RNA, 21 nt, synthetic construct
  source 1..21: mol_type = other RNA; note = GPSZRA207 antisense strand
atactcccttctcattaggca

SEQ ID NO: 208 - RNA, 21 nt, synthetic construct
  source 1..21: mol_type = other RNA; note = GPSZRA208 antisense strand
gatactcccttctcattaggc

SEQ ID NO: 209 - RNA, 21 nt, synthetic construct
  source 1..21: mol_type = other RNA; note = GPSZRA209 antisense strand
agatactcccttctcattagg

SEQ ID NO: 210 - RNA, 21 nt, synthetic construct
  source 1..21: mol_type = other RNA; note = GPSZRA210 antisense strand
cagatactcccttctcattag

SEQ ID NO: 211 - RNA, 21 nt, synthetic construct
  source 1..21: mol_type = other RNA; note = GPSZRA211 antisense strand
acagatactcccttctcatta

SEQ ID NO: 212 - RNA, 21 nt, synthetic construct
  source 1..21: mol_type = other RNA; note = GPSZRA212 antisense strand
cacagatactcccttctcatt

SEQ ID NO: 213 - RNA, 21 nt, synthetic construct
  source 1..21: mol_type = other RNA; note = GPSZRA213 antisense strand
tcacagatactcccttctcat

SEQ ID NO: 214 - RNA, 21 nt, synthetic construct
  source 1..21: mol_type = other RNA; note = GPSZRA214 antisense strand
ttcacagatactcccttctca

SEQ ID NO: 215 - RNA, 21 nt, synthetic construct
  source 1..21: mol_type = other RNA; note = GPSZRA215 antisense strand
cttcacagatactcccttctc

SEQ ID NO: 216 - RNA, 21 nt, synthetic construct
  source 1..21: mol_type = other RNA; note = GPSZRA216 antisense strand
ccttcacagatactcccttct

SEQ ID NO: 217 - RNA, 21 nt, synthetic construct
  source 1..21: mol_type = other RNA; note = GPSZRA217 antisense strand
tccttcacagatactcccttc

SEQ ID NO: 218 - RNA, 21 nt, synthetic construct
  source 1..21: mol_type = other RNA; note = GPSZRA218 antisense strand
ttccttcacagatactccctt

SEQ ID NO: 219 - RNA, 21 nt, synthetic construct
  source 1..21: mol_type = other RNA; note = GPSZRA219 antisense strand
tctcagggtgtctcctggtct

SEQ ID NO: 220 - RNA, 21 nt, synthetic construct
  source 1..21: mol_type = other RNA; note = GPSZRA220 antisense strand
cgactgcagtgtgaagagccc

SEQ ID NO: 221 - RNA, 21 nt, synthetic construct
  source 1..21: mol_type = other RNA; note = GPSZRA221 antisense strand
ccgactgcagtgtgaagagcc

SEQ ID NO: 222 - RNA, 21 nt, synthetic construct
  source 1..21: mol_type = other RNA; note = GPSZRA222 antisense strand
tccgactgcagtgtgaagagc

SEQ ID NO: 223 - RNA, 21 nt, synthetic construct
  source 1..21: mol_type = other RNA; note = GPSZRA223 antisense strand
ctccgactgcagtgtgaagag

SEQ ID NO: 224 - RNA, 21 nt, synthetic construct
  source 1..21: mol_type = other RNA; note = GPSZRA224 antisense strand
gctccgactgcagtgtgaaga

SEQ ID NO: 225 - RNA, 21 nt, synthetic construct
  source 1..21: mol_type = other RNA; note = GPSZRA225 antisense strand
agctccgactgcagtgtgaag

SEQ ID NO: 226 - RNA, 21 nt, synthetic construct
  source 1..21: mol_type = other RNA; note = GPSZRA226 antisense strand
tagctccgactgcagtgtgaa

SEQ ID NO: 227 - RNA, 21 nt, synthetic construct
  source 1..21: mol_type = other RNA; note = GPSZRA227 antisense strand
ttagctccgactgcagtgtga

SEQ ID NO: 228 - RNA, 21 nt, synthetic construct
  source 1..21: mol_type = other RNA; note = GPSZRA228 antisense strand
attagctccgactgcagtgtg

SEQ ID NO: 229 - RNA, 21 nt, synthetic construct
  source 1..21: mol_type = other RNA; note = GPSZRA229 antisense strand
cattagctccgactgcagtgt

SEQ ID NO: 230 - RNA, 21 nt, synthetic construct
  source 1..21: mol_type = other RNA; note = GPSZRA230 antisense strand
ccattagctccgactgcagtg

SEQ ID NO: 231 - RNA, 21 nt, synthetic construct
  source 1..21: mol_type = other RNA; note = GPSZRA231 antisense strand
accattagctccgactgcagt

SEQ ID NO: 232 - RNA, 21 nt, synthetic construct
  source 1..21: mol_type = other RNA; note = GPSZRA232 antisense strand
caccattagctccgactgcag

SEQ ID NO: 233 - RNA, 21 nt, synthetic construct
  source 1..21: mol_type = other RNA; note = GPSZRA233 antisense strand
tcaccattagctccgactgca

SEQ ID NO: 234 - RNA, 21 nt, synthetic construct
  source 1..21: mol_type = other RNA; note = GPSZRA234 antisense strand
gtcaccattagctccgactgc

SEQ ID NO: 235 - RNA, 21 nt, synthetic construct
  source 1..21: mol_type = other RNA; note = GPSZRA235 antisense strand
ggtcaccattagctccgactg

SEQ ID NO: 236 - RNA, 21 nt, synthetic construct
  source 1..21: mol_type = other RNA; note = GPSZRA236 antisense strand
gggtcaccattagctccgact

SEQ ID NO: 237 - RNA, 21 nt, synthetic construct
  source 1..21: mol_type = other RNA; note = GPSZRA237 antisense strand
tggggtcaccattagctccga

SEQ ID NO: 238 - RNA, 21 nt, synthetic construct
  source 1..21: mol_type = other RNA; note = GPSZRA238 antisense strand
ctggggtcaccattagctccg

SEQ ID NO: 239 - RNA, 21 nt, synthetic construct
  source 1..21: mol_type = other RNA; note = GPSZRA239 antisense strand
gctggggtcaccattagctcc

SEQ ID NO: 240 - RNA, 21 nt, synthetic construct
  source 1..21: mol_type = other RNA; note = GPSZRA240 antisense strand
aagctacaggagaaggtggga

SEQ ID NO: 241 - RNA, 21 nt, synthetic construct
  source 1..21: mol_type = other RNA; note = GPSZRA241 antisense strand
gaagctacaggagaaggtggg

SEQ ID NO: 242 - RNA, 21 nt, synthetic construct
  source 1..21: mol_type = other RNA; note = GPSZRA242 antisense strand
tgaagctacaggagaaggtgg

SEQ ID NO: 243 - RNA, 21 nt, synthetic construct
  source 1..21: mol_type = other RNA; note = GPSZRA243 antisense strand
ctgaagctacaggagaaggtg

SEQ ID NO: 244 - RNA, 21 nt, synthetic construct
  source 1..21: mol_type = other RNA; note = GPSZRA244 antisense strand
gctgaagctacaggagaaggt

SEQ ID NO: 245 - RNA, 21 nt, synthetic construct
  source 1..21: mol_type = other RNA; note = GPSZRA245 antisense strand
ggctgaagctacaggagaagg

SEQ ID NO: 246 - RNA, 21 nt, synthetic construct
  source 1..21: mol_type = other RNA; note = GPSZRA246 antisense strand
gggctgaagctacaggagaag

SEQ ID NO: 247 - RNA, 21 nt, synthetic construct
  source 1..21: mol_type = other RNA; note = GPSZRA247 antisense strand
tgggctgaagctacaggagaa

SEQ ID NO: 248 - RNA, 21 nt, synthetic construct
  source 1..21: mol_type = other RNA; note = GPSZRA248 antisense strand
ctgggctgaagctacaggaga

SEQ ID NO: 249 - RNA, 21 nt, synthetic construct
  source 1..21: mol_type = other RNA; note = GPSZRA249 antisense strand
aaggcctgggctgaagctaca

SEQ ID NO: 250 - RNA, 21 nt, synthetic construct
  source 1..21: mol_type = other RNA; note = GPSZRA250 antisense strand
attggacctcctccagaggca

SEQ ID NO: 251 - RNA, 21 nt, synthetic construct
  source 1..21: mol_type = other RNA; note = GPSZRA251 antisense strand
aattggacctcctccagaggc

SEQ ID NO: 252 - RNA, 21 nt, synthetic construct
  source 1..21: mol_type = other RNA; note = GPSZRA252 antisense strand
caattggacctcctccagagg

SEQ ID NO: 253 - RNA, 21 nt, synthetic construct
  source 1..21: mol_type = other RNA; note = GPSZRA253 antisense strand
ccaattggacctcctccagag

SEQ ID NO: 254 - RNA, 21 nt, synthetic construct
  source 1..21: mol_type = other RNA; note = GPSZRA254 antisense strand
accaattggacctcctccaga

SEQ ID NO: 255 - RNA, 21 nt, synthetic construct
  source 1..21: mol_type = other RNA; note = GPSZRA255 antisense strand
caccaattggacctcctccag

SEQ ID NO: 256 - RNA, 21 nt, synthetic construct
  source 1..21: mol_type = other RNA; note = GPSZRA256 antisense strand
ccaccaattggacctcctcca

SEQ ID NO: 257 - RNA, 21 nt, synthetic construct
  source 1..21: mol_type = other RNA; note = GPSZRA257 antisense strand
accaccaattggacctcctcc

SEQ ID NO: 258 - RNA, 21 nt, synthetic construct
  source 1..21: mol_type = other RNA; note = GPSZRA258 antisense strand
tactgctccaccttctggctc

SEQ ID NO: 259 - RNA, 21 nt, synthetic construct
  source 1..21: mol_type = other RNA; note = GPSZRA259 antisense strand
ctactgctccaccttctggct

SEQ ID NO: 260 - RNA, 21 nt, synthetic construct
  source 1..21: mol_type = other RNA; note = GPSZRA260 antisense strand
gctactgctccaccttctggc

SEQ ID NO: 261 - RNA, 21 nt, synthetic construct
  source 1..21: mol_type = other RNA; note = GPSZRA261 antisense strand
agctactgctccaccttctgg

SEQ ID NO: 262 - RNA, 21 nt, synthetic construct
  source 1..21: mol_type = other RNA; note = GPSZRA262 antisense strand
gagctactgctccaccttctg

SEQ ID NO: 263 - RNA, 21 nt, synthetic construct
  source 1..21: mol_type = other RNA; note = GPSZRA263 antisense strand
ggagctactgctccaccttct

SEQ ID NO: 264 - RNA, 21 nt, synthetic construct
  source 1..21: mol_type = other RNA; note = GPSZRA264 antisense strand
aggagctactgctccaccttc

SEQ ID NO: 265 - RNA, 21 nt, synthetic construct
  source 1..21: mol_type = other RNA; note = GPSZRA265 antisense strand
accaggagctactgctccacc

SEQ ID NO: 266 - RNA, 21 nt, synthetic construct
  source 1..21: mol_type = other RNA; note = GPSZRA266 antisense strand
tccaccaggagctactgctcc

SEQ ID NO: 267 - RNA, 21 nt, synthetic construct
  source 1..21: mol_type = other RNA; note = GPSZRA267 antisense strand
ttccaccaggagctactgctc

SEQ ID NO: 268 - RNA, 21 nt, synthetic construct
  source 1..21: mol_type = other RNA; note = GPSZRA268 antisense strand
gttccaccaggagctactgct

SEQ ID NO: 269 - RNA, 21 nt, synthetic construct
  source 1..21: mol_type = other RNA; note = GPSZRA269 antisense strand
ggttccaccaggagctactgc

SEQ ID NO: 270 - RNA, 21 nt, synthetic construct
  source 1..21: mol_type = other RNA; note = GPSZRA270 antisense strand
acggttccaccaggagctact

SEQ ID NO: 271 - RNA, 21 nt, synthetic construct
  source 1..21: mol_type = other RNA; note = GPSZRA271 antisense strand
tacggttccaccaggagctac

SEQ ID NO: 272 - RNA, 21 nt, synthetic construct
  source 1..21: mol_type = other RNA; note = GPSZRA272 antisense strand
ttacggttccaccaggagcta

SEQ ID NO: 273 - RNA, 21 nt, synthetic construct
  source 1..21: mol_type = other RNA; note = GPSZRA273 antisense strand
gttacggttccaccaggagct

SEQ ID NO: 274 - RNA, 21 nt, synthetic construct
  source 1..21: mol_type = other RNA; note = GPSZRA274 antisense strand
ggttacggttccaccaggagc

SEQ ID NO: 275 - RNA, 21 nt, synthetic construct
  source 1..21: mol_type = other RNA; note = GPSZRA275 antisense strand
agggttacggttccaccagga

SEQ ID NO: 276 - RNA, 21 nt, synthetic construct
  source 1..21: mol_type = other RNA; note = GPSZRA276 antisense strand
cagggttacggttccaccagg

SEQ ID NO: 277 - RNA, 21 nt, synthetic construct
  source 1..21: mol_type = other RNA; note = GPSZRA277 antisense strand
tcagggttacggttccaccag

SEQ ID NO: 278 - RNA, 21 nt, synthetic construct
  source 1..21: mol_type = other RNA; note = GPSZRA278 antisense strand
gtcagggttacggttccacca

SEQ ID NO: 279 - RNA, 21 nt, synthetic construct
  source 1..21: mol_type = other RNA; note = GPSZRA279 antisense strand
ggtcagggttacggttccacc

SEQ ID NO: 280 - RNA, 21 nt, synthetic construct
  source 1..21: mol_type = other RNA; note = GPSZRA280 antisense strand
aggtcagggttacggttccac

SEQ ID NO: 281 - RNA, 21 nt, synthetic construct
  source 1..21: mol_type = other RNA; note = GPSZRA281 antisense strand
caggtcagggttacggttcca

SEQ ID NO: 282 - RNA, 21 nt, synthetic construct
  source 1..21: mol_type = other RNA; note = GPSZRA282 antisense strand
acaggtcagggttacggttcc

SEQ ID NO: 283 - RNA, 21 nt, synthetic construct
  source 1..21: mol_type = other RNA; note = GPSZRA283 antisense strand
cacaggtcagggttacggttc

SEQ ID NO: 284 - RNA, 21 nt, synthetic construct
  source 1..21: mol_type = other RNA; note = GPSZRA284 antisense strand
tcacaggtcagggttacggtt

SEQ ID NO: 285 - RNA, 21 nt, synthetic construct
  source 1..21: mol_type = other RNA; note = GPSZRA285 antisense strand
ttcacaggtcagggttacggt

SEQ ID NO: 286 - RNA, 21 nt, synthetic construct
  source 1..21: mol_type = other RNA; note = GPSZRA286 antisense strand
cttcacaggtcagggttacgg

SEQ ID NO: 287 - RNA, 21 nt, synthetic construct
  source 1..21: mol_type = other RNA; note = GPSZRA287 antisense strand
acttcacaggtcagggttacg

SEQ ID NO: 288 - RNA, 21 nt, synthetic construct
  source 1..21: mol_type = other RNA; note = GPSZRA288 antisense strand
gacttcacaggtcagggttac

SEQ ID NO: 289 - RNA, 21 nt, synthetic construct
  source 1..21: mol_type = other RNA; note = GPSZRA289 antisense strand
ggacttcacaggtcagggtta

SEQ ID NO: 290 - RNA, 21 nt, synthetic construct
  source 1..21: mol_type = other RNA; note = GPSZRA290 antisense strand
agggacttcacaggtcagggt

SEQ ID NO: 291 - RNA, 21 nt, synthetic construct
  source 1..21: mol_type = other RNA; note = GPSZRA291 antisense strand
cagggacttcacaggtcaggg

SEQ ID NO: 292 - RNA, 21 nt, synthetic construct
  source 1..21: mol_type = other RNA; note = GPSZRA292 antisense strand
gcagggacttcacaggtcagg

SEQ ID NO: 293 - RNA, 21 nt, synthetic construct
  source 1..21: mol_type = other RNA; note = GPSZRA293 antisense strand
atttgaggagagggctgggca

SEQ ID NO: 294 - RNA, 21 nt, synthetic construct
  source 1..21: mol_type = other RNA; note = GPSZRA294 antisense strand
gatttgaggagagggctgggc

SEQ ID NO: 295 - RNA, 21 nt, synthetic construct
  source 1..21: mol_type = other RNA; note = GPSZRA295 antisense strand
ggatttgaggagagggctggg

SEQ ID NO: 296 - RNA, 21 nt, synthetic construct
  source 1..21: mol_type = other RNA; note = GPSZRA296 antisense strand
tggatttgaggagagggctgg

SEQ ID NO: 297 - RNA, 21 nt, synthetic construct
  source 1..21: mol_type = other RNA; note = GPSZRA297 antisense strand
gtggatttgaggagagggctg

SEQ ID NO: 298 - RNA, 21 nt, synthetic construct
  source 1..21: mol_type = other RNA; note = GPSZRA298 antisense strand
agtggatttgaggagagggct

SEQ ID NO: 299 - RNA, 21 nt, synthetic construct
  source 1..21: mol_type = other RNA; note = GPSZRA299 antisense strand
cagtggatttgaggagagggc

SEQ ID NO: 300 - RNA, 21 nt, synthetic construct
  source 1..21: mol_type = other RNA; note = GPSZRA300 antisense strand
ccagtggatttgaggagaggg

SEQ ID NO: 301 - RNA, 21 nt, synthetic construct
  source 1..21: mol_type = other RNA; note = GPSZRA301 antisense strand
tccagtggatttgaggagagg

SEQ ID NO: 302 - RNA, 21 nt, synthetic construct
  source 1..21: mol_type = other RNA; note = GPSZRA302 antisense strand
atccagtggatttgaggagag

SEQ ID NO: 303 - RNA, 21 nt, synthetic construct
  source 1..21: mol_type = other RNA; note = GPSZRA303 antisense strand
catccagtggatttgaggaga

SEQ ID NO: 304 - RNA, 21 nt, synthetic construct
  source 1..21: mol_type = other RNA; note = GPSZRA304 antisense strand
tcatccagtggatttgaggag

SEQ ID NO: 305 - RNA, 21 nt, synthetic construct
  source 1..21: mol_type = other RNA; note = GPSZRA305 antisense strand
ttcatccagtggatttgagga

SEQ ID NO: 306 - RNA, 21 nt, synthetic construct
  source 1..21: mol_type = other RNA; note = GPSZRA306 antisense strand
cttcatccagtggatttgagg

SEQ ID NO: 307 - RNA, 21 nt, synthetic construct
  source 1..21: mol_type = other RNA; note = GPSZRA307 antisense strand
ccttcatccagtggatttgag

SEQ ID NO: 308 - RNA, 21 nt, synthetic construct
  source 1..21: mol_type = other RNA; note = GPSZRA308 antisense strand
tccttcatccagtggatttga

SEQ ID NO: 309 - RNA, 21 nt, synthetic construct
  source 1..21: mol_type = other RNA; note = GPSZRA309 antisense strand
atccttcatccagtggatttg

SEQ ID NO: 310 - RNA, 21 nt, synthetic construct
  source 1..21: mol_type = other RNA; note = GPSZRA310 antisense strand
catccttcatccagtggattt

SEQ ID NO: 311 - RNA, 21 nt, synthetic construct
  source 1..21: mol_type = other RNA; note = GPSZRA311 antisense strand
ccatccttcatccagtggatt

SEQ ID NO: 312 - RNA, 21 nt, synthetic construct
  source 1..21: mol_type = other RNA; note = GPSZRA312 antisense strand
accatccttcatccagtggat

SEQ ID NO: 313 - RNA, 21 nt, synthetic construct
  source 1..21: mol_type = other RNA; note = GPSZRA313 antisense strand
caccatccttcatccagtgga

SEQ ID NO: 314 - RNA, 21 nt, synthetic construct
  source 1..21: mol_type = other RNA; note = GPSZRA314 antisense strand
acaccatccttcatccagtgg

SEQ ID NO: 315 - RNA, 21 nt, synthetic construct
  source 1..21: mol_type = other RNA; note = GPSZRA315 antisense strand
cacaccatccttcatccagtg

SEQ ID NO: 316 - RNA, 21 nt, synthetic construct
  source 1..21: mol_type = other RNA; note = GPSZRA316 antisense strand
gcacaccatccttcatccagt

SEQ ID NO: 317 - RNA, 21 nt, synthetic construct
  source 1..21: mol_type = other RNA; note = GPSZRA317 antisense strand
ggcacaccatccttcatccag

SEQ ID NO: 318 - RNA, 21 nt, synthetic construct
  source 1..21: mol_type = other RNA; note = GPSZRA318 antisense strand
gggcacaccatccttcatcca

SEQ ID NO: 319 - RNA, 21 nt, synthetic construct
  source 1..21: mol_type = other RNA; note = GPSZRA319 antisense strand
agggcacaccatccttcatcc

SEQ ID NO: 320 - RNA, 21 nt, synthetic construct
  source 1..21: mol_type = other RNA; note = GPSZRA320 antisense strand
aagggcacaccatccttcatc

SEQ ID NO: 321 - RNA, 21 nt, synthetic construct
  source 1..21: mol_type = other RNA; note = GPSZRA321 antisense strand
tcagggaggatcagcacaggg

SEQ ID NO: 322 - RNA, 21 nt, synthetic construct
  source 1..21: mol_type = other RNA; note = GPSZRA322 antisense strand
ctcagggaggatcagcacagg

SEQ ID NO: 323 - RNA, 21 nt, synthetic construct
  source 1..21: mol_type = other RNA; note = GPSZRA323 antisense strand
tctcagggaggatcagcacag

SEQ ID NO: 324 - RNA, 21 nt, synthetic construct
  source 1..21: mol_type = other RNA; note = GPSZRA324 antisense strand
atctcagggaggatcagcaca

SEQ ID NO: 325 - RNA, 21 nt, synthetic construct
  source 1..21: mol_type = other RNA; note = GPSZRA325 antisense strand
tatctcagggaggatcagcac

SEQ ID NO: 326 - RNA, 21 nt, synthetic construct
  source 1..21: mol_type = other RNA; note = GPSZRA326 antisense strand
ctatctcagggaggatcagca

SEQ ID NO: 327 - RNA, 21 nt, synthetic construct
  source 1..21: mol_type = other RNA; note = GPSZRA327 antisense strand
cctatctcagggaggatcagc

SEQ ID NO: 328 - RNA, 21 nt, synthetic construct
  source 1..21: mol_type = other RNA; note = GPSZRA328 antisense strand
ccctatctcagggaggatcag

SEQ ID NO: 329 - RNA, 21 nt, synthetic construct
  source 1..21: mol_type = other RNA; note = GPSZRA329 antisense strand
gccctatctcagggaggatca

SEQ ID NO: 330 - RNA, 21 nt, synthetic construct
  source 1..21: mol_type = other RNA; note = GPSZRA330 antisense strand
ctgtaggttccctggtcctga

SEQ ID NO: 331 - RNA, 21 nt, synthetic construct
  source 1..21: mol_type = other RNA; note = GPSZRA331 antisense strand
tgacagcacggctttcctggg

SEQ ID NO: 332 - RNA, 21 nt, synthetic construct
  source 1..21: mol_type = other RNA; note = GPSZRA332 antisense strand
ctgacagcacggctttcctgg

SEQ ID NO: 333 - RNA, 21 nt, synthetic construct
  source 1..21: mol_type = other RNA; note = GPSZRA333 antisense strand
tgctgacagcacggctttcct

SEQ ID NO: 334 - RNA, 21 nt, synthetic construct
  source 1..21: mol_type = other RNA; note = GPSZRA334 antisense strand
atgctgacagcacggctttcc

SEQ ID NO: 335 - RNA, 21 nt, synthetic construct
  source 1..21: mol_type = other RNA; note = GPSZRA335 antisense strand
gatgctgacagcacggctttc

SEQ ID NO: 336 - RNA, 21 nt, synthetic construct
  source 1..21: mol_type = other RNA; note = GPSZRA336 antisense strand
tgatgctgacagcacggcttt

SEQ ID NO: 337 - RNA, 21 nt, synthetic construct
  source 1..21: mol_type = other RNA; note = GPSZRA337 antisense strand
tgctgatgctgacagcacggc

SEQ ID NO: 338 - RNA, 21 nt, synthetic construct
  source 1..21: mol_type = other RNA; note = GPSZRA338 antisense strand
atgctgatgctgacagcacgg

SEQ ID NO: 339 - RNA, 21 nt, synthetic construct
  source 1..21: mol_type = other RNA; note = GPSZRA339 antisense strand
gatgctgatgctgacagcacg

SEQ ID NO: 340 - RNA, 21 nt, synthetic construct
  source 1..21: mol_type = other RNA; note = GPSZRA340 antisense strand
tgatgctgatgctgacagcac

SEQ ID NO: 341 - RNA, 21 nt, synthetic construct
  source 1..21: mol_type = other RNA; note = GPSZRA341 antisense strand
atgatgctgatgctgacagca

SEQ ID NO: 342 - RNA, 21 nt, synthetic construct
  source 1..21: mol_type = other RNA; note = GPSZRA342 antisense strand
gatgatgctgatgctgacagc

SEQ ID NO: 343 - RNA, 21 nt, synthetic construct
  source 1..21: mol_type = other RNA; note = GPSZRA343 antisense strand
cgatgatgctgatgctgacag

SEQ ID NO: 344 - RNA, 21 nt, synthetic construct
  source 1..21: mol_type = other RNA; note = GPSZRA344 antisense strand
tcgatgatgctgatgctgaca

SEQ ID NO: 345 - RNA, 21 nt, synthetic construct
  source 1..21: mol_type = other RNA; note = GPSZRA345 antisense strand
ttcgatgatgctgatgctgac

SEQ ID NO: 346 - RNA, 21 nt, synthetic construct
  source 1..21: mol_type = other RNA; note = GPSZRA346 antisense strand
gttcgatgatgctgatgctga

SEQ ID NO: 347 - RNA, 21 nt, synthetic construct
  source 1..21: mol_type = other RNA; note = GPSZRA347 antisense strand
ggttcgatgatgctgatgctg

SEQ ID NO: 348 - RNA, 21 nt, synthetic construct
  source 1..21: mol_type = other RNA; note = GPSZRA348 antisense strand
tggttcgatgatgctgatgct

SEQ ID NO: 349 - RNA, 21 nt, synthetic construct
  source 1..21: mol_type = other RNA; note = GPSZRA349 antisense strand
ctggttcgatgatgctgatgc

SEQ ID NO: 350 - RNA, 21 nt, synthetic construct
  source 1..21: mol_type = other RNA; note = GPSZRA350 antisense strand
cctggttcgatgatgctgatg

SEQ ID NO: 351 - RNA, 21 nt, synthetic construct
  source 1..21: mol_type = other RNA; note = GPSZRA351 antisense strand
gcctggttcgatgatgctgat

SEQ ID NO: 352 - RNA, 21 nt, synthetic construct
  source 1..21: mol_type = other RNA; note = GPSZRA352 antisense strand
cgcctggttcgatgatgctga

SEQ ID NO: 353 - RNA, 21 nt, synthetic construct
  source 1..21: mol_type = other RNA; note = GPSZRA353 antisense strand
tcgcctggttcgatgatgctg

SEQ ID NO: 354 - RNA, 21 nt, synthetic construct
  source 1..21: mol_type = other RNA; note = GPSZRA354 antisense strand
ctcgcctggttcgatgatgct

SEQ ID NO: 355 - RNA, 21 nt, synthetic construct
  source 1..21: mol_type = other RNA; note = GPSZRA355 antisense strand
cctcgcctggttcgatgatgc

SEQ ID NO: 356 - RNA, 21 nt, synthetic construct
  source 1..21: mol_type = other RNA; note = GPSZRA356 antisense strand
tcctcgcctggttcgatgatg

SEQ ID NO: 357 - RNA, 21 nt, synthetic construct
  source 1..21: mol_type = other RNA; note = GPSZRA357 antisense strand
tcccacagagcctgcagttgg

SEQ ID NO: 358 - RNA, 21 nt, synthetic construct
  source 1..21: mol_type = other RNA; note = GPSZRA358 antisense strand
tgatcctcccacagagcctgc

SEQ ID NO: 359 - RNA, 21 nt, synthetic construct
  source 1..21: mol_type = other RNA; note = GPSZRA359 antisense strand
caagatgaccccaatgagcag

SEQ ID NO: 360 - RNA, 21 nt, synthetic construct
  source 1..21: mol_type = other RNA; note = GPSZRA360 antisense strand
acaagatgaccccaatgagca

SEQ ID NO: 361 - RNA, 21 nt, synthetic construct
  source 1..21: mol_type = other RNA; note = GPSZRA361 antisense strand
cacaagatgaccccaatgagc

SEQ ID NO: 362 - RNA, 21 nt, synthetic construct
  source 1..21: mol_type = other RNA; note = GPSZRA362 antisense strand
ccacaagatgaccccaatgag

SEQ ID NO: 363 - RNA, 21 nt, synthetic construct
  source 1..21: mol_type = other RNA; note = GPSZRA363 antisense strand
gccacaagatgaccccaatga

SEQ ID NO: 364 - RNA, 21 nt, synthetic construct
  source 1..21: mol_type = other RNA; note = GPSZRA364 antisense strand
tgccacaagatgaccccaatg

SEQ ID NO: 365 - RNA, 21 nt, synthetic construct
  source 1..21: mol_type = other RNA; note = GPSZRA365 antisense strand
ttgccacaagatgaccccaat

SEQ ID NO: 366 - RNA, 21 nt, synthetic construct
  source 1..21: mol_type = other RNA; note = GPSZRA366 antisense strand
tttgccacaagatgaccccaa

SEQ ID NO: 367 - RNA, 21 nt, synthetic construct
  source 1..21: mol_type = other RNA; note = GPSZRA367 antisense strand
ctttgccacaagatgacccca

SEQ ID NO: 368 - RNA, 21 nt, synthetic construct
  source 1..21: mol_type = other RNA; note = GPSZRA368 antisense strand
cctttgccacaagatgacccc

SEQ ID NO: 369 - RNA, 21 nt, synthetic construct
  source 1..21: mol_type = other RNA; note = GPSZRA369 antisense strand
gcctttgccacaagatgaccc

SEQ ID NO: 370 - RNA, 21 nt, synthetic construct
  source 1..21: mol_type = other RNA; note = GPSZRA370 antisense strand
cgcctttgccacaagatgacc

SEQ ID NO: 371 - RNA, 21 nt, synthetic construct
  source 1..21: mol_type = other RNA; note = GPSZRA371 antisense strand
ccgcctttgccacaagatgac

SEQ ID NO: 372 - RNA, 21 nt, synthetic construct
  source 1..21: mol_type = other RNA; note = GPSZRA372 antisense strand
gccgcctttgccacaagatga

SEQ ID NO: 373 - RNA, 21 nt, synthetic construct
  source 1..21: mol_type = other RNA; note = GPSZRA373 antisense strand
cctcttcctcctggttttctg

SEQ ID NO: 374 - RNA, 21 nt, synthetic construct
  source 1..21: mol_type = other RNA; note = GPSZRA374 antisense strand
tcctcttcctcctggttttct

SEQ ID NO: 375 - RNA, 21 nt, synthetic construct
  source 1..21: mol_type = other RNA; note = GPSZRA375 antisense strand
ctcctcttcctcctggttttc

SEQ ID NO: 376 - RNA, 21 nt, synthetic construct
  source 1..21: mol_type = other RNA; note = GPSZRA376 antisense strand
cctcctcttcctcctggtttt

SEQ ID NO: 377 - RNA, 21 nt, synthetic construct
  source 1..21: mol_type = other RNA; note = GPSZRA377 antisense strand
tcctcctcttcctcctggttt

SEQ ID NO: 378 - RNA, 21 nt, synthetic construct
  source 1..21: mol_type = other RNA; note = GPSZRA378 antisense strand
tctgcacgctcctcctcttcc

SEQ ID NO: 379 - RNA, 21 nt, synthetic construct
  source 1..21: mol_type = other RNA; note = GPSZRA379 antisense strand
aggttcctccgactgattcag

SEQ ID NO: 380 - RNA, 21 nt, synthetic construct
  source 1..21: mol_type = other RNA; note = GPSZRA380 antisense strand
caggttcctccgactgattca

SEQ ID NO: 381 - RNA, 21 nt, synthetic construct
  source 1..21: mol_type = other RNA; note = GPSZRA381 antisense strand
tcaggttcctccgactgattc

SEQ ID NO: 382 - RNA, 21 nt, synthetic construct
  source 1..21: mol_type = other RNA; note = GPSZRA382 antisense strand
ctcaggttcctccgactgatt

SEQ ID NO: 383 - RNA, 21 nt, synthetic construct
  source 1..21: mol_type = other RNA; note = GPSZRA383 antisense strand
gggaaaaagaaaagggagctg

SEQ ID NO: 384 - RNA, 21 nt, synthetic construct
  source 1..21: mol_type = other RNA; note = GPSZRA384 antisense strand
agggaaaaagaaaagggagct

SEQ ID NO: 385 - RNA, 21 nt, synthetic construct
  source 1..21: mol_type = other RNA; note = GPSZRA385 antisense strand
aagggaaaaagaaaagggagc

SEQ ID NO: 386 - RNA, 21 nt, synthetic construct
  source 1..21: mol_type = other RNA; note = GPSZRA386 antisense strand
caagggaaaaagaaaagggag

SEQ ID NO: 387 - RNA, 21 nt, synthetic construct
  source 1..21: mol_type = other RNA; note = GPSZRA387 antisense strand
tcaagggaaaaagaaaaggga

SEQ ID NO: 388 - RNA, 21 nt, synthetic construct
  source 1..21: mol_type = other RNA; note = GPSZRA388 antisense strand
ttcaagggaaaaagaaaaggg

SEQ ID NO: 389 - RNA, 21 nt, synthetic construct
  source 1..21: mol_type = other RNA; note = GPSZRA389 antisense strand
gttcaagggaaaaagaaaagg

SEQ ID NO: 390 - RNA, 21 nt, synthetic construct
  source 1..21: mol_type = other RNA; note = GPSZRA390 antisense strand
agttcaagggaaaaagaaaag

SEQ ID NO: 391 - RNA, 21 nt, synthetic construct
  source 1..21: mol_type = other RNA; note = GPSZRA391 antisense strand
cagttcaagggaaaaagaaaa

SEQ ID NO: 392 - RNA, 21 nt, synthetic construct
  source 1..21: mol_type = other RNA; note = GPSZRA392 antisense strand
acagttcaagggaaaaagaaa

SEQ ID NO: 393 - RNA, 21 nt, synthetic construct
  source 1..21: mol_type = other RNA; note = GPSZRA393 antisense strand
aacagttcaagggaaaaagaa

SEQ ID NO: 394 - RNA, 21 nt, synthetic construct
  source 1..21: mol_type = other RNA; note = GPSZRA394 antisense strand
gaacagttcaagggaaaaaga

SEQ ID NO: 395 - RNA, 21 nt, synthetic construct
  source 1..21: mol_type = other RNA; note = GPSZRA395 antisense strand
agaacagttcaagggaaaaag

SEQ ID NO: 396 - RNA, 21 nt, synthetic construct
  source 1..21: mol_type = other RNA; note = GPSZRA396 antisense strand
cagaacagttcaagggaaaaa

SEQ ID NO: 397 - RNA, 21 nt, synthetic construct
  source 1..21: mol_type = other RNA; note = GPSZRA397 antisense strand
ccagaacagttcaagggaaaa

SEQ ID NO: 398 - RNA, 21 nt, synthetic construct
  source 1..21: mol_type = other RNA; note = GPSZRA398 antisense strand
gccagaacagttcaagggaaa

SEQ ID NO: 399 - RNA, 21 nt, synthetic construct
  source 1..21: mol_type = other RNA; note = GPSZRA399 antisense strand
ggccagaacagttcaagggaa

SEQ ID NO: 400 - RNA, 21 nt, synthetic construct
  source 1..21: mol_type = other RNA; note = GPSZRA400 antisense strand
atacaggagagagttggtctg

SEQ ID NO: 401 - RNA, 21 nt, synthetic construct
  source 1..21: mol_type = other RNA; note = GPSZRA401 antisense strand
tatacaggagagagttggtct

SEQ ID NO: 402 - RNA, 21 nt, synthetic construct
  source 1..21: mol_type = other RNA; note = GPSZRA402 antisense strand
ttatacaggagagagttggtc

SEQ ID NO: 403 - RNA, 21 nt, synthetic construct
  source 1..21: mol_type = other RNA; note = GPSZRA403 antisense strand
gtggggttatacaggagagag

SEQ ID NO: 404 - RNA, 21 nt, synthetic construct
  source 1..21: mol_type = other RNA; note = GPSZRA404 antisense strand
ggtggggttatacaggagaga

SEQ ID NO: 405 - RNA, 21 nt, synthetic construct
  source 1..21: mol_type = other RNA; note = GPSZRA405 antisense strand
aggtggggttatacaggagag

SEQ ID NO: 406 - RNA, 21 nt, synthetic construct
  source 1..21: mol_type = other RNA; note = GPSZRA406 antisense strand
aaggtggggttatacaggaga

SEQ ID NO: 407 - RNA, 21 nt, synthetic construct
  source 1..21: mol_type = other RNA; note = GPSZRA407 antisense strand
caaggtggggttatacaggag

SEQ ID NO: 408 - RNA, 21 nt, synthetic construct
  source 1..21: mol_type = other RNA; note = GPSZRA408 antisense strand
gcaaggtggggttatacagga

SEQ ID NO: 409 - RNA, 21 nt, synthetic construct
  source 1..21: mol_type = other RNA; note = GPSZRA409 antisense strand
ggcaaggtggggttatacagg

SEQ ID NO: 410 - RNA, 21 nt, synthetic construct
  source 1..21: mol_type = other RNA; note = GPSZRA410 antisense strand
tggcaaggtggggttatacag

SEQ ID NO: 411 - RNA, 21 nt, synthetic construct
  source 1..21: mol_type = other RNA; note = GPSZRA411 antisense strand
ttggcaaggtggggttataca

SEQ ID NO: 412 - RNA, 21 nt, synthetic construct
  source 1..21: mol_type = other RNA; note = GPSZRA412 antisense strand
ggctctggttgtagaagaaag

SEQ ID NO: 413 - RNA, 21 nt, synthetic construct
  source 1..21: mol_type = other RNA; note = GPSZRA413 antisense strand
gggctctggttgtagaagaaa

SEQ ID NO: 414 - RNA, 21 nt, synthetic construct
  source 1..21: mol_type = other RNA; note = GPSZRA414 antisense strand
ggggctctggttgtagaagaa

SEQ ID NO: 415 - RNA, 21 nt, synthetic construct
  source 1..21: mol_type = other RNA; note = GPSZRA415 antisense strand
gggggctctggttgtagaaga

SEQ ID NO: 416 - RNA, 21 nt, synthetic construct
  source 1..21: mol_type = other RNA; note = GPSZRA416 antisense strand
attgtggggggctctggttgt

SEQ ID NO: 417 - RNA, 21 nt, synthetic construct
  source 1..21: mol_type = other RNA; note = GPSZRA417 antisense strand
atcattgtggggggctctggt

SEQ ID NO: 418 - RNA, 21 nt, synthetic construct
  source 1..21: mol_type = other RNA; note = GPSZRA418 antisense strand
catcattgtggggggctctgg

SEQ ID NO: 419 - RNA, 21 nt, synthetic construct
  source 1..21: mol_type = other RNA; note = GPSZRA419 antisense strand
tcatcattgtggggggctctg

SEQ ID NO: 420 - RNA, 19 nt, synthetic construct
  source 1..19: mol_type = other RNA; note = GPSZRA001 sense strand
tggaaggaagcaggatggc

SEQ ID NO: 421 - RNA, 19 nt, synthetic construct
  source 1..19: mol_type = other RNA; note = GPSZRA002 sense strand
gtgctggtcctcagtctgt

SEQ ID NO: 422 - RNA, 19 nt, synthetic construct
  source 1..19: mol_type = other RNA; note = GPSZRA003 sense strand
tgctggtcctcagtctgtg

SEQ ID NO: 423 - RNA, 19 nt, synthetic construct
  source 1..19: mol_type = other RNA; note = GPSZRA004 sense strand
agtagtaggtgctcaaaac

SEQ ID NO: 424 - RNA, 19 nt, synthetic construct
  source 1..19: mol_type = other RNA; note = GPSZRA005 sense strand
gtagtaggtgctcaaaaca

SEQ ID NO: 425 - RNA, 19 nt, synthetic construct
  source 1..19: mol_type = other RNA; note = GPSZRA006 sense strand
tagtaggtgctcaaaacat

SEQ ID NO: 426 - RNA, 19 nt, synthetic construct
  source 1..19: mol_type = other RNA; note = GPSZRA007 sense strand
agtaggtgctcaaaacatc

SEQ ID NO: 427 - RNA, 19 nt, synthetic construct
  source 1..19: mol_type = other RNA; note = GPSZRA008 sense strand
gtaggtgctcaaaacatca

SEQ ID NO: 428 - RNA, 19 nt, synthetic construct
  source 1..19: mol_type = other RNA; note = GPSZRA009 sense strand
taggtgctcaaaacatcac

SEQ ID NO: 429 - RNA, 19 nt, synthetic construct
  source 1..19: mol_type = other RNA; note = GPSZRA010 sense strand
aggtgctcaaaacatcaca

SEQ ID NO: 430 - RNA, 19 nt, synthetic construct
  source 1..19: mol_type = other RNA; note = GPSZRA011 sense strand
ggtgctcaaaacatcacag

SEQ ID NO: 431 - RNA, 19 nt, synthetic construct
  source 1..19: mol_type = other RNA; note = GPSZRA012 sense strand
gtgctcaaaacatcacagc

SEQ ID NO: 432 - RNA, 19 nt, synthetic construct
  source 1..19: mol_type = other RNA; note = GPSZRA013 sense strand
tgctcaaaacatcacagcc

SEQ ID NO: 433 - RNA, 19 nt, synthetic construct
  source 1..19: mol_type = other RNA; note = GPSZRA014 sense strand
gctcaaaacatcacagccc

SEQ ID NO: 434 - RNA, 19 nt, synthetic construct
  source 1..19: mol_type = other RNA; note = GPSZRA015 sense strand
ctcaaaacatcacagcccg

SEQ ID NO: 435 - RNA, 19 nt, synthetic construct
  source 1..19: mol_type = other RNA; note = GPSZRA016 sense strand
tcaaaacatcacagcccgg

SEQ ID NO: 436 - RNA, 19 nt, synthetic construct
  source 1..19: mol_type = other RNA; note = GPSZRA017 sense strand
caaaacatcacagcccgga

SEQ ID NO: 437 - RNA, 19 nt, synthetic construct
  source 1..19: mol_type = other RNA; note = GPSZRA018 sense strand
aaaacatcacagcccggat

SEQ ID NO: 438 - RNA, 19 nt, synthetic construct
  source 1..19: mol_type = other RNA; note = GPSZRA019 sense strand
gccactggtgctgaagtgt

SEQ ID NO: 439 - RNA, 19 nt, synthetic construct
  source 1..19: mol_type = other RNA; note = GPSZRA020 sense strand
ccactggtgctgaagtgta

SEQ ID NO: 440 - RNA, 19 nt, synthetic construct
  source 1..19: mol_type = other RNA; note = GPSZRA021 sense strand
cactggtgctgaagtgtaa

SEQ ID NO: 441 - RNA, 19 nt, synthetic construct
  source 1..19: mol_type = other RNA; note = GPSZRA022 sense strand
actggtgctgaagtgtaag

SEQ ID NO: 442 - RNA, 19 nt, synthetic construct
  source 1..19: mol_type = other RNA; note = GPSZRA023 sense strand
ctggtgctgaagtgtaagg

SEQ ID NO: 443 - RNA, 19 nt, synthetic construct
  source 1..19: mol_type = other RNA; note = GPSZRA024 sense strand
tggtgctgaagtgtaaggg

SEQ ID NO: 444 - RNA, 19 nt, synthetic construct
  source 1..19: mol_type = other RNA; note = GPSZRA025 sense strand
ggtgctgaagtgtaagggg

SEQ ID NO: 445 - RNA, 19 nt, synthetic construct
  source 1..19: mol_type = other RNA; note = GPSZRA026 sense strand
gtgctgaagtgtaaggggg

SEQ ID NO: 446 - RNA, 19 nt, synthetic construct
  source 1..19: mol_type = other RNA; note = GPSZRA027 sense strand
tgctgaagtgtaagggggc

SEQ ID NO: 447 - RNA, 19 nt, synthetic construct
  source 1..19: mol_type = other RNA; note = GPSZRA028 sense strand
taagggggcccccaagaaa

SEQ ID NO: 448 - RNA, 19 nt, synthetic construct
  source 1..19: mol_type = other RNA; note = GPSZRA029 sense strand
gccggacagaagcttggaa

SEQ ID NO: 449 - RNA, 19 nt, synthetic construct
  source 1..19: mol_type = other RNA; note = GPSZRA030 sense strand
ccggacagaagcttggaag

SEQ ID NO: 450 - RNA, 19 nt, synthetic construct
  source 1..19: mol_type = other RNA; note = GPSZRA031 sense strand
cggacagaagcttggaagg

SEQ ID NO: 451 - RNA, 19 nt, synthetic construct
  source 1..19: mol_type = other RNA; note = GPSZRA032 sense strand
ggacagaagcttggaaggt

SEQ ID NO: 452 - RNA, 19 nt, synthetic construct
  source 1..19: mol_type = other RNA; note = GPSZRA033 sense strand
gacagaagcttggaaggtc

SEQ ID NO: 453 - RNA, 19 nt, synthetic construct
  source 1..19: mol_type = other RNA; note = GPSZRA034 sense strand
acagaagcttggaaggtcc

SEQ ID NO: 454 - RNA, 19 nt, synthetic construct
  source 1..19: mol_type = other RNA; note = GPSZRA035 sense strand
cagaagcttggaaggtcct

SEQ ID NO: 455 - RNA, 19 nt, synthetic construct
  source 1..19: mol_type = other RNA; note = GPSZRA036 sense strand
tggctcgtgtccttcccaa

SEQ ID NO: 456 - RNA, 19 nt, synthetic construct
  source 1..19: mol_type = other RNA; note = GPSZRA037 sense strand
ttcccaacggctccctctt

SEQ ID NO: 457 - RNA, 19 nt, synthetic construct
  source 1..19: mol_type = other RNA; note = GPSZRA038 sense strand
caacggctccctcttcctt

SEQ ID NO: 458 - RNA, 19 nt, synthetic construct
  source 1..19: mol_type = other RNA; note = GPSZRA039 sense strand
aacggctccctcttccttc

SEQ ID NO: 459 - RNA, 19 nt, synthetic construct
  source 1..19: mol_type = other RNA; note = GPSZRA040 sense strand
ctgtcgggatccaggatga

SEQ ID NO: 460 - RNA, 19 nt, synthetic construct
  source 1..19: mol_type = other RNA; note = GPSZRA041 sense strand
tgtcgggatccaggatgag

SEQ ID NO: 461 - RNA, 19 nt, synthetic construct
  source 1..19: mol_type = other RNA; note = GPSZRA042 sense strand
ggatccaggatgaggggat

SEQ ID NO: 462 - RNA, 19 nt, synthetic construct
  source 1..19: mol_type = other RNA; note = GPSZRA043 sense strand
gatccaggatgaggggatt

SEQ ID NO: 463 - RNA, 19 nt, synthetic construct
  source 1..19: mol_type = other RNA; note = GPSZRA044 sense strand
atccaggatgaggggattt

SEQ ID NO: 464 - RNA, 19 nt, synthetic construct
  source 1..19: mol_type = other RNA; note = GPSZRA045 sense strand
tccaggatgaggggatttt

SEQ ID NO: 465 - RNA, 19 nt, synthetic construct
  source 1..19: mol_type = other RNA; note = GPSZRA046 sense strand
ccaggatgaggggattttc

SEQ ID NO: 466 - RNA, 19 nt, synthetic construct
  source 1..19: mol_type = other RNA; note = GPSZRA047 sense strand
caggatgaggggattttcc

SEQ ID NO: 467 - RNA, 19 nt, synthetic construct
  source 1..19: mol_type = other RNA; note = GPSZRA048 sense strand
aggatgaggggattttccg

SEQ ID NO: 468 - RNA, 19 nt, synthetic construct
  source 1..19: mol_type = other RNA; note = GPSZRA049 sense strand
ggatgaggggattttccgg

SEQ ID NO: 469 - RNA, 19 nt, synthetic construct
  source 1..19: mol_type = other RNA; note = GPSZRA050 sense strand
gatgaggggattttccggt

SEQ ID NO: 470 - RNA, 19 nt, synthetic construct
  source 1..19: mol_type = other RNA; note = GPSZRA051 sense strand
atgaggggattttccggtg

SEQ ID NO: 471 - RNA, 19 nt, synthetic construct
  source 1..19: mol_type = other RNA; note = GPSZRA052 sense strand
tgaggggattttccggtgc

SEQ ID NO: 472 - RNA, 19 nt, synthetic construct
  source 1..19: mol_type = other RNA; note = GPSZRA053 sense strand
aggggattttccggtgcca

SEQ ID NO: 473 - RNA, 19 nt, synthetic construct
  source 1..19: mol_type = other RNA; note = GPSZRA054 sense strand
gattttccggtgccaggca

SEQ ID NO: 474 - RNA, 19 nt, synthetic construct
  source 1..19: mol_type = other RNA; note = GPSZRA055 sense strand
attttccggtgccaggcaa

SEQ ID NO: 475 - RNA, 19 nt, synthetic construct
  source 1..19: mol_type = other RNA; note = GPSZRA056 sense strand
ttttccggtgccaggcaat

SEQ ID NO: 476 - RNA, 19 nt, synthetic construct
  source 1..19: mol_type = other RNA; note = GPSZRA057 sense strand
tttccggtgccaggcaatg

SEQ ID NO: 477 - RNA, 19 nt, synthetic construct
  source 1..19: mol_type = other RNA; note = GPSZRA058 sense strand
ttccggtgccaggcaatga

SEQ ID NO: 478 - RNA, 19 nt, synthetic construct
  source 1..19: mol_type = other RNA; note = GPSZRA059 sense strand
tccggtgccaggcaatgaa

SEQ ID NO: 479 - RNA, 19 nt, synthetic construct
  source 1..19: mol_type = other RNA; note = GPSZRA060 sense strand
cggtgccaggcaatgaaca

SEQ ID NO: 480 - RNA, 19 nt, synthetic construct
  source 1..19: mol_type = other RNA; note = GPSZRA061 sense strand
ggtgccaggcaatgaacag

SEQ ID NO: 481 - RNA, 19 nt, synthetic construct
  source 1..19: mol_type = other RNA; note = GPSZRA062 sense strand
gtgccaggcaatgaacagg

SEQ ID NO: 482 - RNA, 19 nt, synthetic construct
  source 1..19: mol_type = other RNA; note = GPSZRA063 sense strand
tgccaggcaatgaacagga

SEQ ID NO: 483 - RNA, 19 nt, synthetic construct
  source 1..19: mol_type = other RNA; note = GPSZRA064 sense strand
gccaggcaatgaacaggaa

SEQ ID NO: 484 - RNA, 19 nt, synthetic construct
  source 1..19: mol_type = other RNA; note = GPSZRA065 sense strand
ccaggcaatgaacaggaat

SEQ ID NO: 485 - RNA, 19 nt, synthetic construct
  source 1..19: mol_type = other RNA; note = GPSZRA066 sense strand
caggcaatgaacaggaatg

SEQ ID NO: 486 - RNA, 19 nt, synthetic construct
  source 1..19: mol_type = other RNA; note = GPSZRA067 sense strand
aggcaatgaacaggaatgg

SEQ ID NO: 487 - RNA, 19 nt, synthetic construct
  source 1..19: mol_type = other RNA; note = GPSZRA068 sense strand
ggcaatgaacaggaatgga

SEQ ID NO: 488 - RNA, 19 nt, synthetic construct
  source 1..19: mol_type = other RNA; note = GPSZRA069 sense strand
gcaatgaacaggaatggaa

SEQ ID NO: 489 - RNA, 19 nt, synthetic construct
  source 1..19: mol_type = other RNA; note = GPSZRA070 sense strand
caatgaacaggaatggaaa

SEQ ID NO: 490 - RNA, 19 nt, synthetic construct
  source 1..19: mol_type = other RNA; note = GPSZRA071 sense strand
aatgaacaggaatggaaag

SEQ ID NO: 491 - RNA, 19 nt, synthetic construct
  source 1..19: mol_type = other RNA; note = GPSZRA072 sense strand
atgaacaggaatggaaagg

SEQ ID NO: 492 - RNA, 19 nt, synthetic construct
  source 1..19: mol_type = other RNA; note = GPSZRA073 sense strand
tgaacaggaatggaaagga

SEQ ID NO: 493 - RNA, 19 nt, synthetic construct
  source 1..19: mol_type = other RNA; note = GPSZRA074 sense strand
gaacaggaatggaaaggag

SEQ ID NO: 494 - RNA, 19 nt, synthetic construct
  source 1..19: mol_type = other RNA; note = GPSZRA075 sense strand
aacaggaatggaaaggaga

SEQ ID NO: 495 - RNA, 19 nt, synthetic construct
  source 1..19: mol_type = other RNA; note = GPSZRA076 sense strand
acaggaatggaaaggagac

SEQ ID NO: 496 - RNA, 19 nt, synthetic construct
  source 1..19: mol_type = other RNA; note = GPSZRA077 sense strand
caggaatggaaaggagacc

SEQ ID NO: 497 - RNA, 19 nt, synthetic construct
  source 1..19: mol_type = other RNA; note = GPSZRA078 sense strand
aggaatggaaaggagacca

SEQ ID NO: 498 - RNA, 19 nt, synthetic construct
  source 1..19: mol_type = other RNA; note = GPSZRA079 sense strand
ggaatggaaaggagaccaa

SEQ ID NO: 499 - RNA, 19 nt, synthetic construct
  source 1..19: mol_type = other RNA; note = GPSZRA080 sense strand
gaatggaaaggagaccaag

SEQ ID NO: 500 - RNA, 19 nt, synthetic construct
  source 1..19: mol_type = other RNA; note = GPSZRA081 sense strand
aatggaaaggagaccaagt

SEQ ID NO: 501 - RNA, 19 nt, synthetic construct
  source 1..19: mol_type = other RNA; note = GPSZRA082 sense strand
atggaaaggagaccaagtc

SEQ ID NO: 502 - RNA, 19 nt, synthetic construct
  source 1..19: mol_type = other RNA; note = GPSZRA083 sense strand
tggaaaggagaccaagtcc

SEQ ID NO: 503 - RNA, 19 nt, synthetic construct
  source 1..19: mol_type = other RNA; note = GPSZRA084 sense strand
ggaaaggagaccaagtcca

SEQ ID NO: 504 - RNA, 19 nt, synthetic construct
  source 1..19: mol_type = other RNA; note = GPSZRA085 sense strand
gaaaggagaccaagtccaa

SEQ ID NO: 505 - RNA, 19 nt, synthetic construct
  source 1..19: mol_type = other RNA; note = GPSZRA086 sense strand
aaaggagaccaagtccaac

SEQ ID NO: 506 - RNA, 19 nt, synthetic construct
  source 1..19: mol_type = other RNA; note = GPSZRA087 sense strand
aaggagaccaagtccaact

SEQ ID NO: 507 - RNA, 19 nt, synthetic construct
  source 1..19: mol_type = other RNA; note = GPSZRA088 sense strand
aggagaccaagtccaacta

SEQ ID NO: 508 - RNA, 19 nt, synthetic construct
  source 1..19: mol_type = other RNA; note = GPSZRA089 sense strand
ggagaccaagtccaactac

SEQ ID NO: 509 - RNA, 19 nt, synthetic construct
  source 1..19: mol_type = other RNA; note = GPSZRA090 sense strand
gagaccaagtccaactacc

SEQ ID NO: 510 - RNA, 19 nt, synthetic construct
  source 1..19: mol_type = other RNA; note = GPSZRA091 sense strand
agaccaagtccaactaccg

SEQ ID NO: 511 - RNA, 19 nt, synthetic construct
  source 1..19: mol_type = other RNA; note = GPSZRA092 sense strand
gaccaagtccaactaccga

SEQ ID NO: 512 - RNA, 19 nt, synthetic construct
  source 1..19: mol_type = other RNA; note = GPSZRA093 sense strand
accaagtccaactaccgag

SEQ ID NO: 513 - RNA, 19 nt, synthetic construct
  source 1..19: mol_type = other RNA; note = GPSZRA094 sense strand
ccaagtccaactaccgagt

SEQ ID NO: 514 - RNA, 19 nt, synthetic construct
  source 1..19: mol_type = other RNA; note = GPSZRA095 sense strand
caagtccaactaccgagtc

SEQ ID NO: 515 - RNA, 19 nt, synthetic construct
  source 1..19: mol_type = other RNA; note = GPSZRA096 sense strand
aagtccaactaccgagtcc

SEQ ID NO: 516 - RNA, 19 nt, synthetic construct
  source 1..19: mol_type = other RNA; note = GPSZRA097 sense strand
agtccaactaccgagtccg

SEQ ID NO: 517 - RNA, 19 nt, synthetic construct
  source 1..19: mol_type = other RNA; note = GPSZRA098 sense strand
gtccaactaccgagtccgt

SEQ ID NO: 518 - RNA, 19 nt, synthetic construct
  source 1..19: mol_type = other RNA; note = GPSZRA099 sense strand
tccaactaccgagtccgtg

SEQ ID NO: 519 - RNA, 19 nt, synthetic construct
  source 1..19: mol_type = other RNA; note = GPSZRA100 sense strand
ccaactaccgagtccgtgt

SEQ ID NO: 520 - RNA, 19 nt, synthetic construct
  source 1..19: mol_type = other RNA; note = GPSZRA101 sense strand
caactaccgagtccgtgtc

SEQ ID NO: 521 - RNA, 19 nt, synthetic construct
  source 1..19: mol_type = other RNA; note = GPSZRA102 sense strand
aactaccgagtccgtgtct

SEQ ID NO: 522 - RNA, 19 nt, synthetic construct
  source 1..19: mol_type = other RNA; note = GPSZRA103 sense strand
actaccgagtccgtgtcta

SEQ ID NO: 523 - RNA, 19 nt, synthetic construct
  source 1..19: mol_type = other RNA; note = GPSZRA104 sense strand
ctaccgagtccgtgtctac

SEQ ID NO: 524 - RNA, 19 nt, synthetic construct
  source 1..19: mol_type = other RNA; note = GPSZRA105 sense strand
taccgagtccgtgtctacc

SEQ ID NO: 525 - RNA, 19 nt, synthetic construct
  source 1..19: mol_type = other RNA; note = GPSZRA106 sense strand
accgagtccgtgtctacca

SEQ ID NO: 526 - RNA, 19 nt, synthetic construct
  source 1..19: mol_type = other RNA; note = GPSZRA107 sense strand
cgagtccgtgtctaccaga

SEQ ID NO: 527 - RNA, 19 nt, synthetic construct
  source 1..19: mol_type = other RNA; note = GPSZRA108 sense strand
gagtccgtgtctaccagat

SEQ ID NO: 528 - RNA, 19 nt, synthetic construct
  source 1..19: mol_type = other RNA; note = GPSZRA109 sense strand
agtccgtgtctaccagatt

SEQ ID NO: 529 - RNA, 19 nt, synthetic construct
  source 1..19: mol_type = other RNA; note = GPSZRA110 sense strand
gtccgtgtctaccagattc

SEQ ID NO: 530 - RNA, 19 nt, synthetic construct
  source 1..19: mol_type = other RNA; note = GPSZRA111 sense strand
tccgtgtctaccagattcc

SEQ ID NO: 531 - RNA, 19 nt, synthetic construct
  source 1..19: mol_type = other RNA; note = GPSZRA112 sense strand
ccgtgtctaccagattcct

SEQ ID NO: 532 - RNA, 19 nt, synthetic construct
  source 1..19: mol_type = other RNA; note = GPSZRA113 sense strand
cgtgtctaccagattcctg

SEQ ID NO: 533 - RNA, 19 nt, synthetic construct
  source 1..19: mol_type = other RNA; note = GPSZRA114 sense strand
gtgtctaccagattcctgg

SEQ ID NO: 534 - RNA, 19 nt, synthetic construct
  source 1..19: mol_type = other RNA; note = GPSZRA115 sense strand
tgtctaccagattcctggg

SEQ ID NO: 535 - RNA, 19 nt, synthetic construct
  source 1..19: mol_type = other RNA; note = GPSZRA116 sense strand
gtctaccagattcctggga

SEQ ID NO: 536 - RNA, 19 nt, synthetic construct
  source 1..19: mol_type = other RNA; note = GPSZRA117 sense strand
tctaccagattcctgggaa

SEQ ID NO: 537 - RNA, 19 nt, synthetic construct
  source 1..19: mol_type = other RNA; note = GPSZRA118 sense strand
ctaccagattcctgggaag

SEQ ID NO: 538 - RNA, 19 nt, synthetic construct
  source 1..19: mol_type = other RNA; note = GPSZRA119 sense strand
taccagattcctgggaagc

SEQ ID NO: 539 - RNA, 19 nt, synthetic construct
  source 1..19: mol_type = other RNA; note = GPSZRA120 sense strand
accagattcctgggaagcc

SEQ ID NO: 540 - RNA, 19 nt, synthetic construct
  source 1..19: mol_type = other RNA; note = GPSZRA121 sense strand
gattctgcctctgaactca

SEQ ID NO: 541 - RNA, 19 nt, synthetic construct
  source 1..19: mol_type = other RNA; note = GPSZRA122 sense strand
attctgcctctgaactcac

SEQ ID NO: 542 - RNA, 19 nt, synthetic construct
  source 1..19: mol_type = other RNA; note = GPSZRA123 sense strand
ttctgcctctgaactcacg

SEQ ID NO: 543 - RNA, 19 nt, synthetic construct
  source 1..19: mol_type = other RNA; note = GPSZRA124 sense strand
tctgcctctgaactcacgg

SEQ ID NO: 544 - RNA, 19 nt, synthetic construct
  source 1..19: mol_type = other RNA; note = GPSZRA125 sense strand
tgcctctgaactcacggct

SEQ ID NO: 545 - RNA, 19 nt, synthetic construct
  source 1..19: mol_type = other RNA; note = GPSZRA126 sense strand
ctctgaactcacggctggt

SEQ ID NO: 546 - RNA, 19 nt, synthetic construct
  source 1..19: mol_type = other RNA; note = GPSZRA127 sense strand
tctgaactcacggctggtg

SEQ ID NO: 547 - RNA, 19 nt, synthetic construct
  source 1..19: mol_type = other RNA; note = GPSZRA128 sense strand
ctgaactcacggctggtgt

SEQ ID NO: 548 - RNA, 19 nt, synthetic construct
  source 1..19: mol_type = other RNA; note = GPSZRA129 sense strand
tgaactcacggctggtgtt

SEQ ID NO: 549 - RNA, 19 nt, synthetic construct
  source 1..19: mol_type = other RNA; note = GPSZRA130 sense strand
gaactcacggctggtgttc

SEQ ID NO: 550 - RNA, 19 nt, synthetic construct
  source 1..19: mol_type = other RNA; note = GPSZRA131 sense strand
aactcacggctggtgttcc

SEQ ID NO: 551 - RNA, 19 nt, synthetic construct
  source 1..19: mol_type = other RNA; note = GPSZRA132 sense strand
tcacggctggtgttcccaa

SEQ ID NO: 552 - RNA, 19 nt, synthetic construct
  source 1..19: mol_type = other RNA; note = GPSZRA133 sense strand
cacggctggtgttcccaat

SEQ ID NO: 553 - RNA, 19 nt, synthetic construct
  source 1..19: mol_type = other RNA; note = GPSZRA134 sense strand
acggctggtgttcccaata

SEQ ID NO: 554 - RNA, 19 nt, synthetic construct
  source 1..19: mol_type = other RNA; note = GPSZRA135 sense strand
cggctggtgttcccaataa

SEQ ID NO: 555 - RNA, 19 nt, synthetic construct
  source 1..19: mol_type = other RNA; note = GPSZRA136 sense strand
ggctggtgttcccaataag

SEQ ID NO: 556 - RNA, 19 nt, synthetic construct
  source 1..19: mol_type = other RNA; note = GPSZRA137 sense strand
gctggtgttcccaataagg

SEQ ID NO: 557 - RNA, 19 nt, synthetic construct
  source 1..19: mol_type = other RNA; note = GPSZRA138 sense strand
ctggtgttcccaataaggt

SEQ ID NO: 558 - RNA, 19 nt, synthetic construct
  source 1..19: mol_type = other RNA; note = GPSZRA139 sense strand
tggtgttcccaataaggtg

SEQ ID NO: 559 - RNA, 19 nt, synthetic construct
  source 1..19: mol_type = other RNA; note = GPSZRA140 sense strand
ggtgttcccaataaggtgg

SEQ ID NO: 560 - RNA, 19 nt, synthetic construct
  source 1..19: mol_type = other RNA; note = GPSZRA141 sense strand
gtgttcccaataaggtggg

SEQ ID NO: 561 - RNA, 19 nt, synthetic construct
  source 1..19: mol_type = other RNA; note = GPSZRA142 sense strand
tgttcccaataaggtgggg

SEQ ID NO: 562 - RNA, 19 nt, synthetic construct
  source 1..19: mol_type = other RNA; note = GPSZRA143 sense strand
gttcccaataaggtgggga

SEQ ID NO: 563 - RNA, 19 nt, synthetic construct
  source 1..19: mol_type = other RNA; note = GPSZRA144 sense strand
ttcccaataaggtggggac

SEQ ID NO: 564 - RNA, 19 nt, synthetic construct
  source 1..19: mol_type = other RNA; note = GPSZRA145 sense strand
tcccaataaggtggggaca

SEQ ID NO: 565 - RNA, 19 nt, synthetic construct
  source 1..19: mol_type = other RNA; note = GPSZRA146 sense strand
cccaataaggtggggacat

SEQ ID NO: 566 - RNA, 19 nt, synthetic construct
  source 1..19: mol_type = other RNA; note = GPSZRA147 sense strand
ccaataaggtggggacatg

SEQ ID NO: 567 - RNA, 19 nt, synthetic construct
  source 1..19: mol_type = other RNA; note = GPSZRA148 sense strand
caataaggtggggacatgt

SEQ ID NO: 568 - RNA, 19 nt, synthetic construct
  source 1..19: mol_type = other RNA; note = GPSZRA149 sense strand
aataaggtggggacatgtg

SEQ ID NO: 569 - RNA, 19 nt, synthetic construct
  source 1..19: mol_type = other RNA; note = GPSZRA150 sense strand
ataaggtggggacatgtgt

SEQ ID NO: 570 - RNA, 19 nt, synthetic construct
  source 1..19: mol_type = other RNA; note = GPSZRA151 sense strand
taaggtggggacatgtgtg

SEQ ID NO: 571 - RNA, 19 nt, synthetic construct
  source 1..19: mol_type = other RNA; note = GPSZRA152 sense strand
aaggtggggacatgtgtgt

SEQ ID NO: 572 - RNA, 19 nt, synthetic construct
  source 1..19: mol_type = other RNA; note = GPSZRA153 sense strand
aggtggggacatgtgtgtc

SEQ ID NO: 573 - RNA, 19 nt, synthetic construct
  source 1..19: mol_type = other RNA; note = GPSZRA154 sense strand
ggtggggacatgtgtgtca

SEQ ID NO: 574 - RNA, 19 nt, synthetic construct
  source 1..19: mol_type = other RNA; note = GPSZRA155 sense strand
gtggggacatgtgtgtcag

SEQ ID NO: 575 - RNA, 19 nt, synthetic construct
  source 1..19: mol_type = other RNA; note = GPSZRA156 sense strand
tggggacatgtgtgtcaga

SEQ ID NO: 576 - RNA, 19 nt, synthetic construct
  source 1..19: mol_type = other RNA; note = GPSZRA157 sense strand
ggggacatgtgtgtcagag

SEQ ID NO: 577 - RNA, 19 nt, synthetic construct
  source 1..19: mol_type = other RNA; note = GPSZRA158 sense strand
gggacatgtgtgtcagagg

SEQ ID NO: 578 - RNA, 19 nt, synthetic construct
  source 1..19: mol_type = other RNA; note = GPSZRA159 sense strand
ggacatgtgtgtcagaggg

SEQ ID NO: 579 - RNA, 19 nt, synthetic construct
  source 1..19: mol_type = other RNA; note = GPSZRA160 sense strand
gacatgtgtgtcagaggga

SEQ ID NO: 580 - RNA, 19 nt, synthetic construct
  source 1..19: mol_type = other RNA; note = GPSZRA161 sense strand
acatgtgtgtcagagggaa

SEQ ID NO: 581 - RNA, 19 nt, synthetic construct
  source 1..19: mol_type = other RNA; note = GPSZRA162 sense strand
catgtgtgtcagagggaag

SEQ ID NO: 582 - RNA, 19 nt, synthetic construct
  source 1..19: mol_type = other RNA; note = GPSZRA163 sense strand
atgtgtgtcagagggaagc

SEQ ID NO: 583 - RNA, 19 nt, synthetic construct
  source 1..19: mol_type = other RNA; note = GPSZRA164 sense strand
tgtgtgtcagagggaagct

SEQ ID NO: 584 - RNA, 19 nt, synthetic construct
  source 1..19: mol_type = other RNA; note = GPSZRA165 sense strand
gtgtgtcagagggaagcta

SEQ ID NO: 585 - RNA, 19 nt, synthetic construct
  source 1..19: mol_type = other RNA; note = GPSZRA166 sense strand
tgtgtcagagggaagctac

SEQ ID NO: 586 - RNA, 19 nt, synthetic construct
  source 1..19: mol_type = other RNA; note = GPSZRA167 sense strand
gtgtcagagggaagctacc

SEQ ID NO: 587 - RNA, 19 nt, synthetic construct
  source 1..19: mol_type = other RNA; note = GPSZRA168 sense strand
tgtcagagggaagctaccc

SEQ ID NO: 588 - RNA, 19 nt, synthetic construct
  source 1..19: mol_type = other RNA; note = GPSZRA169 sense strand
gtcagagggaagctaccct

SEQ ID NO: 589 - RNA, 19 nt, synthetic construct
  source 1..19: mol_type = other RNA; note = GPSZRA170 sense strand
tcagagggaagctaccctg

SEQ ID NO: 590 - RNA, 19 nt, synthetic construct
  source 1..19: mol_type = other RNA; note = GPSZRA171 sense strand
agagggaagctaccctgca

SEQ ID NO: 591 - RNA, 19 nt, synthetic construct
  source 1..19: mol_type = other RNA; note = GPSZRA172 sense strand
aagctaccctgcagggact

SEQ ID NO: 592 - RNA, 19 nt, synthetic construct
  source 1..19: mol_type = other RNA; note = GPSZRA173 sense strand
ctaccctgcagggactctt

SEQ ID NO: 593 - RNA, 19 nt, synthetic construct
  source 1..19: mol_type = other RNA; note = GPSZRA174 sense strand
taccctgcagggactctta

SEQ ID NO: 594 - RNA, 19 nt, synthetic construct
  source 1..19: mol_type = other RNA; note = GPSZRA175 sense strand
accctgcagggactcttag

SEQ ID NO: 595 - RNA, 19 nt, synthetic construct
  source 1..19: mol_type = other RNA; note = GPSZRA176 sense strand
cctgcagggactcttagct

SEQ ID NO: 596 - RNA, 19 nt, synthetic construct
  source 1..19: mol_type = other RNA; note = GPSZRA177 sense strand
ctgcagggactcttagctg

SEQ ID NO: 597 - RNA, 19 nt, synthetic construct
  source 1..19: mol_type = other RNA; note = GPSZRA178 sense strand
tgcagggactcttagctgg

SEQ ID NO: 598 - RNA, 19 nt, synthetic construct
  source 1..19: mol_type = other RNA; note = GPSZRA179 sense strand
cagggactcttagctggca

SEQ ID NO: 599 - RNA, 19 nt, synthetic construct
  source 1..19: mol_type = other RNA; note = GPSZRA180 sense strand
agggactcttagctggcac

SEQ ID NO: 600 - RNA, 19 nt, synthetic construct
  source 1..19: mol_type = other RNA; note = GPSZRA181 sense strand
gggactcttagctggcact

SEQ ID NO: 601 - RNA, 19 nt, synthetic construct
  source 1..19: mol_type = other RNA; note = GPSZRA182 sense strand
ggactcttagctggcactt

SEQ ID NO: 602 - RNA, 19 nt, synthetic construct
  source 1..19: mol_type = other RNA; note = GPSZRA183 sense strand
gactcttagctggcacttg

SEQ ID NO: 603 - RNA, 19 nt, synthetic construct
  source 1..19: mol_type = other RNA; note = GPSZRA184 sense strand
actcttagctggcacttgg

SEQ ID NO: 604 - RNA, 19 nt, synthetic construct
  source 1..19: mol_type = other RNA; note = GPSZRA185 sense strand
ctcttagctggcacttgga

SEQ ID NO: 605 - RNA, 19 nt, synthetic construct
  source 1..19: mol_type = other RNA; note = GPSZRA186 sense strand
tcttagctggcacttggat

SEQ ID NO: 606 - RNA, 19 nt, synthetic construct
  source 1..19: mol_type = other RNA; note = GPSZRA187 sense strand
cttagctggcacttggatg

SEQ ID NO: 607 - RNA, 19 nt, synthetic construct
  source 1..19: mol_type = other RNA; note = GPSZRA188 sense strand
ttagctggcacttggatgg

SEQ ID NO: 608 - RNA, 19 nt, synthetic construct
  source 1..19: mol_type = other RNA; note = GPSZRA189 sense strand
tagctggcacttggatggg

SEQ ID NO: 609 - RNA, 19 nt, synthetic construct
  source 1..19: mol_type = other RNA; note = GPSZRA190 sense strand
agctggcacttggatggga

SEQ ID NO: 610 - RNA, 19 nt, synthetic construct
  source 1..19: mol_type = other RNA; note = GPSZRA191 sense strand
gctggcacttggatgggaa

SEQ ID NO: 611 - RNA, 19 nt, synthetic construct
  source 1..19: mol_type = other RNA; note = GPSZRA192 sense strand
ctggcacttggatgggaag

SEQ ID NO: 612 - RNA, 19 nt, synthetic construct
  source 1..19: mol_type = other RNA; note = GPSZRA193 sense strand
tggcacttggatgggaagc

SEQ ID NO: 613 - RNA, 19 nt, synthetic construct
  source 1..19: mol_type = other RNA; note = GPSZRA194 sense strand
acttggatgggaagcccct

SEQ ID NO: 614 - RNA, 19 nt, synthetic construct
  source 1..19: mol_type = other RNA; note = GPSZRA195 sense strand
gaagcccctggtgcctaat

SEQ ID NO: 615 - RNA, 19 nt, synthetic construct
  source 1..19: mol_type = other RNA; note = GPSZRA196 sense strand
aagcccctggtgcctaatg

SEQ ID NO: 616 - RNA, 19 nt, synthetic construct
  source 1..19: mol_type = other RNA; note = GPSZRA197 sense strand
agcccctggtgcctaatga

SEQ ID NO: 617 - RNA, 19 nt, synthetic construct
  source 1..19: mol_type = other RNA; note = GPSZRA198 sense strand
cccctggtgcctaatgaga

SEQ ID NO: 618 - RNA, 19 nt, synthetic construct
  source 1..19: mol_type = other RNA; note = GPSZRA199 sense strand
ccctggtgcctaatgagaa

SEQ ID NO: 619 - RNA, 19 nt, synthetic construct
  source 1..19: mol_type = other RNA; note = GPSZRA200 sense strand
cctggtgcctaatgagaag

SEQ ID NO: 620 - RNA, 19 nt, synthetic construct
  source 1..19: mol_type = other RNA; note = GPSZRA201 sense strand
ctggtgcctaatgagaagg

SEQ ID NO: 621 - RNA, 19 nt, synthetic construct
  source 1..19: mol_type = other RNA; note = GPSZRA202 sense strand
tggtgcctaatgagaaggg

SEQ ID NO: 622 - RNA, 19 nt, synthetic construct
  source 1..19: mol_type = other RNA; note = GPSZRA203 sense strand
ggtgcctaatgagaaggga

SEQ ID NO: 623 - RNA, 19 nt, synthetic construct
  source 1..19: mol_type = other RNA; note = GPSZRA204 sense strand
gtgcctaatgagaagggag

SEQ ID NO: 624 - RNA, 19 nt, synthetic construct
  source 1..19: mol_type = other RNA; note = GPSZRA205 sense strand
tgcctaatgagaagggagt

SEQ ID NO: 625 - RNA, 19 nt, synthetic construct
  source 1..19: mol_type = other RNA; note = GPSZRA206 sense strand
gcctaatgagaagggagta

SEQ ID NO: 626 - RNA, 19 nt, synthetic construct
  source 1..19: mol_type = other RNA; note = GPSZRA207 sense strand
cctaatgagaagggagtat

SEQ ID NO: 627 - RNA, 19 nt, synthetic construct
  source 1..19: mol_type = other RNA; note = GPSZRA208 sense strand
ctaatgagaagggagtatc

SEQ ID NO: 628 - RNA, 19 nt, synthetic construct
  source 1..19: mol_type = other RNA; note = GPSZRA209 sense strand
taatgagaagggagtatct

SEQ ID NO: 629 - RNA, 19 nt, synthetic construct
  source 1..19: mol_type = other RNA; note = GPSZRA210 sense strand
aatgagaagggagtatctg

SEQ ID NO: 630 - RNA, 19 nt, synthetic construct
  source 1..19: mol_type = other RNA; note = GPSZRA211 sense strand
atgagaagggagtatctgt

SEQ ID NO: 631 - RNA, 19 nt, synthetic construct
  source 1..19: mol_type = other RNA; note = GPSZRA212 sense strand
tgagaagggagtatctgtg

SEQ ID NO: 632 - RNA, 19 nt, synthetic construct
  source 1..19: mol_type = other RNA; note = GPSZRA213 sense strand
gagaagggagtatctgtga

SEQ ID NO: 633 - RNA, 19 nt, synthetic construct
  source 1..19: mol_type = other RNA; note = GPSZRA214 sense strand
agaagggagtatctgtgaa

SEQ ID NO: 634 - RNA, 19 nt, synthetic construct
  source 1..19: mol_type = other RNA; note = GPSZRA215 sense strand
gaagggagtatctgtgaag

SEQ ID NO: 635 - RNA, 19 nt, synthetic construct
  source 1..19: mol_type = other RNA; note = GPSZRA216 sense strand
aagggagtatctgtgaagg

SEQ ID NO: 636 - RNA, 19 nt, synthetic construct
  source 1..19: mol_type = other RNA; note = GPSZRA217 sense strand
agggagtatctgtgaagga

SEQ ID NO: 637 - RNA, 19 nt, synthetic construct
  source 1..19: mol_type = other RNA; note = GPSZRA218 sense strand
gggagtatctgtgaaggaa

SEQ ID NO: 638 - RNA, 19 nt, synthetic construct
  source 1..19: mol_type = other RNA; note = GPSZRA219 sense strand
accaggagacaccctgaga

SEQ ID NO: 639 - RNA, 19 nt, synthetic construct
  source 1..19: mol_type = other RNA; note = GPSZRA220 sense strand
gctcttcacactgcagtcg

SEQ ID NO: 640 - RNA, 19 nt, synthetic construct
  source 1..19: mol_type = other RNA; note = GPSZRA221 sense strand
ctcttcacactgcagtcgg

SEQ ID NO: 641 - RNA, 19 nt, synthetic construct
  source 1..19: mol_type = other RNA; note = GPSZRA222 sense strand
tcttcacactgcagtcgga

SEQ ID NO: 642 - RNA, 19 nt, synthetic construct
  source 1..19: mol_type = other RNA; note = GPSZRA223 sense strand
cttcacactgcagtcggag

SEQ ID NO: 643 - RNA, 19 nt, synthetic construct
  source 1..19: mol_type = other RNA; note = GPSZRA224 sense strand
ttcacactgcagtcggagc

SEQ ID NO: 644 - RNA, 19 nt, synthetic construct
  source 1..19: mol_type = other RNA; note = GPSZRA225 sense strand
tcacactgcagtcggagct

SEQ ID NO: 645 - RNA, 19 nt, synthetic construct
  source 1..19: mol_type = other RNA; note = GPSZRA226 sense strand
cacactgcagtcggagcta

SEQ ID NO: 646 - RNA, 19 nt, synthetic construct
  source 1..19: mol_type = other RNA; note = GPSZRA227 sense strand
acactgcagtcggagctaa

SEQ ID NO: 647 - RNA, 19 nt, synthetic construct
  source 1..19: mol_type = other RNA; note = GPSZRA228 sense strand
cactgcagtcggagctaat

SEQ ID NO: 648 - RNA, 19 nt, synthetic construct
  source 1..19: mol_type = other RNA; note = GPSZRA229 sense strand
actgcagtcggagctaatg

SEQ ID NO: 649 - RNA, 19 nt, synthetic construct
  source 1..19: mol_type = other RNA; note = GPSZRA230 sense strand
ctgcagtcggagctaatgg

SEQ ID NO: 650 - RNA, 19 nt, synthetic construct
  source 1..19: mol_type = other RNA; note = GPSZRA231 sense strand
tgcagtcggagctaatggt

SEQ ID NO: 651 - RNA, 19 nt, synthetic construct
  source 1..19: mol_type = other RNA; note = GPSZRA232 sense strand
gcagtcggagctaatggtg

SEQ ID NO: 652 - RNA, 19 nt, synthetic construct
  source 1..19: mol_type = other RNA; note = GPSZRA233 sense strand
cagtcggagctaatggtga

SEQ ID NO: 653 - RNA, 19 nt, synthetic construct
  source 1..19: mol_type = other RNA; note = GPSZRA234 sense strand
agtcggagctaatggtgac

SEQ ID NO: 654 - RNA, 19 nt, synthetic construct
  source 1..19: mol_type = other RNA; note = GPSZRA235 sense strand
gtcggagctaatggtgacc

SEQ ID NO: 655 - RNA, 19 nt, synthetic construct
  source 1..19: mol_type = other RNA; note = GPSZRA236 sense strand
tcggagctaatggtgaccc

SEQ ID NO: 656 - RNA, 19 nt, synthetic construct
  source 1..19: mol_type = other RNA; note = GPSZRA237 sense strand
ggagctaatggtgacccca

SEQ ID NO: 657 - RNA, 19 nt, synthetic construct
  source 1..19: mol_type = other RNA; note = GPSZRA238 sense strand
gagctaatggtgaccccag

SEQ ID NO: 658 - RNA, 19 nt, synthetic construct
  source 1..19: mol_type = other RNA; note = GPSZRA239 sense strand
agctaatggtgaccccagc

SEQ ID NO: 659 - RNA, 19 nt, synthetic construct
  source 1..19: mol_type = other RNA; note = GPSZRA240 sense strand
ccaccttctcctgtagctt

SEQ ID NO: 660 - RNA, 19 nt, synthetic construct
  source 1..19: mol_type = other RNA; note = GPSZRA241 sense strand
caccttctcctgtagcttc

SEQ ID NO: 661 - RNA, 19 nt, synthetic construct
  source 1..19: mol_type = other RNA; note = GPSZRA242 sense strand
accttctcctgtagcttca

SEQ ID NO: 662 - RNA, 19 nt, synthetic construct
  source 1..19: mol_type = other RNA; note = GPSZRA243 sense strand
ccttctcctgtagcttcag

SEQ ID NO: 663 - RNA, 19 nt, synthetic construct
  source 1..19: mol_type = other RNA; note = GPSZRA244 sense strand
cttctcctgtagcttcagc

SEQ ID NO: 664 - RNA, 19 nt, synthetic construct
  source 1..19: mol_type = other RNA; note = GPSZRA245 sense strand
ttctcctgtagcttcagcc

SEQ ID NO: 665 - RNA, 19 nt, synthetic construct
  source 1..19: mol_type = other RNA; note = GPSZRA246 sense strand
tctcctgtagcttcagccc

SEQ ID NO: 666 - RNA, 19 nt, synthetic construct
  source 1..19: mol_type = other RNA; note = GPSZRA247 sense strand
ctcctgtagcttcagccca

SEQ ID NO: 667 - RNA, 19 nt, synthetic construct
  source 1..19: mol_type = other RNA; note = GPSZRA248 sense strand
tcctgtagcttcagcccag

SEQ ID NO: 668 - RNA, 19 nt, synthetic construct
  source 1..19: mol_type = other RNA; note = GPSZRA249 sense strand
tagcttcagcccaggcctt

SEQ ID NO: 669 - RNA, 19 nt, synthetic construct
  source 1..19: mol_type = other RNA; note = GPSZRA250 sense strand
cctctggaggaggtccaat

SEQ ID NO: 670 - RNA, 19 nt, synthetic construct
  source 1..19: mol_type = other RNA; note = GPSZRA251 sense strand
ctctggaggaggtccaatt

SEQ ID NO: 671 - RNA, 19 nt, synthetic construct
  source 1..19: mol_type = other RNA; note = GPSZRA252 sense strand
tctggaggaggtccaattg

SEQ ID NO: 672 - RNA, 19 nt, synthetic construct
  source 1..19: mol_type = other RNA; note = GPSZRA253 sense strand
ctggaggaggtccaattgg

SEQ ID NO: 673 - RNA, 19 nt, synthetic construct
  source 1..19: mol_type = other RNA; note = GPSZRA254 sense strand
tggaggaggtccaattggt

SEQ ID NO: 674 - RNA, 19 nt, synthetic construct
  source 1..19: mol_type = other RNA; note = GPSZRA255 sense strand
ggaggaggtccaattggtg

SEQ ID NO: 675 - RNA, 19 nt, synthetic construct
  source 1..19: mol_type = other RNA; note = GPSZRA256 sense strand
gaggaggtccaattggtgg

SEQ ID NO: 676 - RNA, 19 nt, synthetic construct
  source 1..19: mol_type = other RNA; note = GPSZRA257 sense strand
aggaggtccaattggtggt

SEQ ID NO: 677 - RNA, 19 nt, synthetic construct
  source 1..19: mol_type = other RNA; note = GPSZRA258 sense strand
gccagaaggtggagcagta

SEQ ID NO: 678 - RNA, 19 nt, synthetic construct
  source 1..19: mol_type = other RNA; note = GPSZRA259 sense strand
ccagaaggtggagcagtag

SEQ ID NO: 679 - RNA, 19 nt, synthetic construct
  source 1..19: mol_type = other RNA; note = GPSZRA260 sense strand
cagaaggtggagcagtagc

SEQ ID NO: 680 - RNA, 19 nt, synthetic construct
  source 1..19: mol_type = other RNA; note = GPSZRA261 sense strand
agaaggtggagcagtagct

SEQ ID NO: 681 - RNA, 19 nt, synthetic construct
  source 1..19: mol_type = other RNA; note = GPSZRA262 sense strand
gaaggtggagcagtagctc

SEQ ID NO: 682 - RNA, 19 nt, synthetic construct
  source 1..19: mol_type = other RNA; note = GPSZRA263 sense strand
aaggtggagcagtagctcc

SEQ ID NO: 683 - RNA, 19 nt, synthetic construct
  source 1..19: mol_type = other RNA; note = GPSZRA264 sense strand
aggtggagcagtagctcct

SEQ ID NO: 684 - RNA, 19 nt, synthetic construct
  source 1..19: mol_type = other RNA; note = GPSZRA265 sense strand
tggagcagtagctcctggt

SEQ ID NO: 685 - RNA, 19 nt, synthetic construct
  source 1..19: mol_type = other RNA; note = GPSZRA266 sense strand
agcagtagctcctggtgga

SEQ ID NO: 686 - RNA, 19 nt, synthetic construct
  source 1..19: mol_type = other RNA; note = GPSZRA267 sense strand
gcagtagctcctggtggaa

SEQ ID NO: 687 - RNA, 19 nt, synthetic construct
  source 1..19: mol_type = other RNA; note = GPSZRA268 sense strand
cagtagctcctggtggaac

SEQ ID NO: 688 - RNA, 19 nt, synthetic construct
  source 1..19: mol_type = other RNA; note = GPSZRA269 sense strand
agtagctcctggtggaacc

SEQ ID NO: 689 - RNA, 19 nt, synthetic construct
  source 1..19: mol_type = other RNA; note = GPSZRA270 sense strand
tagctcctggtggaaccgt

SEQ ID NO: 690 - RNA, 19 nt, synthetic construct
  source 1..19: mol_type = other RNA; note = GPSZRA271 sense strand
agctcctggtggaaccgta

SEQ ID NO: 691 - RNA, 19 nt, synthetic construct
  source 1..19: mol_type = other RNA; note = GPSZRA272 sense strand
gctcctggtggaaccgtaa

SEQ ID NO: 692 - RNA, 19 nt, synthetic construct
  source 1..19: mol_type = other RNA; note = GPSZRA273 sense strand
ctcctggtggaaccgtaac

SEQ ID NO: 693 - RNA, 19 nt, synthetic construct
  source 1..19: mol_type = other RNA; note = GPSZRA274 sense strand
tcctggtggaaccgtaacc

SEQ ID NO: 694 - RNA, 19 nt, synthetic construct
  source 1..19: mol_type = other RNA; note = GPSZRA275 sense strand
ctggtggaaccgtaaccct

SEQ ID NO: 695 - RNA, 19 nt, synthetic construct
  source 1..19: mol_type = other RNA; note = GPSZRA276 sense strand
tggtggaaccgtaaccctg

SEQ ID NO: 696 - RNA, 19 nt, synthetic construct
  source 1..19: mol_type = other RNA; note = GPSZRA277 sense strand
ggtggaaccgtaaccctga

SEQ ID NO: 697 - RNA, 19 nt, synthetic construct
  source 1..19: mol_type = other RNA; note = GPSZRA278 sense strand
gtggaaccgtaaccctgac

SEQ ID NO: 698 - RNA, 19 nt, synthetic construct
  source 1..19: mol_type = other RNA; note = GPSZRA279 sense strand
tggaaccgtaaccctgacc

SEQ ID NO: 699 - RNA, 19 nt, synthetic construct
  source 1..19: mol_type = other RNA; note = GPSZRA280 sense strand
ggaaccgtaaccctgacct

SEQ ID NO: 700 - RNA, 19 nt, synthetic construct
  source 1..19: mol_type = other RNA; note = GPSZRA281 sense strand
gaaccgtaaccctgacctg

SEQ ID NO: 701 - RNA, 19 nt, synthetic construct
  source 1..19: mol_type = other RNA; note = GPSZRA282 sense strand
aaccgtaaccctgacctgt

SEQ ID NO: 702 - RNA, 19 nt, synthetic construct
  source 1..19: mol_type = other RNA; note = GPSZRA283 sense strand
accgtaaccctgacctgtg

SEQ ID NO: 703 - RNA, 19 nt, synthetic construct
  source 1..19: mol_type = other RNA; note = GPSZRA284 sense strand
ccgtaaccctgacctgtga

SEQ ID NO: 704 - RNA, 19 nt, synthetic construct
  source 1..19: mol_type = other RNA; note = GPSZRA285 sense strand
cgtaaccctgacctgtgaa

SEQ ID NO: 705 - RNA, 19 nt, synthetic construct
  source 1..19: mol_type = other RNA; note = GPSZRA286 sense strand
gtaaccctgacctgtgaag

SEQ ID NO: 706 - RNA, 19 nt, synthetic construct
  source 1..19: mol_type = other RNA; note = GPSZRA287 sense strand
taaccctgacctgtgaagt

SEQ ID NO: 707 - RNA, 19 nt, synthetic construct
  source 1..19: mol_type = other RNA; note = GPSZRA288 sense strand
aaccctgacctgtgaagtc

SEQ ID NO: 708 - RNA, 19 nt, synthetic construct
  source 1..19: mol_type = other RNA; note = GPSZRA289 sense strand
accctgacctgtgaagtcc

SEQ ID NO: 709 - RNA, 19 nt, synthetic construct
  source 1..19: mol_type = other RNA; note = GPSZRA290 sense strand
cctgacctgtgaagtccct

SEQ ID NO: 710 - RNA, 19 nt, synthetic construct
  source 1..19: mol_type = other RNA; note = GPSZRA291 sense strand
ctgacctgtgaagtccctg

SEQ ID NO: 711 - RNA, 19 nt, synthetic construct
  source 1..19: mol_type = other RNA; note = GPSZRA292 sense strand
tgacctgtgaagtccctgc

SEQ ID NO: 712 - RNA, 19 nt, synthetic construct
  source 1..19: mol_type = other RNA; note = GPSZRA293 sense strand
cccagccctctcctcaaat

SEQ ID NO: 713 - RNA, 19 nt, synthetic construct
  source 1..19: mol_type = other RNA; note = GPSZRA294 sense strand
ccagccctctcctcaaatc

SEQ ID NO: 714 - RNA, 19 nt, synthetic construct
  source 1..19: mol_type = other RNA; note = GPSZRA295 sense strand
cagccctctcctcaaatcc

SEQ ID NO: 715 - RNA, 19 nt, synthetic construct
  source 1..19: mol_type = other RNA; note = GPSZRA296 sense strand
agccctctcctcaaatcca

SEQ ID NO: 716 - RNA, 19 nt, synthetic construct
  source 1..19: mol_type = other RNA; note = GPSZRA297 sense strand
gccctctcctcaaatccac

SEQ ID NO: 717 - RNA, 19 nt, synthetic construct
  source 1..19: mol_type = other RNA; note = GPSZRA298 sense strand
ccctctcctcaaatccact

SEQ ID NO: 718 - RNA, 19 nt, synthetic construct
  source 1..19: mol_type = other RNA; note = GPSZRA299 sense strand
cctctcctcaaatccactg

SEQ ID NO: 719 - RNA, 19 nt, synthetic construct
  source 1..19: mol_type = other RNA; note = GPSZRA300 sense strand
ctctcctcaaatccactgg

SEQ ID NO: 720 - RNA, 19 nt, synthetic construct
  source 1..19: mol_type = other RNA; note = GPSZRA301 sense strand
tctcctcaaatccactgga

SEQ ID NO: 721 - RNA, 19 nt, synthetic construct
  source 1..19: mol_type = other RNA; note = GPSZRA302 sense strand
ctcctcaaatccactggat

SEQ ID NO: 722 - RNA, 19 nt, synthetic construct
  source 1..19: mol_type = other RNA; note = GPSZRA303 sense strand
tcctcaaatccactggatg

SEQ ID NO: 723 - RNA, 19 nt, synthetic construct
  source 1..19: mol_type = other RNA; note = GPSZRA304 sense strand
cctcaaatccactggatga

SEQ ID NO: 724 - RNA, 19 nt, synthetic construct
  source 1..19: mol_type = other RNA; note = GPSZRA305 sense strand
ctcaaatccactggatgaa

SEQ ID NO: 725 - RNA, 19 nt, synthetic construct
  source 1..19: mol_type = other RNA; note = GPSZRA306 sense strand
tcaaatccactggatgaag

SEQ ID NO: 726 - RNA, 19 nt, synthetic construct
  source 1..19: mol_type = other RNA; note = GPSZRA307 sense strand
caaatccactggatgaagg

SEQ ID NO: 727 - RNA, 19 nt, synthetic construct
  source 1..19: mol_type = other RNA; note = GPSZRA308 sense strand
aaatccactggatgaagga

SEQ ID NO: 728 - RNA, 19 nt, synthetic construct
  source 1..19: mol_type = other RNA; note = GPSZRA309 sense strand
aatccactggatgaaggat

SEQ ID NO: 729 - RNA, 19 nt, synthetic construct
  source 1..19: mol_type = other RNA; note = GPSZRA310 sense strand
atccactggatgaaggatg

SEQ ID NO: 730 - RNA, 19 nt, synthetic construct
  source 1..19: mol_type = other RNA; note = GPSZRA311 sense strand
tccactggatgaaggatgg

SEQ ID NO: 731 - RNA, 19 nt, synthetic construct
  source 1..19: mol_type = other RNA; note = GPSZRA312 sense strand
ccactggatgaaggatggt

SEQ ID NO: 732 - RNA, 19 nt, synthetic construct
  source 1..19: mol_type = other RNA; note = GPSZRA313 sense strand
cactggatgaaggatggtg

SEQ ID NO: 733 - RNA, 19 nt, synthetic construct
  source 1..19: mol_type = other RNA; note = GPSZRA314 sense strand
actggatgaaggatggtgt

SEQ ID NO: 734 - RNA, 19 nt, synthetic construct
  source 1..19: mol_type = other RNA; note = GPSZRA315 sense strand
ctggatgaaggatggtgtg

SEQ ID NO: 735 - RNA, 19 nt, synthetic construct
  source 1..19: mol_type = other RNA; note = GPSZRA316 sense strand
tggatgaaggatggtgtgc

SEQ ID NO: 736 - RNA, 19 nt, synthetic construct
  source 1..19: mol_type = other RNA; note = GPSZRA317 sense strand
ggatgaaggatggtgtgcc

SEQ ID NO: 737 - RNA, 19 nt, synthetic construct
  source 1..19: mol_type = other RNA; note = GPSZRA318 sense strand
gatgaaggatggtgtgccc

SEQ ID NO: 738 - RNA, 19 nt, synthetic construct
  source 1..19: mol_type = other RNA; note = GPSZRA319 sense strand
atgaaggatggtgtgccct

SEQ ID NO: 739 - RNA, 19 nt, synthetic construct
  source 1..19: mol_type = other RNA; note = GPSZRA320 sense strand
tgaaggatggtgtgccctt

SEQ ID NO: 740 - RNA, 19 nt, synthetic construct
  source 1..19: mol_type = other RNA; note = GPSZRA321 sense strand
ctgtgctgatcctccctga

SEQ ID NO: 741 - RNA, 19 nt, synthetic construct
  source 1..19: mol_type = other RNA; note = GPSZRA322 sense strand
tgtgctgatcctccctgag

SEQ ID NO: 742 - RNA, 19 nt, synthetic construct
  source 1..19: mol_type = other RNA; note = GPSZRA323 sense strand
gtgctgatcctccctgaga

SEQ ID NO: 743 - RNA, 19 nt, synthetic construct
  source 1..19: mol_type = other RNA; note = GPSZRA324 sense strand
tgctgatcctccctgagat

SEQ ID NO: 744 - RNA, 19 nt, synthetic construct
  source 1..19: mol_type = other RNA; note = GPSZRA325 sense strand
gctgatcctccctgagata

SEQ ID NO: 745 - RNA, 19 nt, synthetic construct
  source 1..19: mol_type = other RNA; note = GPSZRA326 sense strand
ctgatcctccctgagatag

SEQ ID NO: 746 - RNA, 19 nt, synthetic construct
  source 1..19: mol_type = other RNA; note = GPSZRA327 sense strand
tgatcctccctgagatagg

SEQ ID NO: 747 - RNA, 19 nt, synthetic construct
  source 1..19: mol_type = other RNA; note = GPSZRA328 sense strand
gatcctccctgagataggg

SEQ ID NO: 748 - RNA, 19 nt, synthetic construct
  source 1..19: mol_type = other RNA; note = GPSZRA329 sense strand
atcctccctgagatagggc

SEQ ID NO: 749 - RNA, 19 nt, synthetic construct
  source 1..19: mol_type = other RNA; note = GPSZRA330 sense strand
aggaccagggaacctacag

SEQ ID NO: 750 - RNA, 19 nt, synthetic construct
  source 1..19: mol_type = other RNA; note = GPSZRA331 sense strand
caggaaagccgtgctgtca

SEQ ID NO: 751 - RNA, 19 nt, synthetic construct
  source 1..19: mol_type = other RNA; note = GPSZRA332 sense strand
aggaaagccgtgctgtcag

SEQ ID NO: 752 - RNA, 19 nt, synthetic construct
  source 1..19: mol_type = other RNA; note = GPSZRA333 sense strand
gaaagccgtgctgtcagca

SEQ ID NO: 753 - RNA, 19 nt, synthetic construct
  source 1..19: mol_type = other RNA; note = GPSZRA334 sense strand
aaagccgtgctgtcagcat

SEQ ID NO: 754 - RNA, 19 nt, synthetic construct
  source 1..19: mol_type = other RNA; note = GPSZRA335 sense strand
aagccgtgctgtcagcatc

SEQ ID NO: 755 - RNA, 19 nt, synthetic construct
  source 1..19: mol_type = other RNA; note = GPSZRA336 sense strand
agccgtgctgtcagcatca

SEQ ID NO: 756 - RNA, 19 nt, synthetic construct
  source 1..19: mol_type = other RNA; note = GPSZRA337 sense strand
cgtgctgtcagcatcagca

SEQ ID NO: 757 - RNA, 19 nt, synthetic construct
  source 1..19: mol_type = other RNA; note = GPSZRA338 sense strand
gtgctgtcagcatcagcat

SEQ ID NO: 758 - RNA, 19 nt, synthetic construct
  source 1..19: mol_type = other RNA; note = GPSZRA339 sense strand
tgctgtcagcatcagcatc

SEQ ID NO: 759 - RNA, 19 nt, synthetic construct
  source 1..19: mol_type = other RNA; note = GPSZRA340 sense strand
gctgtcagcatcagcatca

SEQ ID NO: 760 - RNA, 19 nt, synthetic construct
  source 1..19: mol_type = other RNA; note = GPSZRA341 sense strand
ctgtcagcatcagcatcat

SEQ ID NO: 761 - RNA, 19 nt, synthetic construct
  source 1..19: mol_type = other RNA; note = GPSZRA342 sense strand
tgtcagcatcagcatcatc

SEQ ID NO: 762 - RNA, 19 nt, synthetic construct
  source 1..19: mol_type = other RNA; note = GPSZRA343 sense strand
gtcagcatcagcatcatcg

SEQ ID NO: 763 - RNA, 19 nt, synthetic construct
  source 1..19: mol_type = other RNA; note = GPSZRA344 sense strand
tcagcatcagcatcatcga

SEQ ID NO: 764 - RNA, 19 nt, synthetic construct
  source 1..19: mol_type = other RNA; note = GPSZRA345 sense strand
cagcatcagcatcatcgaa

SEQ ID NO: 765 - RNA, 19 nt, synthetic construct
  source 1..19: mol_type = other RNA; note = GPSZRA346 sense strand
agcatcagcatcatcgaac

SEQ ID NO: 766 - RNA, 19 nt, synthetic construct
  source 1..19: mol_type = other RNA; note = GPSZRA347 sense strand
gcatcagcatcatcgaacc

SEQ ID NO: 767 - RNA, 19 nt, synthetic construct
  source 1..19: mol_type = other RNA; note = GPSZRA348 sense strand
catcagcatcatcgaacca

SEQ ID NO: 768 - RNA, 19 nt, synthetic construct
  source 1..19: mol_type = other RNA; note = GPSZRA349 sense strand
atcagcatcatcgaaccag

SEQ ID NO: 769 - RNA, 19 nt, synthetic construct
  source 1..19: mol_type = other RNA; note = GPSZRA350 sense strand
tcagcatcatcgaaccagg

SEQ ID NO: 770 - RNA, 19 nt, synthetic construct
  source 1..19: mol_type = other RNA; note = GPSZRA351 sense strand
cagcatcatcgaaccaggc

SEQ ID NO: 771 - RNA, 19 nt, synthetic construct
  source 1..19: mol_type = other RNA; note = GPSZRA352 sense strand
agcatcatcgaaccaggcg

SEQ ID NO: 772 - RNA, 19 nt, synthetic construct
  source 1..19: mol_type = other RNA; note = GPSZRA353 sense strand
gcatcatcgaaccaggcga

SEQ ID NO: 773 - RNA, 19 nt, synthetic construct
  source 1..19: mol_type = other RNA; note = GPSZRA354 sense strand
catcatcgaaccaggcgag

SEQ ID NO: 774 - RNA, 19 nt, synthetic construct
  source 1..19: mol_type = other RNA; note = GPSZRA355 sense strand
atcatcgaaccaggcgagg

SEQ ID NO: 775 - RNA, 19 nt, synthetic construct
  source 1..19: mol_type = other RNA; note = GPSZRA356 sense strand
tcatcgaaccaggcgagga

SEQ ID NO: 776 - RNA, 19 nt, synthetic construct
  source 1..19: mol_type = other RNA; note = GPSZRA357 sense strand
aactgcaggctctgtggga

SEQ ID NO: 777 - RNA, 19 nt, synthetic construct
  source 1..19: mol_type = other RNA; note = GPSZRA358 sense strand
aggctctgtgggaggatca

SEQ ID NO: 778 - RNA, 19 nt, synthetic construct
  source 1..19: mol_type = other RNA; note = GPSZRA359 sense strand
gctcattggggtcatcttg

SEQ ID NO: 779 - RNA, 19 nt, synthetic construct
  source 1..19: mol_type = other RNA; note = GPSZRA360 sense strand
ctcattggggtcatcttgt

SEQ ID NO: 780 - RNA, 19 nt, synthetic construct
  source 1..19: mol_type = other RNA; note = GPSZRA361 sense strand
tcattggggtcatcttgtg

SEQ ID NO: 781 - RNA, 19 nt, synthetic construct
  source 1..19: mol_type = other RNA; note = GPSZRA362 sense strand
cattggggtcatcttgtgg

SEQ ID NO: 782 - RNA, 19 nt, synthetic construct
  source 1..19: mol_type = other RNA; note = GPSZRA363 sense strand
attggggtcatcttgtggc

SEQ ID NO: 783 - RNA, 19 nt, synthetic construct
  source 1..19: mol_type = other RNA; note = GPSZRA364 sense strand
ttggggtcatcttgtggca

SEQ ID NO: 784 - RNA, 19 nt, synthetic construct
  source 1..19: mol_type = other RNA; note = GPSZRA365 sense strand
tggggtcatcttgtggcaa

SEQ ID NO: 785 - RNA, 19 nt, synthetic construct
  source 1..19: mol_type = other RNA; note = GPSZRA366 sense strand
ggggtcatcttgtggcaaa

SEQ ID NO: 786 - RNA, 19 nt, synthetic construct
  source 1..19: mol_type = other RNA; note = GPSZRA367 sense strand
gggtcatcttgtggcaaag

SEQ ID NO: 787 - RNA, 19 nt, synthetic construct
  source 1..19: mol_type = other RNA; note = GPSZRA368 sense strand
ggtcatcttgtggcaaagg

SEQ ID NO: 788 - RNA, 19 nt, synthetic construct
  source 1..19: mol_type = other RNA; note = GPSZRA369 sense strand
gtcatcttgtggcaaaggc

SEQ ID NO: 789 - RNA, 19 nt, synthetic construct
  source 1..19: mol_type = other RNA; note = GPSZRA370 sense strand
tcatcttgtggcaaaggcg

SEQ ID NO: 790 - RNA, 19 nt, synthetic construct
  source 1..19: mol_type = other RNA; note = GPSZRA371 sense strand
catcttgtggcaaaggcgg

SEQ ID NO: 791 - RNA, 19 nt, synthetic construct
  source 1..19: mol_type = other RNA; note = GPSZRA372 sense strand
atcttgtggcaaaggcggc

SEQ ID NO: 792 - RNA, 19 nt, synthetic construct
  source 1..19: mol_type = other RNA; note = GPSZRA373 sense strand
gaaaaccaggaggaagagg

SEQ ID NO: 793 - RNA, 19 nt, synthetic construct
  source 1..19: mol_type = other RNA; note = GPSZRA374 sense strand
aaaaccaggaggaagagga

SEQ ID NO: 794 - RNA, 19 nt, synthetic construct
  source 1..19: mol_type = other RNA; note = GPSZRA375 sense strand
aaaccaggaggaagaggag

SEQ ID NO: 795 - RNA, 19 nt, synthetic construct
  source 1..19: mol_type = other RNA; note = GPSZRA376 sense strand
aaccaggaggaagaggagg

SEQ ID NO: 796 - RNA, 19 nt, synthetic construct
  source 1..19: mol_type = other RNA; note = GPSZRA377 sense strand
accaggaggaagaggagga

SEQ ID NO: 797 - RNA, 19 nt, synthetic construct
  source 1..19: mol_type = other RNA; note = GPSZRA378 sense strand
aagaggaggagcgtgcaga

SEQ ID NO: 798 - RNA, 19 nt, synthetic construct
  source 1..19: mol_type = other RNA; note = GPSZRA379 sense strand
gaatcagtcggaggaacct

SEQ ID NO: 799 - RNA, 19 nt, synthetic construct
  source 1..19: mol_type = other RNA; note = GPSZRA380 sense strand
aatcagtcggaggaacctg

SEQ ID NO: 800 - RNA, 19 nt, synthetic construct
  source 1..19: mol_type = other RNA; note = GPSZRA381 sense strand
atcagtcggaggaacctga

SEQ ID NO: 801 - RNA, 19 nt, synthetic construct
  source 1..19: mol_type = other RNA; note = GPSZRA382 sense strand
tcagtcggaggaacctgag

SEQ ID NO: 802 - RNA, 19 nt, synthetic construct
  source 1..19: mol_type = other RNA; note = GPSZRA383 sense strand
gctcccttttctttttccc

SEQ ID NO: 803 - RNA, 19 nt, synthetic construct
  source 1..19: mol_type = other RNA; note = GPSZRA384 sense strand
ctcccttttctttttccct

SEQ ID NO: 804 - RNA, 19 nt, synthetic construct
  source 1..19: mol_type = other RNA; note = GPSZRA385 sense strand
tcccttttctttttccctt

SEQ ID NO: 805 - RNA, 19 nt, synthetic construct
  source 1..19: mol_type = other RNA; note = GPSZRA386 sense strand
cccttttctttttcccttg

SEQ ID NO: 806 - RNA, 19 nt, synthetic construct
  source 1..19: mol_type = other RNA; note = GPSZRA387 sense strand
ccttttctttttcccttga

SEQ ID NO: 807 - RNA, 19 nt, synthetic construct
  source 1..19: mol_type = other RNA; note = GPSZRA388 sense strand
cttttctttttcccttgaa

SEQ ID NO: 808 - RNA, 19 nt, synthetic construct
  source 1..19: mol_type = other RNA; note = GPSZRA389 sense strand
ttttctttttcccttgaac

SEQ ID NO: 809 - RNA, 19 nt, synthetic construct
  source 1..19: mol_type = other RNA; note = GPSZRA390 sense strand
tttctttttcccttgaact

SEQ ID NO: 810 - RNA, 19 nt, synthetic construct
  source 1..19: mol_type = other RNA; note = GPSZRA391 sense strand
ttctttttcccttgaactg

SEQ ID NO: 811 - RNA, 19 nt, synthetic construct
  source 1..19: mol_type = other RNA; note = GPSZRA392 sense strand
tctttttcccttgaactgt

SEQ ID NO: 812 - RNA, 19 nt, synthetic construct
  source 1..19: mol_type = other RNA; note = GPSZRA393 sense strand
ctttttcccttgaactgtt

SEQ ID NO: 813 - RNA, 19 nt, synthetic construct
  source 1..19: mol_type = other RNA; note = GPSZRA394 sense strand
tttttcccttgaactgttc

SEQ ID NO: 814 - RNA, 19 nt, synthetic construct
  source 1..19: mol_type = other RNA; note = GPSZRA395 sense strand
ttttcccttgaactgttct

SEQ ID NO: 815 - RNA, 19 nt, synthetic construct
  source 1..19: mol_type = other RNA; note = GPSZRA396 sense strand
tttcccttgaactgttctg

SEQ ID NO: 816 - RNA, 19 nt, synthetic construct
  source 1..19: mol_type = other RNA; note = GPSZRA397 sense strand
ttcccttgaactgttctgg

SEQ ID NO: 817 - RNA, 19 nt, synthetic construct
  source 1..19: mol_type = other RNA; note = GPSZRA398 sense strand
tcccttgaactgttctggc

SEQ ID NO: 818 - RNA, 19 nt, synthetic construct
  source 1..19: mol_type = other RNA; note = GPSZRA399 sense strand
cccttgaactgttctggcc

SEQ ID NO: 819 - RNA, 19 nt, synthetic construct
  source 1..19: mol_type = other RNA; note = GPSZRA400 sense strand
gaccaactctctcctgtat

SEQ ID NO: 820 - RNA, 19 nt, synthetic construct
  source 1..19: mol_type = other RNA; note = GPSZRA401 sense strand
accaactctctcctgtata

SEQ ID NO: 821 - RNA, 19 nt, synthetic construct
  source 1..19: mol_type = other RNA; note = GPSZRA402 sense strand
ccaactctctcctgtataa

SEQ ID NO: 822 - RNA, 19 nt, synthetic construct
  source 1..19: mol_type = other RNA; note = GPSZRA403 sense strand
ctctcctgtataaccccac

SEQ ID NO: 823 - RNA, 19 nt, synthetic construct
  source 1..19: mol_type = other RNA; note = GPSZRA404 sense strand
tctcctgtataaccccacc

SEQ ID NO: 824 - RNA, 19 nt, synthetic construct
  source 1..19: mol_type = other RNA; note = GPSZRA405 sense strand
ctcctgtataaccccacct

SEQ ID NO: 825 - RNA, 19 nt, synthetic construct
  source 1..19: mol_type = other RNA; note = GPSZRA406 sense strand
tcctgtataaccccacctt

SEQ ID NO: 826 - RNA, 19 nt, synthetic construct
  source 1..19: mol_type = other RNA; note = GPSZRA407 sense strand
cctgtataaccccaccttg

SEQ ID NO: 827 - RNA, 19 nt, synthetic construct
  source 1..19: mol_type = other RNA; note = GPSZRA408 sense strand
ctgtataaccccaccttgc

SEQ ID NO: 828 - RNA, 19 nt, synthetic construct
  source 1..19: mol_type = other RNA; note = GPSZRA409 sense strand
tgtataaccccaccttgcc

SEQ ID NO: 829 - RNA, 19 nt, synthetic construct
  source 1..19: mol_type = other RNA; note = GPSZRA410 sense strand
gtataaccccaccttgcca

SEQ ID NO: 830 - RNA, 19 nt, synthetic construct
  source 1..19: mol_type = other RNA; note = GPSZRA411 sense strand
tataaccccaccttgccaa

SEQ ID NO: 831 - RNA, 19 nt, synthetic construct
  source 1..19: mol_type = other RNA; note = GPSZRA412 sense strand
ttcttctacaaccagagcc

SEQ ID NO: 832 - RNA, 19 nt, synthetic construct
  source 1..19: mol_type = other RNA; note = GPSZRA413 sense strand
tcttctacaaccagagccc

SEQ ID NO: 833 - RNA, 19 nt, synthetic construct
  source 1..19: mol_type = other RNA; note = GPSZRA414 sense strand
cttctacaaccagagcccc

SEQ ID NO: 834 - RNA, 19 nt, synthetic construct
  source 1..19: mol_type = other RNA; note = GPSZRA415 sense strand
ttctacaaccagagccccc

SEQ ID NO: 835 - RNA, 19 nt, synthetic construct
  source 1..19: mol_type = other RNA; note = GPSZRA416 sense strand
aaccagagccccccacaat

SEQ ID NO: 836 - RNA, 19 nt, synthetic construct
  source 1..19: mol_type = other RNA; note = GPSZRA417 sense strand
cagagccccccacaatgat

SEQ ID NO: 837 - RNA, 19 nt, synthetic construct
  source 1..19: mol_type = other RNA; note = GPSZRA418 sense strand
agagccccccacaatgatg

SEQ ID NO: 838 - RNA, 19 nt, synthetic construct
  source 1..19: mol_type = other RNA; note = GPSZRA419 sense strand
gagccccccacaatgatga

SEQ ID NO: 839 - RNA, 21 nt, synthetic construct
  source 1..21: mol_type = other RNA; note = GPSZRA084S1 antisense strand
  modified_base order(1,3,5,7,9,11,12,13,15,17,19,20,21): mod_base = OTHER; note = 2'-methoxy-modified
  modified_base order(2,4,6,8,10,14,16,18): mod_base = OTHER; note = 2'-fluoro-modified
  modified_base order(1^2,2^3,19^20,20^21): mod_base = OTHER; note = phosphorothioate linkage
tggacttggtctcctttccat

SEQ ID NO: 840 - RNA, 21 nt, synthetic construct
  source 1..21: mol_type = other RNA; note = GPSZRA087S1 antisense strand
  modified_base order(1,3,5,7,9,11,12,13,15,17,19,20,21): mod_base = OTHER; note = 2'-methoxy-modified
  modified_base order(2,4,6,8,10,14,16,18): mod_base = OTHER; note = 2'-fluoro-modified
  modified_base order(1^2,2^3,19^20,20^21): mod_base = OTHER; note = phosphorothioate linkage
agttggacttggtctcctttc

SEQ ID NO: 841 - RNA, 21 nt, synthetic construct
  source 1..21: mol_type = other RNA; note = GPSZRA092S1 antisense strand
  modified_base order(1,3,5,7,9,11,12,13,15,17,19,20,21): mod_base = OTHER; note = 2'-methoxy-modified
  modified_base order(2,4,6,8,10,14,16,18): mod_base = OTHER; note = 2'-fluoro-modified
  modified_base order(1^2,2^3,19^20,20^21): mod_base = OTHER; note = phosphorothioate linkage
tcggtagttggacttggtctc

SEQ ID NO: 842 - RNA, 21 nt, synthetic construct
  source 1..21: mol_type = other RNA; note = GPSZRA093S1 antisense strand
  modified_base order(1,3,5,7,9,11,12,13,15,17,19,20,21): mod_base = OTHER; note = 2'-methoxy-modified
  modified_base order(2,4,6,8,10,14,16,18): mod_base = OTHER; note = 2'-fluoro-modified
  modified_base order(1^2,2^3,19^20,20^21): mod_base = OTHER; note = phosphorothioate linkage
ctcggtagttggacttggtct

SEQ ID NO: 843 - RNA, 21 nt, synthetic construct
  source 1..21: mol_type = other RNA; note = GPSZRA097S1 antisense strand
  modified_base order(1,3,5,7,9,11,12,13,15,17,19,20,21): mod_base = OTHER; note = 2'-methoxy-modified
  modified_base order(2,4,6,8,10,14,16,18): mod_base = OTHER; note = 2'-fluoro-modified
  modified_base order(1^2,2^3,19^20,20^21): mod_base = OTHER; note = phosphorothioate linkage
cggactcggtagttggacttg

SEQ ID NO: 844 - RNA, 21 nt, synthetic construct
  source 1..21: mol_type = other RNA; note = GPSZRA118S1 antisense strand
  modified_base order(1,3,5,7,9,11,12,13,15,17,19,20,21): mod_base = OTHER; note = 2'-methoxy-modified
  modified_base order(2,4,6,8,10,14,16,18): mod_base = OTHER; note = 2'-fluoro-modified
  modified_base order(1^2,2^3,19^20,20^21): mod_base = OTHER; note = phosphorothioate linkage
cttcccaggaatctggtagac

SEQ ID NO: 845 - RNA, 21 nt, synthetic construct
  source 1..21: mol_type = other RNA; note = GPSZRA217S1 antisense strand
  modified_base order(1,3,5,7,9,11,12,13,15,17,19,20,21): mod_base = OTHER; note = 2'-methoxy-modified
  modified_base order(2,4,6,8,10,14,16,18): mod_base = OTHER; note = 2'-fluoro-modified
  modified_base order(1^2,2^3,19^20,20^21): mod_base = OTHER; note = phosphorothioate linkage
tccttcacagatactcccttc

SEQ ID NO: 846 - RNA, 21 nt, synthetic construct
  source 1..21: mol_type = other RNA; note = GPSZRA222S1 antisense strand
  modified_base order(1,3,5,7,9,11,12,13,15,17,19,20,21): mod_base = OTHER; note = 2'-methoxy-modified
  modified_base order(2,4,6,8,10,14,16,18): mod_base = OTHER; note = 2'-fluoro-modified
  modified_base order(1^2,2^3,19^20,20^21): mod_base = OTHER; note = phosphorothioate linkage
tccgactgcagtgtgaagagc

SEQ ID NO: 847 - RNA, 21 nt, synthetic construct
  source 1..21: mol_type = other RNA; note = GPSZRA227S1 antisense strand
  modified_base order(1,3,5,7,9,11,12,13,15,17,19,20,21): mod_base = OTHER; note = 2'-methoxy-modified
  modified_base order(2,4,6,8,10,14,16,18): mod_base = OTHER; note = 2'-fluoro-modified
  modified_base order(1^2,2^3,19^20,20^21): mod_base = OTHER; note = phosphorothioate linkage
ttagctccgactgcagtgtga

SEQ ID NO: 848 - RNA, 21 nt, synthetic construct
  source 1..21: mol_type = other RNA; note = GPSZRA228S1 antisense strand
  modified_base order(1,3,5,7,9,11,12,13,15,17,19,20,21): mod_base = OTHER; note = 2'-methoxy-modified
  modified_base order(2,4,6,8,10,14,16,18): mod_base = OTHER; note = 2'-fluoro-modified
  modified_base order(1^2,2^3,19^20,20^21): mod_base = OTHER; note = phosphorothioate linkage
attagctccgactgcagtgtg

SEQ ID NO: 849 - RNA, 21 nt, synthetic construct
  source 1..21: mol_type = other RNA; note = GPSZRA229S1 antisense strand
  modified_base order(1,3,5,7,9,11,12,13,15,17,19,20,21): mod_base = OTHER; note = 2'-methoxy-modified
  modified_base order(2,4,6,8,10,14,16,18): mod_base = OTHER; note = 2'-fluoro-modified
  modified_base order(1^2,2^3,19^20,20^21): mod_base = OTHER; note = phosphorothioate linkage
cattagctccgactgcagtgt

SEQ ID NO: 850 - RNA, 21 nt, synthetic construct
  source 1..21: mol_type = other RNA; note = GPSZRA231S1 antisense strand
  modified_base order(1,3,5,7,9,11,12,13,15,17,19,20,21): mod_base = OTHER; note = 2'-methoxy-modified
  modified_base order(2,4,6,8,10,14,16,18): mod_base = OTHER; note = 2'-fluoro-modified
  modified_base order(1^2,2^3,19^20,20^21): mod_base = OTHER; note = phosphorothioate linkage
accattagctccgactgcagt

SEQ ID NO: 851 - RNA, 21 nt, synthetic construct
  source 1..21: mol_type = other RNA; note = GPSZRA232S1 antisense strand
  modified_base order(1,3,5,7,9,11,12,13,15,17,19,20,21): mod_base = OTHER; note = 2'-methoxy-modified
  modified_base order(2,4,6,8,10,14,16,18): mod_base = OTHER; note = 2'-fluoro-modified
  modified_base order(1^2,2^3,19^20,20^21): mod_base = OTHER; note = phosphorothioate linkage
caccattagctccgactgcag

SEQ ID NO: 852 - RNA, 21 nt, synthetic construct
  source 1..21: mol_type = other RNA; note = GPSZRA233S1 antisense strand
  modified_base order(1,3,5,7,9,11,12,13,15,17,19,20,21): mod_base = OTHER; note = 2'-methoxy-modified
  modified_base order(2,4,6,8,10,14,16,18): mod_base = OTHER; note = 2'-fluoro-modified
  modified_base order(1^2,2^3,19^20,20^21): mod_base = OTHER; note = phosphorothioate linkage
tcaccattagctccgactgca

SEQ ID NO: 853 - RNA, 21 nt, synthetic construct
  source 1..21: mol_type = other RNA; note = GPSZRA252S1 antisense strand
  modified_base order(1,3,5,7,9,11,12,13,15,17,19,20,21): mod_base = OTHER; note = 2'-methoxy-modified
  modified_base order(2,4,6,8,10,14,16,18): mod_base = OTHER; note = 2'-fluoro-modified
  modified_base order(1^2,2^3,19^20,20^21): mod_base = OTHER; note = phosphorothioate linkage
caattggacctcctccagagg

SEQ ID NO: 854 - RNA, 21 nt, synthetic construct
  source 1..21: mol_type = other RNA; note = GPSZRA257S1 antisense strand
  modified_base order(1,3,5,7,9,11,12,13,15,17,19,20,21): mod_base = OTHER; note = 2'-methoxy-modified
  modified_base order(2,4,6,8,10,14,16,18): mod_base = OTHER; note = 2'-fluoro-modified
  modified_base order(1^2,2^3,19^20,20^21): mod_base = OTHER; note = phosphorothioate linkage
accaccaattggacctcctcc

SEQ ID NO: 855 - RNA, 21 nt, synthetic construct
  source 1..21: mol_type = other RNA; note = GPSZRA266S1 antisense strand
  modified_base order(1,3,5,7,9,11,12,13,15,17,19,20,21): mod_base = OTHER; note = 2'-methoxy-modified
  modified_base order(2,4,6,8,10,14,16,18): mod_base = OTHER; note = 2'-fluoro-modified
  modified_base order(1^2,2^3,19^20,20^21): mod_base = OTHER; note = phosphorothioate linkage
tccaccaggagctactgctcc

SEQ ID NO: 856 - RNA, 21 nt, synthetic construct
  source 1..21: mol_type = other RNA; note = GPSZRA267S1 antisense strand
  modified_base order(1,3,5,7,9,11,12,13,15,17,19,20,21): mod_base = OTHER; note = 2'-methoxy-modified
  modified_base order(2,4,6,8,10,14,16,18): mod_base = OTHER; note = 2'-fluoro-modified
  modified_base order(1^2,2^3,19^20,20^21): mod_base = OTHER; note = phosphorothioate linkage
ttccaccaggagctactgctc

SEQ ID NO: 857 - RNA, 21 nt, synthetic construct
  source 1..21: mol_type = other RNA; note = GPSZRA271S1 antisense strand
  modified_base order(1,3,5,7,9,11,12,13,15,17,19,20,21): mod_base = OTHER; note = 2'-methoxy-modified
  modified_base order(2,4,6,8,10,14,16,18): mod_base = OTHER; note = 2'-fluoro-modified
  modified_base order(1^2,2^3,19^20,20^21): mod_base = OTHER; note = phosphorothioate linkage
tacggttccaccaggagctac

SEQ ID NO: 858 - RNA, 21 nt, synthetic construct
  source 1..21: mol_type = other RNA; note = GPSZRA272S1 antisense strand
  modified_base order(1,3,5,7,9,11,12,13,15,17,19,20,21): mod_base = OTHER; note = 2'-methoxy-modified
  modified_base order(2,4,6,8,10,14,16,18): mod_base = OTHER; note = 2'-fluoro-modified
  modified_base order(1^2,2^3,19^20,20^21): mod_base = OTHER; note = phosphorothioate linkage
ttacggttccaccaggagcta

SEQ ID NO: 859 - RNA, 21 nt, synthetic construct
  source 1..21: mol_type = other RNA; note = GPSZRA274S1 antisense strand
  modified_base order(1,3,5,7,9,11,12,13,15,17,19,20,21): mod_base = OTHER; note = 2'-methoxy-modified
  modified_base order(2,4,6,8,10,14,16,18): mod_base = OTHER; note = 2'-fluoro-modified
  modified_base order(1^2,2^3,19^20,20^21): mod_base = OTHER; note = phosphorothioate linkage
ggttacggttccaccaggagc

SEQ ID NO: 860 - RNA, 21 nt, synthetic construct
  source 1..21: mol_type = other RNA; note = GPSZRA275S1 antisense strand
  modified_base order(1,3,5,7,9,11,12,13,15,17,19,20,21): mod_base = OTHER; note = 2'-methoxy-modified
  modified_base order(2,4,6,8,10,14,16,18): mod_base = OTHER; note = 2'-fluoro-modified
  modified_base order(1^2,2^3,19^20,20^21): mod_base = OTHER; note = phosphorothioate linkage
agggttacggttccaccagga

SEQ ID NO: 861 - RNA, 21 nt, synthetic construct
  source 1..21: mol_type = other RNA; note = GPSZRA276S1 antisense strand
  modified_base order(1,3,5,7,9,11,12,13,15,17,19,20,21): mod_base = OTHER; note = 2'-methoxy-modified
  modified_base order(2,4,6,8,10,14,16,18): mod_base = OTHER; note = 2'-fluoro-modified
  modified_base order(1^2,2^3,19^20,20^21): mod_base = OTHER; note = phosphorothioate linkage
cagggttacggttccaccagg

SEQ ID NO: 862 - RNA, 21 nt, synthetic construct
  source 1..21: mol_type = other RNA; note = GPSZRA277S1 antisense strand
  modified_base order(1,3,5,7,9,11,12,13,15,17,19,20,21): mod_base = OTHER; note = 2'-methoxy-modified
  modified_base order(2,4,6,8,10,14,16,18): mod_base = OTHER; note = 2'-fluoro-modified
  modified_base order(1^2,2^3,19^20,20^21): mod_base = OTHER; note = phosphorothioate linkage
tcagggttacggttccaccag

SEQ ID NO: 863 - RNA, 21 nt, synthetic construct
  source 1..21: mol_type = other RNA; note = GPSZRA281S1 antisense strand
  modified_base order(1,3,5,7,9,11,12,13,15,17,19,20,21): mod_base = OTHER; note = 2'-methoxy-modified
  modified_base order(2,4,6,8,10,14,16,18): mod_base = OTHER; note = 2'-fluoro-modified
  modified_base order(1^2,2^3,19^20,20^21): mod_base = OTHER; note = phosphorothioate linkage
caggtcagggttacggttcca

SEQ ID NO: 864 - RNA, 21 nt, synthetic construct
  source 1..21: mol_type = other RNA; note = GPSZRA282S1 antisense strand
  modified_base order(1,3,5,7,9,11,12,13,15,17,19,20,21): mod_base = OTHER; note = 2'-methoxy-modified
  modified_base order(2,4,6,8,10,14,16,18): mod_base = OTHER; note = 2'-fluoro-modified
  modified_base order(1^2,2^3,19^20,20^21): mod_base = OTHER; note = phosphorothioate linkage
acaggtcagggttacggttcc

SEQ ID NO: 865 - RNA, 21 nt, synthetic construct
  source 1..21: mol_type = other RNA; note = GPSZRA283S1 antisense strand
  modified_base order(1,3,5,7,9,11,12,13,15,17,19,20,21): mod_base = OTHER; note = 2'-methoxy-modified
  modified_base order(2,4,6,8,10,14,16,18): mod_base = OTHER; note = 2'-fluoro-modified
  modified_base order(1^2,2^3,19^20,20^21): mod_base = OTHER; note = phosphorothioate linkage
cacaggtcagggttacggttc

SEQ ID NO: 866 - RNA, 21 nt, synthetic construct
  source 1..21: mol_type = other RNA; note = GPSZRA284S1 antisense strand
  modified_base order(1,3,5,7,9,11,12,13,15,17,19,20,21): mod_base = OTHER; note = 2'-methoxy-modified
  modified_base order(2,4,6,8,10,14,16,18): mod_base = OTHER; note = 2'-fluoro-modified
  modified_base order(1^2,2^3,19^20,20^21): mod_base = OTHER; note = phosphorothioate linkage
tcacaggtcagggttacggtt

SEQ ID NO: 867 - RNA, 21 nt, synthetic construct
  source 1..21: mol_type = other RNA; note = GPSZRA285S1 antisense strand
  modified_base order(1,3,5,7,9,11,12,13,15,17,19,20,21): mod_base = OTHER; note = 2'-methoxy-modified
  modified_base order(2,4,6,8,10,14,16,18): mod_base = OTHER; note = 2'-fluoro-modified
  modified_base order(1^2,2^3,19^20,20^21): mod_base = OTHER; note = phosphorothioate linkage
ttcacaggtcagggttacggt

SEQ ID NO: 868 - RNA, 21 nt, synthetic construct
  source 1..21: mol_type = other RNA; note = GPSZRA286S1 antisense strand
  modified_base order(1,3,5,7,9,11,12,13,15,17,19,20,21): mod_base = OTHER; note = 2'-methoxy-modified
  modified_base order(2,4,6,8,10,14,16,18): mod_base = OTHER; note = 2'-fluoro-modified
  modified_base order(1^2,2^3,19^20,20^21): mod_base = OTHER; note = phosphorothioate linkage
cttcacaggtcagggttacgg

SEQ ID NO: 869 - RNA, 21 nt, synthetic construct
  source 1..21: mol_type = other RNA; note = GPSZRA287S1 antisense strand
  modified_base order(1,3,5,7,9,11,12,13,15,17,19,20,21): mod_base = OTHER; note = 2'-methoxy-modified
  modified_base order(2,4,6,8,10,14,16,18): mod_base = OTHER; note = 2'-fluoro-modified
  modified_base order(1^2,2^3,19^20,20^21): mod_base = OTHER; note = phosphorothioate linkage
acttcacaggtcagggttacg

SEQ ID NO: 870 - RNA, 21 nt, synthetic construct
  source 1..21: mol_type = other RNA; note = GPSZRA288S1 antisense strand
  modified_base order(1,3,5,7,9,11,12,13,15,17,19,20,21): mod_base = OTHER; note = 2'-methoxy-modified
  modified_base order(2,4,6,8,10,14,16,18): mod_base = OTHER; note = 2'-fluoro-modified
  modified_base order(1^2,2^3,19^20,20^21): mod_base = OTHER; note = phosphorothioate linkage
gacttcacaggtcagggttac

SEQ ID NO: 871 - RNA, 21 nt, synthetic construct
  source 1..21: mol_type = other RNA; note = GPSZRA290S1 antisense strand
  modified_base order(1,3,5,7,9,11,12,13,15,17,19,20,21): mod_base = OTHER; note = 2'-methoxy-modified
  modified_base order(2,4,6,8,10,14,16,18): mod_base = OTHER; note = 2'-fluoro-modified
  modified_base order(1^2,2^3,19^20,20^21): mod_base = OTHER; note = phosphorothioate linkage
agggacttcacaggtcagggt

SEQ ID NO: 872 - RNA, 21 nt, synthetic construct
  source 1..21: mol_type = other RNA; note = GPSZRA292S1 antisense strand
  modified_base order(1,3,5,7,9,11,12,13,15,17,19,20,21): mod_base = OTHER; note = 2'-methoxy-modified
  modified_base order(2,4,6,8,10,14,16,18): mod_base = OTHER; note = 2'-fluoro-modified
  modified_base order(1^2,2^3,19^20,20^21): mod_base = OTHER; note = phosphorothioate linkage
gcagggacttcacaggtcagg

SEQ ID NO: 873 - RNA, 21 nt, synthetic construct
  source 1..21: mol_type = other RNA; note = GPSZRA301S1 antisense strand
  modified_base order(1,3,5,7,9,11,12,13,15,17,19,20,21): mod_base = OTHER; note = 2'-methoxy-modified
  modified_base order(2,4,6,8,10,14,16,18): mod_base = OTHER; note = 2'-fluoro-modified
  modified_base order(1^2,2^3,19^20,20^21): mod_base = OTHER; note = phosphorothioate linkage
tccagtggatttgaggagagg

SEQ ID NO: 874 - RNA, 21 nt, synthetic construct
  source 1..21: mol_type = other RNA; note = GPSZRA308S1 antisense strand
  modified_base order(1,3,5,7,9,11,12,13,15,17,19,20,21): mod_base = OTHER; note = 2'-methoxy-modified
  modified_base order(2,4,6,8,10,14,16,18): mod_base = OTHER; note = 2'-fluoro-modified
  modified_base order(1^2,2^3,19^20,20^21): mod_base = OTHER; note = phosphorothioate linkage
tccttcatccagtggatttga

SEQ ID NO: 875 - RNA, 21 nt, synthetic construct
  source 1..21: mol_type = other RNA; note = GPSZRA311S1 antisense strand
  modified_base order(1,3,5,7,9,11,12,13,15,17,19,20,21): mod_base = OTHER; note = 2'-methoxy-modified
  modified_base order(2,4,6,8,10,14,16,18): mod_base = OTHER; note = 2'-fluoro-modified
  modified_base order(1^2,2^3,19^20,20^21): mod_base = OTHER; note = phosphorothioate linkage
ccatccttcatccagtggatt

SEQ ID NO: 876 - RNA, 21 nt, synthetic construct
  source 1..21: mol_type = other RNA; note = GPSZRA312S1 antisense strand
  modified_base order(1,3,5,7,9,11,12,13,15,17,19,20,21): mod_base = OTHER; note = 2'-methoxy-modified
  modified_base order(2,4,6,8,10,14,16,18): mod_base = OTHER; note = 2'-fluoro-modified
  modified_base order(1^2,2^3,19^20,20^21): mod_base = OTHER; note = phosphorothioate linkage
accatccttcatccagtggat

SEQ ID NO: 877 - RNA, 21 nt, synthetic construct
  source 1..21: mol_type = other RNA; note = GPSZRA313S1 antisense strand
  modified_base order(1,3,5,7,9,11,12,13,15,17,19,20,21): mod_base = OTHER; note = 2'-methoxy-modified
  modified_base order(2,4,6,8,10,14,16,18): mod_base = OTHER; note = 2'-fluoro-modified
  modified_base order(1^2,2^3,19^20,20^21): mod_base = OTHER; note = phosphorothioate linkage
caccatccttcatccagtgga

SEQ ID NO: 878 - RNA, 21 nt, synthetic construct
  source 1..21: mol_type = other RNA; note = GPSZRA314S1 antisense strand
  modified_base order(1,3,5,7,9,11,12,13,15,17,19,20,21): mod_base = OTHER; note = 2'-methoxy-modified
  modified_base order(2,4,6,8,10,14,16,18): mod_base = OTHER; note = 2'-fluoro-modified
  modified_base order(1^2,2^3,19^20,20^21): mod_base = OTHER; note = phosphorothioate linkage
acaccatccttcatccagtgg

SEQ ID NO: 879 - RNA, 21 nt, synthetic construct
  source 1..21: mol_type = other RNA; note = GPSZRA315S1 antisense strand
  modified_base order(1,3,5,7,9,11,12,13,15,17,19,20,21): mod_base = OTHER; note = 2'-methoxy-modified
  modified_base order(2,4,6,8,10,14,16,18): mod_base = OTHER; note = 2'-fluoro-modified
  modified_base order(1^2,2^3,19^20,20^21): mod_base = OTHER; note = phosphorothioate linkage
cacaccatccttcatccagtg

SEQ ID NO: 880 - RNA, 21 nt, synthetic construct
  source 1..21: mol_type = other RNA; note = GPSZRA316S1 antisense strand
  modified_base order(1,3,5,7,9,11,12,13,15,17,19,20,21): mod_base = OTHER; note = 2'-methoxy-modified
  modified_base order(2,4,6,8,10,14,16,18): mod_base = OTHER; note = 2'-fluoro-modified
  modified_base order(1^2,2^3,19^20,20^21): mod_base = OTHER; note = phosphorothioate linkage
gcacaccatccttcatccagt

SEQ ID NO: 881 - RNA, 21 nt, synthetic construct
  source 1..21: mol_type = other RNA; note = GPSZRA317S1 antisense strand
  modified_base order(1,3,5,7,9,11,12,13,15,17,19,20,21): mod_base = OTHER; note = 2'-methoxy-modified
  modified_base order(2,4,6,8,10,14,16,18): mod_base = OTHER; note = 2'-fluoro-modified
  modified_base order(1^2,2^3,19^20,20^21): mod_base = OTHER; note = phosphorothioate linkage
ggcacaccatccttcatccag

SEQ ID NO: 882 - RNA, 21 nt, synthetic construct
  source 1..21: mol_type = other RNA; note = GPSZRA318S1 antisense strand
  modified_base order(1,3,5,7,9,11,12,13,15,17,19,20,21): mod_base = OTHER; note = 2'-methoxy-modified
  modified_base order(2,4,6,8,10,14,16,18): mod_base = OTHER; note = 2'-fluoro-modified
  modified_base order(1^2,2^3,19^20,20^21): mod_base = OTHER; note = phosphorothioate linkage
gggcacaccatccttcatcca

SEQ ID NO: 883 - RNA, 21 nt, synthetic construct
  source 1..21: mol_type = other RNA; note = GPSZRA320S1 antisense strand
  modified_base order(1,3,5,7,9,11,12,13,15,17,19,20,21): mod_base = OTHER; note = 2'-methoxy-modified
  modified_base order(2,4,6,8,10,14,16,18): mod_base = OTHER; note = 2'-fluoro-modified
  modified_base order(1^2,2^3,19^20,20^21): mod_base = OTHER; note = phosphorothioate linkage
aagggcacaccatccttcatc

SEQ ID NO: 884 - RNA, 21 nt, synthetic construct
  source 1..21: mol_type = other RNA; note = GPSZRA333S1 antisense strand
  modified_base order(1,3,5,7,9,11,12,13,15,17,19,20,21): mod_base = OTHER; note = 2'-methoxy-modified
  modified_base order(2,4,6,8,10,14,16,18): mod_base = OTHER; note = 2'-fluoro-modified
  modified_base order(1^2,2^3,19^20,20^21): mod_base = OTHER; note = phosphorothioate linkage
tgctgacagcacggctttcct

SEQ ID NO: 885 - RNA, 21 nt, synthetic construct
  source 1..21: mol_type = other RNA; note = GPSZRA342S1 antisense strand
  modified_base order(1,3,5,7,9,11,12,13,15,17,19,20,21): mod_base = OTHER; note = 2'-methoxy-modified
  modified_base order(2,4,6,8,10,14,16,18): mod_base = OTHER; note = 2'-fluoro-modified
  modified_base order(1^2,2^3,19^20,20^21): mod_base = OTHER; note = phosphorothioate linkage
gatgatgctgatgctgacagc

SEQ ID NO: 886 - RNA, 21 nt, synthetic construct
  source 1..21: mol_type = other RNA; note = GPSZRA378S1 antisense strand
  modified_base order(1,3,5,7,9,11,12,13,15,17,19,20,21): mod_base = OTHER; note = 2'-methoxy-modified
  modified_base order(2,4,6,8,10,14,16,18): mod_base = OTHER; note = 2'-fluoro-modified
  modified_base order(1^2,2^3,19^20,20^21): mod_base = OTHER; note = phosphorothioate linkage
tctgcacgctcctcctcttcc

SEQ ID NO: 887 - RNA, 21 nt, synthetic construct
  source 1..21: mol_type = other RNA; note = GPSZRA379S1 antisense strand
  modified_base order(1,3,5,7,9,11,12,13,15,17,19,20,21): mod_base = OTHER; note = 2'-methoxy-modified
  modified_base order(2,4,6,8,10,14,16,18): mod_base = OTHER; note = 2'-fluoro-modified
  modified_base order(1^2,2^3,19^20,20^21): mod_base = OTHER; note = phosphorothioate linkage
aggttcctccgactgattcag

SEQ ID NO: 888 - RNA, 21 nt, synthetic construct
  source 1..21: mol_type = other RNA; note = GPSZRA380S1 antisense strand
  modified_base order(1,3,5,7,9,11,12,13,15,17,19,20,21): mod_base = OTHER; note = 2'-methoxy-modified
  modified_base order(2,4,6,8,10,14,16,18): mod_base = OTHER; note = 2'-fluoro-modified
  modified_base order(1^2,2^3,19^20,20^21): mod_base = OTHER; note = phosphorothioate linkage
caggttcctccgactgattca

SEQ ID NO: 889 - RNA, 21 nt, synthetic construct
  source 1..21: mol_type = other RNA; note = GPSZRA381S1 antisense strand
  modified_base order(1,3,5,7,9,11,12,13,15,17,19,20,21): mod_base = OTHER; note = 2'-methoxy-modified
  modified_base order(2,4,6,8,10,14,16,18): mod_base = OTHER; note = 2'-fluoro-modified
  modified_base order(1^2,2^3,19^20,20^21): mod_base = OTHER; note = phosphorothioate linkage
tcaggttcctccgactgattc

SEQ ID NO: 890 - RNA, 21 nt, synthetic construct
  source 1..21: mol_type = other RNA; note = GPSZRA402S1 antisense strand
  modified_base order(1,3,5,7,9,11,12,13,15,17,19,20,21): mod_base = OTHER; note = 2'-methoxy-modified
  modified_base order(2,4,6,8,10,14,16,18): mod_base = OTHER; note = 2'-fluoro-modified
  modified_base order(1^2,2^3,19^20,20^21): mod_base = OTHER; note = phosphorothioate linkage
ttatacaggagagagttggtc

SEQ ID NO: 891 - RNA, 21 nt, synthetic construct
  source 1..21: mol_type = other RNA; note = GPSZRA407S1 antisense strand
  modified_base order(1,3,5,7,9,11,12,13,15,17,19,20,21): mod_base = OTHER; note = 2'-methoxy-modified
  modified_base order(2,4,6,8,10,14,16,18): mod_base = OTHER; note = 2'-fluoro-modified
  modified_base order(1^2,2^3,19^20,20^21): mod_base = OTHER; note = phosphorothioate linkage
caaggtggggttatacaggag

SEQ ID NO: 892 - RNA, 21 nt, synthetic construct
  source 1..21: mol_type = other RNA; note = GPSZRA408S1 antisense strand
  modified_base order(1,3,5,7,9,11,12,13,15,17,19,20,21): mod_base = OTHER; note = 2'-methoxy-modified
  modified_base order(2,4,6,8,10,14,16,18): mod_base = OTHER; note = 2'-fluoro-modified
  modified_base order(1^2,2^3,19^20,20^21): mod_base = OTHER; note = phosphorothioate linkage
gcaaggtggggttatacagga

SEQ ID NO: 893 - RNA, 21 nt, synthetic construct
  source 1..21: mol_type = other RNA; note = GPSZRA409S1 antisense strand
  modified_base order(1,3,5,7,9,11,12,13,15,17,19,20,21): mod_base = OTHER; note = 2'-methoxy-modified
  modified_base order(2,4,6,8,10,14,16,18): mod_base = OTHER; note = 2'-fluoro-modified
  modified_base order(1^2,2^3,19^20,20^21): mod_base = OTHER; note = phosphorothioate linkage
ggcaaggtggggttatacagg

SEQ ID NO: 894 - RNA, 21 nt, synthetic construct
  source 1..21: mol_type = other RNA; note = GPSZRA410S1 antisense strand
  modified_base order(1,3,5,7,9,11,12,13,15,17,19,20,21): mod_base = OTHER; note = 2'-methoxy-modified
  modified_base order(2,4,6,8,10,14,16,18): mod_base = OTHER; note = 2'-fluoro-modified
  modified_base order(1^2,2^3,19^20,20^21): mod_base = OTHER; note = phosphorothioate linkage
tggcaaggtggggttatacag

SEQ ID NO: 895 - RNA, 21 nt, synthetic construct
  source 1..21: mol_type = other RNA; note = GPSZRA411S1 antisense strand
  modified_base order(1,3,5,7,9,11,12,13,15,17,19,20,21): mod_base = OTHER; note = 2'-methoxy-modified
  modified_base order(2,4,6,8,10,14,16,18): mod_base = OTHER; note = 2'-fluoro-modified
  modified_base order(1^2,2^3,19^20,20^21): mod_base = OTHER; note = phosphorothioate linkage
ttggcaaggtggggttataca

SEQ ID NO: 896 - RNA, 21 nt, synthetic construct
  source 1..21: mol_type = other RNA; note = GPSZRA084S2 antisense strand
  modified_base order(1^2,2^3,19^20,20^21): mod_base = OTHER; note = phosphorothioate linkage
  modified_base order(1,3,4,5,7,9,10,11,12,13,15,17,18,19,20,21): mod_base = OTHER; note = 2'-methoxy-modified
  modified_base order(2,6,8,14,16): mod_base = OTHER; note = 2'-fluoro-modified
tggacttggtctcctttccat

SEQ ID NO: 897 - RNA, 21 nt, synthetic construct
  source 1..21: mol_type = other RNA; note = GPSZRA087S2 antisense strand
  modified_base order(1^2,2^3,19^20,20^21): mod_base = OTHER; note = phosphorothioate linkage
  modified_base order(1,3,4,5,7,9,10,11,12,13,15,17,18,19,20,21): mod_base = OTHER; note = 2'-methoxy-modified
  modified_base order(2,6,8,14,16): mod_base = OTHER; note = 2'-fluoro-modified
agttggacttggtctcctttc

SEQ ID NO: 898 - RNA, 21 nt, synthetic construct
  source 1..21: mol_type = other RNA; note = GPSZRA092S2 antisense strand
  modified_base order(1^2,2^3,19^20,20^21): mod_base = OTHER; note = phosphorothioate linkage
  modified_base order(1,3,4,5,7,9,10,11,12,13,15,17,18,19,20,21): mod_base = OTHER; note = 2'-methoxy-modified
  modified_base order(2,6,8,14,16): mod_base = OTHER; note = 2'-fluoro-modified
tcggtagttggacttggtctc

SEQ ID NO: 899 - RNA, 21 nt, synthetic construct
  source 1..21: mol_type = other RNA; note = GPSZRA093S2 antisense strand
  modified_base order(1^2,2^3,19^20,20^21): mod_base = OTHER; note = phosphorothioate linkage
  modified_base order(1,3,4,5,7,9,10,11,12,13,15,17,18,19,20,21): mod_base = OTHER; note = 2'-methoxy-modified
  modified_base order(2,6,8,14,16): mod_base = OTHER; note = 2'-fluoro-modified
ctcggtagttggacttggtct

SEQ ID NO: 900 - RNA, 21 nt, synthetic construct
  source 1..21: mol_type = other RNA; note = GPSZRA097S2 antisense strand
  modified_base order(1^2,2^3,19^20,20^21): mod_base = OTHER; note = phosphorothioate linkage
  modified_base order(1,3,4,5,7,9,10,11,12,13,15,17,18,19,20,21): mod_base = OTHER; note = 2'-methoxy-modified
  modified_base order(2,6,8,14,16): mod_base = OTHER; note = 2'-fluoro-modified
cggactcggtagttggacttg

SEQ ID NO: 901 - RNA, 21 nt, synthetic construct
  source 1..21: mol_type = other RNA; note = GPSZRA118S2 antisense strand
  modified_base order(1^2,2^3,19^20,20^21): mod_base = OTHER; note = phosphorothioate linkage
  modified_base order(1,3,4,5,7,9,10,11,12,13,15,17,18,19,20,21): mod_base = OTHER; note = 2'-methoxy-modified
  modified_base order(2,6,8,14,16): mod_base = OTHER; note = 2'-fluoro-modified
cttcccaggaatctggtagac

SEQ ID NO: 902 - RNA, 21 nt, synthetic construct
  source 1..21: mol_type = other RNA; note = GPSZRA217S2 antisense strand
  modified_base order(1^2,2^3,19^20,20^21): mod_base = OTHER; note = phosphorothioate linkage
  modified_base order(1,3,4,5,7,9,10,11,12,13,15,17,18,19,20,21): mod_base = OTHER; note = 2'-methoxy-modified
  modified_base order(2,6,8,14,16): mod_base = OTHER; note = 2'-fluoro-modified
tccttcacagatactcccttc

SEQ ID NO: 903 - RNA, 21 nt, synthetic construct
  source 1..21: mol_type = other RNA; note = GPSZRA222S2 antisense strand
  modified_base order(1^2,2^3,19^20,20^21): mod_base = OTHER; note = phosphorothioate linkage
  modified_base order(1,3,4,5,7,9,10,11,12,13,15,17,18,19,20,21): mod_base = OTHER; note = 2'-methoxy-modified
  modified_base order(2,6,8,14,16): mod_base = OTHER; note = 2'-fluoro-modified
tccgactgcagtgtgaagagc

SEQ ID NO: 904 - RNA, 21 nt, synthetic construct
  source 1..21: mol_type = other RNA; note = GPSZRA227S2 antisense strand
  modified_base order(1^2,2^3,19^20,20^21): mod_base = OTHER; note = phosphorothioate linkage
  modified_base order(1,3,4,5,7,9,10,11,12,13,15,17,18,19,20,21): mod_base = OTHER; note = 2'-methoxy-modified
  modified_base order(2,6,8,14,16): mod_base = OTHER; note = 2'-fluoro-modified
ttagctccgactgcagtgtga

SEQ ID NO: 905 - RNA, 21 nt, synthetic construct
  source 1..21: mol_type = other RNA; note = GPSZRA228S2 antisense strand
  modified_base order(1^2,2^3,19^20,20^21): mod_base = OTHER; note = phosphorothioate linkage
  modified_base order(1,3,4,5,7,9,10,11,12,13,15,17,18,19,20,21): mod_base = OTHER; note = 2'-methoxy-modified
  modified_base order(2,6,8,14,16): mod_base = OTHER; note = 2'-fluoro-modified
attagctccgactgcagtgtg

SEQ ID NO: 906 - RNA, 21 nt, synthetic construct
  source 1..21: mol_type = other RNA; note = GPSZRA229S2 antisense strand
  modified_base order(1^2,2^3,19^20,20^21): mod_base = OTHER; note = phosphorothioate linkage
  modified_base order(1,3,4,5,7,9,10,11,12,13,15,17,18,19,20,21): mod_base = OTHER; note = 2'-methoxy-modified
  modified_base order(2,6,8,14,16): mod_base = OTHER; note = 2'-fluoro-modified
cattagctccgactgcagtgt

SEQ ID NO: 907 - RNA, 21 nt, synthetic construct
  source 1..21: mol_type = other RNA; note = GPSZRA231S2 antisense strand
  modified_base order(1^2,2^3,19^20,20^21): mod_base = OTHER; note = phosphorothioate linkage
  modified_base order(1,3,4,5,7,9,10,11,12,13,15,17,18,19,20,21): mod_base = OTHER; note = 2'-methoxy-modified
  modified_base order(2,6,8,14,16): mod_base = OTHER; note = 2'-fluoro-modified
accattagctccgactgcagt

SEQ ID NO: 908 - RNA, 21 nt, synthetic construct
  source 1..21: mol_type = other RNA; note = GPSZRA232S2 antisense strand
  modified_base order(1^2,2^3,19^20,20^21): mod_base = OTHER; note = phosphorothioate linkage
  modified_base order(1,3,4,5,7,9,10,11,12,13,15,17,18,19,20,21): mod_base = OTHER; note = 2'-methoxy-modified
  modified_base order(2,6,8,14,16): mod_base = OTHER; note = 2'-fluoro-modified
caccattagctccgactgcag

SEQ ID NO: 909 - RNA, 21 nt, synthetic construct
  source 1..21: mol_type = other RNA; note = GPSZRA233S2 antisense strand
  modified_base order(1^2,2^3,19^20,20^21): mod_base = OTHER; note = phosphorothioate linkage
  modified_base order(1,3,4,5,7,9,10,11,12,13,15,17,18,19,20,21): mod_base = OTHER; note = 2'-methoxy-modified
  modified_base order(2,6,8,14,16): mod_base = OTHER; note = 2'-fluoro-modified
tcaccattagctccgactgca

SEQ ID NO: 910 - RNA, 21 nt, synthetic construct
  source 1..21: mol_type = other RNA; note = GPSZRA252S2 antisense strand
  modified_base order(1^2,2^3,19^20,20^21): mod_base = OTHER; note = phosphorothioate linkage
  modified_base order(1,3,4,5,7,9,10,11,12,13,15,17,18,19,20,21): mod_base = OTHER; note = 2'-methoxy-modified
  modified_base order(2,6,8,14,16): mod_base = OTHER; note = 2'-fluoro-modified
caattggacctcctccagagg

SEQ ID NO: 911 - RNA, 21 nt, synthetic construct
  source 1..21: mol_type = other RNA; note = GPSZRA257S2 antisense strand
  modified_base order(1^2,2^3,19^20,20^21): mod_base = OTHER; note = phosphorothioate linkage
  modified_base order(1,3,4,5,7,9,10,11,12,13,15,17,18,19,20,21): mod_base = OTHER; note = 2'-methoxy-modified
  modified_base order(2,6,8,14,16): mod_base = OTHER; note = 2'-fluoro-modified
accaccaattggacctcctcc

SEQ ID NO: 912 - RNA, 21 nt, synthetic construct
  source 1..21: mol_type = other RNA; note = GPSZRA266S2 antisense strand
  modified_base order(1^2,2^3,19^20,20^21): mod_base = OTHER; note = phosphorothioate linkage
  modified_base order(1,3,4,5,7,9,10,11,12,13,15,17,18,19,20,21): mod_base = OTHER; note = 2'-methoxy-modified
  modified_base order(2,6,8,14,16): mod_base = OTHER; note = 2'-fluoro-modified
tccaccaggagctactgctcc

SEQ ID NO: 913 - RNA, 21 nt, synthetic construct
  source 1..21: mol_type = other RNA; note = GPSZRA267S2 antisense strand
  modified_base order(1^2,2^3,19^20,20^21): mod_base = OTHER; note = phosphorothioate linkage
  modified_base order(1,3,4,5,7,9,10,11,12,13,15,17,18,19,20,21): mod_base = OTHER; note = 2'-methoxy-modified
  modified_base order(2,6,8,14,16): mod_base = OTHER; note = 2'-fluoro-modified
ttccaccaggagctactgctc

SEQ ID NO: 914 - RNA, 21 nt, synthetic construct
  source 1..21: mol_type = other RNA; note = GPSZRA271S2 antisense strand
  modified_base order(1^2,2^3,19^20,20^21): mod_base = OTHER; note = phosphorothioate linkage
  modified_base order(1,3,4,5,7,9,10,11,12,13,15,17,18,19,20,21): mod_base = OTHER; note = 2'-methoxy-modified
  modified_base order(2,6,8,14,16): mod_base = OTHER; note = 2'-fluoro-modified
tacggttccaccaggagctac

SEQ ID NO: 915 - RNA, 21 nt, synthetic construct
  source 1..21: mol_type = other RNA; note = GPSZRA272S2 antisense strand
  modified_base order(1^2,2^3,19^20,20^21): mod_base = OTHER; note = phosphorothioate linkage
  modified_base order(1,3,4,5,7,9,10,11,12,13,15,17,18,19,20,21): mod_base = OTHER; note = 2'-methoxy-modified
  modified_base order(2,6,8,14,16): mod_base = OTHER; note = 2'-fluoro-modified
ttacggttccaccaggagcta

SEQ ID NO: 916 - RNA, 21 nt, synthetic construct
  source 1..21: mol_type = other RNA; note = GPSZRA274S2 antisense strand
  modified_base order(1^2,2^3,19^20,20^21): mod_base = OTHER; note = phosphorothioate linkage
  modified_base order(1,3,4,5,7,9,10,11,12,13,15,17,18,19,20,21): mod_base = OTHER; note = 2'-methoxy-modified
  modified_base order(2,6,8,14,16): mod_base = OTHER; note = 2'-fluoro-modified
ggttacggttccaccaggagc

SEQ ID NO: 917 - RNA, 21 nt, synthetic construct
  source 1..21: mol_type = other RNA; note = GPSZRA275S2 antisense strand
  modified_base order(1^2,2^3,19^20,20^21): mod_base = OTHER; note = phosphorothioate linkage
  modified_base order(1,3,4,5,7,9,10,11,12,13,15,17,18,19,20,21): mod_base = OTHER; note = 2'-methoxy-modified
  modified_base order(2,6,8,14,16): mod_base = OTHER; note = 2'-fluoro-modified
agggttacggttccaccagga

SEQ ID NO: 918 - RNA, 21 nt, synthetic construct
  source 1..21: mol_type = other RNA; note = GPSZRA276S2 antisense strand
  modified_base order(1^2,2^3,19^20,20^21): mod_base = OTHER; note = phosphorothioate linkage
  modified_base order(1,3,4,5,7,9,10,11,12,13,15,17,18,19,20,21): mod_base = OTHER; note = 2'-methoxy-modified
  modified_base order(2,6,8,14,16): mod_base = OTHER; note = 2'-fluoro-modified
cagggttacggttccaccagg

SEQ ID NO: 919 - RNA, 21 nt, synthetic construct
  source 1..21: mol_type = other RNA; note = GPSZRA277S2 antisense strand
  modified_base order(1^2,2^3,19^20,20^21): mod_base = OTHER; note = phosphorothioate linkage
  modified_base order(1,3,4,5,7,9,10,11,12,13,15,17,18,19,20,21): mod_base = OTHER; note = 2'-methoxy-modified
  modified_base order(2,6,8,14,16): mod_base = OTHER; note = 2'-fluoro-modified
tcagggttacggttccaccag

SEQ ID NO: 920 - RNA, 21 nt, synthetic construct
  source 1..21: mol_type = other RNA; note = GPSZRA281S2 antisense strand
  modified_base order(1^2,2^3,19^20,20^21): mod_base = OTHER; note = phosphorothioate linkage
  modified_base order(1,3,4,5,7,9,10,11,12,13,15,17,18,19,20,21): mod_base = OTHER; note = 2'-methoxy-modified
  modified_base order(2,6,8,14,16): mod_base = OTHER; note = 2'-fluoro-modified
caggtcagggttacggttcca

SEQ ID NO: 921 - RNA, 21 nt, synthetic construct
  source 1..21: mol_type = other RNA; note = GPSZRA282S2 antisense strand
  modified_base order(1^2,2^3,19^20,20^21): mod_base = OTHER; note = phosphorothioate linkage
  modified_base order(1,3,4,5,7,9,10,11,12,13,15,17,18,19,20,21): mod_base = OTHER; note = 2'-methoxy-modified
  modified_base order(2,6,8,14,16): mod_base = OTHER; note = 2'-fluoro-modified
acaggtcagggttacggttcc

SEQ ID NO: 922 - RNA, 21 nt, synthetic construct
  source 1..21: mol_type = other RNA; note = GPSZRA283S2 antisense strand
  modified_base order(1^2,2^3,19^20,20^21): mod_base = OTHER; note = phosphorothioate linkage
  modified_base order(1,3,4,5,7,9,10,11,12,13,15,17,18,19,20,21): mod_base = OTHER; note = 2'-methoxy-modified
  modified_base order(2,6,8,14,16): mod_base = OTHER; note = 2'-fluoro-modified
cacaggtcagggttacggttc

SEQ ID NO: 923 - RNA, 21 nt, synthetic construct
  source 1..21: mol_type = other RNA; note = GPSZRA284S2 antisense strand
  modified_base order(1^2,2^3,19^20,20^21): mod_base = OTHER; note = phosphorothioate linkage
  modified_base order(1,3,4,5,7,9,10,11,12,13,15,17,18,19,20,21): mod_base = OTHER; note = 2'-methoxy-modified
  modified_base order(2,6,8,14,16): mod_base = OTHER; note = 2'-fluoro-modified
tcacaggtcagggttacggtt

SEQ ID NO: 924 - RNA, 21 nt, synthetic construct
  source 1..21: mol_type = other RNA; note = GPSZRA285S2 antisense strand
  modified_base order(1^2,2^3,19^20,20^21): mod_base = OTHER; note = phosphorothioate linkage
  modified_base order(1,3,4,5,7,9,10,11,12,13,15,17,18,19,20,21): mod_base = OTHER; note = 2'-methoxy-modified
  modified_base order(2,6,8,14,16): mod_base = OTHER; note = 2'-fluoro-modified
ttcacaggtcagggttacggt

SEQ ID NO: 925 - RNA, 21 nt, synthetic construct
  source 1..21: mol_type = other RNA; note = GPSZRA286S2 antisense strand
  modified_base order(1^2,2^3,19^20,20^21): mod_base = OTHER; note = phosphorothioate linkage
  modified_base order(1,3,4,5,7,9,10,11,12,13,15,17,18,19,20,21): mod_base = OTHER; note = 2'-methoxy-modified
  modified_base order(2,6,8,14,16): mod_base = OTHER; note = 2'-fluoro-modified
cttcacaggtcagggttacgg

SEQ ID NO: 926 - RNA, 21 nt, synthetic construct
  source 1..21: mol_type = other RNA; note = GPSZRA287S2 antisense strand
  modified_base order(1^2,2^3,19^20,20^21): mod_base = OTHER; note = phosphorothioate linkage
  modified_base order(1,3,4,5,7,9,10,11,12,13,15,17,18,19,20,21): mod_base = OTHER; note = 2'-methoxy-modified
  modified_base order(2,6,8,14,16): mod_base = OTHER; note = 2'-fluoro-modified
acttcacaggtcagggttacg

SEQ ID NO: 927 - RNA, 21 nt, synthetic construct
  source 1..21: mol_type = other RNA; note = GPSZRA288S2 antisense strand
  modified_base order(1^2,2^3,19^20,20^21): mod_base = OTHER; note = phosphorothioate linkage
  modified_base order(1,3,4,5,7,9,10,11,12,13,15,17,18,19,20,21): mod_base = OTHER; note = 2'-methoxy-modified
  modified_base order(2,6,8,14,16): mod_base = OTHER; note = 2'-fluoro-modified
gacttcacaggtcagggttac

SEQ ID NO: 928 - RNA, 21 nt, synthetic construct
  source 1..21: mol_type = other RNA; note = GPSZRA290S2 antisense strand
  modified_base order(1^2,2^3,19^20,20^21): mod_base = OTHER; note = phosphorothioate linkage
  modified_base order(1,3,4,5,7,9,10,11,12,13,15,17,18,19,20,21): mod_base = OTHER; note = 2'-methoxy-modified
  modified_base order(2,6,8,14,16): mod_base = OTHER; note = 2'-fluoro-modified
agggacttcacaggtcagggt

SEQ ID NO: 929 - RNA, 21 nt, synthetic construct
  source 1..21: mol_type = other RNA; note = GPSZRA292S2 antisense strand
  modified_base order(1^2,2^3,19^20,20^21): mod_base = OTHER; note = phosphorothioate linkage
  modified_base order(1,3,4,5,7,9,10,11,12,13,15,17,18,19,20,21): mod_base = OTHER; note = 2'-methoxy-modified
  modified_base order(2,6,8,14,16): mod_base = OTHER; note = 2'-fluoro-modified
gcagggacttcacaggtcagg

SEQ ID NO: 930 - RNA, 21 nt, synthetic construct
  source 1..21: mol_type = other RNA; note = GPSZRA301S2 antisense strand
  modified_base order(1^2,2^3,19^20,20^21): mod_base = OTHER; note = phosphorothioate linkage
  modified_base order(1,3,4,5,7,9,10,11,12,13,15,17,18,19,20,21): mod_base = OTHER; note = 2'-methoxy-modified
  modified_base order(2,6,8,14,16): mod_base = OTHER; note = 2'-fluoro-modified
tccagtggatttgaggagagg

SEQ ID NO: 931 - RNA, 21 nt, synthetic construct
  source 1..21: mol_type = other RNA; note = GPSZRA308S2 antisense strand
  modified_base order(1^2,2^3,19^20,20^21): mod_base = OTHER; note = phosphorothioate linkage
  modified_base order(1,3,4,5,7,9,10,11,12,13,15,17,18,19,20,21): mod_base = OTHER; note = 2'-methoxy-modified
  modified_base order(2,6,8,14,16): mod_base = OTHER; note = 2'-fluoro-modified
tccttcatccagtggatttga

SEQ ID NO: 932 - RNA, 21 nt, synthetic construct
  source 1..21: mol_type = other RNA; note = GPSZRA311S2 antisense strand
  modified_base order(1^2,2^3,19^20,20^21): mod_base = OTHER; note = phosphorothioate linkage
  modified_base order(1,3,4,5,7,9,10,11,12,13,15,17,18,19,20,21): mod_base = OTHER; note = 2'-methoxy-modified
  modified_base order(2,6,8,14,16): mod_base = OTHER; note = 2'-fluoro-modified
ccatccttcatccagtggatt

SEQ ID NO: 933 - RNA, 21 nt, synthetic construct
  source 1..21: mol_type = other RNA; note = GPSZRA312S2 antisense strand
  modified_base order(1^2,2^3,19^20,20^21): mod_base = OTHER; note = phosphorothioate linkage
  modified_base order(1,3,4,5,7,9,10,11,12,13,15,17,18,19,20,21): mod_base = OTHER; note = 2'-methoxy-modified
  modified_base order(2,6,8,14,16): mod_base = OTHER; note = 2'-fluoro-modified
accatccttcatccagtggat

SEQ ID NO: 934 - RNA, 21 nt, synthetic construct
  source 1..21: mol_type = other RNA; note = GPSZRA313S2 antisense strand
  modified_base order(1^2,2^3,19^20,20^21): mod_base = OTHER; note = phosphorothioate linkage
  modified_base order(1,3,4,5,7,9,10,11,12,13,15,17,18,19,20,21): mod_base = OTHER; note = 2'-methoxy-modified
  modified_base order(2,6,8,14,16): mod_base = OTHER; note = 2'-fluoro-modified
caccatccttcatccagtgga

SEQ ID NO: 935 - RNA, 21 nt, synthetic construct
  source 1..21: mol_type = other RNA; note = GPSZRA314S2 antisense strand
  modified_base order(1^2,2^3,19^20,20^21): mod_base = OTHER; note = phosphorothioate linkage
  modified_base order(1,3,4,5,7,9,10,11,12,13,15,17,18,19,20,21): mod_base = OTHER; note = 2'-methoxy-modified
  modified_base order(2,6,8,14,16): mod_base = OTHER; note = 2'-fluoro-modified
acaccatccttcatccagtgg

SEQ ID NO: 936 - RNA, 21 nt, synthetic construct
  source 1..21: mol_type = other RNA; note = GPSZRA315S2 antisense strand
  modified_base order(1^2,2^3,19^20,20^21): mod_base = OTHER; note = phosphorothioate linkage
  modified_base order(1,3,4,5,7,9,10,11,12,13,15,17,18,19,20,21): mod_base = OTHER; note = 2'-methoxy-modified
  modified_base order(2,6,8,14,16): mod_base = OTHER; note = 2'-fluoro-modified
cacaccatccttcatccagtg

SEQ ID NO: 937 - RNA, 21 nt, synthetic construct
  source 1..21: mol_type = other RNA; note = GPSZRA316S2 antisense strand
  modified_base order(1^2,2^3,19^20,20^21): mod_base = OTHER; note = phosphorothioate linkage
  modified_base order(1,3,4,5,7,9,10,11,12,13,15,17,18,19,20,21): mod_base = OTHER; note = 2'-methoxy-modified
  modified_base order(2,6,8,14,16): mod_base = OTHER; note = 2'-fluoro-modified
gcacaccatccttcatccagt

SEQ ID NO: 938 - RNA, 21 nt, synthetic construct
  source 1..21: mol_type = other RNA; note = GPSZRA317S2 antisense strand
  modified_base order(1^2,2^3,19^20,20^21): mod_base = OTHER; note = phosphorothioate linkage
  modified_base order(1,3,4,5,7,9,10,11,12,13,15,17,18,19,20,21): mod_base = OTHER; note = 2'-methoxy-modified
  modified_base order(2,6,8,14,16): mod_base = OTHER; note = 2'-fluoro-modified
ggcacaccatccttcatccag

SEQ ID NO: 939 - RNA, 21 nt, synthetic construct
  source 1..21: mol_type = other RNA; note = GPSZRA318S2 antisense strand
  modified_base order(1^2,2^3,19^20,20^21): mod_base = OTHER; note = phosphorothioate linkage
  modified_base order(1,3,4,5,7,9,10,11,12,13,15,17,18,19,20,21): mod_base = OTHER; note = 2'-methoxy-modified
  modified_base order(2,6,8,14,16): mod_base = OTHER; note = 2'-fluoro-modified
gggcacaccatccttcatcca

SEQ ID NO: 940 - RNA, 21 nt, synthetic construct
  source 1..21: mol_type = other RNA; note = GPSZRA320S2 antisense strand
  modified_base order(1^2,2^3,19^20,20^21): mod_base = OTHER; note = phosphorothioate linkage
  modified_base order(1,3,4,5,7,9,10,11,12,13,15,17,18,19,20,21): mod_base = OTHER; note = 2'-methoxy-modified
  modified_base order(2,6,8,14,16): mod_base = OTHER; note = 2'-fluoro-modified
aagggcacaccatccttcatc

SEQ ID NO: 941 - RNA, 21 nt, synthetic construct
  source 1..21: mol_type = other RNA; note = GPSZRA333S2 antisense strand
  modified_base order(1^2,2^3,19^20,20^21): mod_base = OTHER; note = phosphorothioate linkage
  modified_base order(1,3,4,5,7,9,10,11,12,13,15,17,18,19,20,21): mod_base = OTHER; note = 2'-methoxy-modified
  modified_base order(2,6,8,14,16): mod_base = OTHER; note = 2'-fluoro-modified
tgctgacagcacggctttcct

SEQ ID NO: 942 - RNA, 21 nt, synthetic construct
  source 1..21: mol_type = other RNA; note = GPSZRA342S2 antisense strand
  modified_base order(1^2,2^3,19^20,20^21): mod_base = OTHER; note = phosphorothioate linkage
  modified_base order(1,3,4,5,7,9,10,11,12,13,15,17,18,19,20,21): mod_base = OTHER; note = 2'-methoxy-modified
  modified_base order(2,6,8,14,16): mod_base = OTHER; note = 2'-fluoro-modified
gatgatgctgatgctgacagc

SEQ ID NO: 943 - RNA, 21 nt, synthetic construct
  source 1..21: mol_type = other RNA; note = GPSZRA378S2 antisense strand
  modified_base order(1^2,2^3,19^20,20^21): mod_base = OTHER; note = phosphorothioate linkage
  modified_base order(1,3,4,5,7,9,10,11,12,13,15,17,18,19,20,21): mod_base = OTHER; note = 2'-methoxy-modified
  modified_base order(2,6,8,14,16): mod_base = OTHER; note = 2'-fluoro-modified
tctgcacgctcctcctcttcc

SEQ ID NO: 944 - RNA, 21 nt, synthetic construct
  source 1..21: mol_type = other RNA; note = GPSZRA379S2 antisense strand
  modified_base order(1^2,2^3,19^20,20^21): mod_base = OTHER; note = phosphorothioate linkage
  modified_base order(1,3,4,5,7,9,10,11,12,13,15,17,18,19,20,21): mod_base = OTHER; note = 2'-methoxy-modified
  modified_base order(2,6,8,14,16): mod_base = OTHER; note = 2'-fluoro-modified
aggttcctccgactgattcag

SEQ ID NO: 945 - RNA, 21 nt, synthetic construct
  source 1..21: mol_type = other RNA; note = GPSZRA380S2 antisense strand
  modified_base order(1^2,2^3,19^20,20^21): mod_base = OTHER; note = phosphorothioate linkage
  modified_base order(1,3,4,5,7,9,10,11,12,13,15,17,18,19,20,21): mod_base = OTHER; note = 2'-methoxy-modified
  modified_base order(2,6,8,14,16): mod_base = OTHER; note = 2'-fluoro-modified
caggttcctccgactgattca

SEQ ID NO: 946 - RNA, 21 nt, synthetic construct
  source 1..21: mol_type = other RNA; note = GPSZRA381S2 antisense strand
  modified_base order(1^2,2^3,19^20,20^21): mod_base = OTHER; note = phosphorothioate linkage
  modified_base order(1,3,4,5,7,9,10,11,12,13,15,17,18,19,20,21): mod_base = OTHER; note = 2'-methoxy-modified
  modified_base order(2,6,8,14,16): mod_base = OTHER; note = 2'-fluoro-modified
tcaggttcctccgactgattc

SEQ ID NO: 947 - RNA, 21 nt, synthetic construct
  source 1..21: mol_type = other RNA; note = GPSZRA402S2 antisense strand
  modified_base order(1^2,2^3,19^20,20^21): mod_base = OTHER; note = phosphorothioate linkage
  modified_base order(1,3,4,5,7,9,10,11,12,13,15,17,18,19,20,21): mod_base = OTHER; note = 2'-methoxy-modified
  modified_base order(2,6,8,14,16): mod_base = OTHER; note = 2'-fluoro-modified
ttatacaggagagagttggtc

SEQ ID NO: 948 - RNA, 21 nt, synthetic construct
  source 1..21: mol_type = other RNA; note = GPSZRA407S2 antisense strand
  modified_base order(1^2,2^3,19^20,20^21): mod_base = OTHER; note = phosphorothioate linkage
  modified_base order(1,3,4,5,7,9,10,11,12,13,15,17,18,19,20,21): mod_base = OTHER; note = 2'-methoxy-modified
  modified_base order(2,6,8,14,16): mod_base = OTHER; note = 2'-fluoro-modified
caaggtggggttatacaggag

SEQ ID NO: 949 - RNA, 21 nt, synthetic construct
  source 1..21: mol_type = other RNA; note = GPSZRA408S2 antisense strand
  modified_base order(1^2,2^3,19^20,20^21): mod_base = OTHER; note = phosphorothioate linkage
  modified_base order(1,3,4,5,7,9,10,11,12,13,15,17,18,19,20,21): mod_base = OTHER; note = 2'-methoxy-modified
  modified_base order(2,6,8,14,16): mod_base = OTHER; note = 2'-fluoro-modified
gcaaggtggggttatacagga

SEQ ID NO: 950 - RNA, 21 nt, synthetic construct
  source 1..21: mol_type = other RNA; note = GPSZRA409S2 antisense strand
  modified_base order(1^2,2^3,19^20,20^21): mod_base = OTHER; note = phosphorothioate linkage
  modified_base order(1,3,4,5,7,9,10,11,12,13,15,17,18,19,20,21): mod_base = OTHER; note = 2'-methoxy-modified
  modified_base order(2,6,8,14,16): mod_base = OTHER; note = 2'-fluoro-modified
ggcaaggtggggttatacagg

SEQ ID NO: 951 - RNA, 21 nt, synthetic construct
  source 1..21: mol_type = other RNA; note = GPSZRA410S2 antisense strand
  modified_base order(1^2,2^3,19^20,20^21): mod_base = OTHER; note = phosphorothioate linkage
  modified_base order(1,3,4,5,7,9,10,11,12,13,15,17,18,19,20,21): mod_base = OTHER; note = 2'-methoxy-modified
  modified_base order(2,6,8,14,16): mod_base = OTHER; note = 2'-fluoro-modified
tggcaaggtggggttatacag

SEQ ID NO: 952 - RNA, 21 nt, synthetic construct
  source 1..21: mol_type = other RNA; note = GPSZRA411S2 antisense strand
  modified_base order(1^2,2^3,19^20,20^21): mod_base = OTHER; note = phosphorothioate linkage
  modified_base order(1,3,4,5,7,9,10,11,12,13,15,17,18,19,20,21): mod_base = OTHER; note = 2'-methoxy-modified
  modified_base order(2,6,8,14,16): mod_base = OTHER; note = 2'-fluoro-modified
ttggcaaggtggggttataca

SEQ ID NO: 953 - RNA, 21 nt, synthetic construct
  source 1..21: mol_type = other RNA; note = GPSZRA084S3 antisense strand
  modified_base order(1^2,2^3,19^20,20^21): mod_base = OTHER; note = phosphorothioate linkage
  modified_base order(1,3,4,5,7,8,9,10,11,12,13,15,17,18,19,20,21): mod_base = OTHER; note = 2'-methoxy-modified
  modified_base order(2,6,14,16): mod_base = OTHER; note = 2'-fluoro-modified
tggacttggtctcctttccat

SEQ ID NO: 954 - RNA, 21 nt, synthetic construct
  source 1..21: mol_type = other RNA; note = GPSZRA087S3 antisense strand
  modified_base order(1^2,2^3,19^20,20^21): mod_base = OTHER; note = phosphorothioate linkage
  modified_base order(1,3,4,5,7,8,9,10,11,12,13,15,17,18,19,20,21): mod_base = OTHER; note = 2'-methoxy-modified
  modified_base order(2,6,14,16): mod_base = OTHER; note = 2'-fluoro-modified
agttggacttggtctcctttc

SEQ ID NO: 955 - RNA, 21 nt, synthetic construct
  source 1..21: mol_type = other RNA; note = GPSZRA092S3 antisense strand
  modified_base order(1^2,2^3,19^20,20^21): mod_base = OTHER; note = phosphorothioate linkage
  modified_base order(1,3,4,5,7,8,9,10,11,12,13,15,17,18,19,20,21): mod_base = OTHER; note = 2'-methoxy-modified
  modified_base order(2,6,14,16): mod_base = OTHER; note = 2'-fluoro-modified
tcggtagttggacttggtctc

SEQ ID NO: 956 - RNA, 21 nt, synthetic construct
  source 1..21: mol_type = other RNA; note = GPSZRA093S3 antisense strand
  modified_base order(1^2,2^3,19^20,20^21): mod_base = OTHER; note = phosphorothioate linkage
  modified_base order(1,3,4,5,7,8,9,10,11,12,13,15,17,18,19,20,21): mod_base = OTHER; note = 2'-methoxy-modified
  modified_base order(2,6,14,16): mod_base = OTHER; note = 2'-fluoro-modified
ctcggtagttggacttggtct

SEQ ID NO: 957 - RNA, 21 nt, synthetic construct
  source 1..21: mol_type = other RNA; note = GPSZRA097S3 antisense strand
  modified_base order(1^2,2^3,19^20,20^21): mod_base = OTHER; note = phosphorothioate linkage
  modified_base order(1,3,4,5,7,8,9,10,11,12,13,15,17,18,19,20,21): mod_base = OTHER; note = 2'-methoxy-modified
  modified_base order(2,6,14,16): mod_base = OTHER; note = 2'-fluoro-modified
cggactcggtagttggacttg

SEQ ID NO: 958 - RNA, 21 nt, synthetic construct
  source 1..21: mol_type = other RNA; note = GPSZRA118S3 antisense strand
  modified_base order(1^2,2^3,19^20,20^21): mod_base = OTHER; note = phosphorothioate linkage
  modified_base order(1,3,4,5,7,8,9,10,11,12,13,15,17,18,19,20,21): mod_base = OTHER; note = 2'-methoxy-modified
  modified_base order(2,6,14,16): mod_base = OTHER; note = 2'-fluoro-modified
cttcccaggaatctggtagac

SEQ ID NO: 959 - RNA, 21 nt, synthetic construct
  source 1..21: mol_type = other RNA; note = GPSZRA217S3 antisense strand
  modified_base order(1^2,2^3,19^20,20^21): mod_base = OTHER; note = phosphorothioate linkage
  modified_base order(1,3,4,5,7,8,9,10,11,12,13,15,17,18,19,20,21): mod_base = OTHER; note = 2'-methoxy-modified
  modified_base order(2,6,14,16): mod_base = OTHER; note = 2'-fluoro-modified
tccttcacagatactcccttc

SEQ ID NO: 960 - RNA, 21 nt, synthetic construct
  source 1..21: mol_type = other RNA; note = GPSZRA222S3 antisense strand
  modified_base order(1^2,2^3,19^20,20^21): mod_base = OTHER; note = phosphorothioate linkage
  modified_base order(1,3,4,5,7,8,9,10,11,12,13,15,17,18,19,20,21): mod_base = OTHER; note = 2'-methoxy-modified
  modified_base order(2,6,14,16): mod_base = OTHER; note = 2'-fluoro-modified
tccgactgcagtgtgaagagc

SEQ ID NO: 961 - RNA, 21 nt, synthetic construct
  source 1..21: mol_type = other RNA; note = GPSZRA227S3 antisense strand
  modified_base order(1^2,2^3,19^20,20^21): mod_base = OTHER; note = phosphorothioate linkage
  modified_base order(1,3,4,5,7,8,9,10,11,12,13,15,17,18,19,20,21): mod_base = OTHER; note = 2'-methoxy-modified
  modified_base order(2,6,14,16): mod_base = OTHER; note = 2'-fluoro-modified
ttagctccgactgcagtgtga

SEQ ID NO: 962 - RNA, 21 nt, synthetic construct
  source 1..21: mol_type = other RNA; note = GPSZRA228S3 antisense strand
  modified_base order(1^2,2^3,19^20,20^21): mod_base = OTHER; note = phosphorothioate linkage
  modified_base order(1,3,4,5,7,8,9,10,11,12,13,15,17,18,19,20,21): mod_base = OTHER; note = 2'-methoxy-modified
  modified_base order(2,6,14,16): mod_base = OTHER; note = 2'-fluoro-modified
attagctccgactgcagtgtg

SEQ ID NO: 963 - RNA, 21 nt, synthetic construct
  source 1..21: mol_type = other RNA; note = GPSZRA229S3 antisense strand
  modified_base order(1^2,2^3,19^20,20^21): mod_base = OTHER; note = phosphorothioate linkage
  modified_base order(1,3,4,5,7,8,9,10,11,12,13,15,17,18,19,20,21): mod_base = OTHER; note = 2'-methoxy-modified
  modified_base order(2,6,14,16): mod_base = OTHER; note = 2'-fluoro-modified
cattagctccgactgcagtgt

SEQ ID NO: 964 - RNA, 21 nt, synthetic construct
  source 1..21: mol_type = other RNA; note = GPSZRA231S3 antisense strand
  modified_base order(1^2,2^3,19^20,20^21): mod_base = OTHER; note = phosphorothioate linkage
  modified_base order(1,3,4,5,7,8,9,10,11,12,13,15,17,18,19,20,21): mod_base = OTHER; note = 2'-methoxy-modified
  modified_base order(2,6,14,16): mod_base = OTHER; note = 2'-fluoro-modified
accattagctccgactgcagt

SEQ ID NO: 965 - RNA, 21 nt, synthetic construct
  source 1..21: mol_type = other RNA; note = GPSZRA232S3 antisense strand
  modified_base order(1^2,2^3,19^20,20^21): mod_base = OTHER; note = phosphorothioate linkage
  modified_base order(1,3,4,5,7,8,9,10,11,12,13,15,17,18,19,20,21): mod_base = OTHER; note = 2'-methoxy-modified
  modified_base order(2,6,14,16): mod_base = OTHER; note = 2'-fluoro-modified
caccattagctccgactgcag

SEQ ID NO: 966 - RNA, 21 nt, synthetic construct
  source 1..21: mol_type = other RNA; note = GPSZRA233S3 antisense strand
  modified_base order(1^2,2^3,19^20,20^21): mod_base = OTHER; note = phosphorothioate linkage
  modified_base order(1,3,4,5,7,8,9,10,11,12,13,15,17,18,19,20,21): mod_base = OTHER; note = 2'-methoxy-modified
  modified_base order(2,6,14,16): mod_base = OTHER; note = 2'-fluoro-modified
tcaccattagctccgactgca

SEQ ID NO: 967 - RNA, 21 nt, synthetic construct
  source 1..21: mol_type = other RNA; note = GPSZRA252S3 antisense strand
  modified_base order(1^2,2^3,19^20,20^21): mod_base = OTHER; note = phosphorothioate linkage
  modified_base order(1,3,4,5,7,8,9,10,11,12,13,15,17,18,19,20,21): mod_base = OTHER; note = 2'-methoxy-modified
  modified_base order(2,6,14,16): mod_base = OTHER; note = 2'-fluoro-modified
caattggacctcctccagagg

SEQ ID NO: 968 - RNA, 21 nt, synthetic construct
  source 1..21: mol_type = other RNA; note = GPSZRA257S3 antisense strand
  modified_base order(1^2,2^3,19^20,20^21): mod_base = OTHER; note = phosphorothioate linkage
  modified_base order(1,3,4,5,7,8,9,10,11,12,13,15,17,18,19,20,21): mod_base = OTHER; note = 2'-methoxy-modified
  modified_base order(2,6,14,16): mod_base = OTHER; note = 2'-fluoro-modified
accaccaattggacctcctcc

SEQ ID NO: 969 - RNA, 21 nt, synthetic construct
  source 1..21: mol_type = other RNA; note = GPSZRA266S3 antisense strand
  modified_base order(1^2,2^3,19^20,20^21): mod_base = OTHER; note = phosphorothioate linkage
  modified_base order(1,3,4,5,7,8,9,10,11,12,13,15,17,18,19,20,21): mod_base = OTHER; note = 2'-methoxy-modified
  modified_base order(2,6,14,16): mod_base = OTHER; note = 2'-fluoro-modified
tccaccaggagctactgctcc

SEQ ID NO: 970 - RNA, 21 nt, synthetic construct
  source 1..21: mol_type = other RNA; note = GPSZRA267S3 antisense strand
  modified_base order(1^2,2^3,19^20,20^21): mod_base = OTHER; note = phosphorothioate linkage
  modified_base order(1,3,4,5,7,8,9,10,11,12,13,15,17,18,19,20,21): mod_base = OTHER; note = 2'-methoxy-modified
  modified_base order(2,6,14,16): mod_base = OTHER; note = 2'-fluoro-modified
ttccaccaggagctactgctc

SEQ ID NO: 971 - RNA, 21 nt, synthetic construct
  source 1..21: mol_type = other RNA; note = GPSZRA271S3 antisense strand
  modified_base order(1^2,2^3,19^20,20^21): mod_base = OTHER; note = phosphorothioate linkage
  modified_base order(1,3,4,5,7,8,9,10,11,12,13,15,17,18,19,20,21): mod_base = OTHER; note = 2'-methoxy-modified
  modified_base order(2,6,14,16): mod_base = OTHER; note = 2'-fluoro-modified
tacggttccaccaggagctac

SEQ ID NO: 972 - RNA, 21 nt, synthetic construct
  source 1..21: mol_type = other RNA; note = GPSZRA272S3 antisense strand
  modified_base order(1^2,2^3,19^20,20^21): mod_base = OTHER; note = phosphorothioate linkage
  modified_base order(1,3,4,5,7,8,9,10,11,12,13,15,17,18,19,20,21): mod_base = OTHER; note = 2'-methoxy-modified
  modified_base order(2,6,14,16): mod_base = OTHER; note = 2'-fluoro-modified
ttacggttccaccaggagcta

SEQ ID NO: 973 - RNA, 21 nt, synthetic construct
  source 1..21: mol_type = other RNA; note = GPSZRA274S3 antisense strand
  modified_base order(1^2,2^3,19^20,20^21): mod_base = OTHER; note = phosphorothioate linkage
  modified_base order(1,3,4,5,7,8,9,10,11,12,13,15,17,18,19,20,21): mod_base = OTHER; note = 2'-methoxy-modified
  modified_base order(2,6,14,16): mod_base = OTHER; note = 2'-fluoro-modified
ggttacggttccaccaggagc

SEQ ID NO: 974 - RNA, 21 nt, synthetic construct
  source 1..21: mol_type = other RNA; note = GPSZRA275S3 antisense strand
  modified_base order(1^2,2^3,19^20,20^21): mod_base = OTHER; note = phosphorothioate linkage
  modified_base order(1,3,4,5,7,8,9,10,11,12,13,15,17,18,19,20,21): mod_base = OTHER; note = 2'-methoxy-modified
  modified_base order(2,6,14,16): mod_base = OTHER; note = 2'-fluoro-modified
agggttacggttccaccagga

SEQ ID NO: 975 - RNA, 21 nt, synthetic construct
  source 1..21: mol_type = other RNA; note = GPSZRA276S3 antisense strand
  modified_base order(1^2,2^3,19^20,20^21): mod_base = OTHER; note = phosphorothioate linkage
  modified_base order(1,3,4,5,7,8,9,10,11,12,13,15,17,18,19,20,21): mod_base = OTHER; note = 2'-methoxy-modified
  modified_base order(2,6,14,16): mod_base = OTHER; note = 2'-fluoro-modified
cagggttacggttccaccagg

SEQ ID NO: 976 - RNA, 21 nt, synthetic construct
  source 1..21: mol_type = other RNA; note = GPSZRA277S3 antisense strand
  modified_base order(1^2,2^3,19^20,20^21): mod_base = OTHER; note = phosphorothioate linkage
  modified_base order(1,3,4,5,7,8,9,10,11,12,13,15,17,18,19,20,21): mod_base = OTHER; note = 2'-methoxy-modified
  modified_base order(2,6,14,16): mod_base = OTHER; note = 2'-fluoro-modified
tcagggttacggttccaccag

SEQ ID NO: 977 - RNA, 21 nt, synthetic construct
  source 1..21: mol_type = other RNA; note = GPSZRA281S3 antisense strand
  modified_base order(1^2,2^3,19^20,20^21): mod_base = OTHER; note = phosphorothioate linkage
  modified_base order(1,3,4,5,7,8,9,10,11,12,13,15,17,18,19,20,21): mod_base = OTHER; note = 2'-methoxy-modified
  modified_base order(2,6,14,16): mod_base = OTHER; note = 2'-fluoro-modified
caggtcagggttacggttcca

SEQ ID NO: 978 - RNA, 21 nt, synthetic construct
  source 1..21: mol_type = other RNA; note = GPSZRA282S3 antisense strand
  modified_base order(1^2,2^3,19^20,20^21): mod_base = OTHER; note = phosphorothioate linkage
  modified_base order(1,3,4,5,7,8,9,10,11,12,13,15,17,18,19,20,21): mod_base = OTHER; note = 2'-methoxy-modified
  modified_base order(2,6,14,16): mod_base = OTHER; note = 2'-fluoro-modified
acaggtcagggttacggttcc

SEQ ID NO: 979 - RNA, 21 nt, synthetic construct
  source 1..21: mol_type = other RNA; note = GPSZRA283S3 antisense strand
  modified_base order(1^2,2^3,19^20,20^21): mod_base = OTHER; note = phosphorothioate linkage
  modified_base order(1,3,4,5,7,8,9,10,11,12,13,15,17,18,19,20,21): mod_base = OTHER; note = 2'-methoxy-modified
  modified_base order(2,6,14,16): mod_base = OTHER; note = 2'-fluoro-modified
cacaggtcagggttacggttc

SEQ ID NO: 980 - RNA, 21 nt, synthetic construct
  source 1..21: mol_type = other RNA; note = GPSZRA284S3 antisense strand
  modified_base order(1^2,2^3,19^20,20^21): mod_base = OTHER; note = phosphorothioate linkage
  modified_base order(1,3,4,5,7,8,9,10,11,12,13,15,17,18,19,20,21): mod_base = OTHER; note = 2'-methoxy-modified
  modified_base order(2,6,14,16): mod_base = OTHER; note = 2'-fluoro-modified
tcacaggtcagggttacggtt

SEQ ID NO: 981 - RNA, 21 nt, synthetic construct
  source 1..21: mol_type = other RNA; note = GPSZRA285S3 antisense strand
  modified_base order(1^2,2^3,19^20,20^21): mod_base = OTHER; note = phosphorothioate linkage
  modified_base order(1,3,4,5,7,8,9,10,11,12,13,15,17,18,19,20,21): mod_base = OTHER; note = 2'-methoxy-modified
  modified_base order(2,6,14,16): mod_base = OTHER; note = 2'-fluoro-modified
ttcacaggtcagggttacggt

SEQ ID NO: 982 - RNA, 21 nt, synthetic construct
  source 1..21: mol_type = other RNA; note = GPSZRA286S3 antisense strand
  modified_base order(1^2,2^3,19^20,20^21): mod_base = OTHER; note = phosphorothioate linkage
  modified_base order(1,3,4,5,7,8,9,10,11,12,13,15,17,18,19,20,21): mod_base = OTHER; note = 2'-methoxy-modified
  modified_base order(2,6,14,16): mod_base = OTHER; note = 2'-fluoro-modified
cttcacaggtcagggttacgg

SEQ ID NO: 983 - RNA, 21 nt, synthetic construct
  source 1..21: mol_type = other RNA; note = GPSZRA287S3 antisense strand
  modified_base order(1^2,2^3,19^20,20^21): mod_base = OTHER; note = phosphorothioate linkage
  modified_base order(1,3,4,5,7,8,9,10,11,12,13,15,17,18,19,20,21): mod_base = OTHER; note = 2'-methoxy-modified
  modified_base order(2,6,14,16): mod_base = OTHER; note = 2'-fluoro-modified
acttcacaggtcagggttacg

SEQ ID NO: 984 - RNA, 21 nt, synthetic construct
  source 1..21: mol_type = other RNA; note = GPSZRA288S3 antisense strand
  modified_base order(1^2,2^3,19^20,20^21): mod_base = OTHER; note = phosphorothioate linkage
  modified_base order(1,3,4,5,7,8,9,10,11,12,13,15,17,18,19,20,21): mod_base = OTHER; note = 2'-methoxy-modified
  modified_base order(2,6,14,16): mod_base = OTHER; note = 2'-fluoro-modified
gacttcacaggtcagggttac

SEQ ID NO: 985 - RNA, 21 nt, synthetic construct
  source 1..21: mol_type = other RNA; note = GPSZRA290S3 antisense strand
  modified_base order(1^2,2^3,19^20,20^21): mod_base = OTHER; note = phosphorothioate linkage
  modified_base order(1,3,4,5,7,8,9,10,11,12,13,15,17,18,19,20,21): mod_base = OTHER; note = 2'-methoxy-modified
  modified_base order(2,6,14,16): mod_base = OTHER; note = 2'-fluoro-modified
agggacttcacaggtcagggt

SEQ ID NO: 986 - RNA, 21 nt, synthetic construct
  source 1..21: mol_type = other RNA; note = GPSZRA292S3 antisense strand
  modified_base order(1^2,2^3,19^20,20^21): mod_base = OTHER; note = phosphorothioate linkage
  modified_base order(1,3,4,5,7,8,9,10,11,12,13,15,17,18,19,20,21): mod_base = OTHER; note = 2'-methoxy-modified
  modified_base order(2,6,14,16): mod_base = OTHER; note = 2'-fluoro-modified
gcagggacttcacaggtcagg

SEQ ID NO: 987 - RNA, 21 nt, synthetic construct
  source 1..21: mol_type = other RNA; note = GPSZRA301S3 antisense strand
  modified_base order(1^2,2^3,19^20,20^21): mod_base = OTHER; note = phosphorothioate linkage
  modified_base order(1,3,4,5,7,8,9,10,11,12,13,15,17,18,19,20,21): mod_base = OTHER; note = 2'-methoxy-modified
  modified_base order(2,6,14,16): mod_base = OTHER; note = 2'-fluoro-modified
tccagtggatttgaggagagg

SEQ ID NO: 988 - RNA, 21 nt, synthetic construct
  source 1..21: mol_type = other RNA; note = GPSZRA308S3 antisense strand
  modified_base order(1^2,2^3,19^20,20^21): mod_base = OTHER; note = phosphorothioate linkage
  modified_base order(1,3,4,5,7,8,9,10,11,12,13,15,17,18,19,20,21): mod_base = OTHER; note = 2'-methoxy-modified
  modified_base order(2,6,14,16): mod_base = OTHER; note = 2'-fluoro-modified
tccttcatccagtggatttga

SEQ ID NO: 989 - RNA, 21 nt, synthetic construct
  source 1..21: mol_type = other RNA; note = GPSZRA311S3 antisense strand
  modified_base order(1^2,2^3,19^20,20^21): mod_base = OTHER; note = phosphorothioate linkage
  modified_base order(1,3,4,5,7,8,9,10,11,12,13,15,17,18,19,20,21): mod_base = OTHER; note = 2'-methoxy-modified
  modified_base order(2,6,14,16): mod_base = OTHER; note = 2'-fluoro-modified
ccatccttcatccagtggatt

SEQ ID NO: 990 - RNA, 21 nt, synthetic construct
  source 1..21: mol_type = other RNA; note = GPSZRA312S3 antisense strand
  modified_base order(1^2,2^3,19^20,20^21): mod_base = OTHER; note = phosphorothioate linkage
  modified_base order(1,3,4,5,7,8,9,10,11,12,13,15,17,18,19,20,21): mod_base = OTHER; note = 2'-methoxy-modified
  modified_base order(2,6,14,16): mod_base = OTHER; note = 2'-fluoro-modified
accatccttcatccagtggat

SEQ ID NO: 991 - RNA, 21 nt, synthetic construct
  source 1..21: mol_type = other RNA; note = GPSZRA313S3 antisense strand
  modified_base order(1^2,2^3,19^20,20^21): mod_base = OTHER; note = phosphorothioate linkage
  modified_base order(1,3,4,5,7,8,9,10,11,12,13,15,17,18,19,20,21): mod_base = OTHER; note = 2'-methoxy-modified
  modified_base order(2,6,14,16): mod_base = OTHER; note = 2'-fluoro-modified
caccatccttcatccagtgga

SEQ ID NO: 992 - RNA, 21 nt, synthetic construct
  source 1..21: mol_type = other RNA; note = GPSZRA314S3 antisense strand
  modified_base order(1^2,2^3,19^20,20^21): mod_base = OTHER; note = phosphorothioate linkage
  modified_base order(1,3,4,5,7,8,9,10,11,12,13,15,17,18,19,20,21): mod_base = OTHER; note = 2'-methoxy-modified
  modified_base order(2,6,14,16): mod_base = OTHER; note = 2'-fluoro-modified
acaccatccttcatccagtgg

SEQ ID NO: 993 - RNA, 21 nt, synthetic construct
  source 1..21: mol_type = other RNA; note = GPSZRA315S3 antisense strand
  modified_base order(1^2,2^3,19^20,20^21): mod_base = OTHER; note = phosphorothioate linkage
  modified_base order(1,3,4,5,7,8,9,10,11,12,13,15,17,18,19,20,21): mod_base = OTHER; note = 2'-methoxy-modified
  modified_base order(2,6,14,16): mod_base = OTHER; note = 2'-fluoro-modified
cacaccatccttcatccagtg

SEQ ID NO: 994 - RNA, 21 nt, synthetic construct
  source 1..21: mol_type = other RNA; note = GPSZRA316S3 antisense strand
  modified_base order(1^2,2^3,19^20,20^21): mod_base = OTHER; note = phosphorothioate linkage
  modified_base order(1,3,4,5,7,8,9,10,11,12,13,15,17,18,19,20,21): mod_base = OTHER; note = 2'-methoxy-modified
  modified_base order(2,6,14,16): mod_base = OTHER; note = 2'-fluoro-modified
gcacaccatccttcatccagt

SEQ ID NO: 995 - RNA, 21 nt, synthetic construct
  source 1..21: mol_type = other RNA; note = GPSZRA317S3 antisense strand
  modified_base order(1^2,2^3,19^20,20^21): mod_base = OTHER; note = phosphorothioate linkage
  modified_base order(1,3,4,5,7,8,9,10,11,12,13,15,17,18,19,20,21): mod_base = OTHER; note = 2'-methoxy-modified
  modified_base order(2,6,14,16): mod_base = OTHER; note = 2'-fluoro-modified
ggcacaccatccttcatccag

SEQ ID NO: 996 - RNA, 21 nt, synthetic construct
  source 1..21: mol_type = other RNA; note = GPSZRA318S3 antisense strand
  modified_base order(1,3,4,5,7,8,9,10,11,12,13,15,17,18,19,20,21): mod_base = OTHER; note = 2'-methoxy-modified
  modified_base order(2,6,14,16): mod_base = OTHER; note = 2'-fluoro-modified
  modified_base order(1^2,2^3,19^20,20^21): mod_base = OTHER; note = phosphorothioate linkage
gggcacaccatccttcatcca

SEQ ID NO: 997 - RNA, 21 nt, synthetic construct
  source 1..21: mol_type = other RNA; note = GPSZRA320S3 antisense strand
  modified_base order(1^2,2^3,19^20,20^21): mod_base = OTHER; note = phosphorothioate linkage
  modified_base order(1,3,4,5,7,8,9,10,11,12,13,15,17,18,19,20,21): mod_base = OTHER; note = 2'-methoxy-modified
  modified_base order(2,6,14,16): mod_base = OTHER; note = 2'-fluoro-modified
aagggcacaccatccttcatc

SEQ ID NO: 998 - RNA, 21 nt, synthetic construct
  source 1..21: mol_type = other RNA; note = GPSZRA333S3 antisense strand
  modified_base order(1^2,2^3,19^20,20^21): mod_base = OTHER; note = phosphorothioate linkage
  modified_base order(1,3,4,5,7,8,9,10,11,12,13,15,17,18,19,20,21): mod_base = OTHER; note = 2'-methoxy-modified
  modified_base order(2,6,14,16): mod_base = OTHER; note = 2'-fluoro-modified
tgctgacagcacggctttcct

SEQ ID NO: 999 - RNA, 21 nt, synthetic construct
  source 1..21: mol_type = other RNA; note = GPSZRA342S3 antisense strand
  modified_base order(1^2,2^3,19^20,20^21): mod_base = OTHER; note = phosphorothioate linkage
  modified_base order(1,3,4,5,7,8,9,10,11,12,13,15,17,18,19,20,21): mod_base = OTHER; note = 2'-methoxy-modified
  modified_base order(2,6,14,16): mod_base = OTHER; note = 2'-fluoro-modified
gatgatgctgatgctgacagc

SEQ ID NO: 1000 - RNA, 21 nt, synthetic construct
  source 1..21: mol_type = other RNA; note = GPSZRA378S3 antisense strand
  modified_base order(1^2,2^3,19^20,20^21): mod_base = OTHER; note = phosphorothioate linkage
  modified_base order(1,3,4,5,7,8,9,10,11,12,13,15,17,18,19,20,21): mod_base = OTHER; note = 2'-methoxy-modified
  modified_base order(2,6,14,16): mod_base = OTHER; note = 2'-fluoro-modified
tctgcacgctcctcctcttcc

SEQ ID NO: 1001 - RNA, 21 nt, synthetic construct
  source 1..21: mol_type = other RNA; note = GPSZRA379S3 antisense strand
  modified_base order(1^2,2^3,19^20,20^21): mod_base = OTHER; note = phosphorothioate linkage
  modified_base order(1,3,4,5,7,8,9,10,11,12,13,15,17,18,19,20,21): mod_base = OTHER; note = 2'-methoxy-modified
  modified_base order(2,6,14,16): mod_base = OTHER; note = 2'-fluoro-modified
aggttcctccgactgattcag

SEQ ID NO: 1002 - RNA, 21 nt, synthetic construct
  source 1..21: mol_type = other RNA; note = GPSZRA380S3 antisense strand
  modified_base order(1^2,2^3,19^20,20^21): mod_base = OTHER; note = phosphorothioate linkage
  modified_base order(1,3,4,5,7,8,9,10,11,12,13,15,17,18,19,20,21): mod_base = OTHER; note = 2'-methoxy-modified
  modified_base order(2,6,14,16): mod_base = OTHER; note = 2'-fluoro-modified
caggttcctccgactgattca

SEQ ID NO: 1003 - RNA, 21 nt, synthetic construct
  source 1..21: mol_type = other RNA; note = GPSZRA381S3 antisense strand
  modified_base order(1^2,2^3,19^20,20^21): mod_base = OTHER; note = phosphorothioate linkage
  modified_base order(1,3,4,5,7,8,9,10,11,12,13,15,17,18,19,20,21): mod_base = OTHER; note = 2'-methoxy-modified
  modified_base order(2,6,14,16): mod_base = OTHER; note = 2'-fluoro-modified
tcaggttcctccgactgattc

SEQ ID NO: 1004 - RNA, 21 nt, synthetic construct
  source 1..21: mol_type = other RNA; note = GPSZRA402S3 antisense strand
  modified_base order(1^2,2^3,19^20,20^21): mod_base = OTHER; note = phosphorothioate linkage
  modified_base order(1,3,4,5,7,8,9,10,11,12,13,15,17,18,19,20,21): mod_base = OTHER; note = 2'-methoxy-modified
  modified_base order(2,6,14,16): mod_base = OTHER; note = 2'-fluoro-modified
ttatacaggagagagttggtc

SEQ ID NO: 1005 - RNA, 21 nt, synthetic construct
  source 1..21: mol_type = other RNA; note = GPSZRA407S3 antisense strand
  modified_base order(1^2,2^3,19^20,20^21): mod_base = OTHER; note = phosphorothioate linkage
  modified_base order(1,3,4,5,7,8,9,10,11,12,13,15,17,18,19,20,21): mod_base = OTHER; note = 2'-methoxy-modified
  modified_base order(2,6,14,16): mod_base = OTHER; note = 2'-fluoro-modified
caaggtggggttatacaggag

SEQ ID NO: 1006 - RNA, 21 nt, synthetic construct
  source 1..21: mol_type = other RNA; note = GPSZRA408S3 antisense strand
  modified_base order(1^2,2^3,19^20,20^21): mod_base = OTHER; note = phosphorothioate linkage
  modified_base order(1,3,4,5,7,8,9,10,11,12,13,15,17,18,19,20,21): mod_base = OTHER; note = 2'-methoxy-modified
  modified_base order(2,6,14,16): mod_base = OTHER; note = 2'-fluoro-modified
gcaaggtggggttatacagga

SEQ ID NO: 1007 - RNA, 21 nt, synthetic construct
  source 1..21: mol_type = other RNA; note = GPSZRA409S3 antisense strand
  modified_base order(1^2,2^3,19^20,20^21): mod_base = OTHER; note = phosphorothioate linkage
  modified_base order(1,3,4,5,7,8,9,10,11,12,13,15,17,18,19,20,21): mod_base = OTHER; note = 2'-methoxy-modified
  modified_base order(2,6,14,16): mod_base = OTHER; note = 2'-fluoro-modified
ggcaaggtggggttatacagg

SEQ ID NO: 1008 - RNA, 21 nt, synthetic construct
  source 1..21: mol_type = other RNA; note = GPSZRA410S3 antisense strand
  modified_base order(1^2,2^3,19^20,20^21): mod_base = OTHER; note = phosphorothioate linkage
  modified_base order(1,3,4,5,7,8,9,10,11,12,13,15,17,18,19,20,21): mod_base = OTHER; note = 2'-methoxy-modified
  modified_base order(2,6,14,16): mod_base = OTHER; note = 2'-fluoro-modified
tggcaaggtggggttatacag

SEQ ID NO: 1009 - RNA, 21 nt, synthetic construct
  source 1..21: mol_type = other RNA; note = GPSZRA411S3 antisense strand
  modified_base order(1^2,2^3,19^20,20^21): mod_base = OTHER; note = phosphorothioate linkage
  modified_base order(1,3,4,5,7,8,9,10,11,12,13,15,17,18,19,20,21): mod_base = OTHER; note = 2'-methoxy-modified
  modified_base order(2,6,14,16): mod_base = OTHER; note = 2'-fluoro-modified
ttggcaaggtggggttataca

SEQ ID NO: 1010 - RNA, 21 nt, synthetic construct
  source 1..21: mol_type = other RNA; note = GPSZRA084S4 antisense strand
  modified_base order(1^2,2^3,19^20,20^21): mod_base = OTHER; note = phosphorothioate linkage
  modified_base order(1,3,4,5,7,9,10,11,12,13,15,17,18,19,20,21): mod_base = OTHER; note = 2'-methoxy-modified
  modified_base order(2,6,8,14,16): mod_base = OTHER; note = 2'-fluoro-modified
tggacttggtctcctttccat

SEQ ID NO: 1011 - RNA, 21 nt, synthetic construct
  source 1..21: mol_type = other RNA; note = GPSZRA087S4 antisense strand
  modified_base order(1^2,2^3,19^20,20^21): mod_base = OTHER; note = phosphorothioate linkage
  modified_base order(1,3,4,5,7,9,10,11,12,13,15,17,18,19,20,21): mod_base = OTHER; note = 2'-methoxy-modified
  modified_base order(2,6,8,14,16): mod_base = OTHER; note = 2'-fluoro-modified
agttggacttggtctcctttc

SEQ ID NO: 1012 - RNA, 21 nt, synthetic construct
  source 1..21: mol_type = other RNA; note = GPSZRA092S4 antisense strand
  modified_base order(1^2,2^3,19^20,20^21): mod_base = OTHER; note = phosphorothioate linkage
  modified_base order(1,3,4,5,7,9,10,11,12,13,15,17,18,19,20,21): mod_base = OTHER; note = 2'-methoxy-modified
  modified_base order(2,6,8,14,16): mod_base = OTHER; note = 2'-fluoro-modified
tcggtagttggacttggtctc

SEQ ID NO: 1013 - RNA, 21 nt, synthetic construct
  source 1..21: mol_type = other RNA; note = GPSZRA093S4 antisense strand
  modified_base order(1^2,2^3,19^20,20^21): mod_base = OTHER; note = phosphorothioate linkage
  modified_base order(1,3,4,5,7,9,10,11,12,13,15,17,18,19,20,21): mod_base = OTHER; note = 2'-methoxy-modified
  modified_base order(2,6,8,14,16): mod_base = OTHER; note = 2'-fluoro-modified
ctcggtagttggacttggtct

SEQ ID NO: 1014 - RNA, 21 nt, synthetic construct
  source 1..21: mol_type = other RNA; note = GPSZRA097S4 antisense strand
  modified_base order(1^2,2^3,19^20,20^21): mod_base = OTHER; note = phosphorothioate linkage
  modified_base order(1,3,4,5,7,9,10,11,12,13,15,17,18,19,20,21): mod_base = OTHER; note = 2'-methoxy-modified
  modified_base order(2,6,8,14,16): mod_base = OTHER; note = 2'-fluoro-modified
cggactcggtagttggacttg

SEQ ID NO: 1015 - RNA, 21 nt, synthetic construct
  source 1..21: mol_type = other RNA; note = GPSZRA118S4 antisense strand
  modified_base order(1^2,2^3,19^20,20^21): mod_base = OTHER; note = phosphorothioate linkage
  modified_base order(1,3,4,5,7,9,10,11,12,13,15,17,18,19,20,21): mod_base = OTHER; note = 2'-methoxy-modified
  modified_base order(2,6,8,14,16): mod_base = OTHER; note = 2'-fluoro-modified
cttcccaggaatctggtagac

SEQ ID NO: 1016 - RNA, 21 nt, synthetic construct
  source 1..21: mol_type = other RNA; note = GPSZRA217S4 antisense strand
  modified_base order(1^2,2^3,19^20,20^21): mod_base = OTHER; note = phosphorothioate linkage
  modified_base order(1,3,4,5,7,9,10,11,12,13,15,17,18,19,20,21): mod_base = OTHER; note = 2'-methoxy-modified
  modified_base order(2,6,8,14,16): mod_base = OTHER; note = 2'-fluoro-modified
tccttcacagatactcccttc

SEQ ID NO: 1017 - RNA, 21 nt, synthetic construct
  source 1..21: mol_type = other RNA; note = GPSZRA222S4 antisense strand
  modified_base order(1^2,2^3,19^20,20^21): mod_base = OTHER; note = phosphorothioate linkage
  modified_base order(1,3,4,5,7,9,10,11,12,13,15,17,18,19,20,21): mod_base = OTHER; note = 2'-methoxy-modified
  modified_base order(2,6,8,14,16): mod_base = OTHER; note = 2'-fluoro-modified
tccgactgcagtgtgaagagc

SEQ ID NO: 1018 - RNA, 21 nt, synthetic construct
  source 1..21: mol_type = other RNA; note = GPSZRA227S4 antisense strand
  modified_base order(1^2,2^3,19^20,20^21): mod_base = OTHER; note = phosphorothioate linkage
  modified_base order(1,3,4,5,7,9,10,11,12,13,15,17,18,19,20,21): mod_base = OTHER; note = 2'-methoxy-modified
  modified_base order(2,6,8,14,16): mod_base = OTHER; note = 2'-fluoro-modified
ttagctccgactgcagtgtga

SEQ ID NO: 1019 - RNA, 21 nt, synthetic construct
  source 1..21: mol_type = other RNA; note = GPSZRA228S4 antisense strand
  modified_base order(1^2,2^3,19^20,20^21): mod_base = OTHER; note = phosphorothioate linkage
  modified_base order(1,3,4,5,7,9,10,11,12,13,15,17,18,19,20,21): mod_base = OTHER; note = 2'-methoxy-modified
  modified_base order(2,6,8,14,16): mod_base = OTHER; note = 2'-fluoro-modified
attagctccgactgcagtgtg

SEQ ID NO: 1020 - RNA, 21 nt, synthetic construct
  source 1..21: mol_type = other RNA; note = GPSZRA229S4 antisense strand
  modified_base order(1^2,2^3,19^20,20^21): mod_base = OTHER; note = phosphorothioate linkage
  modified_base order(1,3,4,5,7,9,10,11,12,13,15,17,18,19,20,21): mod_base = OTHER; note = 2'-methoxy-modified
  modified_base order(2,6,8,14,16): mod_base = OTHER; note = 2'-fluoro-modified
cattagctccgactgcagtgt

SEQ ID NO: 1021 - RNA, 21 nt, synthetic construct
  source 1..21: mol_type = other RNA; note = GPSZRA231S4 antisense strand
  modified_base order(1^2,2^3,19^20,20^21): mod_base = OTHER; note = phosphorothioate linkage
  modified_base order(1,3,4,5,7,9,10,11,12,13,15,17,18,19,20,21): mod_base = OTHER; note = 2'-methoxy-modified
  modified_base order(2,6,8,14,16): mod_base = OTHER; note = 2'-fluoro-modified
accattagctccgactgcagt

SEQ ID NO: 1022 - RNA, 21 nt, synthetic construct
  source 1..21: mol_type = other RNA; note = GPSZRA232S4 antisense strand
  modified_base order(1^2,2^3,19^20,20^21): mod_base = OTHER; note = phosphorothioate linkage
  modified_base order(1,3,4,5,7,9,10,11,12,13,15,17,18,19,20,21): mod_base = OTHER; note = 2'-methoxy-modified
  modified_base order(2,6,8,14,16): mod_base = OTHER; note = 2'-fluoro-modified
caccattagctccgactgcag

SEQ ID NO: 1023 - RNA, 21 nt, synthetic construct
  source 1..21: mol_type = other RNA; note = GPSZRA233S4 antisense strand
  modified_base order(1^2,2^3,19^20,20^21): mod_base = OTHER; note = phosphorothioate linkage
  modified_base order(1,3,4,5,7,9,10,11,12,13,15,17,18,19,20,21): mod_base = OTHER; note = 2'-methoxy-modified
  modified_base order(2,6,8,14,16): mod_base = OTHER; note = 2'-fluoro-modified
tcaccattagctccgactgca

SEQ ID NO: 1024 - RNA, 21 nt, synthetic construct
  source 1..21: mol_type = other RNA; note = GPSZRA252S4 antisense strand
  modified_base order(1^2,2^3,19^20,20^21): mod_base = OTHER; note = phosphorothioate linkage
  modified_base order(1,3,4,5,7,9,10,11,12,13,15,17,18,19,20,21): mod_base = OTHER; note = 2'-methoxy-modified
  modified_base order(2,6,8,14,16): mod_base = OTHER; note = 2'-fluoro-modified
caattggacctcctccagagg

SEQ ID NO: 1025 - RNA, 21 nt, synthetic construct
  source 1..21: mol_type = other RNA; note = GPSZRA257S4 antisense strand
  modified_base order(1^2,2^3,19^20,20^21): mod_base = OTHER; note = phosphorothioate linkage
  modified_base order(1,3,4,5,7,9,10,11,12,13,15,17,18,19,20,21): mod_base = OTHER; note = 2'-methoxy-modified
  modified_base order(2,6,8,14,16): mod_base = OTHER; note = 2'-fluoro-modified
accaccaattggacctcctcc

SEQ ID NO: 1026 - RNA, 21 nt, synthetic construct
  source 1..21: mol_type = other RNA; note = GPSZRA266S4 antisense strand
  modified_base order(1^2,2^3,19^20,20^21): mod_base = OTHER; note = phosphorothioate linkage
  modified_base order(1,3,4,5,7,9,10,11,12,13,15,17,18,19,20,21): mod_base = OTHER; note = 2'-methoxy-modified
  modified_base order(2,6,8,14,16): mod_base = OTHER; note = 2'-fluoro-modified
tccaccaggagctactgctcc

SEQ ID NO: 1027 - RNA, 21 nt, synthetic construct
  source 1..21: mol_type = other RNA; note = GPSZRA267S4 antisense strand
  modified_base order(1^2,2^3,19^20,20^21): mod_base = OTHER; note = phosphorothioate linkage
  modified_base order(1,3,4,5,7,9,10,11,12,13,15,17,18,19,20,21): mod_base = OTHER; note = 2'-methoxy-modified
  modified_base order(2,6,8,14,16): mod_base = OTHER; note = 2'-fluoro-modified
ttccaccaggagctactgctc

SEQ ID NO: 1028 - RNA, 21 nt, synthetic construct
  source 1..21: mol_type = other RNA; note = GPSZRA271S4 antisense strand
  modified_base order(1^2,2^3,19^20,20^21): mod_base = OTHER; note = phosphorothioate linkage
  modified_base order(1,3,4,5,7,9,10,11,12,13,15,17,18,19,20,21): mod_base = OTHER; note = 2'-methoxy-modified
  modified_base order(2,6,8,14,16): mod_base = OTHER; note = 2'-fluoro-modified
tacggttccaccaggagctac

SEQ ID NO: 1029 - RNA, 21 nt, synthetic construct
  source 1..21: mol_type = other RNA; note = GPSZRA272S4 antisense strand
  modified_base order(1^2,2^3,19^20,20^21): mod_base = OTHER; note = phosphorothioate linkage
  modified_base order(1,3,4,5,7,9,10,11,12,13,15,17,18,19,20,21): mod_base = OTHER; note = 2'-methoxy-modified
  modified_base order(2,6,8,14,16): mod_base = OTHER; note = 2'-fluoro-modified
ttacggttccaccaggagcta

SEQ ID NO: 1030 - RNA, 21 nt, synthetic construct
  source 1..21: mol_type = other RNA; note = GPSZRA274S4 antisense strand
  modified_base order(1^2,2^3,19^20,20^21): mod_base = OTHER; note = phosphorothioate linkage
  modified_base order(1,3,4,5,7,9,10,11,12,13,15,17,18,19,20,21): mod_base = OTHER; note = 2'-methoxy-modified
  modified_base order(2,6,8,14,16): mod_base = OTHER; note = 2'-fluoro-modified
ggttacggttccaccaggagc

SEQ ID NO: 1031 - RNA, 21 nt, synthetic construct
  source 1..21: mol_type = other RNA; note = GPSZRA275S4 antisense strand
  modified_base order(1^2,2^3,19^20,20^21): mod_base = OTHER; note = phosphorothioate linkage
  modified_base order(1,3,4,5,7,9,10,11,12,13,15,17,18,19,20,21): mod_base = OTHER; note = 2'-methoxy-modified
  modified_base order(2,6,8,14,16): mod_base = OTHER; note = 2'-fluoro-modified
agggttacggttccaccagga

SEQ ID NO: 1032 - RNA, 21 nt, synthetic construct
  source 1..21: mol_type = other RNA; note = GPSZRA276S4 antisense strand
  modified_base order(1^2,2^3,19^20,20^21): mod_base = OTHER; note = phosphorothioate linkage
  modified_base order(1,3,4,5,7,9,10,11,12,13,15,17,18,19,20,21): mod_base = OTHER; note = 2'-methoxy-modified
  modified_base order(2,6,8,14,16): mod_base = OTHER; note = 2'-fluoro-modified
cagggttacggttccaccagg

SEQ ID NO: 1033 - RNA, 21 nt, synthetic construct
  source 1..21: mol_type = other RNA; note = GPSZRA277S4 antisense strand
  modified_base order(1^2,2^3,19^20,20^21): mod_base = OTHER; note = phosphorothioate linkage
  modified_base order(1,3,4,5,7,9,10,11,12,13,15,17,18,19,20,21): mod_base = OTHER; note = 2'-methoxy-modified
  modified_base order(2,6,8,14,16): mod_base = OTHER; note = 2'-fluoro-modified
tcagggttacggttccaccag

SEQ ID NO: 1034 - RNA, 21 nt, synthetic construct
  source 1..21: mol_type = other RNA; note = GPSZRA281S4 antisense strand
  modified_base order(1^2,2^3,19^20,20^21): mod_base = OTHER; note = phosphorothioate linkage
  modified_base order(1,3,4,5,7,9,10,11,12,13,15,17,18,19,20,21): mod_base = OTHER; note = 2'-methoxy-modified
  modified_base order(2,6,8,14,16): mod_base = OTHER; note = 2'-fluoro-modified
caggtcagggttacggttcca

SEQ ID NO: 1035 - RNA, 21 nt, synthetic construct
  source 1..21: mol_type = other RNA; note = GPSZRA282S4 antisense strand
  modified_base order(1^2,2^3,19^20,20^21): mod_base = OTHER; note = phosphorothioate linkage
  modified_base order(1,3,4,5,7,9,10,11,12,13,15,17,18,19,20,21): mod_base = OTHER; note = 2'-methoxy-modified
  modified_base order(2,6,8,14,16): mod_base = OTHER; note = 2'-fluoro-modified
acaggtcagggttacggttcc

SEQ ID NO: 1036 - RNA, 21 nt, synthetic construct
  source 1..21: mol_type = other RNA; note = GPSZRA283S4 antisense strand
  modified_base order(1^2,2^3,19^20,20^21): mod_base = OTHER; note = phosphorothioate linkage
  modified_base order(1,3,4,5,7,9,10,11,12,13,15,17,18,19,20,21): mod_base = OTHER; note = 2'-methoxy-modified
  modified_base order(2,6,8,14,16): mod_base = OTHER; note = 2'-fluoro-modified
cacaggtcagggttacggttc

SEQ ID NO: 1037 - RNA, 21 nt, synthetic construct
  source 1..21: mol_type = other RNA; note = GPSZRA284S4 antisense strand
  modified_base order(1^2,2^3,19^20,20^21): mod_base = OTHER; note = phosphorothioate linkage
  modified_base order(1,3,4,5,7,9,10,11,12,13,15,17,18,19,20,21): mod_base = OTHER; note = 2'-methoxy-modified
  modified_base order(2,6,8,14,16): mod_base = OTHER; note = 2'-fluoro-modified
tcacaggtcagggttacggtt

SEQ ID NO: 1038 - RNA, 21 nt, synthetic construct
  source 1..21: mol_type = other RNA; note = GPSZRA285S4 antisense strand
  modified_base order(1^2,2^3,19^20,20^21): mod_base = OTHER; note = phosphorothioate linkage
  modified_base order(1,3,4,5,7,9,10,11,12,13,15,17,18,19,20,21): mod_base = OTHER; note = 2'-methoxy-modified
  modified_base order(2,6,8,14,16): mod_base = OTHER; note = 2'-fluoro-modified
ttcacaggtcagggttacggt

SEQ ID NO: 1039 - RNA, 21 nt, synthetic construct
  source 1..21: mol_type = other RNA; note = GPSZRA286S4 antisense strand
  modified_base order(1^2,2^3,19^20,20^21): mod_base = OTHER; note = phosphorothioate linkage
  modified_base order(1,3,4,5,7,9,10,11,12,13,15,17,18,19,20,21): mod_base = OTHER; note = 2'-methoxy-modified
  modified_base order(2,6,8,14,16): mod_base = OTHER; note = 2'-fluoro-modified
cttcacaggtcagggttacgg

SEQ ID NO: 1040 - RNA, 21 nt, synthetic construct
  source 1..21: mol_type = other RNA; note = GPSZRA287S4 antisense strand
  modified_base order(1^2,2^3,19^20,20^21): mod_base = OTHER; note = phosphorothioate linkage
  modified_base order(1,3,4,5,7,9,10,11,12,13,15,17,18,19,20,21): mod_base = OTHER; note = 2'-methoxy-modified
  modified_base order(2,6,8,14,16): mod_base = OTHER; note = 2'-fluoro-modified
acttcacaggtcagggttacg

SEQ ID NO: 1041 - RNA, 21 nt, synthetic construct
  source 1..21: mol_type = other RNA; note = GPSZRA288S4 antisense strand
  modified_base order(1^2,2^3,19^20,20^21): mod_base = OTHER; note = phosphorothioate linkage
  modified_base order(1,3,4,5,7,9,10,11,12,13,15,17,18,19,20,21): mod_base = OTHER; note = 2'-methoxy-modified
  modified_base order(2,6,8,14,16): mod_base = OTHER; note = 2'-fluoro-modified
gacttcacaggtcagggttac

SEQ ID NO: 1042 - RNA, 21 nt, synthetic construct
  source 1..21: mol_type = other RNA; note = GPSZRA290S4 antisense strand
  modified_base order(1^2,2^3,19^20,20^21): mod_base = OTHER; note = phosphorothioate linkage
  modified_base order(1,3,4,5,7,9,10,11,12,13,15,17,18,19,20,21): mod_base = OTHER; note = 2'-methoxy-modified
  modified_base order(2,6,8,14,16): mod_base = OTHER; note = 2'-fluoro-modified
agggacttcacaggtcagggt

SEQ ID NO: 1043 - RNA, 21 nt, synthetic construct
  source 1..21: mol_type = other RNA; note = GPSZRA292S4 antisense strand
  modified_base order(1^2,2^3,19^20,20^21): mod_base = OTHER; note = phosphorothioate linkage
  modified_base order(1,3,4,5,7,9,10,11,12,13,15,17,18,19,20,21): mod_base = OTHER; note = 2'-methoxy-modified
  modified_base order(2,6,8,14,16): mod_base = OTHER; note = 2'-fluoro-modified
gcagggacttcacaggtcagg

SEQ ID NO: 1044 - RNA, 21 nt, synthetic construct
  source 1..21: mol_type = other RNA; note = GPSZRA301S4 antisense strand
  modified_base order(1^2,2^3,19^20,20^21): mod_base = OTHER; note = phosphorothioate linkage
  modified_base order(1,3,4,5,7,9,10,11,12,13,15,17,18,19,20,21): mod_base = OTHER; note = 2'-methoxy-modified
  modified_base order(2,6,8,14,16): mod_base = OTHER; note = 2'-fluoro-modified
tccagtggatttgaggagagg

SEQ ID NO: 1045 - RNA, 21 nt, synthetic construct
  source 1..21: mol_type = other RNA; note = GPSZRA308S4 antisense strand
  modified_base order(1^2,2^3,19^20,20^21): mod_base = OTHER; note = phosphorothioate linkage
  modified_base order(1,3,4,5,7,9,10,11,12,13,15,17,18,19,20,21): mod_base = OTHER; note = 2'-methoxy-modified
  modified_base order(2,6,8,14,16): mod_base = OTHER; note = 2'-fluoro-modified
tccttcatccagtggatttga

SEQ ID NO: 1046 - RNA, 21 nt, synthetic construct
  source 1..21: mol_type = other RNA; note = GPSZRA311S4 antisense strand
  modified_base order(1^2,2^3,19^20,20^21): mod_base = OTHER; note = phosphorothioate linkage
  modified_base order(1,3,4,5,7,9,10,11,12,13,15,17,18,19,20,21): mod_base = OTHER; note = 2'-methoxy-modified
  modified_base order(2,6,8,14,16): mod_base = OTHER; note = 2'-fluoro-modified
ccatccttcatccagtggatt

SEQ ID NO: 1047 - RNA, 21 nt, synthetic construct
  source 1..21: mol_type = other RNA; note = GPSZRA312S4 antisense strand
  modified_base order(1^2,2^3,19^20,20^21): mod_base = OTHER; note = phosphorothioate linkage
  modified_base order(1,3,4,5,7,9,10,11,12,13,15,17,18,19,20,21): mod_base = OTHER; note = 2'-methoxy-modified
  modified_base order(2,6,8,14,16): mod_base = OTHER; note = 2'-fluoro-modified
accatccttcatccagtggat

SEQ ID NO: 1048 - RNA, 21 nt, synthetic construct
  source 1..21: mol_type = other RNA; note = GPSZRA313S4 antisense strand
  modified_base order(1^2,2^3,19^20,20^21): mod_base = OTHER; note = phosphorothioate linkage
  modified_base order(1,3,4,5,7,9,10,11,12,13,15,17,18,19,20,21): mod_base = OTHER; note = 2'-methoxy-modified
  modified_base order(2,6,8,14,16): mod_base = OTHER; note = 2'-fluoro-modified
caccatccttcatccagtgga

SEQ ID NO: 1049 - RNA, 21 nt, synthetic construct
  source 1..21: mol_type = other RNA; note = GPSZRA314S4 antisense strand
  modified_base order(1^2,2^3,19^20,20^21): mod_base = OTHER; note = phosphorothioate linkage
  modified_base order(1,3,4,5,7,9,10,11,12,13,15,17,18,19,20,21): mod_base = OTHER; note = 2'-methoxy-modified
  modified_base order(2,6,8,14,16): mod_base = OTHER; note = 2'-fluoro-modified
acaccatccttcatccagtgg

SEQ ID NO: 1050 - RNA, 21 nt, synthetic construct
  source 1..21: mol_type = other RNA; note = GPSZRA315S4 antisense strand
  modified_base order(1^2,2^3,19^20,20^21): mod_base = OTHER; note = phosphorothioate linkage
  modified_base order(1,3,4,5,7,9,10,11,12,13,15,17,18,19,20,21): mod_base = OTHER; note = 2'-methoxy-modified
  modified_base order(2,6,8,14,16): mod_base = OTHER; note = 2'-fluoro-modified
cacaccatccttcatccagtg

SEQ ID NO: 1051 - RNA, 21 nt, synthetic construct
  source 1..21: mol_type = other RNA; note = GPSZRA316S4 antisense strand
  modified_base order(1^2,2^3,19^20,20^21): mod_base = OTHER; note = phosphorothioate linkage
  modified_base order(1,3,4,5,7,9,10,11,12,13,15,17,18,19,20,21): mod_base = OTHER; note = 2'-methoxy-modified
  modified_base order(2,6,8,14,16): mod_base = OTHER; note = 2'-fluoro-modified
gcacaccatccttcatccagt

SEQ ID NO: 1052 - RNA, 21 nt, synthetic construct
  source 1..21: mol_type = other RNA; note = GPSZRA317S4 antisense strand
  modified_base order(1^2,2^3,19^20,20^21): mod_base = OTHER; note = phosphorothioate linkage
  modified_base order(1,3,4,5,7,9,10,11,12,13,15,17,18,19,20,21): mod_base = OTHER; note = 2'-methoxy-modified
  modified_base order(2,6,8,14,16): mod_base = OTHER; note = 2'-fluoro-modified
ggcacaccatccttcatccag

SEQ ID NO: 1053 - RNA, 21 nt, synthetic construct
  source 1..21: mol_type = other RNA; note = GPSZRA318S4 antisense strand
  modified_base order(1^2,2^3,19^20,20^21): mod_base = OTHER; note = phosphorothioate linkage
  modified_base order(1,3,4,5,7,9,10,11,12,13,15,17,18,19,20,21): mod_base = OTHER; note = 2'-methoxy-modified
  modified_base order(2,6,8,14,16): mod_base = OTHER; note = 2'-fluoro-modified
gggcacaccatccttcatcca

SEQ ID NO: 1054 - RNA, 21 nt, synthetic construct
  source 1..21: mol_type = other RNA; note = GPSZRA320S4 antisense strand
  modified_base order(1^2,2^3,19^20,20^21): mod_base = OTHER; note = phosphorothioate linkage
  modified_base order(1,3,4,5,7,9,10,11,12,13,15,17,18,19,20,21): mod_base = OTHER; note = 2'-methoxy-modified
  modified_base order(2,6,8,14,16): mod_base = OTHER; note = 2'-fluoro-modified
aagggcacaccatccttcatc

SEQ ID NO: 1055 - RNA, 21 nt, synthetic construct
  source 1..21: mol_type = other RNA; note = GPSZRA333S4 antisense strand
  modified_base order(1^2,2^3,19^20,20^21): mod_base = OTHER; note = phosphorothioate linkage
  modified_base order(1,3,4,5,7,9,10,11,12,13,15,17,18,19,20,21): mod_base = OTHER; note = 2'-methoxy-modified
  modified_base order(2,6,8,14,16): mod_base = OTHER; note = 2'-fluoro-modified
tgctgacagcacggctttcct

SEQ ID NO: 1056 - RNA, 21 nt, synthetic construct
  source 1..21: mol_type = other RNA; note = GPSZRA342S4 antisense strand
  modified_base order(1^2,2^3,19^20,20^21): mod_base = OTHER; note = phosphorothioate linkage
  modified_base order(1,3,4,5,7,9,10,11,12,13,15,17,18,19,20,21): mod_base = OTHER; note = 2'-methoxy-modified
  modified_base order(2,6,8,14,16): mod_base = OTHER; note = 2'-fluoro-modified
gatgatgctgatgctgacagc

SEQ ID NO: 1057 - RNA, 21 nt, synthetic construct
  source 1..21: mol_type = other RNA; note = GPSZRA378S4 antisense strand
  modified_base order(1^2,2^3,19^20,20^21): mod_base = OTHER; note = phosphorothioate linkage
  modified_base order(1,3,4,5,7,9,10,11,12,13,15,17,18,19,20,21): mod_base = OTHER; note = 2'-methoxy-modified
  modified_base order(2,6,8,14,16): mod_base = OTHER; note = 2'-fluoro-modified
tctgcacgctcctcctcttcc

SEQ ID NO: 1058 - RNA, 21 nt, synthetic construct
  source 1..21: mol_type = other RNA; note = GPSZRA379S4 antisense strand
  modified_base order(1^2,2^3,19^20,20^21): mod_base = OTHER; note = phosphorothioate linkage
  modified_base order(1,3,4,5,7,9,10,11,12,13,15,17,18,19,20,21): mod_base = OTHER; note = 2'-methoxy-modified
  modified_base order(2,6,8,14,16): mod_base = OTHER; note = 2'-fluoro-modified
aggttcctccgactgattcag

SEQ ID NO: 1059 - RNA, 21 nt, synthetic construct
  source 1..21: mol_type = other RNA; note = GPSZRA380S4 antisense strand
  modified_base order(1^2,2^3,19^20,20^21): mod_base = OTHER; note = phosphorothioate linkage
  modified_base order(1,3,4,5,7,9,10,11,12,13,15,17,18,19,20,21): mod_base = OTHER; note = 2'-methoxy-modified
  modified_base order(2,6,8,14,16): mod_base = OTHER; note = 2'-fluoro-modified
caggttcctccgactgattca

SEQ ID NO: 1060 - RNA, 21 nt, synthetic construct
  source 1..21: mol_type = other RNA; note = GPSZRA381S4 antisense strand
  modified_base order(1^2,2^3,19^20,20^21): mod_base = OTHER; note = phosphorothioate linkage
  modified_base order(1,3,4,5,7,9,10,11,12,13,15,17,18,19,20,21): mod_base = OTHER; note = 2'-methoxy-modified
  modified_base order(2,6,8,14,16): mod_base = OTHER; note = 2'-fluoro-modified
tcaggttcctccgactgattc

SEQ ID NO: 1061 - RNA, 21 nt, synthetic construct
  source 1..21: mol_type = other RNA; note = GPSZRA402S4 antisense strand
  modified_base order(1^2,2^3,19^20,20^21): mod_base = OTHER; note = phosphorothioate linkage
  modified_base order(1,3,4,5,7,9,10,11,12,13,15,17,18,19,20,21): mod_base = OTHER; note = 2'-methoxy-modified
  modified_base order(2,6,8,14,16): mod_base = OTHER; note = 2'-fluoro-modified
ttatacaggagagagttggtc

SEQ ID NO: 1062 - RNA, 21 nt, synthetic construct
  source 1..21: mol_type = other RNA; note = GPSZRA407S4 antisense strand
  modified_base order(1^2,2^3,19^20,20^21): mod_base = OTHER; note = phosphorothioate linkage
  modified_base order(1,3,4,5,7,9,10,11,12,13,15,17,18,19,20,21): mod_base = OTHER; note = 2'-methoxy-modified
  modified_base order(2,6,8,14,16): mod_base = OTHER; note = 2'-fluoro-modified
caaggtggggttatacaggag

SEQ ID NO: 1063 - RNA, 21 nt, synthetic construct
  source 1..21: mol_type = other RNA; note = GPSZRA408S4 antisense strand
  modified_base order(1^2,2^3,19^20,20^21): mod_base = OTHER; note = phosphorothioate linkage
  modified_base order(1,3,4,5,7,9,10,11,12,13,15,17,18,19,20,21): mod_base = OTHER; note = 2'-methoxy-modified
  modified_base order(2,6,8,14,16): mod_base = OTHER; note = 2'-fluoro-modified
gcaaggtggggttatacagga

SEQ ID NO: 1064 - RNA, 21 nt, synthetic construct
  source 1..21: mol_type = other RNA; note = GPSZRA409S4 antisense strand
  modified_base order(1^2,2^3,19^20,20^21): mod_base = OTHER; note = phosphorothioate linkage
  modified_base order(1,3,4,5,7,9,10,11,12,13,15,17,18,19,20,21): mod_base = OTHER; note = 2'-methoxy-modified
  modified_base order(2,6,8,14,16): mod_base = OTHER; note = 2'-fluoro-modified
ggcaaggtggggttatacagg

SEQ ID NO: 1065 - RNA, 21 nt, synthetic construct
  source 1..21: mol_type = other RNA; note = GPSZRA410S4 antisense strand
  modified_base order(1^2,2^3,19^20,20^21): mod_base = OTHER; note = phosphorothioate linkage
  modified_base order(1,3,4,5,7,9,10,11,12,13,15,17,18,19,20,21): mod_base = OTHER; note = 2'-methoxy-modified
  modified_base order(2,6,8,14,16): mod_base = OTHER; note = 2'-fluoro-modified
tggcaaggtggggttatacag

SEQ ID NO: 1066 - RNA, 21 nt, synthetic construct
  source 1..21: mol_type = other RNA; note = GPSZRA411S4 antisense strand
  modified_base order(1^2,2^3,19^20,20^21): mod_base = OTHER; note = phosphorothioate linkage
  modified_base order(1,3,4,5,7,9,10,11,12,13,15,17,18,19,20,21): mod_base = OTHER; note = 2'-methoxy-modified
  modified_base order(2,6,8,14,16): mod_base = OTHER; note = 2'-fluoro-modified
ttggcaaggtggggttataca

SEQ ID NO: 1067 - RNA, 21 nt, synthetic construct
  source 1..21: mol_type = other RNA; note = GPSZRA084S5 antisense strand
  modified_base order(1^2,2^3,19^20,20^21): mod_base = OTHER; note = phosphorothioate linkage
  modified_base order(1,3,4,5,7,9,10,11,12,13,15,17,18,19,20,21): mod_base = OTHER; note = 2'-methoxy-modified
  modified_base order(2,6,8,14,16): mod_base = OTHER; note = 2'-fluoro-modified
tggacttggtctcctttccat

SEQ ID NO: 1068 - RNA, 21 nt, synthetic construct
  source 1..21: mol_type = other RNA; note = GPSZRA087S5 antisense strand
  modified_base order(1^2,2^3,19^20,20^21): mod_base = OTHER; note = phosphorothioate linkage
  modified_base order(1,3,4,5,7,9,10,11,12,13,15,17,18,19,20,21): mod_base = OTHER; note = 2'-methoxy-modified
  modified_base order(2,6,8,14,16): mod_base = OTHER; note = 2'-fluoro-modified
agttggacttggtctcctttc

SEQ ID NO: 1069 - RNA, 21 nt, synthetic construct
  source 1..21: mol_type = other RNA; note = GPSZRA092S5 antisense strand
  modified_base order(1^2,2^3,19^20,20^21): mod_base = OTHER; note = phosphorothioate linkage
  modified_base order(1,3,4,5,7,9,10,11,12,13,15,17,18,19,20,21): mod_base = OTHER; note = 2'-methoxy-modified
  modified_base order(2,6,8,14,16): mod_base = OTHER; note = 2'-fluoro-modified
tcggtagttggacttggtctc

SEQ ID NO: 1070 - RNA, 21 nt, synthetic construct
  source 1..21: mol_type = other RNA; note = GPSZRA093S5 antisense strand
  modified_base order(1^2,2^3,19^20,20^21): mod_base = OTHER; note = phosphorothioate linkage
  modified_base order(1,3,4,5,7,9,10,11,12,13,15,17,18,19,20,21): mod_base = OTHER; note = 2'-methoxy-modified
  modified_base order(2,6,8,14,16): mod_base = OTHER; note = 2'-fluoro-modified
ctcggtagttggacttggtct

SEQ ID NO: 1071 - RNA, 21 nt, synthetic construct
  source 1..21: mol_type = other RNA; note = GPSZRA097S5 antisense strand
  modified_base order(1^2,2^3,19^20,20^21): mod_base = OTHER; note = phosphorothioate linkage
  modified_base order(1,3,4,5,7,9,10,11,12,13,15,17,18,19,20,21): mod_base = OTHER; note = 2'-methoxy-modified
  modified_base order(2,6,8,14,16): mod_base = OTHER; note = 2'-fluoro-modified
cggactcggtagttggacttg

SEQ ID NO: 1072 - RNA, 21 nt, synthetic construct
  source 1..21: mol_type = other RNA; note = GPSZRA118S5 antisense strand
  modified_base order(1^2,2^3,19^20,20^21): mod_base = OTHER; note = phosphorothioate linkage
  modified_base order(1,3,4,5,7,9,10,11,12,13,15,17,18,19,20,21): mod_base = OTHER; note = 2'-methoxy-modified
  modified_base order(2,6,8,14,16): mod_base = OTHER; note = 2'-fluoro-modified
cttcccaggaatctggtagac

SEQ ID NO: 1073 - RNA, 21 nt, synthetic construct
  source 1..21: mol_type = other RNA; note = GPSZRA217S5 antisense strand
  modified_base order(1^2,2^3,19^20,20^21): mod_base = OTHER; note = phosphorothioate linkage
  modified_base order(1,3,4,5,7,9,10,11,12,13,15,17,18,19,20,21): mod_base = OTHER; note = 2'-methoxy-modified
  modified_base order(2,6,8,14,16): mod_base = OTHER; note = 2'-fluoro-modified
tccttcacagatactcccttc

SEQ ID NO: 1074 - RNA, 21 nt, synthetic construct
  source 1..21: mol_type = other RNA; note = GPSZRA222S5 antisense strand
  modified_base order(1^2,2^3,19^20,20^21): mod_base = OTHER; note = phosphorothioate linkage
  modified_base order(1,3,4,5,7,9,10,11,12,13,15,17,18,19,20,21): mod_base = OTHER; note = 2'-methoxy-modified
  modified_base order(2,6,8,14,16): mod_base = OTHER; note = 2'-fluoro-modified
tccgactgcagtgtgaagagc

SEQ ID NO: 1075 - RNA, 21 nt, synthetic construct
  source 1..21: mol_type = other RNA; note = GPSZRA227S5 antisense strand
  modified_base order(1^2,2^3,19^20,20^21): mod_base = OTHER; note = phosphorothioate linkage
  modified_base order(1,3,4,5,7,9,10,11,12,13,15,17,18,19,20,21): mod_base = OTHER; note = 2'-methoxy-modified
  modified_base order(2,6,8,14,16): mod_base = OTHER; note = 2'-fluoro-modified
ttagctccgactgcagtgtga

SEQ ID NO: 1076 - RNA, 21 nt, synthetic construct
  source 1..21: mol_type = other RNA; note = GPSZRA228S5 antisense strand
  modified_base order(1^2,2^3,19^20,20^21): mod_base = OTHER; note = phosphorothioate linkage
  modified_base order(1,3,4,5,7,9,10,11,12,13,15,17,18,19,20,21): mod_base = OTHER; note = 2'-methoxy-modified
  modified_base order(2,6,8,14,16): mod_base = OTHER; note = 2'-fluoro-modified
attagctccgactgcagtgtg

SEQ ID NO: 1077 - RNA, 21 nt, synthetic construct
  source 1..21: mol_type = other RNA; note = GPSZRA229S5 antisense strand
  modified_base order(1^2,2^3,19^20,20^21): mod_base = OTHER; note = phosphorothioate linkage
  modified_base order(1,3,4,5,7,9,10,11,12,13,15,17,18,19,20,21): mod_base = OTHER; note = 2'-methoxy-modified
  modified_base order(2,6,8,14,16): mod_base = OTHER; note = 2'-fluoro-modified
cattagctccgactgcagtgt

SEQ ID NO: 1078 - RNA, 21 nt, synthetic construct
  source 1..21: mol_type = other RNA; note = GPSZRA231S5 antisense strand
  modified_base order(1^2,2^3,19^20,20^21): mod_base = OTHER; note = phosphorothioate linkage
  modified_base order(1,3,4,5,7,9,10,11,12,13,15,17,18,19,20,21): mod_base = OTHER; note = 2'-methoxy-modified
  modified_base order(2,6,8,14,16): mod_base = OTHER; note = 2'-fluoro-modified
accattagctccgactgcagt

SEQ ID NO: 1079 - RNA, 21 nt, synthetic construct
  source 1..21: mol_type = other RNA; note = GPSZRA232S5 antisense strand
  modified_base order(1^2,2^3,19^20,20^21): mod_base = OTHER; note = phosphorothioate linkage
  modified_base order(1,3,4,5,7,9,10,11,12,13,15,17,18,19,20,21): mod_base = OTHER; note = 2'-methoxy-modified
  modified_base order(2,6,8,14,16): mod_base = OTHER; note = 2'-fluoro-modified
caccattagctccgactgcag

SEQ ID NO: 1080 - RNA, 21 nt, synthetic construct
  source 1..21: mol_type = other RNA; note = GPSZRA233S5 antisense strand
  modified_base order(1^2,2^3,19^20,20^21): mod_base = OTHER; note = phosphorothioate linkage
  modified_base order(1,3,4,5,7,9,10,11,12,13,15,17,18,19,20,21): mod_base = OTHER; note = 2'-methoxy-modified
  modified_base order(2,6,8,14,16): mod_base = OTHER; note = 2'-fluoro-modified
tcaccattagctccgactgca

SEQ ID NO: 1081 - RNA, 21 nt, synthetic construct
  source 1..21: mol_type = other RNA; note = GPSZRA252S5 antisense strand
  modified_base order(1^2,2^3,19^20,20^21): mod_base = OTHER; note = phosphorothioate linkage
  modified_base order(1,3,4,5,7,9,10,11,12,13,15,17,18,19,20,21): mod_base = OTHER; note = 2'-methoxy-modified
  modified_base order(2,6,8,14,16): mod_base = OTHER; note = 2'-fluoro-modified
caattggacctcctccagagg

SEQ ID NO: 1082 - RNA, 21 nt, synthetic construct
  source 1..21: mol_type = other RNA; note = GPSZRA257S5 antisense strand
  modified_base order(1^2,2^3,19^20,20^21): mod_base = OTHER; note = phosphorothioate linkage
  modified_base order(1,3,4,5,7,9,10,11,12,13,15,17,18,19,20,21): mod_base = OTHER; note = 2'-methoxy-modified
  modified_base order(2,6,8,14,16): mod_base = OTHER; note = 2'-fluoro-modified
accaccaattggacctcctcc

SEQ ID NO: 1083 - RNA, 21 nt, synthetic construct
  source 1..21: mol_type = other RNA; note = GPSZRA266S5 antisense strand
  modified_base order(1^2,2^3,19^20,20^21): mod_base = OTHER; note = phosphorothioate linkage
  modified_base order(1,3,4,5,7,9,10,11,12,13,15,17,18,19,20,21): mod_base = OTHER; note = 2'-methoxy-modified
  modified_base order(2,6,8,14,16): mod_base = OTHER; note = 2'-fluoro-modified
tccaccaggagctactgctcc

SEQ ID NO: 1084 - RNA, 21 nt, synthetic construct
  source 1..21: mol_type = other RNA; note = GPSZRA267S5 antisense strand
  modified_base order(1^2,2^3,19^20,20^21): mod_base = OTHER; note = phosphorothioate linkage
  modified_base order(1,3,4,5,7,9,10,11,12,13,15,17,18,19,20,21): mod_base = OTHER; note = 2'-methoxy-modified
  modified_base order(2,6,8,14,16): mod_base = OTHER; note = 2'-fluoro-modified
ttccaccaggagctactgctc

SEQ ID NO: 1085 - RNA, 21 nt, synthetic construct
  source 1..21: mol_type = other RNA; note = GPSZRA271S5 antisense strand
  modified_base order(1^2,2^3,19^20,20^21): mod_base = OTHER; note = phosphorothioate linkage
  modified_base order(1,3,4,5,7,9,10,11,12,13,15,17,18,19,20,21): mod_base = OTHER; note = 2'-methoxy-modified
  modified_base order(2,6,8,14,16): mod_base = OTHER; note = 2'-fluoro-modified
tacggttccaccaggagctac

SEQ ID NO: 1086 - RNA, 21 nt, synthetic construct
  source 1..21: mol_type = other RNA; note = GPSZRA272S5 antisense strand
  modified_base order(1^2,2^3,19^20,20^21): mod_base = OTHER; note = phosphorothioate linkage
  modified_base order(1,3,4,5,7,9,10,11,12,13,15,17,18,19,20,21): mod_base = OTHER; note = 2'-methoxy-modified
  modified_base order(2,6,8,14,16): mod_base = OTHER; note = 2'-fluoro-modified
ttacggttccaccaggagcta

SEQ ID NO: 1087 - RNA, 21 nt, synthetic construct
  source 1..21: mol_type = other RNA; note = GPSZRA274S5 antisense strand
  modified_base order(1^2,2^3,19^20,20^21): mod_base = OTHER; note = phosphorothioate linkage
  modified_base order(1,3,4,5,7,9,10,11,12,13,15,17,18,19,20,21): mod_base = OTHER; note = 2'-methoxy-modified
  modified_base order(2,6,8,14,16): mod_base = OTHER; note = 2'-fluoro-modified
ggttacggttccaccaggagc

SEQ ID NO: 1088 - RNA, 21 nt, synthetic construct
  source 1..21: mol_type = other RNA; note = GPSZRA275S5 antisense strand
  modified_base order(1^2,2^3,19^20,20^21): mod_base = OTHER; note = phosphorothioate linkage
  modified_base order(1,3,4,5,7,9,10,11,12,13,15,17,18,19,20,21): mod_base = OTHER; note = 2'-methoxy-modified
  modified_base order(2,6,8,14,16): mod_base = OTHER; note = 2'-fluoro-modified
agggttacggttccaccagga

SEQ ID NO: 1089 - RNA, 21 nt, synthetic construct
  source 1..21: mol_type = other RNA; note = GPSZRA276S5 antisense strand
  modified_base order(1^2,2^3,19^20,20^21): mod_base = OTHER; note = phosphorothioate linkage
  modified_base order(1,3,4,5,7,9,10,11,12,13,15,17,18,19,20,21): mod_base = OTHER; note = 2'-methoxy-modified
  modified_base order(2,6,8,14,16): mod_base = OTHER; note = 2'-fluoro-modified
cagggttacggttccaccagg

SEQ ID NO: 1090 - RNA, 21 nt, synthetic construct
  source 1..21: mol_type = other RNA; note = GPSZRA277S5 antisense strand
  modified_base order(1^2,2^3,19^20,20^21): mod_base = OTHER; note = phosphorothioate linkage
  modified_base order(1,3,4,5,7,9,10,11,12,13,15,17,18,19,20,21): mod_base = OTHER; note = 2'-methoxy-modified
  modified_base order(2,6,8,14,16): mod_base = OTHER; note = 2'-fluoro-modified
tcagggttacggttccaccag

SEQ ID NO: 1091 - RNA, 21 nt, synthetic construct
  source 1..21: mol_type = other RNA; note = GPSZRA281S5 antisense strand
  modified_base order(1^2,2^3,19^20,20^21): mod_base = OTHER; note = phosphorothioate linkage
  modified_base order(1,3,4,5,7,9,10,11,12,13,15,17,18,19,20,21): mod_base = OTHER; note = 2'-methoxy-modified
  modified_base order(2,6,8,14,16): mod_base = OTHER; note = 2'-fluoro-modified
caggtcagggttacggttcca

SEQ ID NO: 1092 - RNA, 21 nt, synthetic construct
  source 1..21: mol_type = other RNA; note = GPSZRA282S5 antisense strand
  modified_base order(1^2,2^3,19^20,20^21): mod_base = OTHER; note = phosphorothioate linkage
  modified_base order(1,3,4,5,7,9,10,11,12,13,15,17,18,19,20,21): mod_base = OTHER; note = 2'-methoxy-modified
  modified_base order(2,6,8,14,16): mod_base = OTHER; note = 2'-fluoro-modified
acaggtcagggttacggttcc

SEQ ID NO: 1093 - RNA, 21 nt, synthetic construct
  source 1..21: mol_type = other RNA; note = GPSZRA283S5 antisense strand
  modified_base order(1^2,2^3,19^20,20^21): mod_base = OTHER; note = phosphorothioate linkage
  modified_base order(1,3,4,5,7,9,10,11,12,13,15,17,18,19,20,21): mod_base = OTHER; note = 2'-methoxy-modified
  modified_base order(2,6,8,14,16): mod_base = OTHER; note = 2'-fluoro-modified
cacaggtcagggttacggttc

SEQ ID NO: 1094 - RNA, 21 nt, synthetic construct
  source 1..21: mol_type = other RNA; note = GPSZRA284S5 antisense strand
  modified_base order(1^2,2^3,19^20,20^21): mod_base = OTHER; note = phosphorothioate linkage
  modified_base order(1,3,4,5,7,9,10,11,12,13,15,17,18,19,20,21): mod_base = OTHER; note = 2'-methoxy-modified
  modified_base order(2,6,8,14,16): mod_base = OTHER; note = 2'-fluoro-modified
tcacaggtcagggttacggtt

SEQ ID NO: 1095 - RNA, 21 nt, synthetic construct
  source 1..21: mol_type = other RNA; note = GPSZRA285S5 antisense strand
  modified_base order(1^2,2^3,19^20,20^21): mod_base = OTHER; note = phosphorothioate linkage
  modified_base order(1,3,4,5,7,9,10,11,12,13,15,17,18,19,20,21): mod_base = OTHER; note = 2'-methoxy-modified
  modified_base order(2,6,8,14,16): mod_base = OTHER; note = 2'-fluoro-modified
ttcacaggtcagggttacggt

SEQ ID NO: 1096 - RNA, 21 nt, synthetic construct
  source 1..21: mol_type = other RNA; note = GPSZRA286S5 antisense strand
  modified_base order(1^2,2^3,19^20,20^21): mod_base = OTHER; note = phosphorothioate linkage
  modified_base order(1,3,4,5,7,9,10,11,12,13,15,17,18,19,20,21): mod_base = OTHER; note = 2'-methoxy-modified
  modified_base order(2,6,8,14,16): mod_base = OTHER; note = 2'-fluoro-modified
cttcacaggtcagggttacgg

SEQ ID NO: 1097 - RNA, 21 nt, synthetic construct
  source 1..21: mol_type = other RNA; note = GPSZRA287S5 antisense strand
  modified_base order(1^2,2^3,19^20,20^21): mod_base = OTHER; note = phosphorothioate linkage
  modified_base order(1,3,4,5,7,9,10,11,12,13,15,17,18,19,20,21): mod_base = OTHER; note = 2'-methoxy-modified
  modified_base order(2,6,8,14,16): mod_base = OTHER; note = 2'-fluoro-modified
acttcacaggtcagggttacg

SEQ ID NO: 1098 - RNA, 21 nt, synthetic construct
  source 1..21: mol_type = other RNA; note = GPSZRA288S5 antisense strand
  modified_base order(1^2,2^3,19^20,20^21): mod_base = OTHER; note = phosphorothioate linkage
  modified_base order(1,3,4,5,7,9,10,11,12,13,15,17,18,19,20,21): mod_base = OTHER; note = 2'-methoxy-modified
  modified_base order(2,6,8,14,16): mod_base = OTHER; note = 2'-fluoro-modified
gacttcacaggtcagggttac

SEQ ID NO: 1099 - RNA, 21 nt, synthetic construct
  source 1..21: mol_type = other RNA; note = GPSZRA290S5 antisense strand
  modified_base order(1^2,2^3,19^20,20^21): mod_base = OTHER; note = phosphorothioate linkage
  modified_base order(1,3,4,5,7,9,10,11,12,13,15,17,18,19,20,21): mod_base = OTHER; note = 2'-methoxy-modified
  modified_base order(2,6,8,14,16): mod_base = OTHER; note = 2'-fluoro-modified
agggacttcacaggtcagggt

SEQ ID NO: 1100 - RNA, 21 nt, synthetic construct
  source 1..21: mol_type = other RNA; note = GPSZRA292S5 antisense strand
  modified_base order(1^2,2^3,19^20,20^21): mod_base = OTHER; note = phosphorothioate linkage
  modified_base order(1,3,4,5,7,9,10,11,12,13,15,17,18,19,20,21): mod_base = OTHER; note = 2'-methoxy-modified
  modified_base order(2,6,8,14,16): mod_base = OTHER; note = 2'-fluoro-modified
gcagggacttcacaggtcagg

SEQ ID NO: 1101 - RNA, 21 nt, synthetic construct
  source 1..21: mol_type = other RNA; note = GPSZRA301S5 antisense strand
  modified_base order(1^2,2^3,19^20,20^21): mod_base = OTHER; note = phosphorothioate linkage
  modified_base order(1,3,4,5,7,9,10,11,12,13,15,17,18,19,20,21): mod_base = OTHER; note = 2'-methoxy-modified
  modified_base order(2,6,8,14,16): mod_base = OTHER; note = 2'-fluoro-modified
tccagtggatttgaggagagg

SEQ ID NO: 1102 - RNA, 21 nt, synthetic construct
  source 1..21: mol_type = other RNA; note = GPSZRA308S5 antisense strand
  modified_base order(1^2,2^3,19^20,20^21): mod_base = OTHER; note = phosphorothioate linkage
  modified_base order(1,3,4,5,7,9,10,11,12,13,15,17,18,19,20,21): mod_base = OTHER; note = 2'-methoxy-modified
  modified_base order(2,6,8,14,16): mod_base = OTHER; note = 2'-fluoro-modified
tccttcatccagtggatttga

SEQ ID NO: 1103 - RNA, 21 nt, synthetic construct
  source 1..21: mol_type = other RNA; note = GPSZRA311S5 antisense strand
  modified_base order(1^2,2^3,19^20,20^21): mod_base = OTHER; note = phosphorothioate linkage
  modified_base order(1,3,4,5,7,9,10,11,12,13,15,17,18,19,20,21): mod_base = OTHER; note = 2'-methoxy-modified
  modified_base order(2,6,8,14,16): mod_base = OTHER; note = 2'-fluoro-modified
ccatccttcatccagtggatt

SEQ ID NO: 1104 - RNA, 21 nt, synthetic construct
  source 1..21: mol_type = other RNA; note = GPSZRA312S5 antisense strand
  modified_base order(1^2,2^3,19^20,20^21): mod_base = OTHER; note = phosphorothioate linkage
  modified_base order(1,3,4,5,7,9,10,11,12,13,15,17,18,19,20,21): mod_base = OTHER; note = 2'-methoxy-modified
  modified_base order(2,6,8,14,16): mod_base = OTHER; note = 2'-fluoro-modified
accatccttcatccagtggat

SEQ ID NO: 1105 - RNA, 21 nt, synthetic construct
  source 1..21: mol_type = other RNA; note = GPSZRA313S5 antisense strand
  modified_base order(1^2,2^3,19^20,20^21): mod_base = OTHER; note = phosphorothioate linkage
  modified_base order(1,3,4,5,7,9,10,11,12,13,15,17,18,19,20,21): mod_base = OTHER; note = 2'-methoxy-modified
  modified_base order(2,6,8,14,16): mod_base = OTHER; note = 2'-fluoro-modified
caccatccttcatccagtgga

SEQ ID NO: 1106 - RNA, 21 nt, synthetic construct
  source 1..21: mol_type = other RNA; note = GPSZRA314S5 antisense strand
  modified_base order(1^2,2^3,19^20,20^21): mod_base = OTHER; note = phosphorothioate linkage
  modified_base order(1,3,4,5,7,9,10,11,12,13,15,17,18,19,20,21): mod_base = OTHER; note = 2'-methoxy-modified
  modified_base order(2,6,8,14,16): mod_base = OTHER; note = 2'-fluoro-modified
acaccatccttcatccagtgg

SEQ ID NO: 1107 - RNA, 21 nt, synthetic construct
  source 1..21: mol_type = other RNA; note = GPSZRA315S5 antisense strand
  modified_base order(1^2,2^3,19^20,20^21): mod_base = OTHER; note = phosphorothioate linkage
  modified_base order(1,3,4,5,7,9,10,11,12,13,15,17,18,19,20,21): mod_base = OTHER; note = 2'-methoxy-modified
  modified_base order(2,6,8,14,16): mod_base = OTHER; note = 2'-fluoro-modified
cacaccatccttcatccagtg

SEQ ID NO: 1108 - RNA, 21 nt, synthetic construct
  source 1..21: mol_type = other RNA; note = GPSZRA316S5 antisense strand
  modified_base order(1^2,2^3,19^20,20^21): mod_base = OTHER; note = phosphorothioate linkage
  modified_base order(1,3,4,5,7,9,10,11,12,13,15,17,18,19,20,21): mod_base = OTHER; note = 2'-methoxy-modified
  modified_base order(2,6,8,14,16): mod_base = OTHER; note = 2'-fluoro-modified
gcacaccatccttcatccagt

SEQ ID NO: 1109 - RNA, 21 nt, synthetic construct
  source 1..21: mol_type = other RNA; note = GPSZRA317S5 antisense strand
  modified_base order(1^2,2^3,19^20,20^21): mod_base = OTHER; note = phosphorothioate linkage
  modified_base order(1,3,4,5,7,9,10,11,12,13,15,17,18,19,20,21): mod_base = OTHER; note = 2'-methoxy-modified
  modified_base order(2,6,8,14,16): mod_base = OTHER; note = 2'-fluoro-modified
ggcacaccatccttcatccag

SEQ ID NO: 1110 - RNA, 21 nt, synthetic construct
  source 1..21: mol_type = other RNA; note = GPSZRA318S5 antisense strand
  modified_base order(1^2,2^3,19^20,20^21): mod_base = OTHER; note = phosphorothioate linkage
  modified_base order(1,3,4,5,7,9,10,11,12,13,15,17,18,19,20,21): mod_base = OTHER; note = 2'-methoxy-modified
  modified_base order(2,6,8,14,16): mod_base = OTHER; note = 2'-fluoro-modified
gggcacaccatccttcatcca

SEQ ID NO: 1111 - RNA, 21 nt, synthetic construct
  source 1..21: mol_type = other RNA; note = GPSZRA320S5 antisense strand
  modified_base order(1^2,2^3,19^20,20^21): mod_base = OTHER; note = phosphorothioate linkage
  modified_base order(1,3,4,5,7,9,10,11,12,13,15,17,18,19,20,21): mod_base = OTHER; note = 2'-methoxy-modified
  modified_base order(2,6,8,14,16): mod_base = OTHER; note = 2'-fluoro-modified
aagggcacaccatccttcatc

SEQ ID NO: 1112 - RNA, 21 nt, synthetic construct
  source 1..21: mol_type = other RNA; note = GPSZRA333S5 antisense strand
  modified_base order(1^2,2^3,19^20,20^21): mod_base = OTHER; note = phosphorothioate linkage
  modified_base order(1,3,4,5,7,9,10,11,12,13,15,17,18,19,20,21): mod_base = OTHER; note = 2'-methoxy-modified
  modified_base order(2,6,8,14,16): mod_base = OTHER; note = 2'-fluoro-modified
tgctgacagcacggctttcct

SEQ ID NO: 1113 - RNA, 21 nt, synthetic construct
  source 1..21: mol_type = other RNA; note = GPSZRA342S5 antisense strand
  modified_base order(1^2,2^3,19^20,20^21): mod_base = OTHER; note = phosphorothioate linkage
  modified_base order(1,3,4,5,7,9,10,11,12,13,15,17,18,19,20,21): mod_base = OTHER; note = 2'-methoxy-modified
  modified_base order(2,6,8,14,16): mod_base = OTHER; note = 2'-fluoro-modified
gatgatgctgatgctgacagc

SEQ ID NO: 1114 - RNA, 21 nt, synthetic construct
  source 1..21: mol_type = other RNA; note = GPSZRA378S5 antisense strand
  modified_base order(1^2,2^3,19^20,20^21): mod_base = OTHER; note = phosphorothioate linkage
  modified_base order(1,3,4,5,7,9,10,11,12,13,15,17,18,19,20,21): mod_base = OTHER; note = 2'-methoxy-modified
  modified_base order(2,6,8,14,16): mod_base = OTHER; note = 2'-fluoro-modified
tctgcacgctcctcctcttcc

SEQ ID NO: 1115 - RNA, 21 nt, synthetic construct
  source 1..21: mol_type = other RNA; note = GPSZRA379S5 antisense strand
  modified_base order(1^2,2^3,19^20,20^21): mod_base = OTHER; note = phosphorothioate linkage
  modified_base order(1,3,4,5,7,9,10,11,12,13,15,17,18,19,20,21): mod_base = OTHER; note = 2'-methoxy-modified
  modified_base order(2,6,8,14,16): mod_base = OTHER; note = 2'-fluoro-modified
aggttcctccgactgattcag

SEQ ID NO: 1116 - RNA, 21 nt, synthetic construct
  source 1..21: mol_type = other RNA; note = GPSZRA380S5 antisense strand
  modified_base order(1^2,2^3,19^20,20^21): mod_base = OTHER; note = phosphorothioate linkage
  modified_base order(1,3,4,5,7,9,10,11,12,13,15,17,18,19,20,21): mod_base = OTHER; note = 2'-methoxy-modified
  modified_base order(2,6,8,14,16): mod_base = OTHER; note = 2'-fluoro-modified
caggttcctccgactgattca

SEQ ID NO: 1117 - RNA, 21 nt, synthetic construct
  source 1..21: mol_type = other RNA; note = GPSZRA381S5 antisense strand
  modified_base order(1^2,2^3,19^20,20^21): mod_base = OTHER; note = phosphorothioate linkage
  modified_base order(1,3,4,5,7,9,10,11,12,13,15,17,18,19,20,21): mod_base = OTHER; note = 2'-methoxy-modified
  modified_base order(2,6,8,14,16): mod_base = OTHER; note = 2'-fluoro-modified
tcaggttcctccgactgattc

SEQ ID NO: 1118 - RNA, 21 nt, synthetic construct
  source 1..21: mol_type = other RNA; note = GPSZRA402S5 antisense strand
  modified_base order(1^2,2^3,19^20,20^21): mod_base = OTHER; note = phosphorothioate linkage
  modified_base order(1,3,4,5,7,9,10,11,12,13,15,17,18,19,20,21): mod_base = OTHER; note = 2'-methoxy-modified
  modified_base order(2,6,8,14,16): mod_base = OTHER; note = 2'-fluoro-modified
ttatacaggagagagttggtc

SEQ ID NO: 1119 - RNA, 21 nt, synthetic construct
  source 1..21: mol_type = other RNA; note = GPSZRA407S5 antisense strand
  modified_base order(1^2,2^3,19^20,20^21): mod_base = OTHER; note = phosphorothioate linkage
  modified_base order(1,3,4,5,7,9,10,11,12,13,15,17,18,19,20,21): mod_base = OTHER; note = 2'-methoxy-modified
  modified_base order(2,6,8,14,16): mod_base = OTHER; note = 2'-fluoro-modified
caaggtggggttatacaggag

SEQ ID NO: 1120 - RNA, 21 nt, synthetic construct
  source 1..21: mol_type = other RNA; note = GPSZRA408S5 antisense strand
  modified_base order(1^2,2^3,19^20,20^21): mod_base = OTHER; note = phosphorothioate linkage
  modified_base order(1,3,4,5,7,9,10,11,12,13,15,17,18,19,20,21): mod_base = OTHER; note = 2'-methoxy-modified
  modified_base order(2,6,8,14,16): mod_base = OTHER; note = 2'-fluoro-modified
gcaaggtggggttatacagga

SEQ ID NO: 1121 - RNA, 21 nt, synthetic construct
  source 1..21: mol_type = other RNA; note = GPSZRA409S5 antisense strand
  modified_base order(1^2,2^3,19^20,20^21): mod_base = OTHER; note = phosphorothioate linkage
  modified_base order(1,3,4,5,7,9,10,11,12,13,15,17,18,19,20,21): mod_base = OTHER; note = 2'-methoxy-modified
  modified_base order(2,6,8,14,16): mod_base = OTHER; note = 2'-fluoro-modified
ggcaaggtggggttatacagg

SEQ ID NO: 1122 - RNA, 21 nt, synthetic construct
  source 1..21: mol_type = other RNA; note = GPSZRA410S5 antisense strand
  modified_base order(1^2,2^3,19^20,20^21): mod_base = OTHER; note = phosphorothioate linkage
  modified_base order(1,3,4,5,7,9,10,11,12,13,15,17,18,19,20,21): mod_base = OTHER; note = 2'-methoxy-modified
  modified_base order(2,6,8,14,16): mod_base = OTHER; note = 2'-fluoro-modified
tggcaaggtggggttatacag

SEQ ID NO: 1123 - RNA, 21 nt, synthetic construct
  source 1..21: mol_type = other RNA; note = GPSZRA411S5 antisense strand
  modified_base order(1^2,2^3,19^20,20^21): mod_base = OTHER; note = phosphorothioate linkage
  modified_base order(1,3,4,5,7,9,10,11,12,13,15,17,18,19,20,21): mod_base = OTHER; note = 2'-methoxy-modified
  modified_base order(2,6,8,14,16): mod_base = OTHER; note = 2'-fluoro-modified
ttggcaaggtggggttataca

SEQ ID NO: 1124 - RNA, 19 nt, synthetic construct
  source 1..19: mol_type = other RNA; note = GPSZRA084S1 sense strand
  modified_base order(1^2,18^19): mod_base = OTHER; note = phosphorothioate linkage
  modified_base order(1,2,4,6,10,12,14,16,18): mod_base = OTHER; note = 2'-methoxy-modified
  modified_base order(3,5,7,8,9,11,13,15,17,19): mod_base = OTHER; note = 2'-fluoro-modified
ggaaaggagaccaagtcca

SEQ ID NO: 1125 - RNA, 19 nt, synthetic construct
  source 1..19: mol_type = other RNA; note = GPSZRA087S1 sense strand
  modified_base order(1^2,18^19): mod_base = OTHER; note = phosphorothioate linkage
  modified_base order(1,2,4,6,10,12,14,16,18): mod_base = OTHER; note = 2'-methoxy-modified
  modified_base order(3,5,7,8,9,11,13,15,17,19): mod_base = OTHER; note = 2'-fluoro-modified
aaggagaccaagtccaact

SEQ ID NO: 1126 - RNA, 19 nt, synthetic construct
  source 1..19: mol_type = other RNA; note = GPSZRA092S1 sense strand
  modified_base order(1^2,18^19): mod_base = OTHER; note = phosphorothioate linkage
  modified_base order(1,2,4,6,10,12,14,16,18): mod_base = OTHER; note = 2'-methoxy-modified
  modified_base order(3,5,7,8,9,11,13,15,17,19): mod_base = OTHER; note = 2'-fluoro-modified
gaccaagtccaactaccga

SEQ ID NO: 1127 - RNA, 19 nt, synthetic construct
  source 1..19: mol_type = other RNA; note = GPSZRA093S1 sense strand
  modified_base order(1^2,18^19): mod_base = OTHER; note = phosphorothioate linkage
  modified_base order(1,2,4,6,10,12,14,16,18): mod_base = OTHER; note = 2'-methoxy-modified
  modified_base order(3,5,7,8,9,11,13,15,17,19): mod_base = OTHER; note = 2'-fluoro-modified
accaagtccaactaccgag

SEQ ID NO: 1128 - RNA, 19 nt, synthetic construct
  source 1..19: mol_type = other RNA; note = GPSZRA097S1 sense strand
  modified_base order(1^2,18^19): mod_base = OTHER; note = phosphorothioate linkage
  modified_base order(1,2,4,6,10,12,14,16,18): mod_base = OTHER; note = 2'-methoxy-modified
  modified_base order(3,5,7,8,9,11,13,15,17,19): mod_base = OTHER; note = 2'-fluoro-modified
agtccaactaccgagtccg

SEQ ID NO: 1129 - RNA, 19 nt, synthetic construct
  source 1..19: mol_type = other RNA; note = GPSZRA118S1 sense strand
  modified_base order(1^2,18^19): mod_base = OTHER; note = phosphorothioate linkage
  modified_base order(1,2,4,6,10,12,14,16,18): mod_base = OTHER; note = 2'-methoxy-modified
  modified_base order(3,5,7,8,9,11,13,15,17,19): mod_base = OTHER; note = 2'-fluoro-modified
ctaccagattcctgggaag

SEQ ID NO: 1130 - RNA, 19 nt, synthetic construct
  source 1..19: mol_type = other RNA; note = GPSZRA217S1 sense strand
  modified_base order(1^2,18^19): mod_base = OTHER; note = phosphorothioate linkage
  modified_base order(1,2,4,6,10,12,14,16,18): mod_base = OTHER; note = 2'-methoxy-modified
  modified_base order(3,5,7,8,9,11,13,15,17,19): mod_base = OTHER; note = 2'-fluoro-modified
agggagtatctgtgaagga

SEQ ID NO: 1131 - RNA, 19 nt, synthetic construct
  source 1..19: mol_type = other RNA; note = GPSZRA222S1/GPSZRA222S1-VP sense strand
  modified_base order(1^2,18^19): mod_base = OTHER; note = phosphorothioate linkage
  modified_base order(1,2,4,6,10,12,14,16,18): mod_base = OTHER; note = 2'-methoxy-modified
  modified_base order(3,5,7,8,9,11,13,15,17,19): mod_base = OTHER; note = 2'-fluoro-modified
tcttcacactgcagtcgga

SEQ ID NO: 1132 - RNA, 19 nt, synthetic construct
  source 1..19: mol_type = other RNA; note = GPSZRA227S1/GPSZRA227S1-VP sense strand
  modified_base order(1^2,18^19): mod_base = OTHER; note = phosphorothioate linkage
  modified_base order(1,2,4,6,10,12,14,16,18): mod_base = OTHER; note = 2'-methoxy-modified
  modified_base order(3,5,7,8,9,11,13,15,17,19): mod_base = OTHER; note = 2'-fluoro-modified
acactgcagtcggagctaa

SEQ ID NO: 1133 - RNA, 19 nt, synthetic construct
  source 1..19: mol_type = other RNA; note = GPSZRA228S1 sense strand
  modified_base order(1^2,18^19): mod_base = OTHER; note = phosphorothioate linkage
  modified_base order(1,2,4,6,10,12,14,16,18): mod_base = OTHER; note = 2'-methoxy-modified
  modified_base order(3,5,7,8,9,11,13,15,17,19): mod_base = OTHER; note = 2'-fluoro-modified
cactgcagtcggagctaat

SEQ ID NO: 1134 - RNA, 19 nt, synthetic construct
  source 1..19: mol_type = other RNA; note = GPSZRA229S1 sense strand
  modified_base order(1^2,18^19): mod_base = OTHER; note = phosphorothioate linkage
  modified_base order(1,2,4,6,10,12,14,16,18): mod_base = OTHER; note = 2'-methoxy-modified
  modified_base order(3,5,7,8,9,11,13,15,17,19): mod_base = OTHER; note = 2'-fluoro-modified
actgcagtcggagctaatg

SEQ ID NO: 1135 - RNA, 19 nt, synthetic construct
  source 1..19: mol_type = other RNA; note = GPSZRA231S1 sense strand
  modified_base order(1^2,18^19): mod_base = OTHER; note = phosphorothioate linkage
  modified_base order(1,2,4,6,10,12,14,16,18): mod_base = OTHER; note = 2'-methoxy-modified
  modified_base order(3,5,7,8,9,11,13,15,17,19): mod_base = OTHER; note = 2'-fluoro-modified
tgcagtcggagctaatggt

SEQ ID NO: 1136 - RNA, 19 nt, synthetic construct
  source 1..19: mol_type = other RNA; note = GPSZRA232S1 sense strand
  modified_base order(1^2,18^19): mod_base = OTHER; note = phosphorothioate linkage
  modified_base order(1,2,4,6,10,12,14,16,18): mod_base = OTHER; note = 2'-methoxy-modified
  modified_base order(3,5,7,8,9,11,13,15,17,19): mod_base = OTHER; note = 2'-fluoro-modified
gcagtcggagctaatggtg

SEQ ID NO: 1137 - RNA, 19 nt, synthetic construct
  source 1..19: mol_type = other RNA; note = GPSZRA233S1 sense strand
  modified_base order(1^2,18^19): mod_base = OTHER; note = phosphorothioate linkage
  modified_base order(1,2,4,6,10,12,14,16,18): mod_base = OTHER; note = 2'-methoxy-modified
  modified_base order(3,5,7,8,9,11,13,15,17,19): mod_base = OTHER; note = 2'-fluoro-modified
cagtcggagctaatggtga

SEQ ID NO: 1138 - RNA, 19 nt, synthetic construct
  source 1..19: mol_type = other RNA; note = GPSZRA252S1 sense strand
  modified_base order(1^2,18^19): mod_base = OTHER; note = phosphorothioate linkage
  modified_base order(1,2,4,6,10,12,14,16,18): mod_base = OTHER; note = 2'-methoxy-modified
  modified_base order(3,5,7,8,9,11,13,15,17,19): mod_base = OTHER; note = 2'-fluoro-modified
tctggaggaggtccaattg

SEQ ID NO: 1139 - RNA, 19 nt, synthetic construct
  source 1..19: mol_type = other RNA; note = GPSZRA257S1 sense strand
  modified_base order(1^2,18^19): mod_base = OTHER; note = phosphorothioate linkage
  modified_base order(1,2,4,6,10,12,14,16,18): mod_base = OTHER; note = 2'-methoxy-modified
  modified_base order(3,5,7,8,9,11,13,15,17,19): mod_base = OTHER; note = 2'-fluoro-modified
aggaggtccaattggtggt

SEQ ID NO: 1140 - RNA, 19 nt, synthetic construct
  source 1..19: mol_type = other RNA; note = GPSZRA266S1 sense strand
  modified_base order(1^2,18^19): mod_base = OTHER; note = phosphorothioate linkage
  modified_base order(1,2,4,6,10,12,14,16,18): mod_base = OTHER; note = 2'-methoxy-modified
  modified_base order(3,5,7,8,9,11,13,15,17,19): mod_base = OTHER; note = 2'-fluoro-modified
agcagtagctcctggtgga

SEQ ID NO: 1141 - RNA, 19 nt, synthetic construct
  source 1..19: mol_type = other RNA; note = GPSZRA267S1 sense strand
  modified_base order(1^2,18^19): mod_base = OTHER; note = phosphorothioate linkage
  modified_base order(1,2,4,6,10,12,14,16,18): mod_base = OTHER; note = 2'-methoxy-modified
  modified_base order(3,5,7,8,9,11,13,15,17,19): mod_base = OTHER; note = 2'-fluoro-modified
gcagtagctcctggtggaa

SEQ ID NO: 1142 - RNA, 19 nt, synthetic construct
  source 1..19: mol_type = other RNA; note = GPSZRA271S1 sense strand
  modified_base order(1^2,18^19): mod_base = OTHER; note = phosphorothioate linkage
  modified_base order(1,2,4,6,10,12,14,16,18): mod_base = OTHER; note = 2'-methoxy-modified
  modified_base order(3,5,7,8,9,11,13,15,17,19): mod_base = OTHER; note = 2'-fluoro-modified
agctcctggtggaaccgta

SEQ ID NO: 1143 - RNA, 19 nt, synthetic construct
  source 1..19: mol_type = other RNA; note = GPSZRA272S1 sense strand
  modified_base order(1^2,18^19): mod_base = OTHER; note = phosphorothioate linkage
  modified_base order(1,2,4,6,10,12,14,16,18): mod_base = OTHER; note = 2'-methoxy-modified
  modified_base order(3,5,7,8,9,11,13,15,17,19): mod_base = OTHER; note = 2'-fluoro-modified
gctcctggtggaaccgtaa

SEQ ID NO: 1144 - RNA, 19 nt, synthetic construct
  source 1..19: mol_type = other RNA; note = GPSZRA274S1 sense strand
  modified_base order(1^2,18^19): mod_base = OTHER; note = phosphorothioate linkage
  modified_base order(1,2,4,6,10,12,14,16,18): mod_base = OTHER; note = 2'-methoxy-modified
  modified_base order(3,5,7,8,9,11,13,15,17,19): mod_base = OTHER; note = 2'-fluoro-modified
tcctggtggaaccgtaacc

SEQ ID NO: 1145 - RNA, 19 nt, synthetic construct
  source 1..19: mol_type = other RNA; note = GPSZRA275S1 sense strand
  modified_base order(1^2,18^19): mod_base = OTHER; note = phosphorothioate linkage
  modified_base order(1,2,4,6,10,12,14,16,18): mod_base = OTHER; note = 2'-methoxy-modified
  modified_base order(3,5,7,8,9,11,13,15,17,19): mod_base = OTHER; note = 2'-fluoro-modified
ctggtggaaccgtaaccct

SEQ ID NO: 1146 - RNA, 19 nt, synthetic construct
  source 1..19: mol_type = other RNA; note = GPSZRA276S1 sense strand
  modified_base order(1^2,18^19): mod_base = OTHER; note = phosphorothioate linkage
  modified_base order(1,2,4,6,10,12,14,16,18): mod_base = OTHER; note = 2'-methoxy-modified
  modified_base order(3,5,7,8,9,11,13,15,17,19): mod_base = OTHER; note = 2'-fluoro-modified
tggtggaaccgtaaccctg

SEQ ID NO: 1147 - RNA, 19 nt, synthetic construct
  source 1..19: mol_type = other RNA; note = GPSZRA277S1 sense strand
  modified_base order(1^2,18^19): mod_base = OTHER; note = phosphorothioate linkage
  modified_base order(1,2,4,6,10,12,14,16,18): mod_base = OTHER; note = 2'-methoxy-modified
  modified_base order(3,5,7,8,9,11,13,15,17,19): mod_base = OTHER; note = 2'-fluoro-modified
ggtggaaccgtaaccctga

SEQ ID NO: 1148 - RNA, 19 nt, synthetic construct
  source 1..19: mol_type = other RNA; note = GPSZRA281S1 sense strand
  modified_base order(1^2,18^19): mod_base = OTHER; note = phosphorothioate linkage
  modified_base order(1,2,4,6,10,12,14,16,18): mod_base = OTHER; note = 2'-methoxy-modified
  modified_base order(3,5,7,8,9,11,13,15,17,19): mod_base = OTHER; note = 2'-fluoro-modified
gaaccgtaaccctgacctg

SEQ ID NO: 1149 - RNA, 19 nt, synthetic construct
  source 1..19: mol_type = other RNA; note = GPSZRA282S1 sense strand
  modified_base order(1^2,18^19): mod_base = OTHER; note = phosphorothioate linkage
  modified_base order(1,2,4,6,10,12,14,16,18): mod_base = OTHER; note = 2'-methoxy-modified
  modified_base order(3,5,7,8,9,11,13,15,17,19): mod_base = OTHER; note = 2'-fluoro-modified
aaccgtaaccctgacctgt

SEQ ID NO: 1150 - RNA, 19 nt, synthetic construct
  source 1..19: mol_type = other RNA; note = GPSZRA283S1 sense strand
  modified_base order(1^2,18^19): mod_base = OTHER; note = phosphorothioate linkage
  modified_base order(1,2,4,6,10,12,14,16,18): mod_base = OTHER; note = 2'-methoxy-modified
  modified_base order(3,5,7,8,9,11,13,15,17,19): mod_base = OTHER; note = 2'-fluoro-modified
accgtaaccctgacctgtg

SEQ ID NO: 1151 - RNA, 19 nt, synthetic construct
  source 1..19: mol_type = other RNA; note = GPSZRA284S1 sense strand
  modified_base order(1^2,18^19): mod_base = OTHER; note = phosphorothioate linkage
  modified_base order(1,2,4,6,10,12,14,16,18): mod_base = OTHER; note = 2'-methoxy-modified
  modified_base order(3,5,7,8,9,11,13,15,17,19): mod_base = OTHER; note = 2'-fluoro-modified
ccgtaaccctgacctgtga

SEQ ID NO: 1152 - RNA, 19 nt, synthetic construct
  source 1..19: mol_type = other RNA; note = GPSZRA285S1 sense strand
  modified_base order(1^2,18^19): mod_base = OTHER; note = phosphorothioate linkage
  modified_base order(1,2,4,6,10,12,14,16,18): mod_base = OTHER; note = 2'-methoxy-modified
  modified_base order(3,5,7,8,9,11,13,15,17,19): mod_base = OTHER; note = 2'-fluoro-modified
cgtaaccctgacctgtgaa

SEQ ID NO: 1153 - RNA, 19 nt, synthetic construct
  source 1..19: mol_type = other RNA; note = GPSZRA286S1 sense strand
  modified_base order(1^2,18^19): mod_base = OTHER; note = phosphorothioate linkage
  modified_base order(1,2,4,6,10,12,14,16,18): mod_base = OTHER; note = 2'-methoxy-modified
  modified_base order(3,5,7,8,9,11,13,15,17,19): mod_base = OTHER; note = 2'-fluoro-modified
gtaaccctgacctgtgaag

SEQ ID NO: 1154 - RNA, 19 nt, synthetic construct
  source 1..19: mol_type = other RNA; note = GPSZRA287S1 sense strand
  modified_base order(1^2,18^19): mod_base = OTHER; note = phosphorothioate linkage
  modified_base order(1,2,4,6,10,12,14,16,18): mod_base = OTHER; note = 2'-methoxy-modified
  modified_base order(3,5,7,8,9,11,13,15,17,19): mod_base = OTHER; note = 2'-fluoro-modified
taaccctgacctgtgaagt

SEQ ID NO: 1155 - RNA, 19 nt, synthetic construct
  source 1..19: mol_type = other RNA; note = GPSZRA288S1 sense strand
  modified_base order(1^2,18^19): mod_base = OTHER; note = phosphorothioate linkage
  modified_base order(1,2,4,6,10,12,14,16,18): mod_base = OTHER; note = 2'-methoxy-modified
  modified_base order(3,5,7,8,9,11,13,15,17,19): mod_base = OTHER; note = 2'-fluoro-modified
aaccctgacctgtgaagtc

SEQ ID NO: 1156 - RNA, 19 nt, synthetic construct
  source 1..19: mol_type = other RNA; note = GPSZRA290S1 sense strand
  modified_base order(1^2,18^19): mod_base = OTHER; note = phosphorothioate linkage
  modified_base order(1,2,4,6,10,12,14,16,18): mod_base = OTHER; note = 2'-methoxy-modified
  modified_base order(3,5,7,8,9,11,13,15,17,19): mod_base = OTHER; note = 2'-fluoro-modified
cctgacctgtgaagtccct

SEQ ID NO: 1157 - RNA, 19 nt, synthetic construct
  source 1..19: mol_type = other RNA; note = GPSZRA292S1 sense strand
  modified_base order(1^2,18^19): mod_base = OTHER; note = phosphorothioate linkage
  modified_base order(1,2,4,6,10,12,14,16,18): mod_base = OTHER; note = 2'-methoxy-modified
  modified_base order(3,5,7,8,9,11,13,15,17,19): mod_base = OTHER; note = 2'-fluoro-modified
tgacctgtgaagtccctgc

SEQ ID NO: 1158 - RNA, 19 nt, synthetic construct
  source 1..19: mol_type = other RNA; note = GPSZRA301S1 sense strand
  modified_base order(1^2,18^19): mod_base = OTHER; note = phosphorothioate linkage
  modified_base order(1,2,4,6,10,12,14,16,18): mod_base = OTHER; note = 2'-methoxy-modified
  modified_base order(3,5,7,8,9,11,13,15,17,19): mod_base = OTHER; note = 2'-fluoro-modified
tctcctcaaatccactgga

SEQ ID NO: 1159 - RNA, 19 nt, synthetic construct
  source 1..19: mol_type = other RNA; note = GPSZRA308S1 sense strand
  modified_base order(1^2,18^19): mod_base = OTHER; note = phosphorothioate linkage
  modified_base order(1,2,4,6,10,12,14,16,18): mod_base = OTHER; note = 2'-methoxy-modified
  modified_base order(3,5,7,8,9,11,13,15,17,19): mod_base = OTHER; note = 2'-fluoro-modified
aaatccactggatgaagga

SEQ ID NO: 1160 - RNA, 19 nt, synthetic construct
  source 1..19: mol_type = other RNA; note = GPSZRA311S1 sense strand
  modified_base order(1^2,18^19): mod_base = OTHER; note = phosphorothioate linkage
  modified_base order(1,2,4,6,10,12,14,16,18): mod_base = OTHER; note = 2'-methoxy-modified
  modified_base order(3,5,7,8,9,11,13,15,17,19): mod_base = OTHER; note = 2'-fluoro-modified
tccactggatgaaggatgg

SEQ ID NO: 1161 - RNA, 19 nt, synthetic construct
  source 1..19: mol_type = other RNA; note = GPSZRA312S1 sense strand
  modified_base order(1^2,18^19): mod_base = OTHER; note = phosphorothioate linkage
  modified_base order(1,2,4,6,10,12,14,16,18): mod_base = OTHER; note = 2'-methoxy-modified
  modified_base order(3,5,7,8,9,11,13,15,17,19): mod_base = OTHER; note = 2'-fluoro-modified
ccactggatgaaggatggt

SEQ ID NO: 1162 - RNA, 19 nt, synthetic construct
  source 1..19: mol_type = other RNA; note = GPSZRA313S1 sense strand
  modified_base order(1^2,18^19): mod_base = OTHER; note = phosphorothioate linkage
  modified_base order(1,2,4,6,10,12,14,16,18): mod_base = OTHER; note = 2'-methoxy-modified
  modified_base order(3,5,7,8,9,11,13,15,17,19): mod_base = OTHER; note = 2'-fluoro-modified
cactggatgaaggatggtg

SEQ ID NO: 1163 - RNA, 19 nt, synthetic construct
  source 1..19: mol_type = other RNA; note = GPSZRA314S1/GPSZRA314S1-VP sense strand
  modified_base order(1^2,18^19): mod_base = OTHER; note = phosphorothioate linkage
  modified_base order(1,2,4,6,10,12,14,16,18): mod_base = OTHER; note = 2'-methoxy-modified
  modified_base order(3,5,7,8,9,11,13,15,17,19): mod_base = OTHER; note = 2'-fluoro-modified
actggatgaaggatggtgt

SEQ ID NO: 1164 - RNA, 19 nt, synthetic construct
  source 1..19: mol_type = other RNA; note = GPSZRA315S1 sense strand
  modified_base order(1^2,18^19): mod_base = OTHER; note = phosphorothioate linkage
  modified_base order(1,2,4,6,10,12,14,16,18): mod_base = OTHER; note = 2'-methoxy-modified
  modified_base order(3,5,7,8,9,11,13,15,17,19): mod_base = OTHER; note = 2'-fluoro-modified
ctggatgaaggatggtgtg

SEQ ID NO: 1165 - RNA, 19 nt, synthetic construct
  source 1..19: mol_type = other RNA; note = GPSZRA316S1 sense strand
  modified_base order(1^2,18^19): mod_base = OTHER; note = phosphorothioate linkage
  modified_base order(1,2,4,6,10,12,14,16,18): mod_base = OTHER; note = 2'-methoxy-modified
  modified_base order(3,5,7,8,9,11,13,15,17,19): mod_base = OTHER; note = 2'-fluoro-modified
tggatgaaggatggtgtgc

SEQ ID NO: 1166 - RNA, 19 nt, synthetic construct
  source 1..19: mol_type = other RNA; note = GPSZRA317S1 sense strand
  modified_base order(1^2,18^19): mod_base = OTHER; note = phosphorothioate linkage
  modified_base order(1,2,4,6,10,12,14,16,18): mod_base = OTHER; note = 2'-methoxy-modified
  modified_base order(3,5,7,8,9,11,13,15,17,19): mod_base = OTHER; note = 2'-fluoro-modified
ggatgaaggatggtgtgcc

SEQ ID NO: 1167 - RNA, 19 nt, synthetic construct
  source 1..19: mol_type = other RNA; note = GPSZRA318S1 sense strand
  modified_base order(1^2,18^19): mod_base = OTHER; note = phosphorothioate linkage
  modified_base order(1,2,4,6,10,12,14,16,18): mod_base = OTHER; note = 2'-methoxy-modified
  modified_base order(3,5,7,8,9,11,13,15,17,19): mod_base = OTHER; note = 2'-fluoro-modified
gatgaaggatggtgtgccc

SEQ ID NO: 1168 - RNA, 19 nt, synthetic construct
  source 1..19: mol_type = other RNA; note = GPSZRA320S1 sense strand
  modified_base order(1^2,18^19): mod_base = OTHER; note = phosphorothioate linkage
  modified_base order(1,2,4,6,10,12,14,16,18): mod_base = OTHER; note = 2'-methoxy-modified
  modified_base order(3,5,7,8,9,11,13,15,17,19): mod_base = OTHER; note = 2'-fluoro-modified
tgaaggatggtgtgccctt

SEQ ID NO: 1169 - RNA, 19 nt, synthetic construct
  source 1..19: mol_type = other RNA; note = GPSZRA333S1 sense strand
  modified_base order(1^2,18^19): mod_base = OTHER; note = phosphorothioate linkage
  modified_base order(1,2,4,6,10,12,14,16,18): mod_base = OTHER; note = 2'-methoxy-modified
  modified_base order(3,5,7,8,9,11,13,15,17,19): mod_base = OTHER; note = 2'-fluoro-modified
gaaagccgtgctgtcagca

SEQ ID NO: 1170 - RNA, 19 nt, synthetic construct
  source 1..19: mol_type = other RNA; note = GPSZRA342S1 sense strand
  modified_base order(1^2,18^19): mod_base = OTHER; note = phosphorothioate linkage
  modified_base order(1,2,4,6,10,12,14,16,18): mod_base = OTHER; note = 2'-methoxy-modified
  modified_base order(3,5,7,8,9,11,13,15,17,19): mod_base = OTHER; note = 2'-fluoro-modified
tgtcagcatcagcatcatc

SEQ ID NO: 1171 - RNA, 19 nt, synthetic construct
  source 1..19: mol_type = other RNA; note = GPSZRA378S1 sense strand
  modified_base order(1^2,18^19): mod_base = OTHER; note = phosphorothioate linkage
  modified_base order(1,2,4,6,10,12,14,16,18): mod_base = OTHER; note = 2'-methoxy-modified
  modified_base order(3,5,7,8,9,11,13,15,17,19): mod_base = OTHER; note = 2'-fluoro-modified
aagaggaggagcgtgcaga

SEQ ID NO: 1172 - RNA, 19 nt, synthetic construct
  source 1..19: mol_type = other RNA; note = GPSZRA379S1 sense strand
  modified_base order(1^2,18^19): mod_base = OTHER; note = phosphorothioate linkage
  modified_base order(1,2,4,6,10,12,14,16,18): mod_base = OTHER; note = 2'-methoxy-modified
  modified_base order(3,5,7,8,9,11,13,15,17,19): mod_base = OTHER; note = 2'-fluoro-modified
gaatcagtcggaggaacct

SEQ ID NO: 1173 - RNA, 19 nt, synthetic construct
  source 1..19: mol_type = other RNA; note = GPSZRA380S1 sense strand
  modified_base order(1^2,18^19): mod_base = OTHER; note = phosphorothioate linkage
  modified_base order(1,2,4,6,10,12,14,16,18): mod_base = OTHER; note = 2'-methoxy-modified
  modified_base order(3,5,7,8,9,11,13,15,17,19): mod_base = OTHER; note = 2'-fluoro-modified
aatcagtcggaggaacctg

SEQ ID NO: 1174 - RNA, 19 nt, synthetic construct
  source 1..19: mol_type = other RNA; note = GPSZRA381S1 sense strand
  modified_base order(1^2,18^19): mod_base = OTHER; note = phosphorothioate linkage
  modified_base order(1,2,4,6,10,12,14,16,18): mod_base = OTHER; note = 2'-methoxy-modified
  modified_base order(3,5,7,8,9,11,13,15,17,19): mod_base = OTHER; note = 2'-fluoro-modified
atcagtcggaggaacctga

SEQ ID NO: 1175 - RNA, 19 nt, synthetic construct
  source 1..19: mol_type = other RNA; note = GPSZRA402S1 sense strand
  modified_base order(1^2,18^19): mod_base = OTHER; note = phosphorothioate linkage
  modified_base order(1,2,4,6,10,12,14,16,18): mod_base = OTHER; note = 2'-methoxy-modified
  modified_base order(3,5,7,8,9,11,13,15,17,19): mod_base = OTHER; note = 2'-fluoro-modified
ccaactctctcctgtataa

SEQ ID NO: 1176 - RNA, 19 nt, synthetic construct
  source 1..19: mol_type = other RNA; note = GPSZRA407S1 sense strand
  modified_base order(1^2,18^19): mod_base = OTHER; note = phosphorothioate linkage
  modified_base order(1,2,4,6,10,12,14,16,18): mod_base = OTHER; note = 2'-methoxy-modified
  modified_base order(3,5,7,8,9,11,13,15,17,19): mod_base = OTHER; note = 2'-fluoro-modified
cctgtataaccccaccttg

SEQ ID NO: 1177 - RNA, 19 nt, synthetic construct
  source 1..19: mol_type = other RNA; note = GPSZRA408S1 sense strand
  modified_base order(1^2,18^19): mod_base = OTHER; note = phosphorothioate linkage
  modified_base order(1,2,4,6,10,12,14,16,18): mod_base = OTHER; note = 2'-methoxy-modified
  modified_base order(3,5,7,8,9,11,13,15,17,19): mod_base = OTHER; note = 2'-fluoro-modified
ctgtataaccccaccttgc

SEQ ID NO: 1178 - RNA, 19 nt, synthetic construct
  source 1..19: mol_type = other RNA; note = GPSZRA409S1 sense strand
  modified_base order(1^2,18^19): mod_base = OTHER; note = phosphorothioate linkage
  modified_base order(1,2,4,6,10,12,14,16,18): mod_base = OTHER; note = 2'-methoxy-modified
  modified_base order(3,5,7,8,9,11,13,15,17,19): mod_base = OTHER; note = 2'-fluoro-modified
tgtataaccccaccttgcc

SEQ ID NO: 1179 - RNA, 19 nt, synthetic construct
  source 1..19: mol_type = other RNA; note = GPSZRA410S1 sense strand
  modified_base order(1^2,18^19): mod_base = OTHER; note = phosphorothioate linkage
  modified_base order(1,2,4,6,10,12,14,16,18): mod_base = OTHER; note = 2'-methoxy-modified
  modified_base order(3,5,7,8,9,11,13,15,17,19): mod_base = OTHER; note = 2'-fluoro-modified
gtataaccccaccttgcca

SEQ ID NO: 1180 - RNA, 19 nt, synthetic construct
  source 1..19: mol_type = other RNA; note = GPSZRA411S1 sense strand
  modified_base order(1^2,18^19): mod_base = OTHER; note = phosphorothioate linkage
  modified_base order(1,2,4,6,10,12,14,16,18): mod_base = OTHER; note = 2'-methoxy-modified
  modified_base order(3,5,7,8,9,11,13,15,17,19): mod_base = OTHER; note = 2'-fluoro-modified
tataaccccaccttgccaa

SEQ ID NO: 1181 - RNA, 19 nt, synthetic construct
  source 1..19: mol_type = other RNA; note = GPSZRA084S2 sense strand
  modified_base order(1^2,18^19): mod_base = OTHER; note = phosphorothioate linkage
  modified_base order(1,2,4,5,6,10,12,14,16,17,18,19): mod_base = OTHER; note = 2'-methoxy-modified
  modified_base order(3,7,8,9,11,13,15): mod_base = OTHER; note = 2'-fluoro-modified
ggaaaggagaccaagtcca

SEQ ID NO: 1182 - RNA, 19 nt, synthetic construct
  source 1..19: mol_type = other RNA; note = GPSZRA087S2 sense strand
  modified_base order(1^2,18^19): mod_base = OTHER; note = phosphorothioate linkage
  modified_base order(1,2,4,5,6,10,12,14,16,17,18,19): mod_base = OTHER; note = 2'-methoxy-modified
  modified_base order(3,7,8,9,11,13,15): mod_base = OTHER; note = 2'-fluoro-modified
aaggagaccaagtccaact

SEQ ID NO: 1183 - RNA, 19 nt, synthetic construct
  source 1..19: mol_type = other RNA; note = GPSZRA092S2 sense strand
  modified_base order(1^2,18^19): mod_base = OTHER; note = phosphorothioate linkage
  modified_base order(1,2,4,5,6,10,12,14,16,17,18,19): mod_base = OTHER; note = 2'-methoxy-modified
  modified_base order(3,7,8,9,11,13,15): mod_base = OTHER; note = 2'-fluoro-modified
gaccaagtccaactaccga

SEQ ID NO: 1184 - RNA, 19 nt, synthetic construct
  source 1..19: mol_type = other RNA; note = GPSZRA093S2 sense strand
  modified_base order(1^2,18^19): mod_base = OTHER; note = phosphorothioate linkage
  modified_base order(1,2,4,5,6,10,12,14,16,17,18,19): mod_base = OTHER; note = 2'-methoxy-modified
  modified_base order(3,7,8,9,11,13,15): mod_base = OTHER; note = 2'-fluoro-modified
accaagtccaactaccgag

SEQ ID NO: 1185 - RNA, 19 nt, synthetic construct
  source 1..19: mol_type = other RNA; note = GPSZRA097S2 sense strand
  modified_base order(1^2,18^19): mod_base = OTHER; note = phosphorothioate linkage
  modified_base order(1,2,4,5,6,10,12,14,16,17,18,19): mod_base = OTHER; note = 2'-methoxy-modified
  modified_base order(3,7,8,9,11,13,15): mod_base = OTHER; note = 2'-fluoro-modified
agtccaactaccgagtccg

SEQ ID NO: 1186 - RNA, 19 nt, synthetic construct
  source 1..19: mol_type = other RNA; note = GPSZRA118S2 sense strand
  modified_base order(1^2,18^19): mod_base = OTHER; note = phosphorothioate linkage
  modified_base order(1,2,4,5,6,10,12,14,16,17,18,19): mod_base = OTHER; note = 2'-methoxy-modified
  modified_base order(3,7,8,9,11,13,15): mod_base = OTHER; note = 2'-fluoro-modified
ctaccagattcctgggaag

SEQ ID NO: 1187 - RNA, 19 nt, synthetic construct
  source 1..19: mol_type = other RNA; note = GPSZRA217S2 sense strand
  modified_base order(1^2,18^19): mod_base = OTHER; note = phosphorothioate linkage
  modified_base order(1,2,4,5,6,10,12,14,16,17,18,19): mod_base = OTHER; note = 2'-methoxy-modified
  modified_base order(3,7,8,9,11,13,15): mod_base = OTHER; note = 2'-fluoro-modified
agggagtatctgtgaagga

SEQ ID NO: 1188 - RNA, 19 nt, synthetic construct
  source 1..19: mol_type = other RNA; note = GPSZRA222S2 sense strand
  modified_base order(1^2,18^19): mod_base = OTHER; note = phosphorothioate linkage
  modified_base order(1,2,4,5,6,10,12,14,16,17,18,19): mod_base = OTHER; note = 2'-methoxy-modified
  modified_base order(3,7,8,9,11,13,15): mod_base = OTHER; note = 2'-fluoro-modified
tcttcacactgcagtcgga

SEQ ID NO: 1189 - RNA, 19 nt, synthetic construct
  source 1..19: mol_type = other RNA; note = GPSZRA227S2 sense strand
  modified_base order(1^2,18^19): mod_base = OTHER; note = phosphorothioate linkage
  modified_base order(1,2,4,5,6,10,12,14,16,17,18,19): mod_base = OTHER; note = 2'-methoxy-modified
  modified_base order(3,7,8,9,11,13,15): mod_base = OTHER; note = 2'-fluoro-modified
acactgcagtcggagctaa

SEQ ID NO: 1190 - RNA, 19 nt, synthetic construct
  source 1..19: mol_type = other RNA; note = GPSZRA228S2 sense strand
  modified_base order(1^2,18^19): mod_base = OTHER; note = phosphorothioate linkage
  modified_base order(1,2,4,5,6,10,12,14,16,17,18,19): mod_base = OTHER; note = 2'-methoxy-modified
  modified_base order(3,7,8,9,11,13,15): mod_base = OTHER; note = 2'-fluoro-modified
cactgcagtcggagctaat

SEQ ID NO: 1191 - RNA, 19 nt, synthetic construct
  source 1..19: mol_type = other RNA; note = GPSZRA229S2 sense strand
  modified_base order(1^2,18^19): mod_base = OTHER; note = phosphorothioate linkage
  modified_base order(1,2,4,5,6,10,12,14,16,17,18,19): mod_base = OTHER; note = 2'-methoxy-modified
  modified_base order(3,7,8,9,11,13,15): mod_base = OTHER; note = 2'-fluoro-modified
actgcagtcggagctaatg

SEQ ID NO: 1192 - RNA, 19 nt, synthetic construct
  source 1..19: mol_type = other RNA; note = GPSZRA231S2 sense strand
  modified_base order(1^2,18^19): mod_base = OTHER; note = phosphorothioate linkage
  modified_base order(1,2,4,5,6,10,12,14,16,17,18,19): mod_base = OTHER; note = 2'-methoxy-modified
  modified_base order(3,7,8,9,11,13,15): mod_base = OTHER; note = 2'-fluoro-modified
tgcagtcggagctaatggt

SEQ ID NO: 1193 - RNA, 19 nt, synthetic construct
  source 1..19: mol_type = other RNA; note = GPSZRA232S2 sense strand
  modified_base order(1^2,18^19): mod_base = OTHER; note = phosphorothioate linkage
  modified_base order(1,2,4,5,6,10,12,14,16,17,18,19): mod_base = OTHER; note = 2'-methoxy-modified
  modified_base order(3,7,8,9,11,13,15): mod_base = OTHER; note = 2'-fluoro-modified
gcagtcggagctaatggtg

SEQ ID NO: 1194 - RNA, 19 nt, synthetic construct
  source 1..19: mol_type = other RNA; note = GPSZRA233S2 sense strand
  modified_base order(1^2,18^19): mod_base = OTHER; note = phosphorothioate linkage
  modified_base order(1,2,4,5,6,10,12,14,16,17,18,19): mod_base = OTHER; note = 2'-methoxy-modified
  modified_base order(3,7,8,9,11,13,15): mod_base = OTHER; note = 2'-fluoro-modified
cagtcggagctaatggtga

SEQ ID NO: 1195 - RNA, 19 nt, synthetic construct
  source 1..19: mol_type = other RNA; note = GPSZRA252S2 sense strand
  modified_base order(1^2,18^19): mod_base = OTHER; note = phosphorothioate linkage
  modified_base order(1,2,4,5,6,10,12,14,16,17,18,19): mod_base = OTHER; note = 2'-methoxy-modified
  modified_base order(3,7,8,9,11,13,15): mod_base = OTHER; note = 2'-fluoro-modified
tctggaggaggtccaattg

SEQ ID NO: 1196 - RNA, 19 nt, synthetic construct
  source 1..19: mol_type = other RNA; note = GPSZRA257S2 sense strand
  modified_base order(1^2,18^19): mod_base = OTHER; note = phosphorothioate linkage
  modified_base order(1,2,4,5,6,10,12,14,16,17,18,19): mod_base = OTHER; note = 2'-methoxy-modified
  modified_base order(3,7,8,9,11,13,15): mod_base = OTHER; note = 2'-fluoro-modified
aggaggtccaattggtggt

SEQ ID NO: 1197 - RNA, 19 nt, synthetic construct
  source 1..19: mol_type = other RNA; note = GPSZRA266S2 sense strand
  modified_base order(1^2,18^19): mod_base = OTHER; note = phosphorothioate linkage
  modified_base order(1,2,4,5,6,10,12,14,16,17,18,19): mod_base = OTHER; note = 2'-methoxy-modified
  modified_base order(3,7,8,9,11,13,15): mod_base = OTHER; note = 2'-fluoro-modified
agcagtagctcctggtgga

SEQ ID NO: 1198 - RNA, 19 nt, synthetic construct
  source 1..19: mol_type = other RNA; note = GPSZRA267S2/GPSZRA267S2-VP sense strand
  modified_base order(1^2,18^19): mod_base = OTHER; note = phosphorothioate linkage
  modified_base order(1,2,4,5,6,10,12,14,16,17,18,19): mod_base = OTHER; note = 2'-methoxy-modified
  modified_base order(3,7,8,9,11,13,15): mod_base = OTHER; note = 2'-fluoro-modified
gcagtagctcctggtggaa

SEQ ID NO: 1199 - RNA, 19 nt, synthetic construct
  source 1..19: mol_type = other RNA; note = GPSZRA271S2 sense strand
  modified_base order(1^2,18^19): mod_base = OTHER; note = phosphorothioate linkage
  modified_base order(1,2,4,5,6,10,12,14,16,17,18,19): mod_base = OTHER; note = 2'-methoxy-modified
  modified_base order(3,7,8,9,11,13,15): mod_base = OTHER; note = 2'-fluoro-modified
agctcctggtggaaccgta

SEQ ID NO: 1200 - RNA, 19 nt, synthetic construct
  source 1..19: mol_type = other RNA; note = GPSZRA272S2 sense strand
  modified_base order(1^2,18^19): mod_base = OTHER; note = phosphorothioate linkage
  modified_base order(1,2,4,5,6,10,12,14,16,17,18,19): mod_base = OTHER; note = 2'-methoxy-modified
  modified_base order(3,7,8,9,11,13,15): mod_base = OTHER; note = 2'-fluoro-modified
gctcctggtggaaccgtaa

SEQ ID NO: 1201 - RNA, 19 nt, synthetic construct
  source 1..19: mol_type = other RNA; note = GPSZRA274S2 sense strand
  modified_base order(1^2,18^19): mod_base = OTHER; note = phosphorothioate linkage
  modified_base order(1,2,4,5,6,10,12,14,16,17,18,19): mod_base = OTHER; note = 2'-methoxy-modified
  modified_base order(3,7,8,9,11,13,15): mod_base = OTHER; note = 2'-fluoro-modified
tcctggtggaaccgtaacc

SEQ ID NO: 1202 - RNA, 19 nt, synthetic construct
  source 1..19: mol_type = other RNA; note = GPSZRA275S2 sense strand
  modified_base order(1^2,18^19): mod_base = OTHER; note = phosphorothioate linkage
  modified_base order(1,2,4,5,6,10,12,14,16,17,18,19): mod_base = OTHER; note = 2'-methoxy-modified
  modified_base order(3,7,8,9,11,13,15): mod_base = OTHER; note = 2'-fluoro-modified
ctggtggaaccgtaaccct

SEQ ID NO: 1203 - RNA, 19 nt, synthetic construct
  source 1..19: mol_type = other RNA; note = GPSZRA276S2 sense strand
  modified_base order(1^2,18^19): mod_base = OTHER; note = phosphorothioate linkage
  modified_base order(1,2,4,5,6,10,12,14,16,17,18,19): mod_base = OTHER; note = 2'-methoxy-modified
  modified_base order(3,7,8,9,11,13,15): mod_base = OTHER; note = 2'-fluoro-modified
tggtggaaccgtaaccctg

SEQ ID NO: 1204 - RNA, 19 nt, synthetic construct
  source 1..19: mol_type = other RNA; note = GPSZRA277S2 sense strand
  modified_base order(1^2,18^19): mod_base = OTHER; note = phosphorothioate linkage
  modified_base order(1,2,4,5,6,10,12,14,16,17,18,19): mod_base = OTHER; note = 2'-methoxy-modified
  modified_base order(3,7,8,9,11,13,15): mod_base = OTHER; note = 2'-fluoro-modified
ggtggaaccgtaaccctga

SEQ ID NO: 1205 - RNA, 19 nt, synthetic construct
  source 1..19: mol_type = other RNA; note = GPSZRA281S2 sense strand
  modified_base order(1^2,18^19): mod_base = OTHER; note = phosphorothioate linkage
  modified_base order(1,2,4,5,6,10,12,14,16,17,18,19): mod_base = OTHER; note = 2'-methoxy-modified
  modified_base order(3,7,8,9,11,13,15): mod_base = OTHER; note = 2'-fluoro-modified
gaaccgtaaccctgacctg

SEQ ID NO: 1206 - RNA, 19 nt, synthetic construct
  source 1..19: mol_type = other RNA; note = GPSZRA282S2 sense strand
  modified_base order(1^2,18^19): mod_base = OTHER; note = phosphorothioate linkage
  modified_base order(1,2,4,5,6,10,12,14,16,17,18,19): mod_base = OTHER; note = 2'-methoxy-modified
  modified_base order(3,7,8,9,11,13,15): mod_base = OTHER; note = 2'-fluoro-modified
aaccgtaaccctgacctgt

SEQ ID NO: 1207 - RNA, 19 nt, synthetic construct
  source 1..19: mol_type = other RNA; note = GPSZRA283S2 sense strand
  modified_base order(1^2,18^19): mod_base = OTHER; note = phosphorothioate linkage
  modified_base order(1,2,4,5,6,10,12,14,16,17,18,19): mod_base = OTHER; note = 2'-methoxy-modified
  modified_base order(3,7,8,9,11,13,15): mod_base = OTHER; note = 2'-fluoro-modified
accgtaaccctgacctgtg

SEQ ID NO: 1208 - RNA, 19 nt, synthetic construct
  source 1..19: mol_type = other RNA; note = GPSZRA284S2 sense strand
  modified_base order(1^2,18^19): mod_base = OTHER; note = phosphorothioate linkage
  modified_base order(1,2,4,5,6,10,12,14,16,17,18,19): mod_base = OTHER; note = 2'-methoxy-modified
  modified_base order(3,7,8,9,11,13,15): mod_base = OTHER; note = 2'-fluoro-modified
ccgtaaccctgacctgtga

SEQ ID NO: 1209 - RNA, 19 nt, synthetic construct
  source 1..19: mol_type = other RNA; note = GPSZRA285S2 sense strand
  modified_base order(1^2,18^19): mod_base = OTHER; note = phosphorothioate linkage
  modified_base order(1,2,4,5,6,10,12,14,16,17,18,19): mod_base = OTHER; note = 2'-methoxy-modified
  modified_base order(3,7,8,9,11,13,15): mod_base = OTHER; note = 2'-fluoro-modified
cgtaaccctgacctgtgaa

SEQ ID NO: 1210 - RNA, 19 nt, synthetic construct
  source 1..19: mol_type = other RNA; note = GPSZRA286S2 sense strand
  modified_base order(1^2,18^19): mod_base = OTHER; note = phosphorothioate linkage
  modified_base order(1,2,4,5,6,10,12,14,16,17,18,19): mod_base = OTHER; note = 2'-methoxy-modified
  modified_base order(3,7,8,9,11,13,15): mod_base = OTHER; note = 2'-fluoro-modified
gtaaccctgacctgtgaag

SEQ ID NO: 1211 - RNA, 19 nt, synthetic construct
  source 1..19: mol_type = other RNA; note = GPSZRA287S2 sense strand
  modified_base order(1^2,18^19): mod_base = OTHER; note = phosphorothioate linkage
  modified_base order(1,2,4,5,6,10,12,14,16,17,18,19): mod_base = OTHER; note = 2'-methoxy-modified
  modified_base order(3,7,8,9,11,13,15): mod_base = OTHER; note = 2'-fluoro-modified
taaccctgacctgtgaagt

SEQ ID NO: 1212 - RNA, 19 nt, synthetic construct
  source 1..19: mol_type = other RNA; note = GPSZRA288S2 sense strand
  modified_base order(1^2,18^19): mod_base = OTHER; note = phosphorothioate linkage
  modified_base order(1,2,4,5,6,10,12,14,16,17,18,19): mod_base = OTHER; note = 2'-methoxy-modified
  modified_base order(3,7,8,9,11,13,15): mod_base = OTHER; note = 2'-fluoro-modified
aaccctgacctgtgaagtc

SEQ ID NO: 1213 - RNA, 19 nt, synthetic construct
  source 1..19: mol_type = other RNA; note = GPSZRA290S2 sense strand
  modified_base order(1^2,18^19): mod_base = OTHER; note = phosphorothioate linkage
  modified_base order(1,2,4,5,6,10,12,14,16,17,18,19): mod_base = OTHER; note = 2'-methoxy-modified
  modified_base order(3,7,8,9,11,13,15): mod_base = OTHER; note = 2'-fluoro-modified
cctgacctgtgaagtccct

SEQ ID NO: 1214 - RNA, 19 nt, synthetic construct
  source 1..19: mol_type = other RNA; note = GPSZRA292S2 sense strand
  modified_base order(1^2,18^19): mod_base = OTHER; note = phosphorothioate linkage
  modified_base order(1,2,4,5,6,10,12,14,16,17,18,19): mod_base = OTHER; note = 2'-methoxy-modified
  modified_base order(3,7,8,9,11,13,15): mod_base = OTHER; note = 2'-fluoro-modified
tgacctgtgaagtccctgc

SEQ ID NO: 1215 - RNA, 19 nt, synthetic construct
  source 1..19: mol_type = other RNA; note = GPSZRA301S2 sense strand
  modified_base order(1^2,18^19): mod_base = OTHER; note = phosphorothioate linkage
  modified_base order(1,2,4,5,6,10,12,14,16,17,18,19): mod_base = OTHER; note = 2'-methoxy-modified
  modified_base order(3,7,8,9,11,13,15): mod_base = OTHER; note = 2'-fluoro-modified
tctcctcaaatccactgga

SEQ ID NO: 1216 - RNA, 19 nt, synthetic construct
  source 1..19: mol_type = other RNA; note = GPSZRA308S2 sense strand
  modified_base order(1^2,18^19): mod_base = OTHER; note = phosphorothioate linkage
  modified_base order(1,2,4,5,6,10,12,14,16,17,18,19): mod_base = OTHER; note = 2'-methoxy-modified
  modified_base order(3,7,8,9,11,13,15): mod_base = OTHER; note = 2'-fluoro-modified
aaatccactggatgaagga

SEQ ID NO: 1217 - RNA, 19 nt, synthetic construct
  source 1..19: mol_type = other RNA; note = GPSZRA311S2 sense strand
  modified_base order(1^2,18^19): mod_base = OTHER; note = phosphorothioate linkage
  modified_base order(1,2,4,5,6,10,12,14,16,17,18,19): mod_base = OTHER; note = 2'-methoxy-modified
  modified_base order(3,7,8,9,11,13,15): mod_base = OTHER; note = 2'-fluoro-modified
tccactggatgaaggatgg

SEQ ID NO: 1218 - RNA, 19 nt, synthetic construct
  source 1..19: mol_type = other RNA; note = GPSZRA312S2 sense strand
  modified_base order(1^2,18^19): mod_base = OTHER; note = phosphorothioate linkage
  modified_base order(1,2,4,5,6,10,12,14,16,17,18,19): mod_base = OTHER; note = 2'-methoxy-modified
  modified_base order(3,7,8,9,11,13,15): mod_base = OTHER; note = 2'-fluoro-modified
ccactggatgaaggatggt

SEQ ID NO: 1219 - RNA, 19 nt, synthetic construct
  source 1..19: mol_type = other RNA; note = GPSZRA313S2 sense strand
  modified_base order(1^2,18^19): mod_base = OTHER; note = phosphorothioate linkage
  modified_base order(1,2,4,5,6,10,12,14,16,17,18,19): mod_base = OTHER; note = 2'-methoxy-modified
  modified_base order(3,7,8,9,11,13,15): mod_base = OTHER; note = 2'-fluoro-modified
cactggatgaaggatggtg

SEQ ID NO: 1220 - RNA, 19 nt, synthetic construct
  source 1..19: mol_type = other RNA; note = GPSZRA314S2/GPSZRA314S2-VP sense strand
  modified_base order(1^2,18^19): mod_base = OTHER; note = phosphorothioate linkage
  modified_base order(1,2,4,5,6,10,12,14,16,17,18,19): mod_base = OTHER; note = 2'-methoxy-modified
  modified_base order(3,7,8,9,11,13,15): mod_base = OTHER; note = 2'-fluoro-modified
actggatgaaggatggtgt

SEQ ID NO: 1221 - RNA, 19 nt, synthetic construct
  source 1..19: mol_type = other RNA; note = GPSZRA315S2 sense strand
  modified_base order(1^2,18^19): mod_base = OTHER; note = phosphorothioate linkage
  modified_base order(1,2,4,5,6,10,12,14,16,17,18,19): mod_base = OTHER; note = 2'-methoxy-modified
  modified_base order(3,7,8,9,11,13,15): mod_base = OTHER; note = 2'-fluoro-modified
ctggatgaaggatggtgtg

SEQ ID NO: 1222 - RNA, 19 nt, synthetic construct
  source 1..19: mol_type = other RNA; note = GPSZRA316S2 sense strand
  modified_base order(1^2,18^19): mod_base = OTHER; note = phosphorothioate linkage
  modified_base order(1,2,4,5,6,10,12,14,16,17,18,19): mod_base = OTHER; note = 2'-methoxy-modified
  modified_base order(3,7,8,9,11,13,15): mod_base = OTHER; note = 2'-fluoro-modified
tggatgaaggatggtgtgc

SEQ ID NO: 1223 - RNA, 19 nt, synthetic construct
  source 1..19: mol_type = other RNA; note = GPSZRA317S2 sense strand
  modified_base order(1^2,18^19): mod_base = OTHER; note = phosphorothioate linkage
  modified_base order(1,2,4,5,6,10,12,14,16,17,18,19): mod_base = OTHER; note = 2'-methoxy-modified
  modified_base order(3,7,8,9,11,13,15): mod_base = OTHER; note = 2'-fluoro-modified
ggatgaaggatggtgtgcc

SEQ ID NO: 1224 - RNA, 19 nt, synthetic construct
  source 1..19: mol_type = other RNA; note = GPSZRA318S2/GPSZRA318S2-VP sense strand
  modified_base order(1^2,18^19): mod_base = OTHER; note = phosphorothioate linkage
  modified_base order(1,2,4,5,6,10,12,14,16,17,18,19): mod_base = OTHER; note = 2'-methoxy-modified
  modified_base order(3,7,8,9,11,13,15): mod_base = OTHER; note = 2'-fluoro-modified
gatgaaggatggtgtgccc

SEQ ID NO: 1225 - RNA, 19 nt, synthetic construct
  source 1..19: mol_type = other RNA; note = GPSZRA320S2 sense strand
  modified_base order(1^2,18^19): mod_base = OTHER; note = phosphorothioate linkage
  modified_base order(1,2,4,5,6,10,12,14,16,17,18,19): mod_base = OTHER; note = 2'-methoxy-modified
  modified_base order(3,7,8,9,11,13,15): mod_base = OTHER; note = 2'-fluoro-modified
tgaaggatggtgtgccctt

SEQ ID NO: 1226 - RNA, 19 nt, synthetic construct
  source 1..19: mol_type = other RNA; note = GPSZRA333S2 sense strand
  modified_base order(1^2,18^19): mod_base = OTHER; note = phosphorothioate linkage
  modified_base order(1,2,4,5,6,10,12,14,16,17,18,19): mod_base = OTHER; note = 2'-methoxy-modified
  modified_base order(3,7,8,9,11,13,15): mod_base = OTHER; note = 2'-fluoro-modified
gaaagccgtgctgtcagca

SEQ ID NO: 1227 - RNA, 19 nt, synthetic construct
  source 1..19: mol_type = other RNA; note = GPSZRA342S2 sense strand
  modified_base order(1^2,18^19): mod_base = OTHER; note = phosphorothioate linkage
  modified_base order(1,2,4,5,6,10,12,14,16,17,18,19): mod_base = OTHER; note = 2'-methoxy-modified
  modified_base order(3,7,8,9,11,13,15): mod_base = OTHER; note = 2'-fluoro-modified
tgtcagcatcagcatcatc

SEQ ID NO: 1228 - RNA, 19 nt, synthetic construct
  source 1..19: mol_type = other RNA; note = GPSZRA378S2 sense strand
  modified_base order(1^2,18^19): mod_base = OTHER; note = phosphorothioate linkage
  modified_base order(1,2,4,5,6,10,12,14,16,17,18,19): mod_base = OTHER; note = 2'-methoxy-modified
  modified_base order(3,7,8,9,11,13,15): mod_base = OTHER; note = 2'-fluoro-modified
aagaggaggagcgtgcaga

SEQ ID NO: 1229 - RNA, 19 nt, synthetic construct
  source 1..19: mol_type = other RNA; note = GPSZRA379S2 sense strand
  modified_base order(1^2,18^19): mod_base = OTHER; note = phosphorothioate linkage
  modified_base order(1,2,4,5,6,10,12,14,16,17,18,19): mod_base = OTHER; note = 2'-methoxy-modified
  modified_base order(3,7,8,9,11,13,15): mod_base = OTHER; note = 2'-fluoro-modified
gaatcagtcggaggaacct

SEQ ID NO: 1230 - RNA, 19 nt, synthetic construct
  source 1..19: mol_type = other RNA; note = GPSZRA380S2 sense strand
  modified_base order(1^2,18^19): mod_base = OTHER; note = phosphorothioate linkage
  modified_base order(1,2,4,5,6,10,12,14,16,17,18,19): mod_base = OTHER; note = 2'-methoxy-modified
  modified_base order(3,7,8,9,11,13,15): mod_base = OTHER; note = 2'-fluoro-modified
aatcagtcggaggaacctg

SEQ ID NO: 1231 - RNA, 19 nt, synthetic construct
  source 1..19: mol_type = other RNA; note = GPSZRA381S2 sense strand
  modified_base order(1^2,18^19): mod_base = OTHER; note = phosphorothioate linkage
  modified_base order(1,2,4,5,6,10,12,14,16,17,18,19): mod_base = OTHER; note = 2'-methoxy-modified
  modified_base order(3,7,8,9,11,13,15): mod_base = OTHER; note = 2'-fluoro-modified
atcagtcggaggaacctga

SEQ ID NO: 1232 - RNA, 19 nt, synthetic construct
  source 1..19: mol_type = other RNA; note = GPSZRA402S2 sense strand
  modified_base order(1^2,18^19): mod_base = OTHER; note = phosphorothioate linkage
  modified_base order(1,2,4,5,6,10,12,14,16,17,18,19): mod_base = OTHER; note = 2'-methoxy-modified
  modified_base order(3,7,8,9,11,13,15): mod_base = OTHER; note = 2'-fluoro-modified
ccaactctctcctgtataa

SEQ ID NO: 1233 - RNA, 19 nt, synthetic construct
  source 1..19: mol_type = other RNA; note = GPSZRA407S2 sense strand
  modified_base order(1^2,18^19): mod_base = OTHER; note = phosphorothioate linkage
  modified_base order(1,2,4,5,6,10,12,14,16,17,18,19): mod_base = OTHER; note = 2'-methoxy-modified
  modified_base order(3,7,8,9,11,13,15): mod_base = OTHER; note = 2'-fluoro-modified
cctgtataaccccaccttg

SEQ ID NO: 1234 - RNA, 19 nt, synthetic construct
  source 1..19: mol_type = other RNA; note = GPSZRA408S2 sense strand
  modified_base order(1^2,18^19): mod_base = OTHER; note = phosphorothioate linkage
  modified_base order(1,2,4,5,6,10,12,14,16,17,18,19): mod_base = OTHER; note = 2'-methoxy-modified
  modified_base order(3,7,8,9,11,13,15): mod_base = OTHER; note = 2'-fluoro-modified
ctgtataaccccaccttgc

SEQ ID NO: 1235 - RNA, 19 nt, synthetic construct
  source 1..19: mol_type = other RNA; note = GPSZRA409S2 sense strand
  modified_base order(1^2,18^19): mod_base = OTHER; note = phosphorothioate linkage
  modified_base order(1,2,4,5,6,10,12,14,16,17,18,19): mod_base = OTHER; note = 2'-methoxy-modified
  modified_base order(3,7,8,9,11,13,15): mod_base = OTHER; note = 2'-fluoro-modified
tgtataaccccaccttgcc

SEQ ID NO: 1236 - RNA, 19 nt, synthetic construct
  source 1..19: mol_type = other RNA; note = GPSZRA410S2 sense strand
  modified_base order(1^2,18^19): mod_base = OTHER; note = phosphorothioate linkage
  modified_base order(1,2,4,5,6,10,12,14,16,17,18,19): mod_base = OTHER; note = 2'-methoxy-modified
  modified_base order(3,7,8,9,11,13,15): mod_base = OTHER; note = 2'-fluoro-modified
gtataaccccaccttgcca

SEQ ID NO: 1237 - RNA, 19 nt, synthetic construct
  source 1..19: mol_type = other RNA; note = GPSZRA411S2 sense strand
  modified_base order(1^2,18^19): mod_base = OTHER; note = phosphorothioate linkage
  modified_base order(1,2,4,5,6,10,12,14,16,17,18,19): mod_base = OTHER; note = 2'-methoxy-modified
  modified_base order(3,7,8,9,11,13,15): mod_base = OTHER; note = 2'-fluoro-modified
tataaccccaccttgccaa

SEQ ID NO: 1238 - RNA, 19 nt, synthetic construct
  source 1..19: mol_type = other RNA; note = GPSZRA084S3 sense strand
  modified_base order(1^2,18^19): mod_base = OTHER; note = phosphorothioate linkage
  modified_base order(1,2,3,4,5,6,10,11,12,13,14,15,16,17,18,19): mod_base = OTHER; note = 2'-methoxy-modified
  modified_base order(7,8,9): mod_base = OTHER; note = 2'-fluoro-modified
ggaaaggagaccaagtcca

SEQ ID NO: 1239 - RNA, 19 nt, synthetic construct
  source 1..19: mol_type = other RNA; note = GPSZRA087S3 sense strand
  modified_base order(1^2,18^19): mod_base = OTHER; note = phosphorothioate linkage
  modified_base order(1,2,3,4,5,6,10,11,12,13,14,15,16,17,18,19): mod_base = OTHER; note = 2'-methoxy-modified
  modified_base order(7,8,9): mod_base = OTHER; note = 2'-fluoro-modified
aaggagaccaagtccaact

SEQ ID NO: 1240 - RNA, 19 nt, synthetic construct
  source 1..19: mol_type = other RNA; note = GPSZRA092S3 sense strand
  modified_base order(1^2,18^19): mod_base = OTHER; note = phosphorothioate linkage
  modified_base order(1,2,3,4,5,6,10,11,12,13,14,15,16,17,18,19): mod_base = OTHER; note = 2'-methoxy-modified
  modified_base order(7,8,9): mod_base = OTHER; note = 2'-fluoro-modified
gaccaagtccaactaccga

SEQ ID NO: 1241 - RNA, 19 nt, synthetic construct
  source 1..19: mol_type = other RNA; note = GPSZRA093S3 sense strand
  modified_base order(1^2,18^19): mod_base = OTHER; note = phosphorothioate linkage
  modified_base order(1,2,3,4,5,6,10,11,12,13,14,15,16,17,18,19): mod_base = OTHER; note = 2'-methoxy-modified
  modified_base order(7,8,9): mod_base = OTHER; note = 2'-fluoro-modified
accaagtccaactaccgag

SEQ ID NO: 1242 - RNA, 19 nt, synthetic construct
  source 1..19: mol_type = other RNA; note = GPSZRA097S3 sense strand
  modified_base order(1^2,18^19): mod_base = OTHER; note = phosphorothioate linkage
  modified_base order(1,2,3,4,5,6,10,11,12,13,14,15,16,17,18,19): mod_base = OTHER; note = 2'-methoxy-modified
  modified_base order(7,8,9): mod_base = OTHER; note = 2'-fluoro-modified
agtccaactaccgagtccg

SEQ ID NO: 1243 - RNA, 19 nt, synthetic construct
  source 1..19: mol_type = other RNA; note = GPSZRA118S3 sense strand
  modified_base order(1^2,18^19): mod_base = OTHER; note = phosphorothioate linkage
  modified_base order(1,2,3,4,5,6,10,11,12,13,14,15,16,17,18,19): mod_base = OTHER; note = 2'-methoxy-modified
  modified_base order(7,8,9): mod_base = OTHER; note = 2'-fluoro-modified
ctaccagattcctgggaag

SEQ ID NO: 1244 - RNA, 19 nt, synthetic construct
  source 1..19: mol_type = other RNA; note = GPSZRA217S3 sense strand
  modified_base order(1^2,18^19): mod_base = OTHER; note = phosphorothioate linkage
  modified_base order(1,2,3,4,5,6,10,11,12,13,14,15,16,17,18,19): mod_base = OTHER; note = 2'-methoxy-modified
  modified_base order(7,8,9): mod_base = OTHER; note = 2'-fluoro-modified
agggagtatctgtgaagga

SEQ ID NO: 1245 - RNA, 19 nt, synthetic construct
  source 1..19: mol_type = other RNA; note = GPSZRA222S3/GPSZRA222S3-VP sense strand
  modified_base order(1^2,18^19): mod_base = OTHER; note = phosphorothioate linkage
  modified_base order(1,2,3,4,5,6,10,11,12,13,14,15,16,17,18,19): mod_base = OTHER; note = 2'-methoxy-modified
  modified_base order(7,8,9): mod_base = OTHER; note = 2'-fluoro-modified
tcttcacactgcagtcgga

SEQ ID NO: 1246 - RNA, 19 nt, synthetic construct
  source 1..19: mol_type = other RNA; note = GPSZRA227S3 sense strand
  modified_base order(1^2,18^19): mod_base = OTHER; note = phosphorothioate linkage
  modified_base order(1,2,3,4,5,6,10,11,12,13,14,15,16,17,18,19): mod_base = OTHER; note = 2'-methoxy-modified
  modified_base order(7,8,9): mod_base = OTHER; note = 2'-fluoro-modified
acactgcagtcggagctaa

SEQ ID NO: 1247 - RNA, 19 nt, synthetic construct
  source 1..19: mol_type = other RNA; note = GPSZRA228S3 sense strand
  modified_base order(1^2,18^19): mod_base = OTHER; note = phosphorothioate linkage
  modified_base order(1,2,3,4,5,6,10,11,12,13,14,15,16,17,18,19): mod_base = OTHER; note = 2'-methoxy-modified
  modified_base order(7,8,9): mod_base = OTHER; note = 2'-fluoro-modified
cactgcagtcggagctaat

SEQ ID NO: 1248 - RNA, 19 nt, synthetic construct
  source 1..19: mol_type = other RNA; note = GPSZRA229S3 sense strand
  modified_base order(1^2,18^19): mod_base = OTHER; note = phosphorothioate linkage
  modified_base order(1,2,3,4,5,6,10,11,12,13,14,15,16,17,18,19): mod_base = OTHER; note = 2'-methoxy-modified
  modified_base order(7,8,9): mod_base = OTHER; note = 2'-fluoro-modified
actgcagtcggagctaatg

SEQ ID NO: 1249 - RNA, 19 nt, synthetic construct
  source 1..19: mol_type = other RNA; note = GPSZRA231S3 sense strand
  modified_base order(1^2,18^19): mod_base = OTHER; note = phosphorothioate linkage
  modified_base order(1,2,3,4,5,6,10,11,12,13,14,15,16,17,18,19): mod_base = OTHER; note = 2'-methoxy-modified
  modified_base order(7,8,9): mod_base = OTHER; note = 2'-fluoro-modified
tgcagtcggagctaatggt

SEQ ID NO: 1250 - RNA, 19 nt, synthetic construct
  source 1..19: mol_type = other RNA; note = GPSZRA232S3 sense strand
  modified_base order(1^2,18^19): mod_base = OTHER; note = phosphorothioate linkage
  modified_base order(1,2,3,4,5,6,10,11,12,13,14,15,16,17,18,19): mod_base = OTHER; note = 2'-methoxy-modified
  modified_base order(7,8,9): mod_base = OTHER; note = 2'-fluoro-modified
gcagtcggagctaatggtg

SEQ ID NO: 1251 - RNA, 19 nt, synthetic construct
  source 1..19: mol_type = other RNA; note = GPSZRA233S3 sense strand
  modified_base order(1^2,18^19): mod_base = OTHER; note = phosphorothioate linkage
  modified_base order(1,2,3,4,5,6,10,11,12,13,14,15,16,17,18,19): mod_base = OTHER; note = 2'-methoxy-modified
  modified_base order(7,8,9): mod_base = OTHER; note = 2'-fluoro-modified
cagtcggagctaatggtga

SEQ ID NO: 1252 - RNA, 19 nt, synthetic construct
  source 1..19: mol_type = other RNA; note = GPSZRA252S3 sense strand
  modified_base order(1^2,18^19): mod_base = OTHER; note = phosphorothioate linkage
  modified_base order(1,2,3,4,5,6,10,11,12,13,14,15,16,17,18,19): mod_base = OTHER; note = 2'-methoxy-modified
  modified_base order(7,8,9): mod_base = OTHER; note = 2'-fluoro-modified
tctggaggaggtccaattg

SEQ ID NO: 1253 - RNA, 19 nt, synthetic construct
  source 1..19: mol_type = other RNA; note = GPSZRA257S3 sense strand
  modified_base order(1^2,18^19): mod_base = OTHER; note = phosphorothioate linkage
  modified_base order(1,2,3,4,5,6,10,11,12,13,14,15,16,17,18,19): mod_base = OTHER; note = 2'-methoxy-modified
  modified_base order(7,8,9): mod_base = OTHER; note = 2'-fluoro-modified
aggaggtccaattggtggt

SEQ ID NO: 1254 - RNA, 19 nt, synthetic construct
  source 1..19: mol_type = other RNA; note = GPSZRA266S3 sense strand
  modified_base order(1^2,18^19): mod_base = OTHER; note = phosphorothioate linkage
  modified_base order(1,2,3,4,5,6,10,11,12,13,14,15,16,17,18,19): mod_base = OTHER; note = 2'-methoxy-modified
  modified_base order(7,8,9): mod_base = OTHER; note = 2'-fluoro-modified
agcagtagctcctggtgga

SEQ ID NO: 1255 - RNA, 19 nt, synthetic construct
  source 1..19: mol_type = other RNA; note = GPSZRA267S3 sense strand
  modified_base order(1^2,18^19): mod_base = OTHER; note = phosphorothioate linkage
  modified_base order(1,2,3,4,5,6,10,11,12,13,14,15,16,17,18,19): mod_base = OTHER; note = 2'-methoxy-modified
  modified_base order(7,8,9): mod_base = OTHER; note = 2'-fluoro-modified
gcagtagctcctggtggaa

SEQ ID NO: 1256 - RNA, 19 nt, synthetic construct
  source 1..19: mol_type = other RNA; note = GPSZRA271S3 sense strand
  modified_base order(1^2,18^19): mod_base = OTHER; note = phosphorothioate linkage
  modified_base order(1,2,3,4,5,6,10,11,12,13,14,15,16,17,18,19): mod_base = OTHER; note = 2'-methoxy-modified
  modified_base order(7,8,9): mod_base = OTHER; note = 2'-fluoro-modified
agctcctggtggaaccgta

SEQ ID NO: 1257 - RNA, 19 nt, synthetic construct
  source 1..19: mol_type = other RNA; note = GPSZRA272S3 sense strand
  modified_base order(1^2,18^19): mod_base = OTHER; note = phosphorothioate linkage
  modified_base order(1,2,3,4,5,6,10,11,12,13,14,15,16,17,18,19): mod_base = OTHER; note = 2'-methoxy-modified
  modified_base order(7,8,9): mod_base = OTHER; note = 2'-fluoro-modified
gctcctggtggaaccgtaa

SEQ ID NO: 1258 - RNA, 19 nt, synthetic construct
  source 1..19: mol_type = other RNA; note = GPSZRA274S3 sense strand
  modified_base order(1^2,18^19): mod_base = OTHER; note = phosphorothioate linkage
  modified_base order(1,2,3,4,5,6,10,11,12,13,14,15,16,17,18,19): mod_base = OTHER; note = 2'-methoxy-modified
  modified_base order(7,8,9): mod_base = OTHER; note = 2'-fluoro-modified
tcctggtggaaccgtaacc

SEQ ID NO: 1259 - RNA, 19 nt, synthetic construct
  source 1..19: mol_type = other RNA; note = GPSZRA275S3 sense strand
  modified_base order(1^2,18^19): mod_base = OTHER; note = phosphorothioate linkage
  modified_base order(1,2,3,4,5,6,10,11,12,13,14,15,16,17,18,19): mod_base = OTHER; note = 2'-methoxy-modified
  modified_base order(7,8,9): mod_base = OTHER; note = 2'-fluoro-modified
ctggtggaaccgtaaccct

SEQ ID NO: 1260 - RNA, 19 nt, synthetic construct
  source 1..19: mol_type = other RNA; note = GPSZRA276S3 sense strand
  modified_base order(1^2,18^19): mod_base = OTHER; note = phosphorothioate linkage
  modified_base order(1,2,3,4,5,6,10,11,12,13,14,15,16,17,18,19): mod_base = OTHER; note = 2'-methoxy-modified
  modified_base order(7,8,9): mod_base = OTHER; note = 2'-fluoro-modified
tggtggaaccgtaaccctg

SEQ ID NO: 1261 - RNA, 19 nt, synthetic construct
  source 1..19: mol_type = other RNA; note = GPSZRA277S3 sense strand
  modified_base order(1^2,18^19): mod_base = OTHER; note = phosphorothioate linkage
  modified_base order(1,2,3,4,5,6,10,11,12,13,14,15,16,17,18,19): mod_base = OTHER; note = 2'-methoxy-modified
  modified_base order(7,8,9): mod_base = OTHER; note = 2'-fluoro-modified
ggtggaaccgtaaccctga

SEQ ID NO: 1262 - RNA, 19 nt, synthetic construct
  source 1..19: mol_type = other RNA; note = GPSZRA281S3 sense strand
  modified_base order(1^2,18^19): mod_base = OTHER; note = phosphorothioate linkage
  modified_base order(1,2,3,4,5,6,10,11,12,13,14,15,16,17,18,19): mod_base = OTHER; note = 2'-methoxy-modified
  modified_base order(7,8,9): mod_base = OTHER; note = 2'-fluoro-modified
gaaccgtaaccctgacctg

SEQ ID NO: 1263 - RNA, 19 nt, synthetic construct
  source 1..19: mol_type = other RNA; note = GPSZRA282S3 sense strand
  modified_base order(1^2,18^19): mod_base = OTHER; note = phosphorothioate linkage
  modified_base order(1,2,3,4,5,6,10,11,12,13,14,15,16,17,18,19): mod_base = OTHER; note = 2'-methoxy-modified
  modified_base order(7,8,9): mod_base = OTHER; note = 2'-fluoro-modified
aaccgtaaccctgacctgt

SEQ ID NO: 1264 - RNA, 19 nt, synthetic construct
  source 1..19: mol_type = other RNA; note = GPSZRA283S3 sense strand
  modified_base order(1^2,18^19): mod_base = OTHER; note = phosphorothioate linkage
  modified_base order(1,2,3,4,5,6,10,11,12,13,14,15,16,17,18,19): mod_base = OTHER; note = 2'-methoxy-modified
  modified_base order(7,8,9): mod_base = OTHER; note = 2'-fluoro-modified
accgtaaccctgacctgtg

SEQ ID NO: 1265 - RNA, 19 nt, synthetic construct
  source 1..19: mol_type = other RNA; note = GPSZRA284S3/GPSZRA284S3-VP sense strand
  modified_base order(1^2,18^19): mod_base = OTHER; note = phosphorothioate linkage
  modified_base order(1,2,3,4,5,6,10,11,12,13,14,15,16,17,18,19): mod_base = OTHER; note = 2'-methoxy-modified
  modified_base order(7,8,9): mod_base = OTHER; note = 2'-fluoro-modified
ccgtaaccctgacctgtga

SEQ ID NO: 1266 - RNA, 19 nt, synthetic construct
  source 1..19: mol_type = other RNA; note = GPSZRA285S3 sense strand
  modified_base order(1^2,18^19): mod_base = OTHER; note = phosphorothioate linkage
  modified_base order(1,2,3,4,5,6,10,11,12,13,14,15,16,17,18,19): mod_base = OTHER; note = 2'-methoxy-modified
  modified_base order(7,8,9): mod_base = OTHER; note = 2'-fluoro-modified
cgtaaccctgacctgtgaa

SEQ ID NO: 1267 - RNA, 19 nt, synthetic construct
  source 1..19: mol_type = other RNA; note = GPSZRA286S3 sense strand
  modified_base order(1^2,18^19): mod_base = OTHER; note = phosphorothioate linkage
  modified_base order(1,2,3,4,5,6,10,11,12,13,14,15,16,17,18,19): mod_base = OTHER; note = 2'-methoxy-modified
  modified_base order(7,8,9): mod_base = OTHER; note = 2'-fluoro-modified
gtaaccctgacctgtgaag

SEQ ID NO: 1268 - RNA, 19 nt, synthetic construct
  source 1..19: mol_type = other RNA; note = GPSZRA287S3 sense strand
  modified_base order(1^2,18^19): mod_base = OTHER; note = phosphorothioate linkage
  modified_base order(1,2,3,4,5,6,10,11,12,13,14,15,16,17,18,19): mod_base = OTHER; note = 2'-methoxy-modified
  modified_base order(7,8,9): mod_base = OTHER; note = 2'-fluoro-modified
taaccctgacctgtgaagt

SEQ ID NO: 1269 - RNA, 19 nt, synthetic construct
  source 1..19: mol_type = other RNA; note = GPSZRA288S3 sense strand
  modified_base order(1^2,18^19): mod_base = OTHER; note = phosphorothioate linkage
  modified_base order(1,2,3,4,5,6,10,11,12,13,14,15,16,17,18,19): mod_base = OTHER; note = 2'-methoxy-modified
  modified_base order(7,8,9): mod_base = OTHER; note = 2'-fluoro-modified
aaccctgacctgtgaagtc

SEQ ID NO: 1270 - RNA, 19 nt, synthetic construct
  source 1..19: mol_type = other RNA; note = GPSZRA290S3 sense strand
  modified_base order(1^2,18^19): mod_base = OTHER; note = phosphorothioate linkage
  modified_base order(1,2,3,4,5,6,10,11,12,13,14,15,16,17,18,19): mod_base = OTHER; note = 2'-methoxy-modified
  modified_base order(7,8,9): mod_base = OTHER; note = 2'-fluoro-modified
cctgacctgtgaagtccct

SEQ ID NO: 1271 - RNA, 19 nt, synthetic construct
  source 1..19: mol_type = other RNA; note = GPSZRA292S3 sense strand
  modified_base order(1^2,18^19): mod_base = OTHER; note = phosphorothioate linkage
  modified_base order(1,2,3,4,5,6,10,11,12,13,14,15,16,17,18,19): mod_base = OTHER; note = 2'-methoxy-modified
  modified_base order(7,8,9): mod_base = OTHER; note = 2'-fluoro-modified
tgacctgtgaagtccctgc

SEQ ID NO: 1272 - RNA, 19 nt, synthetic construct
  source 1..19: mol_type = other RNA; note = GPSZRA301S3 sense strand
  modified_base order(1^2,18^19): mod_base = OTHER; note = phosphorothioate linkage
  modified_base order(1,2,3,4,5,6,10,11,12,13,14,15,16,17,18,19): mod_base = OTHER; note = 2'-methoxy-modified
  modified_base order(7,8,9): mod_base = OTHER; note = 2'-fluoro-modified
tctcctcaaatccactgga

SEQ ID NO: 1273 - RNA, 19 nt, synthetic construct
  source 1..19: mol_type = other RNA; note = GPSZRA308S3 sense strand
  modified_base order(1^2,18^19): mod_base = OTHER; note = phosphorothioate linkage
  modified_base order(1,2,3,4,5,6,10,11,12,13,14,15,16,17,18,19): mod_base = OTHER; note = 2'-methoxy-modified
  modified_base order(7,8,9): mod_base = OTHER; note = 2'-fluoro-modified
aaatccactggatgaagga

SEQ ID NO: 1274 - RNA, 19 nt, synthetic construct
  source 1..19: mol_type = other RNA; note = GPSZRA311S3 sense strand
  modified_base order(1^2,18^19): mod_base = OTHER; note = phosphorothioate linkage
  modified_base order(1,2,3,4,5,6,10,11,12,13,14,15,16,17,18,19): mod_base = OTHER; note = 2'-methoxy-modified
  modified_base order(7,8,9): mod_base = OTHER; note = 2'-fluoro-modified
tccactggatgaaggatgg

SEQ ID NO: 1275 - RNA, 19 nt, synthetic construct
  source 1..19: mol_type = other RNA; note = GPSZRA312S3 sense strand
  modified_base order(1^2,18^19): mod_base = OTHER; note = phosphorothioate linkage
  modified_base order(1,2,3,4,5,6,10,11,12,13,14,15,16,17,18,19): mod_base = OTHER; note = 2'-methoxy-modified
  modified_base order(7,8,9): mod_base = OTHER; note = 2'-fluoro-modified
ccactggatgaaggatggt

SEQ ID NO: 1276 - RNA, 19 nt, synthetic construct
  source 1..19: mol_type = other RNA; note = GPSZRA313S3 sense strand
  modified_base order(1^2,18^19): mod_base = OTHER; note = phosphorothioate linkage
  modified_base order(1,2,3,4,5,6,10,11,12,13,14,15,16,17,18,19): mod_base = OTHER; note = 2'-methoxy-modified
  modified_base order(7,8,9): mod_base = OTHER; note = 2'-fluoro-modified
cactggatgaaggatggtg

SEQ ID NO: 1277 - RNA, 19 nt, synthetic construct
  source 1..19: mol_type = other RNA; note = GPSZRA314S3/GPSZRA314S3-VP sense strand
  modified_base order(1^2,18^19): mod_base = OTHER; note = phosphorothioate linkage
  modified_base order(1,2,3,4,5,6,10,11,12,13,14,15,16,17,18,19): mod_base = OTHER; note = 2'-methoxy-modified
  modified_base order(7,8,9): mod_base = OTHER; note = 2'-fluoro-modified
actggatgaaggatggtgt

SEQ ID NO: 1278 - RNA, 19 nt, synthetic construct
  source 1..19: mol_type = other RNA; note = GPSZRA315S3 sense strand
  modified_base order(1^2,18^19): mod_base = OTHER; note = phosphorothioate linkage
  modified_base order(1,2,3,4,5,6,10,11,12,13,14,15,16,17,18,19): mod_base = OTHER; note = 2'-methoxy-modified
  modified_base order(7,8,9): mod_base = OTHER; note = 2'-fluoro-modified
ctggatgaaggatggtgtg

SEQ ID NO: 1279 - RNA, 19 nt, synthetic construct
  source 1..19: mol_type = other RNA; note = GPSZRA316S3 sense strand
  modified_base order(1^2,18^19): mod_base = OTHER; note = phosphorothioate linkage
  modified_base order(1,2,3,4,5,6,10,11,12,13,14,15,16,17,18,19): mod_base = OTHER; note = 2'-methoxy-modified
  modified_base order(7,8,9): mod_base = OTHER; note = 2'-fluoro-modified
tggatgaaggatggtgtgc

SEQ ID NO: 1280 - RNA, 19 nt, synthetic construct
  source 1..19: mol_type = other RNA; note = GPSZRA317S3 sense strand
  modified_base order(1^2,18^19): mod_base = OTHER; note = phosphorothioate linkage
  modified_base order(1,2,3,4,5,6,10,11,12,13,14,15,16,17,18,19): mod_base = OTHER; note = 2'-methoxy-modified
  modified_base order(7,8,9): mod_base = OTHER; note = 2'-fluoro-modified
ggatgaaggatggtgtgcc

SEQ ID NO: 1281 - RNA, 19 nt, synthetic construct
  source 1..19: mol_type = other RNA; note = GPSZRA318S3 sense strand
  modified_base order(1^2,18^19): mod_base = OTHER; note = phosphorothioate linkage
  modified_base order(1,2,3,4,5,6,10,11,12,13,14,15,16,17,18,19): mod_base = OTHER; note = 2'-methoxy-modified
  modified_base order(7,8,9): mod_base = OTHER; note = 2'-fluoro-modified
gatgaaggatggtgtgccc

SEQ ID NO: 1282 - RNA, 19 nt, synthetic construct
  source 1..19: mol_type = other RNA; note = GPSZRA320S3 sense strand
  modified_base order(1^2,18^19): mod_base = OTHER; note = phosphorothioate linkage
  modified_base order(1,2,3,4,5,6,10,11,12,13,14,15,16,17,18,19): mod_base = OTHER; note = 2'-methoxy-modified
  modified_base order(7,8,9): mod_base = OTHER; note = 2'-fluoro-modified
tgaaggatggtgtgccctt

SEQ ID NO: 1283 - RNA, 19 nt, synthetic construct
  source 1..19: mol_type = other RNA; note = GPSZRA333S3 sense strand
  modified_base order(1^2,18^19): mod_base = OTHER; note = phosphorothioate linkage
  modified_base order(1,2,3,4,5,6,10,11,12,13,14,15,16,17,18,19): mod_base = OTHER; note = 2'-methoxy-modified
  modified_base order(7,8,9): mod_base = OTHER; note = 2'-fluoro-modified
gaaagccgtgctgtcagca

SEQ ID NO: 1284 - RNA, 19 nt, synthetic construct
  source 1..19: mol_type = other RNA; note = GPSZRA342S3 sense strand
  modified_base order(1^2,18^19): mod_base = OTHER; note = phosphorothioate linkage
  modified_base order(1,2,3,4,5,6,10,11,12,13,14,15,16,17,18,19): mod_base = OTHER; note = 2'-methoxy-modified
  modified_base order(7,8,9): mod_base = OTHER; note = 2'-fluoro-modified
tgtcagcatcagcatcatc

SEQ ID NO: 1285 - RNA, 19 nt, synthetic construct
  source 1..19: mol_type = other RNA; note = GPSZRA378S3 sense strand
  modified_base order(1^2,18^19): mod_base = OTHER; note = phosphorothioate linkage
  modified_base order(1,2,3,4,5,6,10,11,12,13,14,15,16,17,18,19): mod_base = OTHER; note = 2'-methoxy-modified
  modified_base order(7,8,9): mod_base = OTHER; note = 2'-fluoro-modified
aagaggaggagcgtgcaga

SEQ ID NO: 1286 - RNA, 19 nt, synthetic construct
  source 1..19: mol_type = other RNA; note = GPSZRA379S3 sense strand
  modified_base order(1^2,18^19): mod_base = OTHER; note = phosphorothioate linkage
  modified_base order(1,2,3,4,5,6,10,11,12,13,14,15,16,17,18,19): mod_base = OTHER; note = 2'-methoxy-modified
  modified_base order(7,8,9): mod_base = OTHER; note = 2'-fluoro-modified
gaatcagtcggaggaacct

SEQ ID NO: 1287 - RNA, 19 nt, synthetic construct
  source 1..19: mol_type = other RNA; note = GPSZRA380S3 sense strand
  modified_base order(1^2,18^19): mod_base = OTHER; note = phosphorothioate linkage
  modified_base order(1,2,3,4,5,6,10,11,12,13,14,15,16,17,18,19): mod_base = OTHER; note = 2'-methoxy-modified
  modified_base order(7,8,9): mod_base = OTHER; note = 2'-fluoro-modified
aatcagtcggaggaacctg

SEQ ID NO: 1288 - RNA, 19 nt, synthetic construct
  source 1..19: mol_type = other RNA; note = GPSZRA381S3 sense strand
  modified_base order(1^2,18^19): mod_base = OTHER; note = phosphorothioate linkage
  modified_base order(1,2,3,4,5,6,10,11,12,13,14,15,16,17,18,19): mod_base = OTHER; note = 2'-methoxy-modified
  modified_base order(7,8,9): mod_base = OTHER; note = 2'-fluoro-modified
atcagtcggaggaacctga

SEQ ID NO: 1289 - RNA, 19 nt, synthetic construct
  source 1..19: mol_type = other RNA; note = GPSZRA402S3 sense strand
  modified_base order(1^2,18^19): mod_base = OTHER; note = phosphorothioate linkage
  modified_base order(1,2,3,4,5,6,10,11,12,13,14,15,16,17,18,19): mod_base = OTHER; note = 2'-methoxy-modified
  modified_base order(7,8,9): mod_base = OTHER; note = 2'-fluoro-modified
ccaactctctcctgtataa

SEQ ID NO: 1290 - RNA, 19 nt, synthetic construct
  source 1..19: mol_type = other RNA; note = GPSZRA407S3 sense strand
  modified_base order(1^2,18^19): mod_base = OTHER; note = phosphorothioate linkage
  modified_base order(1,2,3,4,5,6,10,11,12,13,14,15,16,17,18,19): mod_base = OTHER; note = 2'-methoxy-modified
  modified_base order(7,8,9): mod_base = OTHER; note = 2'-fluoro-modified
cctgtataaccccaccttg

SEQ ID NO: 1291 - RNA, 19 nt, synthetic construct
  source 1..19: mol_type = other RNA; note = GPSZRA408S3 sense strand
  modified_base order(1^2,18^19): mod_base = OTHER; note = phosphorothioate linkage
  modified_base order(1,2,3,4,5,6,10,11,12,13,14,15,16,17,18,19): mod_base = OTHER; note = 2'-methoxy-modified
  modified_base order(7,8,9): mod_base = OTHER; note = 2'-fluoro-modified
ctgtataaccccaccttgc

SEQ ID NO: 1292 - RNA, 19 nt, synthetic construct
  source 1..19: mol_type = other RNA; note = GPSZRA409S3 sense strand
  modified_base order(1^2,18^19): mod_base = OTHER; note = phosphorothioate linkage
  modified_base order(1,2,3,4,5,6,10,11,12,13,14,15,16,17,18,19): mod_base = OTHER; note = 2'-methoxy-modified
  modified_base order(7,8,9): mod_base = OTHER; note = 2'-fluoro-modified
tgtataaccccaccttgcc

SEQ ID NO: 1293 - RNA, 19 nt, synthetic construct
  source 1..19: mol_type = other RNA; note = GPSZRA410S3 sense strand
  modified_base order(1^2,18^19): mod_base = OTHER; note = phosphorothioate linkage
  modified_base order(1,2,3,4,5,6,10,11,12,13,14,15,16,17,18,19): mod_base = OTHER; note = 2'-methoxy-modified
  modified_base order(7,8,9): mod_base = OTHER; note = 2'-fluoro-modified
gtataaccccaccttgcca

SEQ ID NO: 1294 - RNA, 19 nt, synthetic construct
  source 1..19: mol_type = other RNA; note = GPSZRA411S3 sense strand
  modified_base order(1^2,18^19): mod_base = OTHER; note = phosphorothioate linkage
  modified_base order(1,2,3,4,5,6,10,11,12,13,14,15,16,17,18,19): mod_base = OTHER; note = 2'-methoxy-modified
  modified_base order(7,8,9): mod_base = OTHER; note = 2'-fluoro-modified
tataaccccaccttgccaa

SEQ ID NO: 1295 - RNA, 19 nt, synthetic construct
  source 1..19: mol_type = other RNA; note = GPSZRA084S4 sense strand
  modified_base order(1^2,18^19): mod_base = OTHER; note = phosphorothioate linkage
  modified_base 1: mod_base = OTHER; note = locked nucleic acid-modified
  modified_base order(2,4,5,6,10,12,14,16,17,18,19): mod_base = OTHER; note = 2'-methoxy-modified
  modified_base order(3,7,8,9,11,13,15): mod_base = OTHER; note = 2'-fluoro-modified
ggaaaggagaccaagtcca

SEQ ID NO: 1296 - RNA, 19 nt, synthetic construct
  source 1..19: mol_type = other RNA; note = GPSZRA087S4 sense strand
  modified_base order(1^2,18^19): mod_base = OTHER; note = phosphorothioate linkage
  modified_base 1: mod_base = OTHER; note = locked nucleic acid-modified
  modified_base order(2,4,5,6,10,12,14,16,17,18,19): mod_base = OTHER; note = 2'-methoxy-modified
  modified_base order(3,7,8,9,11,13,15): mod_base = OTHER; note = 2'-fluoro-modified
aaggagaccaagtccaact

SEQ ID NO: 1297 - RNA, 19 nt, synthetic construct
  source 1..19: mol_type = other RNA; note = GPSZRA092S4 sense strand
  modified_base order(1^2,18^19): mod_base = OTHER; note = phosphorothioate linkage
  modified_base 1: mod_base = OTHER; note = locked nucleic acid-modified
  modified_base order(2,4,5,6,10,12,14,16,17,18,19): mod_base = OTHER; note = 2'-methoxy-modified
  modified_base order(3,7,8,9,11,13,15): mod_base = OTHER; note = 2'-fluoro-modified
gaccaagtccaactaccga

SEQ ID NO: 1298 - RNA, 19 nt, synthetic construct
  source 1..19: mol_type = other RNA; note = GPSZRA093S4 sense strand
  modified_base order(1^2,18^19): mod_base = OTHER; note = phosphorothioate linkage
  modified_base 1: mod_base = OTHER; note = locked nucleic acid-modified
  modified_base order(2,4,5,6,10,12,14,16,17,18,19): mod_base = OTHER; note = 2'-methoxy-modified
  modified_base order(3,7,8,9,11,13,15): mod_base = OTHER; note = 2'-fluoro-modified
accaagtccaactaccgag

SEQ ID NO: 1299 - RNA, 19 nt, synthetic construct
  source 1..19: mol_type = other RNA; note = GPSZRA097S4 sense strand
  modified_base order(1^2,18^19): mod_base = OTHER; note = phosphorothioate linkage
  modified_base 1: mod_base = OTHER; note = locked nucleic acid-modified
  modified_base order(2,4,5,6,10,12,14,16,17,18,19): mod_base = OTHER; note = 2'-methoxy-modified
  modified_base order(3,7,8,9,11,13,15): mod_base = OTHER; note = 2'-fluoro-modified
agtccaactaccgagtccg

SEQ ID NO: 1300 - RNA, 19 nt, synthetic construct
  source 1..19: mol_type = other RNA; note = GPSZRA118S4 sense strand
  modified_base order(1^2,18^19): mod_base = OTHER; note = phosphorothioate linkage
  modified_base 1: mod_base = OTHER; note = locked nucleic acid-modified
  modified_base order(2,4,5,6,10,12,14,16,17,18,19): mod_base = OTHER; note = 2'-methoxy-modified
  modified_base order(3,7,8,9,11,13,15): mod_base = OTHER; note = 2'-fluoro-modified
ctaccagattcctgggaag

SEQ ID NO: 1301 - RNA, 19 nt, synthetic construct
  source 1..19: mol_type = other RNA; note = GPSZRA217S4 sense strand
  modified_base order(1^2,18^19): mod_base = OTHER; note = phosphorothioate linkage
  modified_base 1: mod_base = OTHER; note = locked nucleic acid-modified
  modified_base order(2,4,5,6,10,12,14,16,17,18,19): mod_base = OTHER; note = 2'-methoxy-modified
  modified_base order(3,7,8,9,11,13,15): mod_base = OTHER; note = 2'-fluoro-modified
agggagtatctgtgaagga

SEQ ID NO: 1302 - RNA, 19 nt, synthetic construct
  source 1..19: mol_type = other RNA; note = GPSZRA222S4/GPSZRA222S4-VP sense strand
  modified_base order(1^2,18^19): mod_base = OTHER; note = phosphorothioate linkage
  modified_base 1: mod_base = OTHER; note = locked nucleic acid-modified
  modified_base order(2,4,5,6,10,12,14,16,17,18,19): mod_base = OTHER; note = 2'-methoxy-modified
  modified_base order(3,7,8,9,11,13,15): mod_base = OTHER; note = 2'-fluoro-modified
tcttcacactgcagtcgga

SEQ ID NO: 1303 - RNA, 19 nt, synthetic construct
  source 1..19: mol_type = other RNA; note = GPSZRA227S4 sense strand
  modified_base order(1^2,18^19): mod_base = OTHER; note = phosphorothioate linkage
  modified_base 1: mod_base = OTHER; note = locked nucleic acid-modified
  modified_base order(2,4,5,6,10,12,14,16,17,18,19): mod_base = OTHER; note = 2'-methoxy-modified
  modified_base order(3,7,8,9,11,13,15): mod_base = OTHER; note = 2'-fluoro-modified
acactgcagtcggagctaa

SEQ ID NO: 1304 - RNA, 19 nt, synthetic construct
  source 1..19: mol_type = other RNA; note = GPSZRA228S4 sense strand
  modified_base order(1^2,18^19): mod_base = OTHER; note = phosphorothioate linkage
  modified_base 1: mod_base = OTHER; note = locked nucleic acid-modified
  modified_base order(2,4,5,6,10,12,14,16,17,18,19): mod_base = OTHER; note = 2'-methoxy-modified
  modified_base order(3,7,8,9,11,13,15): mod_base = OTHER; note = 2'-fluoro-modified
cactgcagtcggagctaat

SEQ ID NO: 1305 - RNA, 19 nt, synthetic construct
  source 1..19: mol_type = other RNA; note = GPSZRA229S4 sense strand
  modified_base order(1^2,18^19): mod_base = OTHER; note = phosphorothioate linkage
  modified_base 1: mod_base = OTHER; note = locked nucleic acid-modified
  modified_base order(2,4,5,6,10,12,14,16,17,18,19): mod_base = OTHER; note = 2'-methoxy-modified
  modified_base order(3,7,8,9,11,13,15): mod_base = OTHER; note = 2'-fluoro-modified
actgcagtcggagctaatg

SEQ ID NO: 1306 - RNA, 19 nt, synthetic construct
  source 1..19: mol_type = other RNA; note = GPSZRA231S4 sense strand
  modified_base order(1^2,18^19): mod_base = OTHER; note = phosphorothioate linkage
  modified_base 1: mod_base = OTHER; note = locked nucleic acid-modified
  modified_base order(2,4,5,6,10,12,14,16,17,18,19): mod_base = OTHER; note = 2'-methoxy-modified
  modified_base order(3,7,8,9,11,13,15): mod_base = OTHER; note = 2'-fluoro-modified
tgcagtcggagctaatggt

SEQ ID NO: 1307 - RNA, 19 nt, synthetic construct
  source 1..19: mol_type = other RNA; note = GPSZRA232S4 sense strand
  modified_base order(1^2,18^19): mod_base = OTHER; note = phosphorothioate linkage
  modified_base 1: mod_base = OTHER; note = locked nucleic acid-modified
  modified_base order(2,4,5,6,10,12,14,16,17,18,19): mod_base = OTHER; note = 2'-methoxy-modified
  modified_base order(3,7,8,9,11,13,15): mod_base = OTHER; note = 2'-fluoro-modified
gcagtcggagctaatggtg

SEQ ID NO: 1308 - RNA, 19 nt, synthetic construct
  source 1..19: mol_type = other RNA; note = GPSZRA233S4 sense strand
  modified_base order(1^2,18^19): mod_base = OTHER; note = phosphorothioate linkage
  modified_base 1: mod_base = OTHER; note = locked nucleic acid-modified
  modified_base order(2,4,5,6,10,12,14,16,17,18,19): mod_base = OTHER; note = 2'-methoxy-modified
  modified_base order(3,7,8,9,11,13,15): mod_base = OTHER; note = 2'-fluoro-modified
cagtcggagctaatggtga

SEQ ID NO: 1309 - RNA, 19 nt, synthetic construct
  source 1..19: mol_type = other RNA; note = GPSZRA252S4 sense strand
  modified_base order(1^2,18^19): mod_base = OTHER; note = phosphorothioate linkage
  modified_base 1: mod_base = OTHER; note = locked nucleic acid-modified
  modified_base order(2,4,5,6,10,12,14,16,17,18,19): mod_base = OTHER; note = 2'-methoxy-modified
  modified_base order(3,7,8,9,11,13,15): mod_base = OTHER; note = 2'-fluoro-modified
tctggaggaggtccaattg

SEQ ID NO: 1310 - RNA, 19 nt, synthetic construct
  source 1..19: mol_type = other RNA; note = GPSZRA257S4 sense strand
  modified_base order(1^2,18^19): mod_base = OTHER; note = phosphorothioate linkage
  modified_base 1: mod_base = OTHER; note = locked nucleic acid-modified
  modified_base order(2,4,5,6,10,12,14,16,17,18,19): mod_base = OTHER; note = 2'-methoxy-modified
  modified_base order(3,7,8,9,11,13,15): mod_base = OTHER; note = 2'-fluoro-modified
aggaggtccaattggtggt

SEQ ID NO: 1311 - RNA, 19 nt, synthetic construct
  source 1..19: mol_type = other RNA; note = GPSZRA266S4 sense strand
  modified_base order(1^2,18^19): mod_base = OTHER; note = phosphorothioate linkage
  modified_base 1: mod_base = OTHER; note = locked nucleic acid-modified
  modified_base order(2,4,5,6,10,12,14,16,17,18,19): mod_base = OTHER; note = 2'-methoxy-modified
  modified_base order(3,7,8,9,11,13,15): mod_base = OTHER; note = 2'-fluoro-modified
agcagtagctcctggtgga

SEQ ID NO: 1312 - RNA, 19 nt, synthetic construct
  source 1..19: mol_type = other RNA; note = GPSZRA267S4 sense strand
  modified_base order(1^2,18^19): mod_base = OTHER; note = phosphorothioate linkage
  modified_base 1: mod_base = OTHER; note = locked nucleic acid-modified
  modified_base order(2,4,5,6,10,12,14,16,17,18,19): mod_base = OTHER; note = 2'-methoxy-modified
  modified_base order(3,7,8,9,11,13,15): mod_base = OTHER; note = 2'-fluoro-modified
gcagtagctcctggtggaa

SEQ ID NO: 1313 - RNA, 19 nt, synthetic construct
  source 1..19: mol_type = other RNA; note = GPSZRA271S4 sense strand
  modified_base order(1^2,18^19): mod_base = OTHER; note = phosphorothioate linkage
  modified_base 1: mod_base = OTHER; note = locked nucleic acid-modified
  modified_base order(2,4,5,6,10,12,14,16,17,18,19): mod_base = OTHER; note = 2'-methoxy-modified
  modified_base order(3,7,8,9,11,13,15): mod_base = OTHER; note = 2'-fluoro-modified
agctcctggtggaaccgta

SEQ ID NO: 1314 - RNA, 19 nt, synthetic construct
  source 1..19: mol_type = other RNA; note = GPSZRA272S4 sense strand
  modified_base order(1^2,18^19): mod_base = OTHER; note = phosphorothioate linkage
  modified_base 1: mod_base = OTHER; note = locked nucleic acid-modified
  modified_base order(2,4,5,6,10,12,14,16,17,18,19): mod_base = OTHER; note = 2'-methoxy-modified
  modified_base order(3,7,8,9,11,13,15): mod_base = OTHER; note = 2'-fluoro-modified
gctcctggtggaaccgtaa

SEQ ID NO: 1315 - RNA, 19 nt, synthetic construct
  source 1..19: mol_type = other RNA; note = GPSZRA274S4 sense strand
  modified_base order(1^2,18^19): mod_base = OTHER; note = phosphorothioate linkage
  modified_base 1: mod_base = OTHER; note = locked nucleic acid-modified
  modified_base order(2,4,5,6,10,12,14,16,17,18,19): mod_base = OTHER; note = 2'-methoxy-modified
  modified_base order(3,7,8,9,11,13,15): mod_base = OTHER; note = 2'-fluoro-modified
tcctggtggaaccgtaacc

SEQ ID NO: 1316 - RNA, 19 nt, synthetic construct
  source 1..19: mol_type = other RNA; note = GPSZRA275S4 sense strand
  modified_base order(1^2,18^19): mod_base = OTHER; note = phosphorothioate linkage
  modified_base 1: mod_base = OTHER; note = locked nucleic acid-modified
  modified_base order(2,4,5,6,10,12,14,16,17,18,19): mod_base = OTHER; note = 2'-methoxy-modified
  modified_base order(3,7,8,9,11,13,15): mod_base = OTHER; note = 2'-fluoro-modified
ctggtggaaccgtaaccct

SEQ ID NO: 1317 - RNA, 19 nt, synthetic construct
  source 1..19: mol_type = other RNA; note = GPSZRA276S4 sense strand
  modified_base order(1^2,18^19): mod_base = OTHER; note = phosphorothioate linkage
  modified_base 1: mod_base = OTHER; note = locked nucleic acid-modified
  modified_base order(2,4,5,6,10,12,14,16,17,18,19): mod_base = OTHER; note = 2'-methoxy-modified
  modified_base order(3,7,8,9,11,13,15): mod_base = OTHER; note = 2'-fluoro-modified
tggtggaaccgtaaccctg

SEQ ID NO: 1318 - RNA, 19 nt, synthetic construct
  source 1..19: mol_type = other RNA; note = GPSZRA277S4 sense strand
  modified_base order(1^2,18^19): mod_base = OTHER; note = phosphorothioate linkage
  modified_base 1: mod_base = OTHER; note = locked nucleic acid-modified
  modified_base order(2,4,5,6,10,12,14,16,17,18,19): mod_base = OTHER; note = 2'-methoxy-modified
  modified_base order(3,7,8,9,11,13,15): mod_base = OTHER; note = 2'-fluoro-modified
ggtggaaccgtaaccctga

SEQ ID NO: 1319 - RNA, 19 nt, synthetic construct
  source 1..19: mol_type = other RNA; note = GPSZRA281S4 sense strand
  modified_base order(1^2,18^19): mod_base = OTHER; note = phosphorothioate linkage
  modified_base 1: mod_base = OTHER; note = locked nucleic acid-modified
  modified_base order(2,4,5,6,10,12,14,16,17,18,19): mod_base = OTHER; note = 2'-methoxy-modified
  modified_base order(3,7,8,9,11,13,15): mod_base = OTHER; note = 2'-fluoro-modified
gaaccgtaaccctgacctg

SEQ ID NO: 1320 - RNA, 19 nt, synthetic construct
  source 1..19: mol_type = other RNA; note = GPSZRA282S4 sense strand
  modified_base order(1^2,18^19): mod_base = OTHER; note = phosphorothioate linkage
  modified_base 1: mod_base = OTHER; note = locked nucleic acid-modified
  modified_base order(2,4,5,6,10,12,14,16,17,18,19): mod_base = OTHER; note = 2'-methoxy-modified
  modified_base order(3,7,8,9,11,13,15): mod_base = OTHER; note = 2'-fluoro-modified
aaccgtaaccctgacctgt

SEQ ID NO: 1321 - RNA, 19 nt, synthetic construct
  source 1..19: mol_type = other RNA; note = GPSZRA283S4 sense strand
  modified_base order(1^2,18^19): mod_base = OTHER; note = phosphorothioate linkage
  modified_base 1: mod_base = OTHER; note = locked nucleic acid-modified
  modified_base order(2,4,5,6,10,12,14,16,17,18,19): mod_base = OTHER; note = 2'-methoxy-modified
  modified_base order(3,7,8,9,11,13,15): mod_base = OTHER; note = 2'-fluoro-modified
accgtaaccctgacctgtg

SEQ ID NO: 1322 - RNA, 19 nt, synthetic construct
  source 1..19: mol_type = other RNA; note = GPSZRA284S4 sense strand
  modified_base order(1^2,18^19): mod_base = OTHER; note = phosphorothioate linkage
  modified_base 1: mod_base = OTHER; note = locked nucleic acid-modified
  modified_base order(2,4,5,6,10,12,14,16,17,18,19): mod_base = OTHER; note = 2'-methoxy-modified
  modified_base order(3,7,8,9,11,13,15): mod_base = OTHER; note = 2'-fluoro-modified
ccgtaaccctgacctgtga

SEQ ID NO: 1323 - RNA, 19 nt, synthetic construct
  source 1..19: mol_type = other RNA; note = GPSZRA285S4 sense strand
  modified_base order(1^2,18^19): mod_base = OTHER; note = phosphorothioate linkage
  modified_base 1: mod_base = OTHER; note = locked nucleic acid-modified
  modified_base order(2,4,5,6,10,12,14,16,17,18,19): mod_base = OTHER; note = 2'-methoxy-modified
  modified_base order(3,7,8,9,11,13,15): mod_base = OTHER; note = 2'-fluoro-modified
cgtaaccctgacctgtgaa

SEQ ID NO: 1324 - RNA, 19 nt, synthetic construct
  source 1..19: mol_type = other RNA; note = GPSZRA286S4 sense strand
  modified_base order(1^2,18^19): mod_base = OTHER; note = phosphorothioate linkage
  modified_base 1: mod_base = OTHER; note = locked nucleic acid-modified
  modified_base order(2,4,5,6,10,12,14,16,17,18,19): mod_base = OTHER; note = 2'-methoxy-modified
  modified_base order(3,7,8,9,11,13,15): mod_base = OTHER; note = 2'-fluoro-modified
gtaaccctgacctgtgaag

SEQ ID NO: 1325 - RNA, 19 nt, synthetic construct
  source 1..19: mol_type = other RNA; note = GPSZRA287S4 sense strand
  modified_base order(1^2,18^19): mod_base = OTHER; note = phosphorothioate linkage
  modified_base 1: mod_base = OTHER; note = locked nucleic acid-modified
  modified_base order(2,4,5,6,10,12,14,16,17,18,19): mod_base = OTHER; note = 2'-methoxy-modified
  modified_base order(3,7,8,9,11,13,15): mod_base = OTHER; note = 2'-fluoro-modified
taaccctgacctgtgaagt

SEQ ID NO: 1326 - RNA, 19 nt, synthetic construct
  source 1..19: mol_type = other RNA; note = GPSZRA288S4 sense strand
  modified_base order(1^2,18^19): mod_base = OTHER; note = phosphorothioate linkage
  modified_base 1: mod_base = OTHER; note = locked nucleic acid-modified
  modified_base order(2,4,5,6,10,12,14,16,17,18,19): mod_base = OTHER; note = 2'-methoxy-modified
  modified_base order(3,7,8,9,11,13,15): mod_base = OTHER; note = 2'-fluoro-modified
aaccctgacctgtgaagtc

SEQ ID NO: 1327 - RNA, 19 nt, synthetic construct
  source 1..19: mol_type = other RNA; note = GPSZRA290S4 sense strand
  modified_base order(1^2,18^19): mod_base = OTHER; note = phosphorothioate linkage
  modified_base 1: mod_base = OTHER; note = locked nucleic acid-modified
  modified_base order(2,4,5,6,10,12,14,16,17,18,19): mod_base = OTHER; note = 2'-methoxy-modified
  modified_base order(3,7,8,9,11,13,15): mod_base = OTHER; note = 2'-fluoro-modified
cctgacctgtgaagtccct

SEQ ID NO: 1328 - RNA, 19 nt, synthetic construct
  source 1..19: mol_type = other RNA; note = GPSZRA292S4 sense strand
  modified_base order(1^2,18^19): mod_base = OTHER; note = phosphorothioate linkage
  modified_base 1: mod_base = OTHER; note = locked nucleic acid-modified
  modified_base order(2,4,5,6,10,12,14,16,17,18,19): mod_base = OTHER; note = 2'-methoxy-modified
  modified_base order(3,7,8,9,11,13,15): mod_base = OTHER; note = 2'-fluoro-modified
tgacctgtgaagtccctgc

SEQ ID NO: 1329 - RNA, 19 nt, synthetic construct
  source 1..19: mol_type = other RNA; note = GPSZRA301S4 sense strand
  modified_base order(1^2,18^19): mod_base = OTHER; note = phosphorothioate linkage
  modified_base 1: mod_base = OTHER; note = locked nucleic acid-modified
  modified_base order(2,4,5,6,10,12,14,16,17,18,19): mod_base = OTHER; note = 2'-methoxy-modified
  modified_base order(3,7,8,9,11,13,15): mod_base = OTHER; note = 2'-fluoro-modified
tctcctcaaatccactgga

SEQ ID NO: 1330 - RNA, 19 nt, synthetic construct
  source 1..19: mol_type = other RNA; note = GPSZRA308S4 sense strand
  modified_base order(1^2,18^19): mod_base = OTHER; note = phosphorothioate linkage
  modified_base 1: mod_base = OTHER; note = locked nucleic acid-modified
  modified_base order(2,4,5,6,10,12,14,16,17,18,19): mod_base = OTHER; note = 2'-methoxy-modified
  modified_base order(3,7,8,9,11,13,15): mod_base = OTHER; note = 2'-fluoro-modified
aaatccactggatgaagga

SEQ ID NO: 1331 - RNA, 19 nt, synthetic construct
  source 1..19: mol_type = other RNA; note = GPSZRA311S4 sense strand
  modified_base order(1^2,18^19): mod_base = OTHER; note = phosphorothioate linkage
  modified_base 1: mod_base = OTHER; note = locked nucleic acid-modified
  modified_base order(2,4,5,6,10,12,14,16,17,18,19): mod_base = OTHER; note = 2'-methoxy-modified
  modified_base order(3,7,8,9,11,13,15): mod_base = OTHER; note = 2'-fluoro-modified
tccactggatgaaggatgg

SEQ ID NO: 1332 - RNA, 19 nt, synthetic construct
  source 1..19: mol_type = other RNA; note = GPSZRA312S4 sense strand
  modified_base order(1^2,18^19): mod_base = OTHER; note = phosphorothioate linkage
  modified_base 1: mod_base = OTHER; note = locked nucleic acid-modified
  modified_base order(2,4,5,6,10,12,14,16,17,18,19): mod_base = OTHER; note = 2'-methoxy-modified
  modified_base order(3,7,8,9,11,13,15): mod_base = OTHER; note = 2'-fluoro-modified
ccactggatgaaggatggt

SEQ ID NO: 1333 - RNA, 19 nt, synthetic construct
  source 1..19: mol_type = other RNA; note = GPSZRA313S4 sense strand
  modified_base order(1^2,18^19): mod_base = OTHER; note = phosphorothioate linkage
  modified_base 1: mod_base = OTHER; note = locked nucleic acid-modified
  modified_base order(2,4,5,6,10,12,14,16,17,18,19): mod_base = OTHER; note = 2'-methoxy-modified
  modified_base order(3,7,8,9,11,13,15): mod_base = OTHER; note = 2'-fluoro-modified
cactggatgaaggatggtg

SEQ ID NO: 1334 - RNA, 19 nt, synthetic construct
  source 1..19: mol_type = other RNA; note = GPSZRA314S4 sense strand
  modified_base order(1^2,18^19): mod_base = OTHER; note = phosphorothioate linkage
  modified_base 1: mod_base = OTHER; note = locked nucleic acid-modified
  modified_base order(2,4,5,6,10,12,14,16,17,18,19): mod_base = OTHER; note = 2'-methoxy-modified
  modified_base order(3,7,8,9,11,13,15): mod_base = OTHER; note = 2'-fluoro-modified
actggatgaaggatggtgt

SEQ ID NO: 1335 - RNA, 19 nt, synthetic construct
  source 1..19: mol_type = other RNA; note = GPSZRA315S4 sense strand
  modified_base order(1^2,18^19): mod_base = OTHER; note = phosphorothioate linkage
  modified_base 1: mod_base = OTHER; note = locked nucleic acid-modified
  modified_base order(2,4,5,6,10,12,14,16,17,18,19): mod_base = OTHER; note = 2'-methoxy-modified
  modified_base order(3,7,8,9,11,13,15): mod_base = OTHER; note = 2'-fluoro-modified
ctggatgaaggatggtgtg

SEQ ID NO: 1336 - RNA, 19 nt, synthetic construct
  source 1..19: mol_type = other RNA; note = GPSZRA316S4 sense strand
  modified_base order(1^2,18^19): mod_base = OTHER; note = phosphorothioate linkage
  modified_base 1: mod_base = OTHER; note = locked nucleic acid-modified
  modified_base order(2,4,5,6,10,12,14,16,17,18,19): mod_base = OTHER; note = 2'-methoxy-modified
  modified_base order(3,7,8,9,11,13,15): mod_base = OTHER; note = 2'-fluoro-modified
tggatgaaggatggtgtgc

SEQ ID NO: 1337 - RNA, 19 nt, synthetic construct
  source 1..19: mol_type = other RNA; note = GPSZRA317S4 sense strand
  modified_base order(1^2,18^19): mod_base = OTHER; note = phosphorothioate linkage
  modified_base 1: mod_base = OTHER; note = locked nucleic acid-modified
  modified_base order(2,4,5,6,10,12,14,16,17,18,19): mod_base = OTHER; note = 2'-methoxy-modified
  modified_base order(3,7,8,9,11,13,15): mod_base = OTHER; note = 2'-fluoro-modified
ggatgaaggatggtgtgcc

SEQ ID NO: 1338 - RNA, 19 nt, synthetic construct
  source 1..19: mol_type = other RNA; note = GPSZRA318S4 sense strand
  modified_base order(1^2,18^19): mod_base = OTHER; note = phosphorothioate linkage
  modified_base 1: mod_base = OTHER; note = locked nucleic acid-modified
  modified_base order(2,4,5,6,10,12,14,16,17,18,19): mod_base = OTHER; note = 2'-methoxy-modified
  modified_base order(3,7,8,9,11,13,15): mod_base = OTHER; note = 2'-fluoro-modified
gatgaaggatggtgtgccc

SEQ ID NO: 1339 - RNA, 19 nt, synthetic construct
  source 1..19: mol_type = other RNA; note = GPSZRA320S4 sense strand
  modified_base order(1^2,18^19): mod_base = OTHER; note = phosphorothioate linkage
  modified_base 1: mod_base = OTHER; note = locked nucleic acid-modified
  modified_base order(2,4,5,6,10,12,14,16,17,18,19): mod_base = OTHER; note = 2'-methoxy-modified
  modified_base order(3,7,8,9,11,13,15): mod_base = OTHER; note = 2'-fluoro-modified
tgaaggatggtgtgccctt

SEQ ID NO: 1340 - RNA, 19 nt, synthetic construct
  source 1..19: mol_type = other RNA; note = GPSZRA333S4 sense strand
  modified_base order(1^2,18^19): mod_base = OTHER; note = phosphorothioate linkage
  modified_base 1: mod_base = OTHER; note = locked nucleic acid-modified
  modified_base order(2,4,5,6,10,12,14,16,17,18,19): mod_base = OTHER; note = 2'-methoxy-modified
  modified_base order(3,7,8,9,11,13,15): mod_base = OTHER; note = 2'-fluoro-modified
gaaagccgtgctgtcagca

SEQ ID NO: 1341 - RNA, 19 nt, synthetic construct
  source 1..19: mol_type = other RNA; note = GPSZRA342S4 sense strand
  modified_base order(1^2,18^19): mod_base = OTHER; note = phosphorothioate linkage
  modified_base 1: mod_base = OTHER; note = locked nucleic acid-modified
  modified_base order(2,4,5,6,10,12,14,16,17,18,19): mod_base = OTHER; note = 2'-methoxy-modified
  modified_base order(3,7,8,9,11,13,15): mod_base = OTHER; note = 2'-fluoro-modified
tgtcagcatcagcatcatc

SEQ ID NO: 1342 - RNA, 19 nt, synthetic construct
  source 1..19: mol_type = other RNA; note = GPSZRA378S4 sense strand
  modified_base order(1^2,18^19): mod_base = OTHER; note = phosphorothioate linkage
  modified_base 1: mod_base = OTHER; note = locked nucleic acid-modified
  modified_base order(2,4,5,6,10,12,14,16,17,18,19): mod_base = OTHER; note = 2'-methoxy-modified
  modified_base order(3,7,8,9,11,13,15): mod_base = OTHER; note = 2'-fluoro-modified
aagaggaggagcgtgcaga

SEQ ID NO: 1343 - RNA, 19 nt, synthetic construct
  source 1..19: mol_type = other RNA; note = GPSZRA379S4 sense strand
  modified_base order(1^2,18^19): mod_base = OTHER; note = phosphorothioate linkage
  modified_base 1: mod_base = OTHER; note = locked nucleic acid-modified
  modified_base order(2,4,5,6,10,12,14,16,17,18,19): mod_base = OTHER; note = 2'-methoxy-modified
  modified_base order(3,7,8,9,11,13,15): mod_base = OTHER; note = 2'-fluoro-modified
gaatcagtcggaggaacct

SEQ ID NO: 1344 - RNA, 19 nt, synthetic construct
  source 1..19: mol_type = other RNA; note = GPSZRA380S4 sense strand
  modified_base order(1^2,18^19): mod_base = OTHER; note = phosphorothioate linkage
  modified_base 1: mod_base = OTHER; note = locked nucleic acid-modified
  modified_base order(2,4,5,6,10,12,14,16,17,18,19): mod_base = OTHER; note = 2'-methoxy-modified
  modified_base order(3,7,8,9,11,13,15): mod_base = OTHER; note = 2'-fluoro-modified
aatcagtcggaggaacctg

SEQ ID NO: 1345 - RNA, 19 nt, synthetic construct
  source 1..19: mol_type = other RNA; note = GPSZRA381S4 sense strand
  modified_base order(1^2,18^19): mod_base = OTHER; note = phosphorothioate linkage
  modified_base 1: mod_base = OTHER; note = locked nucleic acid-modified
  modified_base order(2,4,5,6,10,12,14,16,17,18,19): mod_base = OTHER; note = 2'-methoxy-modified
  modified_base order(3,7,8,9,11,13,15): mod_base = OTHER; note = 2'-fluoro-modified
atcagtcggaggaacctga

SEQ ID NO: 1346 - RNA, 19 nt, synthetic construct
  source 1..19: mol_type = other RNA; note = GPSZRA402S4/GPSZRA402S4-VP sense strand
  modified_base order(1^2,18^19): mod_base = OTHER; note = phosphorothioate linkage
  modified_base 1: mod_base = OTHER; note = locked nucleic acid-modified
  modified_base order(2,4,5,6,10,12,14,16,17,18,19): mod_base = OTHER; note = 2'-methoxy-modified
  modified_base order(3,7,8,9,11,13,15): mod_base = OTHER; note = 2'-fluoro-modified
ccaactctctcctgtataa

SEQ ID NO: 1347 - RNA, 19 nt, synthetic construct
  source 1..19: mol_type = other RNA; note = GPSZRA407S4 sense strand
  modified_base order(1^2,18^19): mod_base = OTHER; note = phosphorothioate linkage
  modified_base 1: mod_base = OTHER; note = locked nucleic acid-modified
  modified_base order(2,4,5,6,10,12,14,16,17,18,19): mod_base = OTHER; note = 2'-methoxy-modified
  modified_base order(3,7,8,9,11,13,15): mod_base = OTHER; note = 2'-fluoro-modified
cctgtataaccccaccttg

SEQ ID NO: 1348 - RNA, 19 nt, synthetic construct
  source 1..19: mol_type = other RNA; note = GPSZRA408S4 sense strand
  modified_base order(1^2,18^19): mod_base = OTHER; note = phosphorothioate linkage
  modified_base 1: mod_base = OTHER; note = locked nucleic acid-modified
  modified_base order(2,4,5,6,10,12,14,16,17,18,19): mod_base = OTHER; note = 2'-methoxy-modified
  modified_base order(3,7,8,9,11,13,15): mod_base = OTHER; note = 2'-fluoro-modified
ctgtataaccccaccttgc

SEQ ID NO: 1349 - RNA, 19 nt, synthetic construct
  source 1..19: mol_type = other RNA; note = GPSZRA409S4 sense strand
  modified_base order(1^2,18^19): mod_base = OTHER; note = phosphorothioate linkage
  modified_base 1: mod_base = OTHER; note = locked nucleic acid-modified
  modified_base order(2,4,5,6,10,12,14,16,17,18,19): mod_base = OTHER; note = 2'-methoxy-modified
  modified_base order(3,7,8,9,11,13,15): mod_base = OTHER; note = 2'-fluoro-modified
tgtataaccccaccttgcc

SEQ ID NO: 1350 - RNA, 19 nt, synthetic construct
  source 1..19: mol_type = other RNA; note = GPSZRA410S4 sense strand
  modified_base order(1^2,18^19): mod_base = OTHER; note = phosphorothioate linkage
  modified_base 1: mod_base = OTHER; note = locked nucleic acid-modified
  modified_base order(2,4,5,6,10,12,14,16,17,18,19): mod_base = OTHER; note = 2'-methoxy-modified
  modified_base order(3,7,8,9,11,13,15): mod_base = OTHER; note = 2'-fluoro-modified
gtataaccccaccttgcca

SEQ ID NO: 1351 - RNA, 19 nt, synthetic construct
  source 1..19: mol_type = other RNA; note = GPSZRA411S4 sense strand
  modified_base order(1^2,18^19): mod_base = OTHER; note = phosphorothioate linkage
  modified_base 1: mod_base = OTHER; note = locked nucleic acid-modified
  modified_base order(2,4,5,6,10,12,14,16,17,18,19): mod_base = OTHER; note = 2'-methoxy-modified
  modified_base order(3,7,8,9,11,13,15): mod_base = OTHER; note = 2'-fluoro-modified
tataaccccaccttgccaa

SEQ ID NO: 1352 - RNA, 19 nt, synthetic construct
  source 1..19: mol_type = other RNA; note = GPSZRA084S5 sense strand
  modified_base order(1^2,18^19): mod_base = OTHER; note = phosphorothioate linkage
  modified_base order(1,2,3,4,6,10,11,12,13,14,16,17,18,19): mod_base = OTHER; note = 2'-methoxy-modified
  modified_base order(5,7,8,9,15): mod_base = OTHER; note = 2'-fluoro-modified
ggaaaggagaccaagtcca

SEQ ID NO: 1353 - RNA, 19 nt, synthetic construct
  source 1..19: mol_type = other RNA; note = GPSZRA087S5 sense strand
  modified_base order(1^2,18^19): mod_base = OTHER; note = phosphorothioate linkage
  modified_base order(1,2,3,4,6,10,11,12,13,14,16,17,18,19): mod_base = OTHER; note = 2'-methoxy-modified
  modified_base order(5,7,8,9,15): mod_base = OTHER; note = 2'-fluoro-modified
aaggagaccaagtccaact

SEQ ID NO: 1354 - RNA, 19 nt, synthetic construct
  source 1..19: mol_type = other RNA; note = GPSZRA092S5 sense strand
  modified_base order(1^2,18^19): mod_base = OTHER; note = phosphorothioate linkage
  modified_base order(1,2,3,4,6,10,11,12,13,14,16,17,18,19): mod_base = OTHER; note = 2'-methoxy-modified
  modified_base order(5,7,8,9,15): mod_base = OTHER; note = 2'-fluoro-modified
gaccaagtccaactaccga

SEQ ID NO: 1355 - RNA, 19 nt, synthetic construct
  source 1..19: mol_type = other RNA; note = GPSZRA093S5 sense strand
  modified_base order(1^2,18^19): mod_base = OTHER; note = phosphorothioate linkage
  modified_base order(1,2,3,4,6,10,11,12,13,14,16,17,18,19): mod_base = OTHER; note = 2'-methoxy-modified
  modified_base order(5,7,8,9,15): mod_base = OTHER; note = 2'-fluoro-modified
accaagtccaactaccgag

SEQ ID NO: 1356 - RNA, 19 nt, synthetic construct
  source 1..19: mol_type = other RNA; note = GPSZRA097S5 sense strand
  modified_base order(1^2,18^19): mod_base = OTHER; note = phosphorothioate linkage
  modified_base order(1,2,3,4,6,10,11,12,13,14,16,17,18,19): mod_base = OTHER; note = 2'-methoxy-modified
  modified_base order(5,7,8,9,15): mod_base = OTHER; note = 2'-fluoro-modified
agtccaactaccgagtccg

SEQ ID NO: 1357 - RNA, 19 nt, synthetic construct
  source 1..19: mol_type = other RNA; note = GPSZRA118S5 sense strand
  modified_base order(1^2,18^19): mod_base = OTHER; note = phosphorothioate linkage
  modified_base order(1,2,3,4,6,10,11,12,13,14,16,17,18,19): mod_base = OTHER; note = 2'-methoxy-modified
  modified_base order(5,7,8,9,15): mod_base = OTHER; note = 2'-fluoro-modified
ctaccagattcctgggaag

SEQ ID NO: 1358 - RNA, 19 nt, synthetic construct
  source 1..19: mol_type = other RNA; note = GPSZRA217S5 sense strand
  modified_base order(1^2,18^19): mod_base = OTHER; note = phosphorothioate linkage
  modified_base order(1,2,3,4,6,10,11,12,13,14,16,17,18,19): mod_base = OTHER; note = 2'-methoxy-modified
  modified_base order(5,7,8,9,15): mod_base = OTHER; note = 2'-fluoro-modified
agggagtatctgtgaagga

SEQ ID NO: 1359 - RNA, 19 nt, synthetic construct
  source 1..19: mol_type = other RNA; note = GPSZRA222S5 sense strand
  modified_base order(1^2,18^19): mod_base = OTHER; note = phosphorothioate linkage
  modified_base order(1,2,3,4,6,10,11,12,13,14,16,17,18,19): mod_base = OTHER; note = 2'-methoxy-modified
  modified_base order(5,7,8,9,15): mod_base = OTHER; note = 2'-fluoro-modified
tcttcacactgcagtcgga

SEQ ID NO: 1360 - RNA, 19 nt, synthetic construct
  source 1..19: mol_type = other RNA; note = GPSZRA227S5 sense strand
  modified_base order(1^2,18^19): mod_base = OTHER; note = phosphorothioate linkage
  modified_base order(1,2,3,4,6,10,11,12,13,14,16,17,18,19): mod_base = OTHER; note = 2'-methoxy-modified
  modified_base order(5,7,8,9,15): mod_base = OTHER; note = 2'-fluoro-modified
acactgcagtcggagctaa

SEQ ID NO: 1361 - RNA, 19 nt, synthetic construct
  source 1..19: mol_type = other RNA; note = GPSZRA228S5 sense strand
  modified_base order(1^2,18^19): mod_base = OTHER; note = phosphorothioate linkage
  modified_base order(1,2,3,4,6,10,11,12,13,14,16,17,18,19): mod_base = OTHER; note = 2'-methoxy-modified
  modified_base order(5,7,8,9,15): mod_base = OTHER; note = 2'-fluoro-modified
cactgcagtcggagctaat

SEQ ID NO: 1362 - RNA, 19 nt, synthetic construct
  source 1..19: mol_type = other RNA; note = GPSZRA229S5 sense strand
  modified_base order(1^2,18^19): mod_base = OTHER; note = phosphorothioate linkage
  modified_base order(1,2,3,4,6,10,11,12,13,14,16,17,18,19): mod_base = OTHER; note = 2'-methoxy-modified
  modified_base order(5,7,8,9,15): mod_base = OTHER; note = 2'-fluoro-modified
actgcagtcggagctaatg

SEQ ID NO: 1363 - RNA, 19 nt, synthetic construct
  source 1..19: mol_type = other RNA; note = GPSZRA231S5 sense strand
  modified_base order(1^2,18^19): mod_base = OTHER; note = phosphorothioate linkage
  modified_base order(1,2,3,4,6,10,11,12,13,14,16,17,18,19): mod_base = OTHER; note = 2'-methoxy-modified
  modified_base order(5,7,8,9,15): mod_base = OTHER; note = 2'-fluoro-modified
tgcagtcggagctaatggt

SEQ ID NO: 1364 - RNA, 19 nt, synthetic construct
  source 1..19: mol_type = other RNA; note = GPSZRA232S5 sense strand
  modified_base order(1^2,18^19): mod_base = OTHER; note = phosphorothioate linkage
  modified_base order(1,2,3,4,6,10,11,12,13,14,16,17,18,19): mod_base = OTHER; note = 2'-methoxy-modified
  modified_base order(5,7,8,9,15): mod_base = OTHER; note = 2'-fluoro-modified
gcagtcggagctaatggtg

SEQ ID NO: 1365 - RNA, 19 nt, synthetic construct
  source 1..19: mol_type = other RNA; note = GPSZRA233S5 sense strand
  modified_base order(1^2,18^19): mod_base = OTHER; note = phosphorothioate linkage
  modified_base order(1,2,3,4,6,10,11,12,13,14,16,17,18,19): mod_base = OTHER; note = 2'-methoxy-modified
  modified_base order(5,7,8,9,15): mod_base = OTHER; note = 2'-fluoro-modified
cagtcggagctaatggtga

SEQ ID NO: 1366 - RNA, 19 nt, synthetic construct
  source 1..19: mol_type = other RNA; note = GPSZRA252S5 sense strand
  modified_base order(1^2,18^19): mod_base = OTHER; note = phosphorothioate linkage
  modified_base order(1,2,3,4,6,10,11,12,13,14,16,17,18,19): mod_base = OTHER; note = 2'-methoxy-modified
  modified_base order(5,7,8,9,15): mod_base = OTHER; note = 2'-fluoro-modified
tctggaggaggtccaattg

SEQ ID NO: 1367 - RNA, 19 nt, synthetic construct
  source 1..19: mol_type = other RNA; note = GPSZRA257S5 sense strand
  modified_base order(1^2,18^19): mod_base = OTHER; note = phosphorothioate linkage
  modified_base order(1,2,3,4,6,10,11,12,13,14,16,17,18,19): mod_base = OTHER; note = 2'-methoxy-modified
  modified_base order(5,7,8,9,15): mod_base = OTHER; note = 2'-fluoro-modified
aggaggtccaattggtggt

SEQ ID NO: 1368 - RNA, 19 nt, synthetic construct
  source 1..19: mol_type = other RNA; note = GPSZRA266S5 sense strand
  modified_base order(1^2,18^19): mod_base = OTHER; note = phosphorothioate linkage
  modified_base order(1,2,3,4,6,10,11,12,13,14,16,17,18,19): mod_base = OTHER; note = 2'-methoxy-modified
  modified_base order(5,7,8,9,15): mod_base = OTHER; note = 2'-fluoro-modified
agcagtagctcctggtgga

SEQ ID NO: 1369 - RNA, 19 nt, synthetic construct
  source 1..19: mol_type = other RNA; note = GPSZRA267S5 sense strand
  modified_base order(1^2,18^19): mod_base = OTHER; note = phosphorothioate linkage
  modified_base order(1,2,3,4,6,10,11,12,13,14,16,17,18,19): mod_base = OTHER; note = 2'-methoxy-modified
  modified_base order(5,7,8,9,15): mod_base = OTHER; note = 2'-fluoro-modified
gcagtagctcctggtggaa

SEQ ID NO: 1370 - RNA, 19 nt, synthetic construct
  source 1..19: mol_type = other RNA; note = GPSZRA271S5 sense strand
  modified_base order(1^2,18^19): mod_base = OTHER; note = phosphorothioate linkage
  modified_base order(1,2,3,4,6,10,11,12,13,14,16,17,18,19): mod_base = OTHER; note = 2'-methoxy-modified
  modified_base order(5,7,8,9,15): mod_base = OTHER; note = 2'-fluoro-modified
agctcctggtggaaccgta

SEQ ID NO: 1371 - RNA, 19 nt, synthetic construct
  source 1..19: mol_type = other RNA; note = GPSZRA272S5 sense strand
  modified_base order(1^2,18^19): mod_base = OTHER; note = phosphorothioate linkage
  modified_base order(1,2,3,4,6,10,11,12,13,14,16,17,18,19): mod_base = OTHER; note = 2'-methoxy-modified
  modified_base order(5,7,8,9,15): mod_base = OTHER; note = 2'-fluoro-modified
gctcctggtggaaccgtaa

SEQ ID NO: 1372 - RNA, 19 nt, synthetic construct
  source 1..19: mol_type = other RNA; note = GPSZRA274S5 sense strand
  modified_base order(1^2,18^19): mod_base = OTHER; note = phosphorothioate linkage
  modified_base order(1,2,3,4,6,10,11,12,13,14,16,17,18,19): mod_base = OTHER; note = 2'-methoxy-modified
  modified_base order(5,7,8,9,15): mod_base = OTHER; note = 2'-fluoro-modified
tcctggtggaaccgtaacc

SEQ ID NO: 1373 - RNA, 19 nt, synthetic construct
  source 1..19: mol_type = other RNA; note = GPSZRA275S5 sense strand
  modified_base order(1^2,18^19): mod_base = OTHER; note = phosphorothioate linkage
  modified_base order(1,2,3,4,6,10,11,12,13,14,16,17,18,19): mod_base = OTHER; note = 2'-methoxy-modified
  modified_base order(5,7,8,9,15): mod_base = OTHER; note = 2'-fluoro-modified
ctggtggaaccgtaaccct

SEQ ID NO: 1374 - RNA, 19 nt, synthetic construct
  source 1..19: mol_type = other RNA; note = GPSZRA276S5 sense strand
  modified_base order(1^2,18^19): mod_base = OTHER; note = phosphorothioate linkage
  modified_base order(1,2,3,4,6,10,11,12,13,14,16,17,18,19): mod_base = OTHER; note = 2'-methoxy-modified
  modified_base order(5,7,8,9,15): mod_base = OTHER; note = 2'-fluoro-modified
tggtggaaccgtaaccctg

SEQ ID NO: 1375 - RNA, 19 nt, synthetic construct
  source 1..19: mol_type = other RNA; note = GPSZRA277S5 sense strand
  modified_base order(1^2,18^19): mod_base = OTHER; note = phosphorothioate linkage
  modified_base order(1,2,3,4,6,10,11,12,13,14,16,17,18,19): mod_base = OTHER; note = 2'-methoxy-modified
  modified_base order(5,7,8,9,15): mod_base = OTHER; note = 2'-fluoro-modified
ggtggaaccgtaaccctga

SEQ ID NO: 1376 - RNA, 19 nt, synthetic construct
  source 1..19: mol_type = other RNA; note = GPSZRA281S5 sense strand
  modified_base order(1^2,18^19): mod_base = OTHER; note = phosphorothioate linkage
  modified_base order(1,2,3,4,6,10,11,12,13,14,16,17,18,19): mod_base = OTHER; note = 2'-methoxy-modified
  modified_base order(5,7,8,9,15): mod_base = OTHER; note = 2'-fluoro-modified
gaaccgtaaccctgacctg

SEQ ID NO: 1377 - RNA, 19 nt, synthetic construct
  source 1..19: mol_type = other RNA; note = GPSZRA282S5 sense strand
  modified_base order(1^2,18^19): mod_base = OTHER; note = phosphorothioate linkage
  modified_base order(1,2,3,4,6,10,11,12,13,14,16,17,18,19): mod_base = OTHER; note = 2'-methoxy-modified
  modified_base order(5,7,8,9,15): mod_base = OTHER; note = 2'-fluoro-modified
aaccgtaaccctgacctgt

SEQ ID NO: 1378 - RNA, 19 nt, synthetic construct
  source 1..19: mol_type = other RNA; note = GPSZRA283S5 sense strand
  modified_base order(1^2,18^19): mod_base = OTHER; note = phosphorothioate linkage
  modified_base order(1,2,3,4,6,10,11,12,13,14,16,17,18,19): mod_base = OTHER; note = 2'-methoxy-modified
  modified_base order(5,7,8,9,15): mod_base = OTHER; note = 2'-fluoro-modified
accgtaaccctgacctgtg

SEQ ID NO: 1379 - RNA, 19 nt, synthetic construct
  source 1..19: mol_type = other RNA; note = GPSZRA284S5 sense strand
  modified_base order(1^2,18^19): mod_base = OTHER; note = phosphorothioate linkage
  modified_base order(1,2,3,4,6,10,11,12,13,14,16,17,18,19): mod_base = OTHER; note = 2'-methoxy-modified
  modified_base order(5,7,8,9,15): mod_base = OTHER; note = 2'-fluoro-modified
ccgtaaccctgacctgtga

SEQ ID NO: 1380 - RNA, 19 nt, synthetic construct
  source 1..19: mol_type = other RNA; note = GPSZRA285S5 sense strand
  modified_base order(1^2,18^19): mod_base = OTHER; note = phosphorothioate linkage
  modified_base order(1,2,3,4,6,10,11,12,13,14,16,17,18,19): mod_base = OTHER; note = 2'-methoxy-modified
  modified_base order(5,7,8,9,15): mod_base = OTHER; note = 2'-fluoro-modified
cgtaaccctgacctgtgaa

SEQ ID NO: 1381 - RNA, 19 nt, synthetic construct
  source 1..19: mol_type = other RNA; note = GPSZRA286S5 sense strand
  modified_base order(1^2,18^19): mod_base = OTHER; note = phosphorothioate linkage
  modified_base order(1,2,3,4,6,10,11,12,13,14,16,17,18,19): mod_base = OTHER; note = 2'-methoxy-modified
  modified_base order(5,7,8,9,15): mod_base = OTHER; note = 2'-fluoro-modified
gtaaccctgacctgtgaag

SEQ ID NO: 1382 - RNA, 19 nt, synthetic construct
  source 1..19: mol_type = other RNA; note = GPSZRA287S5 sense strand
  modified_base order(1^2,18^19): mod_base = OTHER; note = phosphorothioate linkage
  modified_base order(1,2,3,4,6,10,11,12,13,14,16,17,18,19): mod_base = OTHER; note = 2'-methoxy-modified
  modified_base order(5,7,8,9,15): mod_base = OTHER; note = 2'-fluoro-modified
taaccctgacctgtgaagt

SEQ ID NO: 1383 - RNA, 19 nt, synthetic construct
  source 1..19: mol_type = other RNA; note = GPSZRA288S5 sense strand
  modified_base order(1^2,18^19): mod_base = OTHER; note = phosphorothioate linkage
  modified_base order(1,2,3,4,6,10,11,12,13,14,16,17,18,19): mod_base = OTHER; note = 2'-methoxy-modified
  modified_base order(5,7,8,9,15): mod_base = OTHER; note = 2'-fluoro-modified
aaccctgacctgtgaagtc

SEQ ID NO: 1384 - RNA, 19 nt, synthetic construct
  source 1..19: mol_type = other RNA; note = GPSZRA290S5 sense strand
  modified_base order(1^2,18^19): mod_base = OTHER; note = phosphorothioate linkage
  modified_base order(1,2,3,4,6,10,11,12,13,14,16,17,18,19): mod_base = OTHER; note = 2'-methoxy-modified
  modified_base order(5,7,8,9,15): mod_base = OTHER; note = 2'-fluoro-modified
cctgacctgtgaagtccct

SEQ ID NO: 1385 - RNA, 19 nt, synthetic construct
  source 1..19: mol_type = other RNA; note = GPSZRA292S5 sense strand
  modified_base order(1^2,18^19): mod_base = OTHER; note = phosphorothioate linkage
  modified_base order(1,2,3,4,6,10,11,12,13,14,16,17,18,19): mod_base = OTHER; note = 2'-methoxy-modified
  modified_base order(5,7,8,9,15): mod_base = OTHER; note = 2'-fluoro-modified
tgacctgtgaagtccctgc

SEQ ID NO: 1386 - RNA, 19 nt, synthetic construct
  source 1..19: mol_type = other RNA; note = GPSZRA301S5 sense strand
  modified_base order(1^2,18^19): mod_base = OTHER; note = phosphorothioate linkage
  modified_base order(1,2,3,4,6,10,11,12,13,14,16,17,18,19): mod_base = OTHER; note = 2'-methoxy-modified
  modified_base order(5,7,8,9,15): mod_base = OTHER; note = 2'-fluoro-modified
tctcctcaaatccactgga

SEQ ID NO: 1387 - RNA, 19 nt, synthetic construct
  source 1..19: mol_type = other RNA; note = GPSZRA308S5 sense strand
  modified_base order(1^2,18^19): mod_base = OTHER; note = phosphorothioate linkage
  modified_base order(1,2,3,4,6,10,11,12,13,14,16,17,18,19): mod_base = OTHER; note = 2'-methoxy-modified
  modified_base order(5,7,8,9,15): mod_base = OTHER; note = 2'-fluoro-modified
aaatccactggatgaagga

SEQ ID NO: 1388 - RNA, 19 nt, synthetic construct
  source 1..19: mol_type = other RNA; note = GPSZRA311S5 sense strand
  modified_base order(1^2,18^19): mod_base = OTHER; note = phosphorothioate linkage
  modified_base order(1,2,3,4,6,10,11,12,13,14,16,17,18,19): mod_base = OTHER; note = 2'-methoxy-modified
  modified_base order(5,7,8,9,15): mod_base = OTHER; note = 2'-fluoro-modified
tccactggatgaaggatgg

SEQ ID NO: 1389 - RNA, 19 nt, synthetic construct
  source 1..19: mol_type = other RNA; note = GPSZRA312S5 sense strand
  modified_base order(1^2,18^19): mod_base = OTHER; note = phosphorothioate linkage
  modified_base order(1,2,3,4,6,10,11,12,13,14,16,17,18,19): mod_base = OTHER; note = 2'-methoxy-modified
  modified_base order(5,7,8,9,15): mod_base = OTHER; note = 2'-fluoro-modified
ccactggatgaaggatggt

SEQ ID NO: 1390 - RNA, 19 nt, synthetic construct
  source 1..19: mol_type = other RNA; note = GPSZRA313S5 sense strand
  modified_base order(1^2,18^19): mod_base = OTHER; note = phosphorothioate linkage
  modified_base order(1,2,3,4,6,10,11,12,13,14,16,17,18,19): mod_base = OTHER; note = 2'-methoxy-modified
  modified_base order(5,7,8,9,15): mod_base = OTHER; note = 2'-fluoro-modified
cactggatgaaggatggtg

SEQ ID NO: 1391 - RNA, 19 nt, synthetic construct
  source 1..19: mol_type = other RNA; note = GPSZRA314S5/GPSZRA314S5-VP sense strand
  modified_base order(1^2,18^19): mod_base = OTHER; note = phosphorothioate linkage
  modified_base order(1,2,3,4,6,10,11,12,13,14,16,17,18,19): mod_base = OTHER; note = 2'-methoxy-modified
  modified_base order(5,7,8,9,15): mod_base = OTHER; note = 2'-fluoro-modified
actggatgaaggatggtgt

SEQ ID NO: 1392 - RNA, 19 nt, synthetic construct
  source 1..19: mol_type = other RNA; note = GPSZRA315S5 sense strand
  modified_base order(1^2,18^19): mod_base = OTHER; note = phosphorothioate linkage
  modified_base order(1,2,3,4,6,10,11,12,13,14,16,17,18,19): mod_base = OTHER; note = 2'-methoxy-modified
  modified_base order(5,7,8,9,15): mod_base = OTHER; note = 2'-fluoro-modified
ctggatgaaggatggtgtg

SEQ ID NO: 1393 - RNA, 19 nt, synthetic construct
  source 1..19: mol_type = other RNA; note = GPSZRA316S5 sense strand
  modified_base order(1^2,18^19): mod_base = OTHER; note = phosphorothioate linkage
  modified_base order(1,2,3,4,6,10,11,12,13,14,16,17,18,19): mod_base = OTHER; note = 2'-methoxy-modified
  modified_base order(5,7,8,9,15): mod_base = OTHER; note = 2'-fluoro-modified
tggatgaaggatggtgtgc

SEQ ID NO: 1394 - RNA, 19 nt, synthetic construct
  source 1..19: mol_type = other RNA; note = GPSZRA317S5 sense strand
  modified_base order(1^2,18^19): mod_base = OTHER; note = phosphorothioate linkage
  modified_base order(1,2,3,4,6,10,11,12,13,14,16,17,18,19): mod_base = OTHER; note = 2'-methoxy-modified
  modified_base order(5,7,8,9,15): mod_base = OTHER; note = 2'-fluoro-modified
ggatgaaggatggtgtgcc

SEQ ID NO: 1395 - RNA, 19 nt, synthetic construct
  source 1..19: mol_type = other RNA; note = GPSZRA318S5 sense strand
  modified_base order(1^2,18^19): mod_base = OTHER; note = phosphorothioate linkage
  modified_base order(1,2,3,4,6,10,11,12,13,14,16,17,18,19): mod_base = OTHER; note = 2'-methoxy-modified
  modified_base order(5,7,8,9,15): mod_base = OTHER; note = 2'-fluoro-modified
gatgaaggatggtgtgccc

SEQ ID NO: 1396 - RNA, 19 nt, synthetic construct
  source 1..19: mol_type = other RNA; note = GPSZRA320S5 sense strand
  modified_base order(1^2,18^19): mod_base = OTHER; note = phosphorothioate linkage
  modified_base order(1,2,3,4,6,10,11,12,13,14,16,17,18,19): mod_base = OTHER; note = 2'-methoxy-modified
  modified_base order(5,7,8,9,15): mod_base = OTHER; note = 2'-fluoro-modified
tgaaggatggtgtgccctt

SEQ ID NO: 1397 - RNA, 19 nt, synthetic construct
  source 1..19: mol_type = other RNA; note = GPSZRA333S5 sense strand
  modified_base order(1^2,18^19): mod_base = OTHER; note = phosphorothioate linkage
  modified_base order(1,2,3,4,6,10,11,12,13,14,16,17,18,19): mod_base = OTHER; note = 2'-methoxy-modified
  modified_base order(5,7,8,9,15): mod_base = OTHER; note = 2'-fluoro-modified
gaaagccgtgctgtcagca

SEQ ID NO: 1398 - RNA, 19 nt, synthetic construct
  source 1..19: mol_type = other RNA; note = GPSZRA342S5 sense strand
  modified_base order(1^2,18^19): mod_base = OTHER; note = phosphorothioate linkage
  modified_base order(1,2,3,4,6,10,11,12,13,14,16,17,18,19): mod_base = OTHER; note = 2'-methoxy-modified
  modified_base order(5,7,8,9,15): mod_base = OTHER; note = 2'-fluoro-modified
tgtcagcatcagcatcatc

SEQ ID NO: 1399 - RNA, 19 nt, synthetic construct
  source 1..19: mol_type = other RNA; note = GPSZRA378S5 sense strand
  modified_base order(1^2,18^19): mod_base = OTHER; note = phosphorothioate linkage
  modified_base order(1,2,3,4,6,10,11,12,13,14,16,17,18,19): mod_base = OTHER; note = 2'-methoxy-modified
  modified_base order(5,7,8,9,15): mod_base = OTHER; note = 2'-fluoro-modified
aagaggaggagcgtgcaga

SEQ ID NO: 1400 - RNA, 19 nt, synthetic construct
  source 1..19: mol_type = other RNA; note = GPSZRA379S5 sense strand
  modified_base order(1^2,18^19): mod_base = OTHER; note = phosphorothioate linkage
  modified_base order(1,2,3,4,6,10,11,12,13,14,16,17,18,19): mod_base = OTHER; note = 2'-methoxy-modified
  modified_base order(5,7,8,9,15): mod_base = OTHER; note = 2'-fluoro-modified
gaatcagtcggaggaacct

SEQ ID NO: 1401 - RNA, 19 nt, synthetic construct
  source 1..19: mol_type = other RNA; note = GPSZRA380S5 sense strand
  modified_base order(1^2,18^19): mod_base = OTHER; note = phosphorothioate linkage
  modified_base order(1,2,3,4,6,10,11,12,13,14,16,17,18,19): mod_base = OTHER; note = 2'-methoxy-modified
  modified_base order(5,7,8,9,15): mod_base = OTHER; note = 2'-fluoro-modified
aatcagtcggaggaacctg

SEQ ID NO: 1402 - RNA, 19 nt, synthetic construct
  source 1..19: mol_type = other RNA; note = GPSZRA381S5 sense strand
  modified_base order(1^2,18^19): mod_base = OTHER; note = phosphorothioate linkage
  modified_base order(1,2,3,4,6,10,11,12,13,14,16,17,18,19): mod_base = OTHER; note = 2'-methoxy-modified
  modified_base order(5,7,8,9,15): mod_base = OTHER; note = 2'-fluoro-modified
atcagtcggaggaacctga

SEQ ID NO: 1403 - RNA, 19 nt, synthetic construct
  source 1..19: mol_type = other RNA; note = GPSZRA402S5/GPSZRA402S5-VP sense strand
  modified_base order(1^2,18^19): mod_base = OTHER; note = phosphorothioate linkage
  modified_base order(1,2,3,4,6,10,11,12,13,14,16,17,18,19): mod_base = OTHER; note = 2'-methoxy-modified
  modified_base order(5,7,8,9,15): mod_base = OTHER; note = 2'-fluoro-modified
ccaactctctcctgtataa

SEQ ID NO: 1404 - RNA, 19 nt, synthetic construct
  source 1..19: mol_type = other RNA; note = GPSZRA407S5 sense strand
  modified_base order(1^2,18^19): mod_base = OTHER; note = phosphorothioate linkage
  modified_base order(1,2,3,4,6,10,11,12,13,14,16,17,18,19): mod_base = OTHER; note = 2'-methoxy-modified
  modified_base order(5,7,8,9,15): mod_base = OTHER; note = 2'-fluoro-modified
cctgtataaccccaccttg

SEQ ID NO: 1405 - RNA, 19 nt, synthetic construct
  source 1..19: mol_type = other RNA; note = GPSZRA408S5 sense strand
  modified_base order(1^2,18^19): mod_base = OTHER; note = phosphorothioate linkage
  modified_base order(1,2,3,4,6,10,11,12,13,14,16,17,18,19): mod_base = OTHER; note = 2'-methoxy-modified
  modified_base order(5,7,8,9,15): mod_base = OTHER; note = 2'-fluoro-modified
ctgtataaccccaccttgc

SEQ ID NO: 1406 - RNA, 19 nt, synthetic construct
  source 1..19: mol_type = other RNA; note = GPSZRA409S5 sense strand
  modified_base order(1^2,18^19): mod_base = OTHER; note = phosphorothioate linkage
  modified_base order(1,2,3,4,6,10,11,12,13,14,16,17,18,19): mod_base = OTHER; note = 2'-methoxy-modified
  modified_base order(5,7,8,9,15): mod_base = OTHER; note = 2'-fluoro-modified
tgtataaccccaccttgcc

SEQ ID NO: 1407 - RNA, 19 nt, synthetic construct
  source 1..19: mol_type = other RNA; note = GPSZRA410S5 sense strand
  modified_base order(1^2,18^19): mod_base = OTHER; note = phosphorothioate linkage
  modified_base order(1,2,3,4,6,10,11,12,13,14,16,17,18,19): mod_base = OTHER; note = 2'-methoxy-modified
  modified_base order(5,7,8,9,15): mod_base = OTHER; note = 2'-fluoro-modified
gtataaccccaccttgcca

SEQ ID NO: 1408 - RNA, 19 nt, synthetic construct
  source 1..19: mol_type = other RNA; note = GPSZRA411S5 sense strand
  modified_base order(1^2,18^19): mod_base = OTHER; note = phosphorothioate linkage
  modified_base order(1,2,3,4,6,10,11,12,13,14,16,17,18,19): mod_base = OTHER; note = 2'-methoxy-modified
  modified_base order(5,7,8,9,15): mod_base = OTHER; note = 2'-fluoro-modified
tataaccccaccttgccaa

SEQ ID NO: 1409-1416 - skipped (8 entries)

SEQ ID NO: 1417 - DNA, 400 bp, synthetic construct
  source 1..400: mol_type = other DNA; note = RAGE mRNA1
agacagagccaggaccctggaaggaagcaggatggctgccggaacagcagttggagcctgggtgctggtcctcagtctgtggggggcagtagtaggtgctcaaaacatcacagcccggattggcgagccactggtgctgaagtgtaagggggcccccaagaaaccaccccagcggctggaatggaaactgaacacaggccggacagaagcttggaaggtcctgtctccccagggaggaggcccctgggacagtgtggctcgtgtccttcccaacggctccctcttccttccggctgtcgggatccaggatgaggggattttccggtgccaggcaatgaacaggaatggaaaggagaccaagtccaactaccgagtccgtgtctaccagattcctgggaag

SEQ ID NO: 1418 - DNA, 400 bp, synthetic construct
  source 1..400: mol_type = other DNA; note = RAGE mRNA2
aggagaccaagtccaactaccgagtccgtgtctaccagattcctgggaagccagaaattgtagattctgcctctgaactcacggctggtgttcccaataaggtggggacatgtgtgtcagagggaagctaccctgcagggactcttagctggcacttggatgggaagcccctggtgcctaatgagaagggagtatctgtgaaggaacagaccaggagacaccctgagacagggctcttcacactgcagtcggagctaatggtgaccccagcccggggaggagatccccgtcccaccttctcctgtagcttcagcccaggccttccccgacaccgggccttgcgcacagcccccatccagccccgtgtctgggagcctgtgcctctggaggaggtccaatt

SEQ ID NO: 1419 - DNA, 400 bp, synthetic construct
  source 1..400: mol_type = other DNA; note = RAGE mRNA3
cccatccagccccgtgtctgggagcctgtgcctctggaggaggtccaattggtggtggagccagaaggtggagcagtagctcctggtggaaccgtaaccctgacctgtgaagtccctgcccagccctctcctcaaatccactggatgaaggatggtgtgcccttgccccttccccccagccctgtgctgatcctccctgagatagggcctcaggaccagggaacctacagctgtgtggccacccattccagccacgggccccaggaaagccgtgctgtcagcatcagcatcatcgaaccaggcgaggaggggccaactgcaggctctgtgggaggatcagggctgggaactctagccctggccctggggatcctgggaggcctggggacagccgccctgc

SEQ ID NO: 1420 - DNA, 400 bp, synthetic construct
  source 1..400: mol_type = other DNA; note = RAGE mRNA4
aggctctgtgggaggatcagggctgggaactctagccctggccctggggatcctgggaggcctggggacagccgccctgctcattggggtcatcttgtggcaaaggcggcaacgccgaggagaggagaggaaggccccagaaaaccaggaggaagaggaggagcgtgcagaactgaatcagtcggaggaacctgaggcaggcgagagtagtactggagggccttgaggggcccacagacagatcccatccatcagctcccttttctttttcccttgaactgttctggcctcagaccaactctctcctgtataatctctctcctgtataaccccaccttgccaagctttcttctacaaccagagccccccacaatgatgattaaacacctgacacatcttg

SEQ ID NO: 1421 - RNA, 23 nt, synthetic construct
  source 1..23: mol_type = other RNA; note = NC1 antisense strand
aaacgtgacacgttcggagaatt

SEQ ID NO: 1422 - RNA, 21 nt, synthetic construct
  source 1..21: mol_type = other RNA; note = NC1 sense strand
ttctccgaacgtgtcacgttt

SEQ ID NO: 1423-1425 - skipped (3 entries)

SEQ ID NO: 1426 - RNA, 21 nt, synthetic construct
  source 1..21: mol_type = other RNA; note = GPSZRA222S1-VP antisense strand
  modified_base order(1,3,5,7,9,11,12,13,15,17,19,20,21): mod_base = OTHER; note = 2'-methoxy-modified
  modified_base order(2,4,6,8,10,14,16,18): mod_base = OTHER; note = 2'-fluoro-modified
  modified_base order(1^2,2^3,19^20,20^21): mod_base = OTHER; note = phosphorothioate linkage
  modified_base 1: mod_base = OTHER; note = 5'-(E)-vinylphosphonate-modified
tccgactgcagtgtgaagagc

SEQ ID NO: 1427 - RNA, 21 nt, synthetic construct
  source 1..21: mol_type = other RNA; note = GPSZRA222S3-VP antisense strand
  modified_base order(1,3,4,5,7,8,9,10,11,12,13,15,17,18,19,20,21): mod_base = OTHER; note = 2'-methoxy-modified
  modified_base order(2,6,14,16): mod_base = OTHER; note = 2'-fluoro-modified
  modified_base order(1^2,2^3,19^20,20^21): mod_base = OTHER; note = phosphorothioate linkage
  modified_base 1: mod_base = OTHER; note = 5'-(E)-vinylphosphonate-modified
tccgactgcagtgtgaagagc

SEQ ID NO: 1428 - RNA, 21 nt, synthetic construct
  source 1..21: mol_type = other RNA; note = GPSZRA222S4-VP antisense strand
  modified_base order(1,3,4,5,7,9,10,11,12,13,15,17,18,19,20,21): mod_base = OTHER; note = 2'-methoxy-modified
  modified_base order(2,6,8,14,16): mod_base = OTHER; note = 2'-fluoro-modified
  modified_base order(1^2,2^3,19^20,20^21): mod_base = OTHER; note = phosphorothioate linkage
  modified_base 1: mod_base = OTHER; note = 5'-(E)-vinylphosphonate-modified
tccgactgcagtgtgaagagc

SEQ ID NO: 1429 - RNA, 21 nt, synthetic construct
  source 1..21: mol_type = other RNA; note = GPSZRA227S1-VP antisense strand
  modified_base order(1,3,5,7,9,11,12,13,15,17,19,20,21): mod_base = OTHER; note = 2'-methoxy-modified
  modified_base order(2,4,6,8,10,14,16,18): mod_base = OTHER; note = 2'-fluoro-modified
  modified_base order(1^2,2^3,19^20,20^21): mod_base = OTHER; note = phosphorothioate linkage
  modified_base 1: mod_base = OTHER; note = 5'-(E)-vinylphosphonate-modified
ttagctccgactgcagtgtga

SEQ ID NO: 1430 - RNA, 21 nt, synthetic construct
  source 1..21: mol_type = other RNA; note = GPSZRA267S2-VP antisense strand
  modified_base order(1,3,4,5,7,9,10,11,12,13,15,17,18,19,20,21): mod_base = OTHER; note = 2'-methoxy-modified
  modified_base order(2,6,8,14,16): mod_base = OTHER; note = 2'-fluoro-modified
  modified_base order(1^2,2^3,19^20,20^21): mod_base = OTHER; note = phosphorothioate linkage
  modified_base 1: mod_base = OTHER; note = 5'-(E)-vinylphosphonate-modified
ttccaccaggagctactgctc

SEQ ID NO: 1431 - RNA, 21 nt, synthetic construct
  source 1..21: mol_type = other RNA; note = GPSZRA284S3-VP antisense strand
  modified_base order(1,3,4,5,7,8,9,10,11,12,13,15,17,18,19,20,21): mod_base = OTHER; note = 2'-methoxy-modified
  modified_base order(2,6,14,16): mod_base = OTHER; note = 2'-fluoro-modified
  modified_base order(1^2,2^3,19^20,20^21): mod_base = OTHER; note = phosphorothioate linkage
  modified_base 1: mod_base = OTHER; note = 5'-(E)-vinylphosphonate-modified
tcacaggtcagggttacggtt

SEQ ID NO: 1432 - RNA, 21 nt, synthetic construct
  source 1..21: mol_type = other RNA; note = GPSZRA314S1-VP antisense strand
  modified_base order(1,3,5,7,9,11,12,13,15,17,19,20,21): mod_base = OTHER; note = 2'-methoxy-modified
  modified_base order(2,4,6,8,10,14,16,18): mod_base = OTHER; note = 2'-fluoro-modified
  modified_base order(1^2,2^3,19^20,20^21): mod_base = OTHER; note = phosphorothioate linkage
  modified_base 1: mod_base = OTHER; note = 5'-(E)-vinylphosphonate-modified
acaccatccttcatccagtgg

SEQ ID NO: 1433 - RNA, 21 nt, synthetic construct
  source 1..21: mol_type = other RNA; note = GPSZRA314S2-VP antisense strand
  modified_base order(1,3,4,5,7,9,10,11,12,13,15,17,18,19,20,21): mod_base = OTHER; note = 2'-methoxy-modified
  modified_base order(2,6,8,14,16): mod_base = OTHER; note = 2'-fluoro-modified
  modified_base order(1^2,2^3,19^20,20^21): mod_base = OTHER; note = phosphorothioate linkage
  modified_base 1: mod_base = OTHER; note = 5'-(E)-vinylphosphonate-modified
acaccatccttcatccagtgg

SEQ ID NO: 1434 - RNA, 21 nt, synthetic construct
  source 1..21: mol_type = other RNA; note = GPSZRA314S3-VP antisense strand
  modified_base order(1,3,4,5,7,8,9,10,11,12,13,15,17,18,19,20,21): mod_base = OTHER; note = 2'-methoxy-modified
  modified_base order(2,6,14,16): mod_base = OTHER; note = 2'-fluoro-modified
  modified_base order(1^2,2^3,19^20,20^21): mod_base = OTHER; note = phosphorothioate linkage
  modified_base 1: mod_base = OTHER; note = 5'-(E)-vinylphosphonate-modified
acaccatccttcatccagtgg

SEQ ID NO: 1435 - RNA, 21 nt, synthetic construct
  source 1..21: mol_type = other RNA; note = GPSZRA314S5-VP antisense strand
  modified_base order(1,3,4,5,7,9,10,11,12,13,15,17,18,19,20,21): mod_base = OTHER; note = 2'-methoxy-modified
  modified_base order(2,6,8,14,16): mod_base = OTHER; note = 2'-fluoro-modified
  modified_base order(1^2,2^3,19^20,20^21): mod_base = OTHER; note = phosphorothioate linkage
  modified_base 1: mod_base = OTHER; note = 5'-(E)-vinylphosphonate-modified
acaccatccttcatccagtgg

SEQ ID NO: 1436 - RNA, 21 nt, synthetic construct
  source 1..21: mol_type = other RNA; note = GPSZRA318S2-VP antisense strand
  modified_base order(1,3,4,5,7,9,10,11,12,13,15,17,18,19,20,21): mod_base = OTHER; note = 2'-methoxy-modified
  modified_base order(2,6,8,14,16): mod_base = OTHER; note = 2'-fluoro-modified
  modified_base order(1^2,2^3,19^20,20^21): mod_base = OTHER; note = phosphorothioate linkage
  modified_base 1: mod_base = OTHER; note = 5'-(E)-vinylphosphonate-modified
gggcacaccatccttcatcca

SEQ ID NO: 1437 - RNA, 21 nt, synthetic construct
  source 1..21: mol_type = other RNA; note = GPSZRA402S4-VP antisense strand
  modified_base order(1,3,4,5,7,9,10,11,12,13,15,17,18,19,20,21): mod_base = OTHER; note = 2'-methoxy-modified
  modified_base order(2,6,8,14,16): mod_base = OTHER; note = 2'-fluoro-modified
  modified_base order(1^2,2^3,19^20,20^21): mod_base = OTHER; note = phosphorothioate linkage
  modified_base 1: mod_base = OTHER; note = 5'-(E)-vinylphosphonate-modified
ttatacaggagagagttggtc

SEQ ID NO: 1438 - RNA, 21 nt, synthetic construct
  source 1..21: mol_type = other RNA; note = GPSZRA402S5-VP antisense strand
  modified_base order(1,3,4,5,7,9,10,11,12,13,15,17,18,19,20,21): mod_base = OTHER; note = 2'-methoxy-modified
  modified_base order(2,6,8,14,16): mod_base = OTHER; note = 2'-fluoro-modified
  modified_base order(1^2,2^3,19^20,20^21): mod_base = OTHER; note = phosphorothioate linkage
  modified_base 1: mod_base = OTHER; note = 5'-(E)-vinylphosphonate-modified
ttatacaggagagagttggtc

SEQ ID NO: 1439 - DNA, 23 bp, synthetic construct
  source 1..23: mol_type = other DNA; note = HGAPDH-FO
catgagaagtatgacaacagcct

SEQ ID NO: 1440 - DNA, 22 bp, synthetic construct
  source 1..22: mol_type = other DNA; note = HGAPDH-RE
agtccttccacgataccaaagt

SEQ ID NO: 1441 - DNA, 21 bp, synthetic construct
  source 1..21: mol_type = other DNA; note = HGAPDH-PR
caatgcctcctgcaccaccaa

SEQ ID NO: 1442 - DNA, 19 bp, synthetic construct
  source 1..19: mol_type = other DNA; note = RAGE-F9; note = RAGE-F9
gtgtccttcccaacggctc

SEQ ID NO: 1443 - DNA, 19 bp, synthetic construct
  source 1..19: mol_type = other DNA; note = RAGE-R9
attgcctggcaccggaaaa

SEQ ID NO: 1444 - DNA, 21 bp, synthetic construct
  source 1..21: mol_type = other DNA; note = RAGE-P9.1
ccggctgtcgggatccaggat

SEQ ID NO: 1445 - RNA, 23 nt, synthetic construct
  source 1..23: mol_type = other RNA; note = NC5 antisense strand
  modified_base order(1,3,5,7,9,11,13,15,17,19,21,23): mod_base = OTHER; note = 2'-methoxy-modified
  modified_base order(2,4,6,8,10,12,14,16,18,20,22): mod_base = OTHER; note = 2'-fluoro-modified
  modified_base order(1^2,2^3,21^22,22^23): mod_base = OTHER; note = phosphorothioate linkage
tcgaagtactcagcgtaagtgat

SEQ ID NO: 1446 - RNA, 21 nt, synthetic construct
  source 1..21: mol_type = other RNA; note = NC5 sense strand
  modified_base order(2,4,6,8,10,12,14,16,18,20): mod_base = OTHER; note = 2'-methoxy-modified
  modified_base order(1,3,5,7,9,11,13,15,17,19,21): mod_base = OTHER; note = 2'-fluoro-modified
  modified_base order(1^2,2^3,19^20,20^21): mod_base = OTHER; note = phosphorothioate linkage
cacttacgctgagtacttcga